European Patent Application EP 4 678 742 A1, published January 14, 2026. Title: IMPROVED CAS9 PROTEINS. Applicant: Astrazeneca AB. The sequence listing filed with the application follows.

SEQUENCE LISTING (215 sequences)

SEQ ID NO: 1 - protein, 1247 aa, Campylobacter lanienae
KSLSINIDMGAINNGIFIATCQDDKIIDKNAFDIKFDKGKLNFSKIDRTLRRHTRRSFDRDRFVLRLLGEILPLENLSNNQKEKLFGLFKNRGFNYLNVNFNAEIDSDNLEILNALDRYYFKDCRVLSDFENSISKIFNELENNEILAFLDDQAQILNQAKEHKNKILNKNINAILEFLESIKNESFKNNKHRKSYLKDIKNEIENSFKDIILKLKIFKNSQELYYFIGNIANFQTRILRRYFNAKFDLVFDDAKLKKNILRNINYLDFISTDEKANKNKILENLNAFSTLEFLKNTDPIVTIPPYENAKNKKPQSCQALVINDEKITPSLKDIAHKILSNSNFECLKTDENGVLADNIKDNEIAKYLQRILDISKGILDDKELYPRLLEKDENAKIFAQEIRLNSVELKEFKDFAKKYYDEVNLAKKGIIKNELLKPCCLHTPHKNKNKNALISALFLKSITQKEIENLEDFFANNKISGNQTFKGFFERLSELKKRYQNRFFHILEHEPTKELEGILKNYKKVMEKIVEHNSNFSFKAPFDDSTISTNFNYLTQLGDIIFDEKSRGFAKTCKFHTLENLIRSSAKSAIASRLASNSARLINGKIEMYLDRLAHEIIKKIDFTDIYNVQINVEMNKFNFESNLSKLGLAKERQKDEESFICPYSGAKISQTNCEYDHILPRSKGLYNSLANLIPTSSTSNQIKSNTKYLLSNLDENYLKYIFAKTQTTDLNSFKAFIDENISKIDENDFTNFKNLSFFEQIAFRHALFLDTDDNSFKKALRLLKLDTIKTHSNGTQKRFINILIEKISKLTKSGIDLNFIDSKLVSSTRKDLAQNDTSIAKQEIQDSHSHCVDASIVFYLANSKIIKGQIEPDYDYFKDIYPKDSDIILPQSKQYLELNQKSQKSKKLFDDSVYSLVYEGKFDEKQKKILTQYELLKENGFVDTHKVFELIFKSFKDKDTIVLKDLKFLDNHLKSYIRKDIFSIFFNEKGELKEAKELKSATKNIDKFYTILSQNQDKIYTIKLDEKAKEKKTLQRNKVIELYKEIFYTKNAKPRARGKNRVTFSLPVYAKDAKYAIKRNSGFAGLKNKDIATKTYIDIDSREILKIPYYSTNVLPIRISDILEILSLQSKNAKQIYKIKIQDNLPKQIVSLDFILSQANRHEVLVSFDKSKLEIQNINDDNGENTFIQKYLCDDFKEFLGKPRDNKIEIIKNNDDILAIKYCVESTSKANKEIIVKALSDETPSA

SEQ ID NO: 2 - protein, 1247 aa, synthetic construct
KSLSINIDMGAINNGIFIATCQDDKIIDKNAFDIKFDKGKLNFSKIDRTLRRHTRRSFDRDRFVLRLLGEILPLENLSNNQKEKLFGLFKNRGFNYLNVNFNAEIDSDNLEILNALDRYYFKDCRVLSDFENSISKIFNELENNEILAFLDDQAQILNQAKEHKNKILNKNINAILEFLESIKNESFKNNKHRKSYLKDIKNEIENSFKDIILKLKIFKNSQELYYFIGNIANFQTRILRRYFNAKFDLVFDDAKLKKNILRNINYLDFISTDEKANKNKILENLNAFSTLEFLKNTDPIVTIPPYENAKNKKPQSCQALVINDEKITPSLKDIAHKILSNSNFECLKTDENGVLADNIKDNEIAKYLQRILDISKGILDDKELYPRLLEKDENAKIFAQEIRLNSVELKEFKDFAKKYYDEVNLAKKGIIKNELLKPCCLHTPHKNKNKNALISALFLKSITQKEIENLEDFFANNKISGNQTFKGFFERLSELKKRYQNRFFHILEHEPTKELEGILKNYKKVMEKIVEHNSNFSFKAPFDDSTISTNFNYLTQLGDIIFDEKSRGFAKTCKFHTLENLIRSSAKSAIASRLASNSARLINGKIEMYLDRLAHEIIKKIDFTDIYNVQINVEMNKFNFESNLSKLGLAKERQKDEESFICPYSGAKISQTNCEYDAILPRSKGLYNSLANLIPTSSTSNQIKSNTKYLLSNLDENYLKYIFAKTQTTDLNSFKAFIDENISKIDENDFTNFKNLSFFEQIAFRHALFLDTDDNSFKKALRLLKLDTIKTHSNGTQKRFINILIEKISKLTKSGIDLNFIDSKLVSSTRKDLAQNDTSIAKQEIQDSHSHCVDASIVFYLANSKIIKGQIEPDYDYFKDIYPKDSDIILPQSKQYLELNQKSQKSKKLFDDSVYSLVYEGKFDEKQKKILTQYELLKENGFVDTHKVFELIFKSFKDKDTIVLKDLKFLDNHLKSYIRKDIFSIFFNEKGELKEAKELKSATKNIDKFYTILSQNQDKIYTIKLDEKAKEKKTLQRNKVIELYKEIFYTKNAKPRARGKNRVTFSLPVYAKDAKYAIKRNSGFAGLKNKDIATKTYIDIDSREILKIPYYSTNVLPIRISDILEILSLQSKNAKQIYKIKIQDNLPKQIVSLDFILSQANRHEVLVSFDKSKLEIQNINDDNGENTFIQKYLCDDFKEFLGKPRDNKIEIIKNNDDILAIKYCVESTSKANKEIIVKALSDETPSA

SEQ ID NO: 3 - protein, 1247 aa, synthetic construct
KSLSINIDMGAINNGIFIATCQDDKIIDKNAFDIKFDKGKLNFSKIDRTLRRHTRRSFDRDRFVLRLLGEILPLENLSNNQKEKLFGLFKNRGFNYLNVNFNAEIDSDNLEILNALDRYYFKDCRVLSDFENSISKIFNELENNEILAFLDDQAQILNQAKEHKNKILNKNINAILEFLESIKNESFKNNKHRKSYLKDIKNEIENSFKDIILKLKIFKNSQELYYFIGNIANFQTRILRRYFNAKFDLVFDDAKLKKNILRNINYLDFISTDEKANKNKILENLNAFSTLEFLKNTDPIVTIPPYENAKNKKPQSCQALVINDEKITPSLKDIAHKILSNSNFECLKTDENGVLADNIKDNEIAKYLQRILDISKGILDDKELYPRLLEKDENAKIFAQEIRLNSVELKEFKDFAKKYYDEVNLAKKGIIKNELLKPCCLHTPHKNKNKNALISALFLKSITQKEIENLEDFFANNKISGNQTFKGFFERLSELKKRYQNRFFHILEHEPTKELEGILKNYKKVMEKIVEHNSNFSFKAPFDDSTISTNFNYLTQLGDIIFDEKSRGFAKTCKFHTLENLIRSSAKSAIASRLASNSARLINGKIEMYLDRLAHEIIKKIDFTDIYNVQINVEMNKFNFESNLSKLGLAKERQKDEESFICPYSGAKISQTNCEYDHILPRSKGLYNSLANLIPTSSTSNQIKSNTKYLLSNLDENYLKYIFAKTQTTDLNSFKAFIDENISKIDENDFTNFKNLSFFEQIAFRHALFLDTDDNSFKKALRLLKLDTIKTHSNGTQKRFINILIEKISKLTKSGIDLNFIDSKLVSSTRKDLAQNDTSIAKQEIQDSHSHCVDASIVFYLANSKIIKGQIEPDYDYFKDIYPKDSDIILPQSKQYLELNQKSQKSKKLFDDSVYSLVYEGKFDEKQKKILTQYELLKENGFVDTHKVFELIFKSFKDKDTIVLKDLKFLDNHLKSYIRKDIFSIFFNEKGELKEAKELKSATKNIDKFYTILSQNQDKIYTIKLDEKAKEKKTLQRNKVIELYKEIFYTKNAKPRARGKNRVTFSLPVYAKDAKYAIKRNSGFAGLKRKDIATKTYIDIDSREILKIPYYSTNVLPIRISDILEILSLQSKNAKQIYKIKIQDNLPKQIVSLDFILSQANRHEVLVSFDKSKLEIQNINDDNGENTFIQKYLCDDFKEFLGKPRDNKIEIIKNNDDILAIKYCVESTSKANKEIIVKALSDETPSA

SEQ ID NO: 4 - protein, 1247 aa, synthetic construct
KSLSINIDMGAINNGIFIATCQDDKIIDKNAFDIKFDKGKLNFSKIDRTLRRHTRRSFDRDRFVLRLLGEILPLENLSNNQKEKLFGLFKNRGFNYLNVNFNAEIDSDNLEILNALDRYYFKDCRVLSDFENSISKIFNELENNEILAFLDDQAQILNQAKEHKNKILNKNINAILEFLESIKNESFKNNKHRKSYLKDIKNEIENSFKDIILKLKIFKNSQELYYFIGNIANFQTRILRRYFNAKFDLVFDDAKLKKNILRNINYLDFISTDEKANKNKILENLNAFSTLEFLKNTDPIVTIPPYENAKNKKPQSCQALVINDEKITPSLKDIAHKILSNSNFECLKTDENGVLADNIKDNEIAKYLQRILDISKGILDDKELYPRLLEKDENAKIFAQEIRLNSVELKEFKDFAKKYYDEVNLAKKGIIKNELLKPCCLHTPHKNKNKNALISALFLKSITQKEIENLEDFFANNKISGNQTFKGFFERLSELKKRYQNRFFHILEHEPTKELEGILKNYKKVMEKIVEHNSNFSFKAPFDDSTISTNFNYLTQLGDIIFDEKSRGFAKTCKFHTLENLIRSSAKSAIASRLASNSARLINGKIEMYLDRLAHEIIKKIDFTDIYNVQINVEMNKFNFESNLSKLGLAKERQKDEESFICPYSGAKISQTNCEYDHILPRSKGLYNSLANLIPTSSTSNQIKSNTKYLLSNLDENYLKYIFAKTQTTDLNSFKAFIDENISKIDENDFTNFKNLSFFEQIAFRHALFLDTDDNSFKKALRLLKLDTIKTHSNGTQKRFINILIEKISKLTKSGIDLNFIDSKLVSSTRKDLAQNDTSIAKQEIQDSHSHCVDASIVFYLANSKIIKGQIEPDYDYFKDIYPKDSDIILPQSKQYLELNQKSQKSKKLFDDSVYSLVYEGKFDEKQKKILTQYELLKENGFVDTHKVFELIFKSFKDKDTIVLKDLKFLDNHLKSYIRKDIFSIFFNEKGELKEAKELKSATKNIDKFYTILSQNQDKIYTIKLDEKAKEKKTLQRNKVIELYKEIFYTKNAKPRARGKNRVTFSLPVYAKDAKYAIKRNSGFAGLKNKDRATKTYIDIDSREILKIPYYSTNVLPIRISDILEILSLQSKNAKQIYKIKIQDNLPKQIVSLDFILSQANRHEVLVSFDKSKLEIQNINDDNGENTFIQKYLCDDFKEFLGKPRDNKIEIIKNNDDILAIKYCVESTSKANKEIIVKALSDETPSA

SEQ ID NO: 5 - protein, 1247 aa, synthetic construct
KSLSINIDMGAINNGIFIATCQDDKIIDKNAFDIKFDKGKLNFSKIDRTLRRHTRRSFDRDRFVLRLLGEILPLENLSNNQKEKLFGLFKNRGFNYLNVNFNAEIDSDNLEILNALDRYYFKDCRVLSDFENSISKIFNELENNEILAFLDDQAQILNQAKEHKNKILNKNINAILEFLESIKNESFKNNKHRKSYLKDIKNEIENSFKDIILKLKIFKNSQELYYFIGNIANFQTRILRRYFNAKFDLVFDDAKLKKNILRNINYLDFISTDEKANKNKILENLNAFSTLEFLKNTDPIVTIPPYENAKNKKPQSCQALVINDEKITPSLKDIAHKILSNSNFECLKTDENGVLADNIKDNEIAKYLQRILDISKGILDDKELYPRLLEKDENAKIFAQEIRLNSVELKEFKDFAKKYYDEVNLAKKGIIKNELLKPCCLHTPHKNKNKNALISALFLKSITQKEIENLEDFFANNKISGNQTFKGFFERLSELKKRYQNRFFHILEHEPTKELEGILKNYKKVMEKIVEHNSNFSFKAPFDDSTISTNFNYLTQLGDIIFDEKSRGFAKTCKFHTLENLIRSSAKSAIASRLASNSARLINGKIEMYLDRLAHEIIKKIDFTDIYNVQINVEMNKFNFESNLSKLGLAKERQKDEESFICPYSGAKISQTNCEYDHILPRSKGLYNSLANLIPTSSTSNQIKSNTKYLLSNLDENYLKYIFAKTQTTDLNSFKAFIDENISKIDENDFTNFKNLSFFEQIAFRHALFLDTDDNSFKKALRLLKLDTIKTHSNGTQKRFINILIEKISKLTKSGIDLNFIDSKLVSSTRKDLAQNDTSIAKQEIQDSHSHCVDASIVFYLANSKIIKGQIEPDYDYFKDIYPKDSDIILPQSKQYLELNQKSQKSKKLFDDSVYSLVYEGKFDEKQKKILTQYELLKENGFVDTHKVFELIFKSFKDKDTIVLKDLKFLDNHLKSYIRKDIFSIFFNEKGELKEAKELKSATKNIDKFYTILSQNQDKIYTIKLDEKAKEKKTLQRNKVIELYKEIFYTKNAKPRARGKNRVTFSLPVYAKDAKYAIKRNSGFAGLKNKDIRTKTYIDIDSREILKIPYYSTNVLPIRISDILEILSLQSKNAKQIYKIKIQDNLPKQIVSLDFILSQANRHEVLVSFDKSKLEIQNINDDNGENTFIQKYLCDDFKEFLGKPRDNKIEIIKNNDDILAIKYCVESTSKANKEIIVKALSDETPSA

SEQ ID NO: 6 - protein, 1247 aa, synthetic construct
KSLSINIDMGAINNGIFIATCQDDKIIDKNAFDIKFDKGKLNFSKIDRTLRRHTRRSFDRDRFVLRLLGEILPLENLSNNQKEKLFGLFKNRGFNYLNVNFNAEIDSDNLEILNALDRYYFKDCRVLSDFENSISKIFNELENNEILAFLDDQAQILNQAKEHKNKILNKNINAILEFLESIKNESFKNNKHRKSYLKDIKNEIENSFKDIILKLKIFKNSQELYYFIGNIANFQTRILRRYFNAKFDLVFDDAKLKKNILRNINYLDFISTDEKANKNKILENLNAFSTLEFLKNTDPIVTIPPYENAKNKKPQSCQALVINDEKITPSLKDIAHKILSNSNFECLKTDENGVLADNIKDNEIAKYLQRILDISKGILDDKELYPRLLEKDENAKIFAQEIRLNSVELKEFKDFAKKYYDEVNLAKKGIIKNELLKPCCLHTPHKNKNKNALISALFLKSITQKEIENLEDFFANNKISGNQTFKGFFERLSELKKRYQNRFFHILEHEPTKELEGILKNYKKVMEKIVEHNSNFSFKAPFDDSTISTNFNYLTQLGDIIFDEKSRGFAKTCKFHTLENLIRSSAKSAIASRLASNSARLINGKIEMYLDRLAHEIIKKIDFTDIYNVQINVEMNKFNFESNLSKLGLAKERQKDEESFICPYSGAKISQTNCEYDHILPRSKGLYNSLANLIPTSSTSNQIKSNTKYLLSNLDENYLKYIFAKTQTTDLNSFKAFIDENISKIDENDFTNFKNLSFFEQIAFRHALFLDTDDNSFKKALRLLKLDTIKTHSNGTQKRFINILIEKISKLTKSGIDLNFIDSKLVSSTRKDLAQNDTSIAKQEIQDSHSHCVDASIVFYLANSKIIKGQIEPDYDYFKDIYPKDSDIILPQSKQYLELNQKSQKSKKLFDDSVYSLVYEGKFDEKQKKILTQYELLKENGFVDTHKVFELIFKSFKDKDTIVLKDLKFLDNHLKSYIRKDIFSIFFNEKGELKEAKELKSATKNIDKFYTILSQNQDKIYTIKLDEKAKEKKTLQRNKVIELYKEIFYTKNAKPRARGKNRVTFSLPVYAKDAKYAIKRNSGFAGLKNKDIKTKTYIDIDSREILKIPYYSTNVLPIRISDILEILSLQSKNAKQIYKIKIQDNLPKQIVSLDFILSQANRHEVLVSFDKSKLEIQNINDDNGENTFIQKYLCDDFKEFLGKPRDNKIEIIKNNDDILAIKYCVESTSKANKEIIVKALSDETPSA

SEQ ID NO: 7 - protein, 1247 aa, synthetic construct
KSLSINIDMGAINNGIFIATCQDDKIIDKNAFDIKFDKGKLNFSKIDRTLRRHTRRSFDRDRFVLRLLGEILPLENLSNNQKEKLFGLFKNRGFNYLNVNFNAEIDSDNLEILNALDRYYFKDCRVLSDFENSISKIFNELENNEILAFLDDQAQILNQAKEHKNKILNKNINAILEFLESIKNESFKNNKHRKSYLKDIKNEIENSFKDIILKLKIFKNSQELYYFIGNIANFQTRILRRYFNAKFDLVFDDAKLKKNILRNINYLDFISTDEKANKNKILENLNAFSTLEFLKNTDPIVTIPPYENAKNKKPQSCQALVINDEKITPSLKDIAHKILSNSNFECLKTDENGVLADNIKDNEIAKYLQRILDISKGILDDKELYPRLLEKDENAKIFAQEIRLNSVELKEFKDFAKKYYDEVNLAKKGIIKNELLKPCCLHTPHKNKNKNALISALFLKSITQKEIENLEDFFANNKISGNQTFKGFFERLSELKKRYQNRFFHILEHEPTKELEGILKNYKKVMEKIVEHNSNFSFKAPFDDSTISTNFNYLTQLGDIIFDEKSRGFAKTCKFHTLENLIRSSAKSAIASRLASNSARLINGKIEMYLDRLAHEIIKKIDFTDIYNVQINVEMNKFNFESNLSKLGLAKERQKDEESFICPYSGAKISQTNCEYDHILPRSKGLYNSLANLIPTSSTSNQIKSNTKYLLSNLDENYLKYIFAKTQTTDLNSFKAFIDENISKIDENDFTNFKNLSFFEQIAFRHALFLDTDDNSFKKALRLLKLDTIKTHSNGTQKRFINILIEKISKLTKSGIDLNFIDSKLVSSTRKDLAQNDTSIAKQEIQDSHSHCVDASIVFYLANSKIIKGQIEPDYDYFKDIYPKDSDIILPQSKQYLELNQKSQKSKKLFDDSVYSLVYEGKFDEKQKKILTQYELLKENGFVDTHKVFELIFKSFKDKDTIVLKDLKFLDNHLKSYIRKDIFSIFFNEKGELKEAKELKSATKNIDKFYTILSQNQDKIYTIKLDEKAKEKKTLQRNKVIELYKEIFYTKNAKPRARGKNRVTFSLPVYAKDAKYAIKRNSGFAGLKNKDIATKTYIDIDSREILKIPYYSTNVLPIRISDILEILSLQSKNAKQIYKIKIQDNLPKQIVSLDFILSQRNRHEVLVSFDKSKLEIQNINDDNGENTFIQKYLCDDFKEFLGKPRDNKIEIIKNNDDILAIKYCVESTSKANKEIIVKALSDETPSA

SEQ ID NO: 8 - protein, 1247 aa, synthetic construct
KSLSINIAMGAINNGIFIATCQDDKIIDKNAFDIKFDKGKLNFSKIDRTLRRHTRRSFDRDRFVLRLLGEILPLENLSNNQKEKLFGLFKNRGFNYLNVNFNAEIDSDNLEILNALDRYYFKDCRVLSDFENSISKIFNELENNEILAFLDDQAQILNQAKEHKNKILNKNINAILEFLESIKNESFKNNKHRKSYLKDIKNEIENSFKDIILKLKIFKNSQELYYFIGNIANFQTRILRRYFNAKFDLVFDDAKLKKNILRNINYLDFISTDEKANKNKILENLNAFSTLEFLKNTDPIVTIPPYENAKNKKPQSCQALVINDEKITPSLKDIAHKILSNSNFECLKTDENGVLADNIKDNEIAKYLQRILDISKGILDDKELYPRLLEKDENAKIFAQEIRLNSVELKEFKDFAKKYYDEVNLAKKGIIKNELLKPCCLHTPHKNKNKNALISALFLKSITQKEIENLEDFFANNKISGNQTFKGFFERLSELKKRYQNRFFHILEHEPTKELEGILKNYKKVMEKIVEHNSNFSFKAPFDDSTISTNFNYLTQLGDIIFDEKSRGFAKTCKFHTLENLIRSSAKSAIASRLASNSARLINGKIEMYLDRLAHEIIKKIDFTDIYNVQINVEMNKFNFESNLSKLGLAKERQKDEESFICPYSGAKISQTNCEYDHILPRSKGLYNSLANLIPTSSTSNQIKSNTKYLLSNLDENYLKYIFAKTQTTDLNSFKAFIDENISKIDENDFTNFKNLSFFEQIAFRHALFLDTDDNSFKKALRLLKLDTIKTHSNGTQKRFINILIEKISKLTKSGIDLNFIDSKLVSSTRKDLAQNDTSIAKQEIQDSHSHCVDASIVFYLANSKIIKGQIEPDYDYFKDIYPKDSDIILPQSKQYLELNQKSQKSKKLFDDSVYSLVYEGKFDEKQKKILTQYELLKENGFVDTHKVFELIFKSFKDKDTIVLKDLKFLDNHLKSYIRKDIFSIFFNEKGELKEAKELKSATKNIDKFYTILSQNQDKIYTIKLDEKAKEKKTLQRNKVIELYKEIFYTKNAKPRARGKNRVTFSLPVYAKDAKYAIKRNSGFAGLKNKDIATKTYIDIDSREILKIPYYSTNVLPIRISDILEILSLQSKNAKQIYKIKIQDNLPKQIVSLDFILSQANRHEVLVSFDKSKLEIQNINDDNGENTFIQKYLCDDFKEFLGKPRDNKIEIIKNNDDILAIKYCVESTSKANKEIIVKALSDETPSA

SEQ ID NO: 9 - protein, 1247 aa, synthetic construct
KSLSINIDMGAINNGIFIATCQDDKIIDKNAFDIKFDKGKLNFSKIDRTLRRHTRRSFDRDRFVLRLLGEILPLENLSNNQKEKLFGLFKNRGFNYLNVNFNAEIDSDNLEILNALDRYYFKDCRVLSDFENSISKIFNELENNEILAFLDDQAQILNQAKEHKNKILNKNINAILEFLESIKNESFKNNKHRKSYLKDIKNEIENSFKDIILKLKIFKNSQELYYFIGNIANFQTRILRRYFNAKFDLVFDDAKLKKNILRNINYLDFISTDEKANKNKILENLNAFSTLEFLKNTDPIVTIPPYENAKNKKPQSCQALVINDEKITPSLKDIAHKILSNSNFECLKTDENGVLADNIKDNEIAKYLQRILDISKGILDDKELYPRLLEKDENAKIFAQEIRLNSVELKEFKDFAKKYYDEVNLAKKGIIKNELLKPCCLHTPHKNKNKNALISALFLKSITQKEIENLEDFFANNKISGNQTFKGFFERLSELKKRYQNRFFHILEHEPTKELEGILKNYKKVMEKIVEHNSNFSFKAPFDDSTISTNFNYLTQLGDIIFDEKSRGFAKTCKFHTLENLIRSSAKSAIASRLASNSARLINGKIEMYLDRLAHEIIKKIDFTDIYNVQINVEMNKFNFESNLSKLGLAKERQKDEESFICPYSGAKISQTNCEYDHILPRSKGLYNSLANLIPTSSTSNQIKSNTKYLLSNLDENYLKYIFAKTQTTDLNSFKAFIDENISKIDENDFTNFKNLSFFEQIAFRHALFLDTDDNSFKKALRLLKLDTIKTHSNGTQKRFINILIEKISKLTKSGIDLNFIDSKLVSSTRKDLAQNDTSIAKQEIQDSHSHCVDASIVFYLANSKIIKGQIEPDYDYFKDIYPKDSDIILPQSKQYLELNQKSQKSKKLFRDSVYSLVYEGKFDEKQKKILTQYELLKENGFVDTHKVFELIFKSFKDKDTIVLKDLKFLDNHLKSYIRKDIFSIFFNEKGELKEAKELKSATKNIDKFYTILSQNQDKIYTIKLDEKAKEKKTLQRNKVIELYKEIFYTKNAKPRARGKNRVTFSLPVYAKDAKYAIKRNSGFAGLKNKDIATKTYIDIDSREILKIPYYSTNVLPIRISDILEILSLQSKNAKQIYKIKIQDNLPKQIVSLDFILSQANRHEVLVSFDKSKLEIQNINDDNGENTFIQKYLCDDFKEFLGKPRDNKIEIIKNNDDILAIKYCVESTSKANKEIIVKALSDETPSA

SEQ ID NO: 10 - protein, 1247 aa, synthetic construct
KSLSINIDMGAINNGIFIATCQDDKIIDKNAFDIKFDKGKLNFSKIDRTLRRHTRRSFDRDRFVLRLLGEILPLENLSNNQKEKLFGLFKNRGFNYLNVNFNAEIDSDNLEILNALDRYYFKDCRVLSDFENSISKIFNELENNEILAFLDDQAQILNQAKEHKNKILNKNINAILEFLESIKNESFKNNKHRKSYLKDIKNEIENSFKDIILKLKIFKNSQELYYFIGNIANFQTRILRRYFNAKFDLVFDDAKLKKNILRNINYLDFISTDEKANKNKILENLNAFSTLEFLKNTDPIVTIPPYENAKNKKPQSCQALVINDEKITPSLKDIAHKILSNSNFECLKTDENGVLADNIKDNEIAKYLQRILDISKGILDDKELYPRLLEKDENAKIFAQEIRLNSVELKEFKDFAKKYYDEVNLAKKGIIKNELLKPCCLHTPHKNKNKNALISALFLKSITQKEIENLEDFFANNKISGNQTFKGFFERLSELKKRYQNRFFHILEHEPTKELEGILKNYKKVMEKIVEHNSNFSFKAPFDDSTISTNFNYLTQLGDIIFDEKSRGFAKTCKFHTLENLIRSSAKSAIASRLASNSARLINGKIEMYLDRLAHEIIKKIDFTDIYNVQINVEMNKFNFESNLSKLGLAKERQKDEESFICPYSGAKISQTNCEYDHILPRSKGLYNSLANLIPTSSTSNQIKSNTKYLLSNLDENYLKYIFAKTQTTDLNSFKAFIDENISKIDENDFTNFKNLSFFEQIAFRHALFLDTDDNSFKKALRLLKLDTIKTHSNGTQKRFINILIEKISKLTKSGIDLNFIDSKLVSSTRKDLAQNDTSIAKQEIQDSHSHCVDASIVFYLANSKIIKGQIEPDYDYFKDIYPKDSDIILPQSKQYLELNQKSQKSKKLFKDSVYSLVYEGKFDEKQKKILTQYELLKENGFVDTHKVFELIFKSFKDKDTIVLKDLKFLDNHLKSYIRKDIFSIFFNEKGELKEAKELKSATKNIDKFYTILSQNQDKIYTIKLDEKAKEKKTLQRNKVIELYKEIFYTKNAKPRARGKNRVTFSLPVYAKDAKYAIKRNSGFAGLKNKDIATKTYIDIDSREILKIPYYSTNVLPIRISDILEILSLQSKNAKQIYKIKIQDNLPKQIVSLDFILSQANRHEVLVSFDKSKLEIQNINDDNGENTFIQKYLCDDFKEFLGKPRDNKIEIIKNNDDILAIKYCVESTSKANKEIIVKALSDETPSA

SEQ ID NO: 11 - protein, 1247 aa, synthetic construct
KSLSINIDMGAINNGIFIATCQDDKIIDKNAFDIKFRKGKLNFSKIDRTLRRHTRRSFDRDRFVLRLLGEILPLENLSNNQKEKLFGLFKNRGFNYLNVNFNAEIDSDNLEILNALDRYYFKDCRVLSDFENSISKIFNELENNEILAFLDDQAQILNQAKEHKNKILNKNINAILEFLESIKNESFKNNKHRKSYLKDIKNEIENSFKDIILKLKIFKNSQELYYFIGNIANFQTRILRRYFNAKFDLVFDDAKLKKNILRNINYLDFISTDEKANKNKILENLNAFSTLEFLKNTDPIVTIPPYENAKNKKPQSCQALVINDEKITPSLKDIAHKILSNSNFECLKTDENGVLADNIKDNEIAKYLQRILDISKGILDDKELYPRLLEKDENAKIFAQEIRLNSVELKEFKDFAKKYYDEVNLAKKGIIKNELLKPCCLHTPHKNKNKNALISALFLKSITQKEIENLEDFFANNKISGNQTFKGFFERLSELKKRYQNRFFHILEHEPTKELEGILKNYKKVMEKIVEHNSNFSFKAPFDDSTISTNFNYLTQLGDIIFDEKSRGFAKTCKFHTLENLIRSSAKSAIASRLASNSARLINGKIEMYLDRLAHEIIKKIDFTDIYNVQINVEMNKFNFESNLSKLGLAKERQKDEESFICPYSGAKISQTNCEYDHILPRSKGLYNSLANLIPTSSTSNQIKSNTKYLLSNLDENYLKYIFAKTQTTDLNSFKAFIDENISKIDENDFTNFKNLSFFEQIAFRHALFLDTDDNSFKKALRLLKLDTIKTHSNGTQKRFINILIEKISKLTKSGIDLNFIDSKLVSSTRKDLAQNDTSIAKQEIQDSHSHCVDASIVFYLANSKIIKGQIEPDYDYFKDIYPKDSDIILPQSKQYLELNQKSQKSKKLFDRSVYSLVYEGKFDEKQKKILTQYELLKENGFVDTHKVFELIFKSFKDKDTIVLKDLKFLDNHLKSYIRKDIFSIFFNEKGELKEAKELKSATKNIDKFYTILSQNQDKIYTIKLDEKAKEKKTLQRNKVIELYKEIFYTKNAKPRARGKNRVTFSLPVYAKDAKYAIKRNSGFAGLKNKRIATKTYIDIDSREILKIPYYSTNVLPIRISDILEILSLQSKNAKQIYKIKIQDNLPKQIVSLDFILSQANRHEVLVSFDKSKLEIQNINDDNGENTFIQKYLCDDFKEFLGKPRDNKIEIIKNNDDILAIKYCVESTSKANKEIIVKALSDETPSA

SEQ ID NO: 12 - protein, 1247 aa, synthetic construct
KSLSINIDMGAINNGIFIATCQDDKIIDKNAFDIKFRKGKLNFSKIDRTLRRHTRRSFDRDRFVLRLLGEILPLENLSNNQKEKLFGLFKNRGFNYLNVNFNAEIDSDNLEILNALDRYYFKDCRVLSDFENSISKIFNELENNEILAFLDDQAQILNQAKEHKNKILNKNINAILEFLESIKNESFKNNKHRKSYLKDIKNEIENSFKDIILKLKIFKNSQELYYFIGNIANFQTRILRRYFNAKFDLVFDDAKLKKNILRNINYLDFISTDEKANKNKILENLNAFSTLEFLKNTDPIVTIPPYENAKNKKPQSCQALVINDEKITPSLKDIAHKILSNSNFECLKTDENGVLADNIKDNEIAKYLQRILDISKGILDDKELYPRLLEKDENAKIFAQEIRLNSVELKEFKDFAKKYYDEVNLAKKGIIKNELLKPCCLHTPHKNKNKNALISALFLKSITQKEIENLEDFFANNKISGNQTFKGFFERLSELKKRYQRRFFHILEHEPTKELEGILKNYKKVMEKIVEHNSNFSFKAPFDDSTISTNFNYLTQLGDIIFDEKSRGFAKTCKFHTLENLIRSSAKSAIASRLASNSARLINGKIEMYLDRLAHEIIKKIDFTDIYNVQINVEMNKFNFESNLSKLGLAKERQKDEESFICPYSGAKISQTNCEYDHILPRSKGLYNSLANLIPTSSTSNQIKSNTKYLLSNLDENYLKYIFAKTQTTDLNSFKAFIDENISKIDENDFTNFKNLSFFEQIAFRHALFLDTDDNSFKKALRLLKLDTIKTHSNGTQKRFINILIEKISKLTKSGIDLNFIDSKLVSSTRKDLAQNDTSIAKQEIQDSHSHCVDASIVFYLANSKIIKGQIEPDYDYFKDIYPKDSDIILPQSKQYLELNQKSQKSKKLFDRSVYSLVYEGKFDEKQKKILTQYELLKENGFVDTHKVFELIFKSFKDKDTIVLKDLKFLDNHLKSYIRKDIFSIFFNEKGELKEAKELKSATKNIDKFYTILSQNQDKIYTIKLDEKAKEKKTLQRNKVIELYKEIFYTKNAKPRARGKNRVTFSLPVYAKDAKYAIKRNSGFAGLKNKDIATKTYIDIDSREILKIPYYSTNVLPIRISDILEILSLQSKNAKQIYKIKIQDNLPKQIVSLDFILSQANRHEVLVSFDKSKLEIQNINDDNGENTFIQKYLCDDFKEFLGKPRDNKIEIIKNNDDILAIKYCVESTSKANKEIIVKALSDETPSA

SEQ ID NO: 13 - protein, 1247 aa, synthetic construct
KSLSINIDMGAINNGIFIATCQDDKIIDKNAFDIKFRKGKLNFSKIDRTLRRHTRRSFDRDRFVLRLLGEILPLENLSNNQKEKLFGLFKNRGFNYLNVNFNAEIDSDNLEILNALDRYYFKDCRVLSDFENSISKIFNELENNEILAFLDDQAQILNQAKEHKNKILNKNINAILEFLESIKNESFKNNKHRKSYLKDIKNEIENSFKDIILKLKIFKNSQELYYFIGNIANFQTRILRRYFNAKFDLVFDDAKLKKNILRNINYLDFISTDEKANKNKILENLNAFSTLEFLKNTDPIVTIPPYENAKNKKPQSCQALVINDEKITPSLKDIAHKILSNSNFECLKTDENGVLADNIKDNEIAKYLQRILDISKGILDDKELYPRLLEKDENAKIFAQEIRLNSVELKEFKDFAKKYYDEVNLAKKGIIKNELLKPCCLHTPHKNKNKNALISALFLKSITQKEIENLEDFFANNKISGNQTFKGFFERLSELKKRYQNRFFHILEHEPTKELEGILKNYKKVMEKIVEHNSNFSFKAPFDDSTISTNFNYLTQLGDIIFDEKSRGFAKTCKFHTLENLIRSSAKSAIASRLASNSARLINGKIEMYLDRLAHEIIKKIDFTDIYNVQINVEMNKFNFESNLSKLGLAKERQKDEESFICPYSGAKISQTNCEYDHILPRSKGLYNSLANLIPTSSTSNQIKSNTKYLLSNLDENYLKYIFAKTQTTDLNSFKAFIDENISKIDENDFTNFKNLSFFEQIAFRHALFLDTDDNSFKKALRLLKLDTIKTHSNGTQKRFINILIEKISKLTKSGIDLNFIDSKLVSSTRKDLAQNDTSIAKQEIQDSHSHCVDASIVFYLANSKIIKGQIEPDYDYFKDIYPKDSDIILPQSKQYLELNQKSQKSKKLFDRSVYSLVYEGKFDEKQKKILTQYELLKENGFVDTHKVFELIFKSFKDKDTIVLKDLKFLDNHLKSYIRKDIFSIFFNEKGELKEAKELKSATKNIDKFYTILSQNQDKIYTIKLDEKAKEKKTLQRNKVIELYKEIFYTKNAKPRARGKNRVTFSLPVYAKDAKYAIKRNSGFAGLKNKSIATKTYIDIDSREILKIPYYSTNVLPIRISDILEILSLQSKNAKQIYKIKIQDNLPKQIVSLDFILSQARRHEVLVSFDKSKLEIQNINDDNGENTFIQKYLCDDFKEFLGKPRDNKIEIIKNNDDILAIKYCVESTRKANKEIIVKALSDETPSA

SEQ ID NO: 14 - protein, 1247 aa, synthetic construct
KSLSINIDMGAINNGIFIATCQDDKIIDKNAFDIKFDKRKLNFSKIDRTLRRHTRRSFDRDRFVLRLLGEILPLENLSNNQKEKLFGLFKNRGFNYLNVNFNAEIDSDNLEILNALDRYYFKDCRVLSDFENSISKIFNELENNEILAFLDDQAQILNQAKEHKNKILNKNINAILEFLESIKNESFKNNKHRKSYLKDIKNEIENSFKDIILKLKIFKNSQELYYFIGNIANFQTRILRRYFNAKFDLVFDDAKLKKNILRNINYLDFISTDEKANKNKILENLNAFSTLEFLKNTDPIVTIPPYENAKNKKPQSCQALVINDEKITPSLKDIAHKILSNSNFECLKTDENGVLADNIKDNEIAKYLQRILDISKGILDDKELYPRLLEKDENAKIFAQEIRLNSVELKEFKDFAKKYYDEVNLAKKGIIKNELLKPCCLHTPHKNKNKNALISALFLKSITQKEIENLEDFFANNKISGNQTFKGFFERLSELKKRYQNRFFHILEHEPTKELEGILKNYKKVMEKIVEHNSNFSFKAPFDDSTISTNFNYLTQLGDIIFDEKSRGFAKTCKFHTLENLIRSSAKSAIASRLASNSARLINGKIEMYLDRLAHEIIKKIDFTDIYNVQINVEMNKFNFESNLSKLGLAKERQKDEESFICPYSGAKISQTNCEYDHILPRSKGLYNSLANLIPTSSTSNQIKSNTKYLLSNLDENYLKYIFAKTQTTDLNSFKAFIDENISKIDENDFTNFKNLSFFEQIAFRHALFLDTDDNSFKKALRLLKLDTIKTHSNGTQKRFINILIEKISKLTKSGIDLNFIDSKLVSSTRKDLAQNDTSIAKQEIQDSHSHCVDASIVFYLANSKIIKGQIEPDYDYFKDIYPKDSDIILPQSKQYLELNQKSQKSKKLFDDSVYSLVYEGKFDEKQKKILTQYELLKENGFVDTHKVFELIFKSFKDKDTIVLKDLKFLDNHLKSYIRKDIFSIFFNEKGELKEAKELKSATKNIDKFYTILSQNQDKIYTIKLDEKAKEKKTLQRNKVIELYKEIFYTKNAKPRARGKNRVTFSLPVYAKDAKYAIKRNSGFAGLKNKDIATKTYIDIDSREILKIPYYSTNVLPIRISDILEILSLQSKNAKQIYKIKIQDNLPKQIVSLDFILSQANRHEVLVSFDKSKLEIQNINDDNGENTFIQKYLCDDFKEFLGKPRDNKIEIIKNNDDILAIKYCVESTSKANKEIIVKALSDETPSA

SEQ ID NO: 15 - protein, 1247 aa, synthetic construct
KSLSINIDMGAINNGIFIATCQDDKIIDKNAFDIKFDKGKLNFSKIDRTLRRHTRRSFDRDRFVLRLLGEILPLENLSNNQKEKLFGLFKNRGFNYLNVNFNAEIDSDNLEILNALDRYYFKDCRVLSDFENSISKIFNELENNEILAFLDDQAQILNQAKEHKNKILNKNINAILEFLESIKNESFKNNKHRKSYLKDIKNEIENSFKDIILKLKIFKNSQELYYFIGNIANFQTRILRRYFNAKFDLVFDDAKLKKNILRNINYLDFISTDEKANKNKILENLNAFSTLEFLKNTDPIVTIPPYENAKNKKPQSCQALVINDEKITPSLKDIAHKILSNSNFECLKTDENGVLADNIKDNEIAKYLQRILDISKGILDDKELYPRLLEKDENAKIFAQEIRLNSVELKEFKDFAKKYYDEVNLAKKGIIKNELLKPCCLHTPHKNKNKNALISALFLKSITQKEIENLEDFFANNKISGNQTFKGFFERLSELKKRYQNRFFHILEHEPTKELEGILKNYKKVMEKIVEHNSNFSFKAPFDDSTISTNFNYLTQLGDIIFDEKSRGFAKTCKFHTLENLIRSSAKSAIASRLASNSARLINGKIEMYLDRLAHEIIKKIDFTDIYNVQINVEMNKFNFESNLSKLGLAKERQKDEESFICPYSGAKISQTNCEYDHILPRSKGLYNSLANLIPTSSTSNQIKSNTKYLLSNLDENYLKYIFAKTQTTDLNSFKAFIDENISKIDENDFTNFKNLSFFEQIAFRHALFLDTDDNSFKKALRLLKLDTIKTHSNGTQKRFINILIEKISKLTKSGIDLNFIDSKLVSSTRKDLAQNDTSIAKQEIQDSHSHCVDASIVFYLANSKIIKGQIEPDYDYFKDIYPKDSDIILPQSKQYLELNQKSQKSKKLFDRSVYSLVYEGKFDEKQKKILTQYELLKENGFVDTHKVFELIFKSFKDKDTIVLKDLKFLDNHLKSYIRKDIFSIFFNEKGELKEAKELKSATKNIDKFYTILSQNQDKIYTIKLDEKAKEKKTLQRNKVIELYKEIFYTKNAKPRARGKNRVTFSLPVYAKDAKYAIKRNSGFAGLKNKDIATKTYIDIDSREILKIPYYSTNVLPIRISDILEILSLQSKNAKQIYKIKIQDNLPKQIVSLDFILSQANRHEVLVSFDKSKLEIQNINDDNGENTFIQKYLCDDFKEFLGKPRDNKIEIIKNNDDILAIKYCVESTSKANKEIIVKALSDETPSA

SEQ ID NO: 16 - protein, 1247 aa, synthetic construct
KSLSINIDMGAINNGIFIATCQDDKIIDKNAFDIKFDKGKLNFSKIDRTLRRHTRRSFDRDRFVLRLLGEILPLENLSNNQKEKLFGLFKNRGFNYLNVNFNAEIDSDNLEILNALDRYYFKDCRVLSDFENSISKIFNELENNEILAFLDDQAQILNQAKEHKNKILNKNINAILEFLESIKNESFKNNKHRKSYLKDIKNEIENSFKDIILKLKIFKNSQELYYFIGNIANFQTRILRRYFNAKFDLVFDDAKLKKNILRNINYLDFISTDEKANKNKILENLNAFSTLEFLKNTDPIVTIPPYENAKNKKPQSCQALVINDEKITPSLKDIAHKILSNSNFECLKTDENGVLADNIKDNEIAKYLQRILDISKGILDDKELYPRLLEKDENAKIFAQEIRLNSVELKEFKDFAKKYYDEVNLAKKGIIKNELLKPCCLHTPHKNKNKNALISALFLKSITQKEIENLEDFFANNKISGNQTFKGFFERLSELKKRYQNRFFHILEHEPTKELEGILKNYKKVMEKIVEHNSNFSFKAPFDDSTISTNFNYLTQLGDIIFDEKSRGFAKTCKFHTLENLIRSSAKSAIASRLASNSARLINGKIEMYLDRLAHEIIKKIDFTDIYNVQINVEMNKFNFESNLSKLGLAKERQKDEESFICPYSGAKISQTNCEYDHILPRSKGLYNSLANLIPTSSTSNQIKSNTKYLLSNLDENYLKYIFAKTQTTDLNSFKAFIDENISKIDENDFTNFKNLSFFEQIAFRHALFLDTDDNSFKKALRLLKLDTIKTHSNGTQKRFINILIEKISKLTKSGIDLNFIDSKLVSSTRKDLAQNDTSIAKQEIQDSHSHCVDASIVFYLANSKIIKGQIEPDYDYFKDIYPKDSDIILPQSKQYLELNQKSQKSKKLFDDSVYSLVYEGKFDEKQKKILTQYELLKENGFVDTHKVFELIFKSFKDKDTIVLKDLKFLDNHLKSYRRKDIFSIFFNEKGELKEAKELKSATKNIDKFYTILSQNQDKIYTIKLDEKAKEKKTLQRNKVIELYKEIFYTKNAKPRARGKNRVTFSLPVYAKDAKYAIKRNSGFAGLKNKDIATKTYIDIDSREILKIPYYSTNVLPIRISDILEILSLQSKNAKQIYKIKIQDNLPKQIVSLDFILSQANRHEVLVSFDKSKLEIQNINDDNGENTFIQKYLCDDFKEFLGKPRDNKIEIIKNNDDILAIKYCVESTSKANKEIIVKALSDETPSA

SEQ ID NO: 17 - protein, 1247 aa, synthetic construct
KSLSINIDMGAINNGIFIATCQDDKIIDKNAFDIKFDKGKLNFSKIDRTLRRHTRRSFDRDRFVLRLLGEILPLENLSNNQKEKLFGLFKNRGFNYLNVNFNAEIDSDNLEILNALDRYYFKDCRVLSDFENSISKIFNELENNEILAFLDDQAQILNQAKEHKNKILNKNINAILEFLESIKNESFKNNKHRKSYLKDIKNEIENSFKDIILKLKIFKNSQELYYFIGNIANFQTRILRRYFNAKFDLVFDDAKLKKNILRNINYLDFISTDEKANKNKILENLNAFSTLEFLKNTDPIVTIPPYENAKNKKPQSCQALVINDEKITPSLKDIAHKILSNSNFECLKTDENGVLADNIKDNEIAKYLQRILDISKGILDDKELYPRLLEKDENAKIFAQEIRLNSVELKEFKDFAKKYYDEVNLAKKGIIKNELLKPCCLHTPHKNKNKNALISALFLKSITQKEIENLEDFFANNKISGNQTFKGFFERLSELKKRYQNRFFHILEHEPTKELEGILKNYKKVMEKIVEHNSNFSFKAPFDDSTISTNFNYLTQLGDIIFDEKSRGFAKTCKFHTLENLIRSSAKSAIASRLASNSARLINGKIEMYLDRLAHEIIKKIDFTDIYNVQINVEMNKFNFESNLSKLGLAKERQKDEESFICPYSGAKISQTNCEYDHILPRSKGLYNSLANLIPTSSTSNQIKSNTKYLLSNLDENYLKYIFAKTQTTDLNSFKAFIDENISKIDENDFTNFKNLSFFEQIAFRHALFLDTDDNSFKKALRLLKLDTIKTHSNGTQKRFINILIEKISKLTKSGIDLNFIDSKLVSSTRKDLAQNDTSIAKQEIQDSHSHCVDASIVFYLANSKIIKGQIEPDYDYFKDIYPKDSDIILPQSKQYLELNQKSQKSKKLFDDSVYSLVYEGKFDEKQKKILTQYELLKENGFVDTHKVFELIFKSFKDKDTIVLKDLKFLDNHLKSYIRKDIFSIFFNEKGELKEAKELKSATKNIDKFYTILSQNQDKIYTIKLDEKAKEKKTLQRNKVIELYKEIFYTKNAKPRARGKNRVTFSLPVYAKDAKYAIKRNSGFAGLKNKDIATKTYIDIDSREILKIPYYSTNVLPIRISDILEILSLQSKNAKQIYKIKIQDNLPKQIVSLDFILSQARRHEVLVSFDKSKLEIQNINDDNGENTFIQKYLCDDFKEFLGKPRDNKIEIIKNNDDILAIKYCVESTSKANKEIIVKALSDETPSA

SEQ ID NO: 18 - protein, 1247 aa, synthetic construct
KSLSINIDMGAINNGIFIATCQDDKIIDKNAFDIKFDKGKLNFSKIDRTLRRHTRRSFDRDRFVLRLLGEILPLENLSNNQKEKLFGLFKNRGFNYLNVNFNAEIDSDNLEILNALDRYYFKDCRVLSDFENSISKIFNELENNEILAFLDDQAQILNQAKEHKNKILNKNINAILEFLESIKNESFKNNKHRKSYLKDIKNEIENSFKDIILKLKIFKNSQELYYFIGNIANFQTRILRRYFNAKFDLVFDDAKLKKNILRNINYLDFISTDEKANKNKILENLNAFSTLEFLKNTDPIVTIPPYENAKNKKPQSCQALVINDEKITPSLKDIAHKILSNSNFECLKTDENGVLADNIKDNEIAKYLQRILDISKGILDDKELYPRLLEKDENAKIFAQEIRLNSVELKEFKDFAKKYYDEVNLAKKGIIKNELLKPCCLHTPHKNKNKNALISALFLKSITQKEIENLEDFFANNKISGNQTFKGFFERLSELKKRYQNRFFHILEHEPTKELEGILKNYKKVMEKIVEHNSNFSFKAPFDDSTISTNFNYLTQLGDIIFDEKSRGFAKTCKFHTLENLIRSSAKSAIASRLASNSARLINGKIEMYLDRLAHEIIKKIDFTDIYNVQINVEMNKFNFESNLSKLGLAKERQKDEESFICPYSGAKISQTNCEYDHILPRSKGLYNSLANLIPTSSTSNQIKSNTKYLLSNLDENYLKYIFAKTQTTDLNSFKAFIDENISKIDENDFTNFKNLSFFEQIAFRHALFLDTDDNSFKKALRLLKLDTIKTHSNGTQKRFINILIEKISKLTKSGIDLNFIDSKLVSSTRKDLAQNDTSIAKQEIQDSHSHCVDASIVFYLANSKIIKGQIEPDYDYFKDIYPKDSDIILPQSKQYLELNQKSQKSKKLFDDSVYSLVYEGKFDEKQKKILTQYELLKENGFVDTHKVFELIFKSFKDKDTIVLKDLKFLDNHLKSYIRKDIFSIFFNEKGELKEAKELKSATKNIDKFYTILSQNQDKIYTIKLDEKAKEKKTLQRNKVIELYKEIFYTKNAKPRARGKNRVTFSLPVYAKDAKYAIKRNSGFAGLKNKDIATKTYIDIDSREILKIPYYSTNVLPIRISDILEILSLQSKNAKQIYKIKIQDNLPKQIVSLDFILSQANRHEVLVSFDKSKLEIQNINDDNGENTFIQKYLCDDFKEFLGKPRDNKIEIIKNNDDILAIKYCVESTRKANKEIIVKALSDETPSA

SEQ ID NO: 19 - protein, 1247 aa, synthetic construct
KSLSINIDMGAINNGIFIATCQDDKIIDKNAFDIKFDKGKLNFSKIDRTLRRHTRRSFDRDRFVLRLLGEILPLENLSNNQKEKLFGLFKNRGFNYLNVNFNAEIDSDNLEILNALDRYYFKDCRVLSDFENSISKIFNELENNEILAFLDDQAQILNQAKEHKNKILNKNINAILEFLESIKNESFKNNKHRKSYLKDIKNEIENSFKDIILKLKIFKNSQELYYFIGNIANFQTRILRRYFNAKFDLVFDDAKLKKNILRNINYLDFISTDEKANKNKILENLNAFSTLEFLKNTDPIVTIPPYENAKNKKPQSCQALVINDEKITPSLKDIAHKILSNSNFECLKTDENGVLADNIKDNEIAKYLQRILDISKGILDDKELYPRLLEKDENAKIFAQEIRLNSVELKEFKDFAKKYYDEVNLAKKGIIKNELLKPCCLHTPHKNKNKNALISALFLKSITQKEIENLEDFFANNKISGNQTFKGFFERLSELKKRYQNRFFHILEHEPTKELEGILKNYKKVMEKIVEHNSNFSFKAPFDDSTISTNFNYLTQLGDIIFDEKSRGFAKTCKFHTLENLIRSSAKSAIASRLASNSARLINGKIEMYLDRLAHEIIKKIDFTDIYNVQINVEMNKFNFESNLSKLGLAKERQKDEESFICPYSGAKISQTNCEYDHILPRSKGLYNSLANLIPTSSTSNQIKSNTKYLLSNLDENYLKYIFAKTQTTDLNSFKAFIDENISKIDENDFTNFKNLSFFEQIAFRHALFLDTDDNSFKKALRLLKLDTIKTHSNGTQKRFINILIEKISKLTKSGIDLNFIDSKLVSSTRKDLAQNDTSIAKQEIQDSHSHCVDASIVFYLANSKIIKGQIEPDYDYFKDIYPKDSDIILPQSKQYLELNQKSQKSKKLFDRSVYSLVYEGKFDEKQKKILTQYELLKENGFVDTHKVFELIFKSFKDKDTIVLKDLKFLDNHLKSYIRKDIFSIFFNEKGELKEAKELKSATKNIDKFYTILSQNQDKIYTIKLDEKAKEKKTLQRNKVIELYKEIFYTKNAKPRARGKNRVTFSLPVYAKDAKYAIKRNSGFAGLKNKRIATKTYIDIDSREILKIPYYSTNVLPIRISDILEILSLQSKNAKQIYKIKIQDNLPKQIVSLDFILSQANRHEVLVSFDKSKLEIQNINDDNGENTFIQKYLCDDFKEFLGKPRDNKIEIIKNNDDILAIKYCVESTSKANKEIIVKALSDETPSA

SEQ ID NO: 20 - protein, 1247 aa, synthetic construct
KSLSINIDMGAINNGIFIATCQDDKIIDKNAFDIKFRKGKLNFSKIDRTLRRHTRRSFDRDRFVLRLLGEILPLENLSNNQKEKLFGLFKNRGFNYLNVNFNAEIDSDNLEILNALDRYYFKDCRVLSDFENSISKIFNELENNEILAFLDDQAQILNQAKEHKNKILNKNINAILEFLESIKNESFKNNKHRKSYLKDIKNEIENSFKDIILKLKIFKNSQELYYFIGNIANFQTRILRRYFNAKFDLVFDDAKLKKNILRNINYLDFISTDEKANKNKILENLNAFSTLEFLKNTDPIVTIPPYENAKNKKPQSCQALVINDEKITPSLKDIAHKILSNSNFECLKTDENGVLADNIKDNEIAKYLQRILDISKGILDDKELYPRLLEKDENAKIFAQEIRLNSVELKEFKDFAKKYYDEVNLAKKGIIKNELLKPCCLHTPHKNKNKNALISALFLKSITQKEIENLEDFFANNKISGNQTFKGFFERLSELKKRYQNRFFHILEHEPTKELEGILKNYKKVMEKIVEHNSNFSFKAPFDDSTISTNFNYLTQLGDIIFDEKSRGFAKTCKFHTLENLIRSSAKSAIASRLASNSARLINGKIEMYLDRLAHEIIKKIDFTDIYNVQINVEMNKFNFESNLSKLGLAKERQKDEESFICPYSGAKISQTNCEYDHILPRSKGLYNSLANLIPTSSTSNQIKSNTKYLLSNLDENYLKYIFAKTQTTDLNSFKAFIDENISKIDENDFTNFKNLSFFEQIAFRHALFLDTDDNSFKKALRLLKLDTIKTHSNGTQKRFINILIEKISKLTKSGIDLNFIDSKLVSSTRKDLAQNDTSIAKQEIQDSHSHCVDASIVFYLANSKIIKGQIEPDYDYFKDIYPKDSDIILPQSKQYLELNQKSQKSKKLFDDSVYSLVYEGKFDEKQKKILTQYELLKENGFVDTHKVFELIFKSFKDKDTIVLKDLKFLDNHLKSYIRKDIFSIFFNEKGELKEAKELKSATKNIDKFYTILSQNQDKIYTIKLDEKAKEKKTLQRNKVIELYKEIFYTKNAKPRARGKNRVTFSLPVYAKDAKYAIKRNSGFAGLKNKRIATKTYIDIDSREILKIPYYSTNVLPIRISDILEILSLQSKNAKQIYKIKIQDNLPKQIVSLDFILSQANRHEVLVSFDKSKLEIQNINDDNGENTFIQKYLCDDFKEFLGKPRDNKIEIIKNNDDILAIKYCVESTRKANKEIIVKALSDETPSA

SEQ ID NO: 21 - protein, 1247 aa, synthetic construct; identical to SEQ ID NO: 20

SEQ ID NO: 22 - protein, 1247 aa, synthetic construct
KSLSINIDMGAINNGIFIATCQDDKIIDKNAFDIKFRKRKLNFSKIDRTLRRHTRRSFDRDRFVLRLLGEILPLENLSNNQKEKLFGLFKNRGFNYLNVNFNAEIDSDNLEILNALDRYYFKDCRVLSDFENSISKIFNELENNEILAFLDDQAQILNQAKEHKNKILNKNINAILEFLESIKNESFKNNKHRKSYLKDIKNEIENSFKDIILKLKIFKNSQELYYFIGNIANFQTRILRRYFNAKFDLVFDDAKLKKNILRNINYLDFISTDEKANKNKILENLNAFSTLEFLKNTDPIVTIPPYENAKNKKPQSCQALVINDEKITPSLKDIAHKILSNSNFECLKTDENGVLADNIKDNEIAKYLQRILDISKGILDDKELYPRLLEKDENAKIFAQEIRLNSVELKEFKDFAKKYYDEVNLAKKGIIKNELLKPCCLHTPHKNKNKNALISALFLKSITQKEIENLEDFFANNKISGNQTFKGFFERLSELKKRYQNRFFHILEHEPTKELEGILKNYKKVMEKIVEHNSNFSFKAPFDDSTISTNFNYLTQLGDIIFDEKSRGFAKTCKFHTLENLIRSSAKSAIASRLASNSARLINGKIEMYLDRLAHEIIKKIDFTDIYNVQINVEMNKFNFESNLSKLGLAKERQKDEESFICPYSGAKISQTNCEYDHILPRSKGLYNSLANLIPTSSTSNQIKSNTKYLLSNLDENYLKYIFAKTQTTDLNSFKAFIDENISKIDENDFTNFKNLSFFEQIAFRHALFLDTDDNSFKKALRLLKLDTIKTHSNGTQKRFINILIEKISKLTKSGIDLNFIDSKLVSSTRKDLAQNDTSIAKQEIQDSHSHCVDASIVFYLANSKIIKGQIEPDYDYFKDIYPKDSDIILPQSKQYLELNQKSQKSKKLFDDSVYSLVYEGKFDEKQKKILTQYELLKENGFVDTHKVFELIFKSFKDKDTIVLKDLKFLDNHLKSYIRKDIFSIFFNEKGELKEAKELKSATKNIDKFYTILSQNQDKIYTIKLDEKAKEKKTLQRNKVIELYKEIFYTKNAKPRARGKNRVTFSLPVYAKDAKYAIKRNSGFAGLKNKRIATKTYIDIDSREILKIPYYSTNVLPIRISDILEILSLQSKNAKQIYKIKIQDNLPKQIVSLDFILSQANRHEVLVSFDKSKLEIQNINDDNGENTFIQKYLCDDFKEFLGKPRDNKIEIIKNNDDILAIKYCVESTSKANKEIIVKALSDETPSA

SEQ ID NO: 23 - protein, 1247 aa, synthetic construct
KSLSINIDMGAINNGIFIATCQDDKIIDKNAFDIKFDKGKLNFSKIDRTLRRHTRRSFDRDRFVLRLLGEILPLENLSNNQKEKLFGLFKNRGFNYLNVNFNAEIDSDNLEILNALDRYYFKDCRVLSDFENSISKIFNELENNEILAFLDDQAQILNQAKEHKNKILNKNINAILEFLESIKNESFKNNKHRKSYLKDIKNEIENSFKDIILKLKIFKNSQELYYFIGNIANFQTRILRRYFNAKFDLVFDDAKLKKNILRNINYLDFISTDEKANKNKILENLNAFSTLEFLKNTDPIVTIPPYENAKNKKPQSCQALVINDEKITPSLKDIAHKILSNSNFECLKTDENGVLADNIKDNEIAKYLQRILDISKGILDDKELYPRLLEKDENAKIFAQEIRLNSVELKEFKDFAKKYYDEVNLAKKGIIKNELLKPCCLHTPHKNKNKNALISALFLKSITQKEIENLEDFFANNKISGNQTFKGFFERLSELKKRYQNRFFHILEHEPTKELEGILKNYKKVMEKIVEHNSNFSFKAPFDDSTISTNFNYLTQLGDIIFDEKSRGFAKTCKFHTLENLIRSSAKSAIASRLASNSARLINGKIEMYLDRLAHEIIKKIDFTDIYNVQINVEMNKFNFESNLSKLGLAKERQKDEESFICPYSGAKISQTNCEYDHILPRSKGLYNSLANLIPTSSTSNQIKSNTKYLLSNLDENYLKYIFAKTQTTDLNSFKAFIDENISKIDENDFTNFKNLSFFEQIAFRHALFLDTDDNSFKKALRLLKLDTIKTHSNGTQKRFINILIEKISKLTKSGIDLNFIDSKLVSSTRKDLAQNDTSIAKQEIQDSHSHCVDASIVFYLANSKIIKGQIEPDYDYFKDIYPKDSDIILPQSKQYLELNQKSQKSKKLFDRSVYSLVYEGKFDEKQKKILTQYELLKENGFVDTHKVFELIFKSFKDKDTIVLKDLKFLDNHLKSYIRKDIFSIFFNEKGELKEAKELKSATKNIDKFYTILSQNQDKIYTIKLDEKAKEKKTLQRNKVIELYKEIFYTKNAKPRARGKNRVTFSLPVYAKDAKYAIKRNSGFAGLKNKRIATKTYIDIDSREILKIPYYSTNVLPIRISDILEILSLQSKNAKQIYKIKIQDNLPKQIVSLDFILSQARRHEVLVSFDKSKLEIQNINDDNGENTFIQKYLCDDFKEFLGKPRDNKIEIIKNNDDILAIKYCVESTSKANKEIIVKALSDETPSA

SEQ ID NO: 24 - protein, 1247 aa, synthetic construct
KSLSINIDMGAINNGIFIATCQDDKIIDKNAFDIKFRKGKLNFSKIRRTLRRHTRRSFDRDRFVLRLLGEILPLENLSNNQKEKLFGLFKNRGFNYLNVNFNAEIDSDNLEILNALDRYYFKDCRVLSDFENSISKIFNELENNEILAFLDDQAQILNQAKEHKNKILNKNINAILEFLESIKNESFKNNKHRKSYLKDIKNEIENSFKDIILKLKIFKNSQELYYFIGNIANFQTRILRRYFNAKFDLVFDDAKLKKNILRNINYLDFISTDEKANKNKILENLNAFSTLEFLKNTDPIVTIPPYENAKNKKPQSCQALVINDEKITPSLKDIAHKILSNSNFECLKTDENGVLADNIKDNEIAKYLQRILDISKGILDDKELYPRLLEKDENAKIFAQEIRLNSVELKEFKDFAKKYYDEVNLAKKGIIKNELLKPCCLHTPHKNKNKNALISALFLKSITQKEIENLEDFFANNKISGNQTFKGFFERLSELKKRYQNRFFHILEHEPTKELEGILKNYKKVMEKIVEHNSNFSFKAPFDDSTISTNFNYLTQLGDIIFDEKSRGFAKTCKFHTLENLIRSSAKSAIASRLASNSARLINGKIEMYLDRLAHEIIKKIDFTDIYNVQINVEMNKFNFESNLSKLGLAKERQKDEESFICPYSGAKISQTNCEYDHILPRSKGLYNSLANLIPTSSTSNQIKSNTKYLLSNLDENYLKYIFAKTQTTDLNSFKAFIDENISKIDENDFTNFKNLSFFEQIAFRHALFLDTDDNSFKKALRLLKLDTIKTHSNGTQKRFINILIEKISKLTKSGIDLNFIDSKLVSSTRKDLAQNDTSIAKQEIQDSHSHCVDASIVFYLANSKIIKGQIEPDYDYFKDIYPKDSDIILPQSKQYLELNQKSQKSKKLFDRSVYSLVYEGKFDEKQKKILTQYELLKENGFVDTHKVFELIFKSFKDKDTIVLKDLKFLDNHLKSYIRKDIFSIFFNEKGELKEAKELKSATKNIDKFYTILSQNQDKIYTIKLDEKAKEKKTLQRNKVIELYKEIFYTKNAKPRARGKNRVTFSLPVYAKDAKYAIKRNSGFAGLKNKDIATKTYIDIDSREILKIPYYSTNVLPIRISDILEILSLQSKNAKQIYKIKIQDNLPKQIVSLDFILSQANRHEVLVSFDKSKLEIQNINDDNGENTFIQKYLCDDFKEFLGKPRDNKIEIIKNNDDILAIKYCVESTSKANKEIIVKALSDETPSA

SEQ ID NO: 25 - protein, 1247 aa, synthetic construct
KSLSINIDMGAINNGIFIATCQDDKIIDKNAFDIKFRKGKLNFSKIDRTLRRHTRRLFDRDRFVLRLLGEILPLENLSNNQKEKLFGLFKNRGFNYLNVNFNAEIDSDNLEILNALDRYYFKDCRVLSDFENSISKIFNELENNEILAFLDDQAQILNQAKEHKNKILNKNINAILEFLESIKNESFKNNKHRKSYLKDIKNEIENSFKDIILKLKIFKNSQELYYFIGNIANFQTRILRRYFNAKFDLVFDDAKLKKNILRNINYLDFISTDEKANKNKILENLNAFSTLEFLKNTDPIVTIPPYENAKNKKPQSCQALVINDEKITPSLKDIAHKILSNSNFECLKTDENGVLADNIKDNEIAKYLQRILDISKGILDDKELYPRLLEKDENAKIFAQEIRLNSVELKEFKDFAKKYYDEVNLAKKGIIKNELLKPCCLHTPHKNKNKNALISALFLKSITQKEIENLEDFFANNKISGNQTFKGFFERLSELKKRYQNRFFHILEHEPTKELEGILKNYKKVMEKIVEHNSNFSFKAPFDDSTISTNFNYLTQLGDIIFDEKSRGFAKTCKFHTLENLIRSSAKSAIASRLASNSARLINGKIEMYLDRLAHEIIKKIDFTDIYNVQINVEMNKFNFESNLSKLGLAKERQKDEESFICPYSGAKISQTNCEYDHILPRSKGLYNSLANLIPTSSTSNQIKSNTKYLLSNLDENYLKYIFAKTQTTDLNSFKAFIDENISKIDENDFTNFKNLSFFEQIAFRHALFLDTDDNSFKKALRLLKLDTIKTHSNGTQKRFINILIEKISKLTKSGIDLNFIDSKLVSSTRKDLAQNDTSIAKQEIQDSHSHCVDASIVFYLANSKIIKGQIEPDYDYFKDIYPKDSDIILPQSKQYLELNQKSQKSKKLFDRSVYSLVYEGKFDEKQKKILTQYELLKENGFVDTHKVFELIFKSFKDKDTIVLKDLKFLDNHLKSYIRKDIFSIFFNEKGELKEAKELKSATKNIDKFYTILSQNQDKIYTIKLDEKAKEKKTLQRNKVIELYKEIFYTKNAKPRARGKNRVTFSLPVYAKDAKYAIKRNSGFAGLKNKDIATKTYIDIDSREILKIPYYSTNVLPIRISDILEILSLQSKNAKQIYKIKIQDNLPKQIVSLDFILSQANRHEVLVSFDKSKLEIQNINDDNGENTFIQKYLCDDFKEFLGKPRDNKIEIIKNNDDILAIKYCVESTSKANKEIIVKALSDETPSA

SEQ ID NO: 26 - protein, 1247 aa, synthetic construct
KSLSINIDMGAINNGIFIATCQDDKIIDKNAFDIKFRKGKLNFSKIDRTLRRHTRRSFDRDRFVLRLLGEILPLENLSNNQKEKLFGLFKNRGFNYLNVNFNAEIDSDNLEILNALDRYYFKDCRVLSDFENSISKIFNELENNEILAFLDDQAQILNQAKEHKNKILNKNINAILEFLESIKNESFKNNKHRKSYLKDIKNEIENSFKDIILKLKIFKNSQELYYFIGNIANFQTRILRRYFNAKFDLVFDDAKLKKNILRNINYLDFISTDEKANKNKILENLNAFSTLEFLKNTDPIVTIPPYENAKNKKPQSCQALVINDEKITPSLKDIAHKILSNSNFECLKTDENGVLADNIKDNEIAKYLQRILDISKGILDDKELYPRLLEKDENAKIFAQEIRLNSVELKEFKDFAKKYYDEVNLAKKGIIKNELLKPCCLHTPHKNKNKNALISALFLKSITQKEIENLEDFFANNKISGNQTFKGFFERLSELKKRYQFRFFHILEHEPTKELEGILKNYKKVMEKIVEHNSNFSFKAPFDDSTISTNFNYLTQLGDIIFDEKSRGFAKTCKFHTLENLIRSSAKSAIASRLASNSARLINGKIEMYLDRLAHEIIKKIDFTDIYNVQINVEMNKFNFESNLSKLGLAKERQKDEESFICPYSGAKISQTNCEYDHILPRSKGLYNSLANLIPTSSTSNQIKSNTKYLLSNLDENYLKYIFAKTQTTDLNSFKAFIDENISKIDENDFTNFKNLSFFEQIAFRHALFLDTDDNSFKKALRLLKLDTIKTHSNGTQKRFINILIEKISKLTKSGIDLNFIDSKLVSSTRKDLAQNDTSIAKQEIQDSHSHCVDASIVFYLANSKIIKGQIEPDYDYFKDIYPKDSDIILPQSKQYLELNQKSQKSKKLFDRSVYSLVYEGKFDEKQKKILTQYELLKENGFVDTHKVFELIFKSFKDKDTIVLKDLKFLDNHLKSYIRKDIFSIFFNEKGELKEAKELKSATKNIDKFYTILSQNQDKIYTIKLDEKAKEKKTLQRNKVIELYKEIFYTKNAKPRARGKNRVTFSLPVYAKDAKYAIKRNSGFAGLKNKDIATKTYIDIDSREILKIPYYSTNVLPIRISDILEILSLQSKNAKQIYKIKIQDNLPKQIVSLDFILSQANRHEVLVSFDKSKLEIQNINDDNGENTFIQKYLCDDFKEFLGKPRDNKIEIIKNNDDILAIKYCVESTSKANKEIIVKALSDETPSA

SEQ ID NO: 27 - protein, 1247 aa, synthetic construct
KSLSINIDMGAINNGIFIATCQDDKIIDKNAFDIKFRKGKLNFSKIDRTLRRHTRRSFDRDRFVLRLLGEILPLENLSNNQKEKLFGLFKNRGFNYLNVNFNAEIDSDNLEILNALDRYYFKDCRVLSDFENSISKIFNELENNEILAFLDDQAQILNQAKEHKNKILNKNINAILEFLESIKNESFKNNKHRKSYLKDIKNEIENSFKDIILKLKIFKNSQELYYFIGNIANFQTRILRRYFNAKFDLVFDDAKLKKNILRNINYLDFISTDEKANKNKILENLNAFSTLEFLKNTDPIVTIPPYENAKNKKPQSCQALVINDEKITPSLKDIAHKILSNSNFECLKTDENGVLADNIKDNEIAKYLQRILDISKGILDDKELYPRLLEKDENAKIFAQEIRLNSVELKEFKDFAKKYYDEVNLAKKGIIKNELLKPCCLHTPHKNKNKNALISALFLKSITQKEIENLEDFFANNKISGNQTFKGFFERLSELKKRYQYRFFHILEHEPTKELEGILKNYKKVMEKIVEHNSNFSFKAPFDDSTISTNFNYLTQLGDIIFDEKSRGFAKTCKFHTLENLIRSSAKSAIASRLASNSARLINGKIEMYLDRLAHEIIKKIDFTDIYNVQINVEMNKFNFESNLSKLGLAKERQKDEESFICPYSGAKISQTNCEYDHILPRSKGLYNSLANLIPTSSTSNQIKSNTKYLLSNLDENYLKYIFAKTQTTDLNSFKAFIDENISKIDENDFTNFKNLSFFEQIAFRHALFLDTDDNSFKKALRLLKLDTIKTHSNGTQKRFINILIEKISKLTKSGIDLNFIDSKLVSSTRKDLAQNDTSIAKQEIQDSHSHCVDASIVFYLANSKIIKGQIEPDYDYFKDIYPKDSDIILPQSKQYLELNQKSQKSKKLFDRSVYSLVYEGKFDEKQKKILTQYELLKENGFVDTHKVFELIFKSFKDKDTIVLKDLKFLDNHLKSYIRKDIFSIFFNEKGELKEAKELKSATKNIDKFYTILSQNQDKIYTIKLDEKAKEKKTLQRNKVIELYKEIFYTKNAKPRARGKNRVTFSLPVYAKDAKYAIKRNSGFAGLKNKDIATKTYIDIDSREILKIPYYSTNVLPIRISDILEILSLQSKNAKQIYKIKIQDNLPKQIVSLDFILSQANRHEVLVSFDKSKLEIQNINDDNGENTFIQKYLCDDFKEFLGKPRDNKIEIIKNNDDILAIKYCVESTSKANKEIIVKALSDETPSA

SEQ ID NO: 28 - protein, 1247 aa, synthetic construct
KSLSINIDMGAINNGIFIATCQDDKIIDKNAFDIKFRKGKLNFSKRDRTLRRHTRRSFDRDRFVLRLLGEILPLENLSNNQKEKLFGLFKNRGFNYLNVNFNAEIDSDNLEILNALDRYYFKDCRVLSDFENSISKIFNELENNEILAFLDDQAQILNQAKEHKNKILNKNINAILEFLESIKNESFKNNKHRKSYLKDIKNEIENSFKDIILKLKIFKNSQELYYFIGNIANFQTRILRRYFNAKFDLVFDDAKLKKNILRNINYLDFISTDEKANKNKILENLNAFSTLEFLKNTDPIVTIPPYENAKNKKPQSCQALVINDEKITPSLKDIAHKILSNSNFECLKTDENGVLADNIKDNEIAKYLQRILDISKGILDDKELYPRLLEKDENAKIFAQEIRLNSVELKEFKDFAKKYYDEVNLAKKGIIKNELLKPCCLHTPHKNKNKNALISALFLKSITQKEIENLEDFFANNKISGNQTFKGFFERLSELKKRYQNRFFHILEHEPTKELEGILKNYKKVMEKIVEHNSNFSFKAPFDDSTISTNFNYLTQLGDIIFDEKSRGFAKTCKFHTLENLIRSSAKSAIASRLASNSARLINGKIEMYLDRLAHEIIKKIDFTDIYNVQINVEMNKFNFESNLSKLGLAKERQKDEESFICPYSGAKISQTNCEYDHILPRSKGLYNSLANLIPTSSTSNQIKSNTKYLLSNLDENYLKYIFAKTQTTDLNSFKAFIDENISKIDENDFTNFKNLSFFEQIAFRHALFLDTDDNSFKKALRLLKLDTIKTHSNGTQKRFINILIEKISKLTKSGIDLNFIDSKLVSSTRKDLAQNDTSIAKQEIQDSHSHCVDASIVFYLANSKIIKGQIEPDYDYFKDIYPKDSDIILPQSKQYLELNQKSQKSKKLFDRSVYSLVYEGKFDEKQKKILTQYELLKENGFVDTHKVFELIFKSFKDKDTIVLKDLKFLDNHLKSYIRKDIFSIFFNEKGELKEAKELKSATKNIDKFYTILSQNQDKIYTIKLDEKAKEKKTLQRNKVIELYKEIFYTKNAKPRARGKNRVTFSLPVYAKDAKYAIKRNSGFAGLKNKSIATKTYIDIDSREILKIPYYSTNVLPIRISDILEILSLQSKNAKQIYKIKIQDNLPKQIVSLDFILSQANRHEVLVSFDKSKLEIQNINDDNGENTFIQKYLCDDFKEFLGKPRDNKIEIIKNNDDILAIKYCVESTSKANKEIIVKALSDETPSA

SEQ ID NO: 29 - protein, 1247 aa, synthetic construct
KSLSINIDMGAINNGIFIATCQDDKIIDKNAFDIKFRKGKLNFSKIDRTLRRHTRRSFDRDRFVLRLLGEILPLENLSNNQKEKLFGLFKNRGFNYLNVNFNAEIDSDNLEILNALDRYYFKDCRVLSDFENSISKIFNELENNEILAFLDDQAQILNQAKEHKNKILNKNINAILEFLESIKNESFKNNKHRKSYLKDIKNEIENSFKDIILKLKIFKNSQELYYFIGNIANFQTRILRRYFNAKFDLVFDDAKLKKNILRNINYLDFISTDEKANKNKILENLNAFSTLEFLKNTDPIVTIPPYENAKNKKPQSCQALVINDEKITPSLKDIAHKILSNSNFECLKTDENGVLADNIKDNEIAKYLQRILDISKGILDDKELYPRLLEKDENAKIFAQEIRLNSVELKEFKDFAKKYYDEVNLAKKGIIKNELLKPCCLHTPHKNKNKNALISALFLKSITQKEIENLEDFFANNKISGNQTFKGFFERLSELKKRYQNRFFHILEHEPTKELEGILKNYKKVMEKIVEHNSNFSFKAPFDDSTISTNFNYLTRLGDIIFDEKSRGFAKTCKFHTLENLIRSSAKSAIASRLASNSARLINGKIEMYLDRLAHEIIKKIDFTDIYNVQINVEMNKFNFESNLSKLGLAKERQKDEESFICPYSGAKISQTNCEYDHILPRSKGLYNSLANLIPTSSTSNQIKSNTKYLLSNLDENYLKYIFAKTQTTDLNSFKAFIDENISKIDENDFTNFKNLSFFEQIAFRHALFLDTDDNSFKKALRLLKLDTIKTHSNGTQKRFINILIEKISKLTKSGIDLNFIDSKLVSSTRKDLAQNDTSIAKQEIQDSHSHCVDASIVFYLANSKIIKGQIEPDYDYFKDIYPKDSDIILPQSKQYLELNQKSQKSKKLFDRSVYSLVYEGKFDEKQKKILTQYELLKENGFVDTHKVFELIFKSFKDKDTIVLKDLKFLDNHLKSYIRKDIFSIFFNEKGELKEAKELKSATKNIDKFYTILSQNQDKIYTIKLDEKAKEKKTLQRNKVIELYKEIFYTKNAKPRARGKNRVTFSLPVYAKDAKYAIKRNSGFAGLKNKSIATKTYIDIDSREILKIPYYSTNVLPIRISDILEILSLQSKNAKQIYKIKIQDNLPKQIVSLDFILSQANRHEVLVSFDKSKLEIQNINDDNGENTFIQKYLCDDFKEFLGKPRDNKIEIIKNNDDILAIKYCVESTSKANKEIIVKALSDETPSA

SEQ ID NO: 30 - protein, 1247 aa, synthetic construct
KSLSINIDMGAINNGIFIATCQDDKIIDKNAFDIKFRKGKLNFSKIDRTLRRHTRRSFDRDRFVLRLLGEILPLENLSNNQKEKLFGLFKNRGFNYLNVNFNAEIDSDNLEILNALDRYYFKDCRVLSDFENSISKIFNELENNEILAFLDDQAQILNQAKEHKNKILNKNINAILEFLESIKNESFKNNKHRKSYLKDIKNEIENSFKDIILKLKIFKNSQELYYFIGNIANFQTRILRRYFNAKFDLVFDDAKLKKNILRNINYLDFISTDEKANKNKILENLNAFSTLEFLKNTDPIVTIPPYENAKNKKPQSCQALVINDEKITPSLKDIAHKILSNSNFECLKTDENGVLADNIKDNEIAKYLQRILDISKGILDDKELYPRLLEKDENAKIFAQEIRLNSVELKEFKDFAKKYYDEVNLAKKGIIKNELLKPCCLHTPHKNKNKNALISALFLKSITQKEIENLEDFFANNKISGNQTFKGFFERLSELKKRYQNRFFHILEHEPTKELEGILKNYKKVMEKIVEHNSNFSFKAPFDDSTISTNFNYLTQLGDIIFDEKSRGFAKTCKFHTLENLIRSSAKSAIASRLASNSARLINGKIEMYLDRLAHEIIKKIDFTDIYNVQINVEMNKFNFESNLSKLGLAKERQKDEESFICPYSGAKISQTNCEYDHILPRSKGLYNSLANLIPTSSTSNQIKSNTKYLLSNLDENYLKYIFAKTQTTDLNSFKAFIDENISKIDENDFTNFKNLSFFEQIAFRHALFLDTDDNSFKKALRLLKLDTIKTHSNGTQKRFINILIEKISKLTKSGIDLNFIDSKLVSSTRKDLAQNDTSIAKQEIQDSHSHCVDASIVFYLANSKIIKGQIEPDYDYFKDIYPKDSDIILPQSKQYLELNQKSQKSKKLFDDSVYSLVYEGKFDEKQKKILTQYELLKENGFVDTHKVFELIFKSFKDKDTIVLKDLKFLDNHLKSYIRKDIFSIFFNEKGELKEAKELKSATKNIDKFYTILSQNQDKIYTIKLDEKAKEKKTLQRNKVIELYKEIFYTKNAKPRARGKNRVTFSLPVYAKDAKYAIKRNSGFAGLKNKDIATKTYIDIDSREILKIPYYSTNVLPIRISDILEILSLQSKNAKQIYKIKIQDNLPKQIVSLDFILSQANRHEVLVSFDKSKLEIQNINDDNGENTFIQKYLCDDFKEFLGKPRDNKIEIIKNNDDILAIKYCVESTSKANKEIIVKALSDETPSA

SEQ ID NO: 31 - protein, 1247 aa, synthetic construct
KSLSINIDMGAINNGIFIATCQDDKIIDKNAFDIKFDKGKLNFSKIDRTLRRHTRRSFDRDRFVLRLLGEILPLENLSNNQKEKLFGLFKNRGFNYLNVNFNAEIDSDNLEILNALDRYYFKDCRVLSDFENSISKIFNELENNEILAFLDDQAQILNQAKEHKNKILNKNINAILEFLESIKNESFKNNKHRKSYLKDIKNEIENSFKDIILKLKIFKNSQELYYFIGNIANFQTRILRRYFNAKFDLVFDDAKLKKNILRNINYLDFISTDEKANKNKILENLNAFSTLEFLKNTDPIVTIPPYENAKNKKPQSCQALVINDEKITPSLKDIAHKILSNSNFECLKTDENGVLADNIKDNEIAKYLQRILDISKGILDDKELYPRLLEKDENAKIFAQEIRLNSVELKEFKDFAKKYYDEVNLAKKGIIKNELLKPCCLHTPHKNKNKNALISALFLKSITQKEIENLEDFFANNKISGNQTFKGFFERLSELKKRYQNRFFHILEHEPTKELEGILKNYKKVMEKIVEHNSNFSFKAPFDDSTISTNFNYLTQLGDIIFDEKSRGFAKTCKFHTLENLIRSSAKSAIASRLASNSARLINGKIEMYLDRLAHEIIKKIDFTDIYNVQINVEMNKFNFESNLSKLGLAKERQKDEESFICPYSGAKISQTNCEYDHILPRSKGLYNSLANLIPTSSTSNQIKSNTKYLLSNLDENYLKYIFAKTQTTDLNSFKAFIDENISKIDENDFTNFKNLSFFEQIAFRHALFLDTDDNSFKKALRLLKLDTIKTHSNGTQKRFINILIEKISKLTKSGIDLNFIDSKLVSSTRKDLAQNDTSIAKQEIQDSHSHCVDASIVFYLANSKIIKGQIEPDYDYFKDIYPKDSDIILPQSKQYLELNQKSQKSKKLFDDSVYSLVYEGKFDEKQKKILTQYELLKENGFVDTHKVFELIFKSFKDKDTIVLKDLKFLDNHLKSYIRKDIFSIFFNEKGELKEAKELKSATKNIDKFYTILSQNQDKIYTIKLDEKAKEKKTLQRNKVIELYKEIFYTKNAKPRARGKNRVTFSLPVYAKDAKYAIKRNSGFAGLKNKRIATKTYIDIDSREILKIPYYSTNVLPIRISDILEILSLQSKNAKQIYKIKIQDNLPKQIVSLDFILSQANRHEVLVSFDKSKLEIQNINDDNGENTFIQKYLCDDFKEFLGKPRDNKIEIIKNNDDILAIKYCVESTSKANKEIIVKALSDETPSA

SEQ ID NO: 32 - protein, 1247 aa, synthetic construct
KSLSINIDMGAINNGIFIATCQDDKIIDKNAFDIKFRKGKLNFSKIDRTLRRHTRRSFDRDRFVLRLLGEILPLENLSNNQKEKLFGLFKNRGFNYLNVNFNAEIDSDNLEILNALDRYYFKDCRVLSDFENSISKIFNELENNEILAFLDDQAQILNQAKEHKNKILNKNINAILEFLESIKNESFKNNKHRKSYLKDIKNEIENSFKDIILKLKIFKNSQELYYFIGNIANFQTRILRRYFNAKFDLVFDDAKLKKNILRNINYLDFISTDEKANKNKILENLNAFSTLEFLKNTDPIVTIPPYENAKNKKPQSCQALVINDEKITPSLKDIAHKILSNSNFECLKTDENGVLADNIKDNEIAKYLQRILDISKGILDDKELYPRLLEKDENAKIFAQEIRLNSVELKEFKDFAKKYYDEVNLAKKGIIKNELLKPCCLHTPHKNKNKNALISALFLKSITQKEIENLEDFFANNKISGNQTFKGFFERLSELKKRYQNRFFHILEHEPTKELEGILKNYKKVMEKIVEHNSNFSFKAPFDDSTISTNFNYLTQLGDIIFDEKSRGFAKTCKFHTLENLIRSSAKSAIASRLASNSARLINGKIEMYLDRLAHEIIKKIDFTDIYNVQINVEMNKFNFESNLSKLGLAKERQKDEESFICPYSGAKISQTNCEYDHILPRSKGLYNSLANLIPTSSTSNQIKSNTKYLLSNLDENYLKYIFAKTQTTDLNSFKAFIDENISKIDENDFTNFKNLSFFEQIAFRHALFLDTDDNSFKKALRLLKLDTIKTHSNGTQKRFINILIEKISKLTKSGIDLNFIDSKLVSSTRKDLAQNDTSIAKQEIQDSHSHCVDASIVFYLANSKIIKGQIEPDYDYFKDIYPKDSDIILPQSKQYLELNQKSQKSKKLFDDSVYSLVYEGKFDEKQKKILTQYELLKENGFVDTHKVFELIFKSFKDKDTIVLKDLKFLDNHLKSYIRKDIFSIFFNEKGELKEAKELKSATKNIDKFYTILSQNQDKIYTIKLDEKAKEKKTLQRNKVIELYKEIFYTKNAKPRARGKNRVTFSLPVYAKDAKYAIKRNSGFAGLKNKRIATKTYIDIDSREILKIPYYSTNVLPIRISDILEILSLQSKNAKQIYKIKIQDNLPKQIVSLDFILSQANRHEVLVSFDKSKLEIQNINDDNGENTFIQKYLCDDFKEFLGKPRDNKIEIIKNNDDILAIKYCVESTSKANKEIIVKALSDETPSA

SEQ ID NO: 33 - protein, 1247 aa, synthetic construct
KSLSINIDMGAINNGIFIATCQDDKIIDKNAFDIKFRKGKLNFSKIDRTLRRHTRRSFDRDRFVLRLLGEILPLENLSNNQKEKLFGLFKNRGFNYLNVNFNAEIDSDNLEILNALDRYYFKDCRVLSDFENSISKIFNELENNEILAFLDDQAQILNQAKEHKNKILNKNINAILEFLESIKNESFKNNKHRKSYLKDIKNEIENSFKDIILKLKIFKNSQELYYFIGNIANFQTRILRRYFNAKFDLVFDDAKLKKNILRNINYLDFISTDEKANKNKILENLNAFSTLEFLKNTDPIVTIPPYENAKNKKPQSCQALVINDEKITPSLKDIAHKILSNSNFECLKTDENGVLADNIKDNEIAKYLQRILDISKGILDDKELYPRLLEKDENAKIFAQEIRLNSVELKEFKDFAKKYYDEVNLAKKGIIKNELLKPCCLHTPHKNKNKNALISALFLKSITQKEIENLEDFFANNKISGNQTFKGFFERLSELKKRYQNRFFHILEHEPTKELEGILKNYKKVMEKIVEHNSNFSFKAPFDDSTISTNFNYLTQLGDIIFDEKSRGFAKTCKFHTLENLIRSSAKSAIASRLASNSARLINGKIEMYLDRLAHEIIKKIDFTDIYNVQINVEMNKFNFESNLSKLGLAKERQKDEESFICPYSGAKISQTNCEYDHILPRSKGLYNSLANLIPTSSTSNQIKSNTKYLLSNLDENYLKYIFAKTQTTDLNSFKAFIDENISKIDENDFTNFKNLSFFEQIAFRHALFLDTDDNSFKKALRLLKLDTIKTHSNGTQKRFINILIEKISKLTKSGIDLNFIDSKLVSSTRKDLAQNDTSIAKQEIQDSHSHCVDASIVFYLANSKIIKGQIEPDYDYFKDIYPKDSDIILPQSKQYLELNQKSQKSKKLFDDSVYSLVYEGKFDEKQKKILTQYELLKENGFVDTHKVFELIFKSFKDKDTIVLKDLKFLDNHLKSYIRKDIFSIFFNEKGELKEAKELKSATKNIDKFYTILSQNQDKIYTIKLDEKAKEKKTLQRNKVIELYKEIFYTKNAKPRARGKNRVTFSLPVYAKDAKYAIKRNSGFAGLKNKRIATKTYIDIDSREILKIPYYSTNVLPIRISDILEILSLQSKNAKQIYKIKIQDNLPKQIVSLDFILSQARRHEVLVSFDKSKLEIQNINDDNGENTFIQKYLCDDFKEFLGKPRDNKIEIIKNNDDILAIKYCVESTSKANKEIIVKALSDETPSA

SEQ ID NO: 34 - protein, 1247 aa, synthetic construct; identical to SEQ ID NO: 33

SEQ ID NO: 35 - protein, 1247 aa, synthetic construct
KSLSINIDMGAINNGIFIATCQDDKIIDKNAFDIKFRKRKLNFSKIDRTLRRHTRRSFDRDRFVLRLLGEILPLENLSNNQKEKLFGLFKNRGFNYLNVNFNAEIDSDNLEILNALDRYYFKDCRVLSDFENSISKIFNELENNEILAFLDDQAQILNQAKEHKNKILNKNINAILEFLESIKNESFKNNKHRKSYLKDIKNEIENSFKDIILKLKIFKNSQELYYFIGNIANFQTRILRRYFNAKFDLVFDDAKLKKNILRNINYLDFISTDEKANKNKILENLNAFSTLEFLKNTDPIVTIPPYENAKNKKPQSCQALVINDEKITPSLKDIAHKILSNSNFECLKTDENGVLADNIKDNEIAKYLQRILDISKGILDDKELYPRLLEKDENAKIFAQEIRLNSVELKEFKDFAKKYYDEVNLAKKGIIKNELLKPCCLHTPHKNKNKNALISALFLKSITQKEIENLEDFFANNKISGNQTFKGFFERLSELKKRYQNRFFHILEHEPTKELEGILKNYKKVMEKIVEHNSNFSFKAPFDDSTISTNFNYLTQLGDIIFDEKSRGFAKTCKFHTLENLIRSSAKSAIASRLASNSARLINGKIEMYLDRLAHEIIKKIDFTDIYNVQINVEMNKFNFESNLSKLGLAKERQKDEESFICPYSGAKISQTNCEYDHILPRSKGLYNSLANLIPTSSTSNQIKSNTKYLLSNLDENYLKYIFAKTQTTDLNSFKAFIDENISKIDENDFTNFKNLSFFEQIAFRHALFLDTDDNSFKKALRLLKLDTIKTHSNGTQKRFINILIEKISKLTKSGIDLNFIDSKLVSSTRKDLAQNDTSIAKQEIQDSHSHCVDASIVFYLANSKIIKGQIEPDYDYFKDIYPKDSDIILPQSKQYLELNQKSQKSKKLFDGSVYSLVYEGKFDEKQKKILTQYELLKENGFVDTHKVFELIFKSFKDKDTIVLKDLKFLDNHLKSYIRKDIFSIFFNEKGELKEAKELKSATKNIDKFYTILSQNQDKIYTIKLDEKAKEKKTLQRNKVIELYKEIFYTKNAKPRARGKNRVTFSLPVYAKDAKYAIKRNSGFAGLKNKDIATKTYIDIDSREILKIPYYSTNVLPIRISDILEILSLQSKNAKQIYKIKIQDNLPKQIVSLDFILSQANRHEVLVSFDKSKLEIQNINDDNGENTFIQKYLCDDFKEFLGKPRDNKIEIIKNNDDILAIKYCVESTSKANKEIIVKALSDETPSA

SEQ ID NO: 36 - protein, 1247 aa, synthetic construct
KSLSINIDMGAINNGIFIATCQDDKIIDKNAFDIKFRKRKLNFSKIDRTLRRHTRRSFDRDRFVLRLLGEILPLENLSNNQKEKLFGLFKNRGFNYLNVNFNAEIDSDNLEILNALDRYYFKDCRVLSDFENSISKIFNELENNEILAFLDDQAQILNQAKEHKNKILNKNINAILEFLESIKNESFKNNKHRKSYLKDIKNEIENSFKDIILKLKIFKNSQELYYFIGNIANFQTRILRRYFNAKFDLVFDDAKLKKNILRNINYLDFISTDEKANKNKILENLNAFSTLEFLKNTDPIVTIPPYENAKNKKPQSCQALVINDEKITPSLKDIAHKILSNSNFECLKTDENGVLADNIKDNEIAKYLQRILDISKGILDDKELYPRLLEKDENAKIFAQEIRLNSVELKEFKDFAKKYYDEVNLAKKGIIKNELLKPCCLHTPHKNKNKNALISALFLKSITQKEIENLEDFFANNKISGNQTFKGFFERLSELKKRYQNRFFHILEHEPTKELEGILKNYKKVMEKIVEHNSNFSFKAPFDDSTISTNFNYLTQLGDIIFDEKSRGFAKTCKFHTLENLIRSSAKSAIASRLASNSARLINGKIEMYLDRLAHEIIKKIDFTDIYNVQINVEMNKFNFESNLSKLGLAKERQKDEESFICPYSGAKISQTNCEYDHILPRSKGLYNSLANLIPTSSTSNQIKSNTKYLLSNLDENYLKYIFAKTQTTDLNSFKAFIDENISKIDENDFTNFKNLSFFEQIAFRHALFLDTDDNSFKKALRLLKLDTIKTHSNGTQKRFINILIEKISKLTKSGIDLNFIDSKLVSSTRKDLAQNDTSIAKQEIQDSHSHCVDASIVFYLANSKIIKGQIEPDYDYFKDIYPKDSDIILPQSKQYLELNQKSQKSKKLFDSSVYSLVYEGKFDEKQKKILTQYELLKENGFVDTHKVFELIFKSFKDKDTIVLKDLKFLDNHLKSYIRKDIFSIFFNEKGELKEAKELKSATKNIDKFYTILSQNQDKIYTIKLDEKAKEKKTLQRNKVIELYKEIFYTKNAKPRARGKNRVTFSLPVYAKDAKYAIKRNSGFAGLKNKDIATKTYIDIDSREILKIPYYSTNVLPIRISDILEILSLQSKNAKQIYKIKIQDNLPKQIVSLDFILSQANRHEVLVSFDKSKLEIQNINDDNGENTFIQKYLCDDFKEFLGKPRDNKIEIIKNNDDILAIKYCVESTSKANKEIIVKALSDETPSA

SEQ ID NO: 37 - protein, 1247 aa, synthetic construct
KSLSINIDMGAINNGIFIATCQDDKIIDKNAFDIKFRKRKLNFSKIDRTLRRHTRRSFDRDRFVLRLLGEILPLENLSNNQKEKLFGLFKNRGFNYLNVNFNAEIDSDNLEILNALDRYYFKDCRVLSDFENSISKIFNELENNEILAFLDDQAQILNQAKEHKNKILNKNINAILEFLESIKNESFKNNKHRKSYLKDIKNEIENSFKDIILKLKIFKNSQELYYFIGNIANFQTRILRRYFNAKFDLVFDDAKLKKNILRNINYLDFISTDEKANKNKILENLNAFSTLEFLKNTDPIVTIPPYENAKNKKPQSCQALVINDEKITPSLKDIAHKILSNSNFECLKTDENGVLADNIKDNEIAKYLQRILDISKGILDDKELYPRLLEKDENAKIFAQEIRLNSVELKEFKDFAKKYYDEVNLAKKGIIKNELLKPCCLHTPHKNKNKNALISALFLKSITQKEIENLEDFFANNKISGNQTFKGFFERLSELKKRYQNRFFHILEHEPTKELEGILKNYKKVMEKIVEHNSNFSFKAPFDDSTISTNFNYLTQLGDIIFDEKSRGFAKTCKFHTLENLIRSSAKSAIASRLASNSARLINGKIEMYLDRLAHEIIKKIDFTDIYNVQINVEMNKFNFESNLSKLGLAKERQKDEESFICPYSGAKISQTNCEYDHILPRSKGLYNSLANLIPTSSTSNQIKSNTKYLLSNLDENYLKYIFAKTQTTDLNSFKAFIDENISKIDENDFTNFKNLSFFEQIAFRHALFLDTDDNSFKKALRLLKLDTIKTHSNGTQKRFINILIEKISKLTKSGIDLNFIDSKLVSSTRKDLAQNDTSIAKQEIQDSHSHCVDASIVFYLANSKIIKGQIEPDYDYFKDIYPKDSDIILPQSKQYLELNQKSQKSKKLFDNSVYSLVYEGKFDEKQKKILTQYELLKENGFVDTHKVFELIFKSFKDKDTIVLKDLKFLDNHLKSYIRKDIFSIFFNEKGELKEAKELKSATKNIDKFYTILSQNQDKIYTIKLDEKAKEKKTLQRNKVIELYKEIFYTKNAKPRARGKNRVTFSLPVYAKDAKYAIKRNSGFAGLKNKDIATKTYIDIDSREILKIPYYSTNVLPIRISDILEILSLQSKNAKQIYKIKIQDNLPKQIVSLDFILSQANRHEVLVSFDKSKLEIQNINDDNGENTFIQKYLCDDFKEFLGKPRDNKIEIIKNNDDILAIKYCVESTSKANKEIIVKALSDETPSA

SEQ ID NO: 38 - protein, 1247 aa, synthetic construct
KSLSINIDMGAINNGIFIATCQDDKIIDKNAFDIKFRKRKLNFSKIDRTLRRHTRRSFDRDRFVLRLLGEILPLENLSNNQKEKLFGLFKNRGFNYLNVNFNAEIDSDNLEILNALDRYYFKDCRVLSDFENSISKIFNELENNEILAFLDDQAQILNQAKEHKNKILNKNINAILEFLESIKNESFKNNKHRKSYLKDIKNEIENSFKDIILKLKIFKNSQELYYFIGNIANFQTRILRRYFNAKFDLVFDDAKLKKNILRNINYLDFISTDEKANKNKILENLNAFSTLEFLKNTDPIVTIPPYENAKNKKPQSCQALVINDEKITPSLKDIAHKILSNSNFECLKTDENGVLADNIKDNEIAKYLQRILDISKGILDDKELYPRLLEKDENAKIFAQEIRLNSVELKEFKDFAKKYYDEVNLAKKGIIKNELLKPCCLHTPHKNKNKNALISALFLKSITQKEIENLEDFFANNKISGNQTFKGFFERLSELKKRYQNRFFHILEHEPTKELEGILKNYKKVMEKIVEHNSNFSFKAPFDDSTISTNFNYLTQLGDIIFDEKSRGFAKTCKFHTLENLIRSSAKSAIASRLASNSARLINGKIEMYLDRLAHEIIKKIDFTDIYNVQINVEMNKFNFESNLSKLGLAKERQKDEESFICPYSGAKISQTNCEYDHILPRSKGLYNSLANLIPTSSTSNQIKSNTKYLLSNLDENYLKYIFAKTQTTDLNSFKAFIDENISKIDENDFTNFKNLSFFEQIAFRHALFLDTDDNSFKKALRLLKLDTIKTHSNGTQKRFINILIEKISKLTKSGIDLNFIDSKLVSSTRKDLAQNDTSIAKQEIQDSHSHCVDASIVFYLANSKIIKGQIEPDYDYFKDIYPKDSDIILPQSKQYLELNQKSQKSKKLFDRSVYSLVYEGKFDEKQKKILTQYELLKENGFVDTHKVFELIFKSFKDKDTIVLKDLKFLDNHLKSYIRKDIFSIFFNEKGELKEAKELKSATKNIDKFYTILSQNQDKIYTIKLDEKAKEKKTLQRNKVIELYKEIFYTKNAKPRARGKNRVTFSLPVYAKDAKYAIKRNSGFAGLKNKDIATKTYIDIDSREILKIPYYSTNVLPIRISDILEILSLQSKNAKQIYKIKIQDNLPKQIVSLDFILSQANRHEVLVSFDKSKLEIQNINDDNGENTFIQKYLCDDFKEFLGKPRDNKIEIIKNNDDILAIKYCVESTSKANKEIIVKALSDETPSA

SEQ ID NO: 39 - protein, 1247 aa, synthetic construct
KSLSINIDMGAINNGIFIATCQDDKIIDKNAFDIKFDKGKLNFSKIDRTLRRHTRRSFDRDRFVLRLLGEILPLENLSNNQKEKLFGLFKNRGFNYLNVNFNAEIDSDNLEILNALDRYYFKDCRVLSDFENSISKIFNELENNEILAFLDDQAQILNQAKEHKNKILNKNINAILEFLESIKNESFKNNKHRKSYLKDIKNEIENSFKDIILKLKIFKNSQELYYFIGNIANFQTRILRRYFNAKFDLVFDDAKLKKNILRNINYLDFISTDEKANKNKILENLNAFSTLEFLKNTDPIVTIPPYENAKNKKPQSCQALVINDEKITPSLKDIAHKILSNSNFECLKTDENGVLADNIKDNEIAKYLQRILDISKGILDDKELYPRLLEKDENAKIFAQEIRLNSVELKEFKDFAKKYYDEVNLAKKGIIKNELLKPCCLHTPHKNKNKNALISALFLKSITQKEIENLEDFFANNKISGNQTFKGFFERLSELKKRYQNRFFHILEHEPTKELEGILKNYKKVMEKIVEHNSNFSFKAPFDDSTISTNFNYLTQLGDIIFDEKSRGFAKTCKFHTLENLIRSSAKSAIASRLASNSARLINGKIEMYLDRLAHEIIKKIDFTDIYNVQINVEMNKFNFESNLSKLGLAKERQKDEESFICPYSGAKISQTNCEYDHILPRSKGLYNSLANLIPTSSTSNQIKSNTKYLLSNLDENYLKYIFAKTQTTDLNSFKAFIDENISKIDENDFTNFKNLSFFEQIAFRHALFLDTDDNSFKKALRLLKLDTIKTHSNGTQKRFINILIEKISKLTKSGIDLNFIDSKLVSSTRKDLAQNDTSIAKQEIQDSHSHCVDASIVFYLANSKIIKGQIEPDYDYFKDIYPKDSDIILPQSKQYLELNQKSQKSKKLFDDSVYSLVYEGKFDEKQKKILTQYELLKENGFVDTHKVFELIFKSFKDKDTIVLKDLKFLDNHLKSYIRKDIFSIFFNEKGELKEAKELKSATKNIDKFYTILSQNQDKIYTIKLDEKAKEKKTLQRNKVIELYKEIFYTKNAKPRARGKNRVTFSLPVYAKDAKYAIKRNSGFAGLKNKRIATKTYIDIDSREILKIPYYSTNVLPIRISDILEILSLQSKNAKQIYKIKIQDNLPKQIVSLDFILSQARRHEVLVSFDKSKLEIQNINDDNGENTFIQKYLCDDFKEFLGKPRDNKIEIIKNNDDILAIKYCVESTRKANKEIIVKALSDETPSA

SEQ ID NO: 40 - protein, 1247 aa, synthetic construct
KSLSINIDMGAINNGIFIATCQDDKIIDKNAFDIKFDKGKLNFSKIDRTLRRHTRRSFDRDRFVLRLLGEILPLENLSNNQKEKLFGLFKNRGFNYLNVNFNAEIDSDNLEILNALDRYYFKDCRVLSDFENSISKIFNELENNEILAFLDDQAQILNQAKEHKNKILNKNINAILEFLESIKNESFKNNKHRKSYLKDIKNEIENSFKDIILKLKIFKNSQELYYFIGNIANFQTRILRRYFNAKFDLVFDDAKLKKNILRNINYLDFISTDEKANKNKILENLNAFSTLEFLKNTDPIVTIPPYENAKNKKPQSCQALVINDEKITPSLKDIAHKILSNSNFECLKTDENGVLADNIKDNEIAKYLQRILDISKGILDDKELYPRLLEKDENAKIFAQEIRLNSVELKEFKDFAKKYYDEVNLAKKGIIKNELLKPCCLHTPHKNKNKNALISALFLKSITQKEIENLEDFFANNKISGNQTFKGFFERLSELKKRYQNRFFHILEHEPTKELEGILKNYKKVMEKIVEHNSNFSFKAPFDDSTISTNFNYLTQLGDIIFDEKSRGFAKTCKFHTLENLIRSSAKSAIASRLASNSARLINGKIEMYLDRLAHEIIKKIDFTDIYNVQINVEMNKFNFESNLSKLGLAKERQKDEESFICPYSGAKISQTNCEYDHILPRSKGLYNSLANLIPTSSTSNQIKSNTKYLLSNLDENYLKYIFAKTQTTDLNSFKAFIDENISKIDENDFTNFKNLSFFEQIAFRHALFLDTDDNSFKKALRLLKLDTIKTHSNGTQKRFINILIEKISKLTKSGIDLNFIDSKLVSSTRKDLAQNDTSIAKQEIQDSHSHCVDASIVFYLANSKIIKGQIEPDYDYFKDIYPKDSDIILPQSKQYLELNQKSQKSKKLFDGSVYSLVYEGKFDEKQKKILTQYELLKENGFVDTHKVFELIFKSFKDKDTIVLKDLKFLDNHLKSYIRKDIFSIFFNEKGELKEAKELKSATKNIDKFYTILSQNQDKIYTIKLDEKAKEKKTLQRNKVIELYKEIFYTKNAKPRARGKNRVTFSLPVYAKDAKYAIKRNSGFAGLKNKRIATKTYIDIDSREILKIPYYSTNVLPIRISDILEILSLQSKNAKQIYKIKIQDNLPKQIVSLDFILSQARRHEVLVSFDKSKLEIQNINDDNGENTFIQKYLCDDFKEFLGKPRDNKIEIIKNNDDILAIKYCVESTSKANKEIIVKALSDETPSA

SEQ ID NO: 41 - protein, 1247 aa, synthetic construct
KSLSINIDMGAINNGIFIATCQDDKIIDKNAFDIKFDKGKLNFSKIDRTLRRHTRRSFDRDRFVLRLLGEILPLENLSNNQKEKLFGLFKNRGFNYLNVNFNAEIDSDNLEILNALDRYYFKDCRVLSDFENSISKIFNELENNEILAFLDDQAQILNQAKEHKNKILNKNINAILEFLESIKNESFKNNKHRKSYLKDIKNEIENSFKDIILKLKIFKNSQELYYFIGNIANFQTRILRRYFNAKFDLVFDDAKLKKNILRNINYLDFISTDEKANKNKILENLNAFSTLEFLKNTDPIVTIPPYENAKNKKPQSCQALVINDEKITPSLKDIAHKILSNSNFECLKTDENGVLADNIKDNEIAKYLQRILDISKGILDDKELYPRLLEKDENAKIFAQEIRLNSVELKEFKDFAKKYYDEVNLAKKGIIKNELLKPCCLHTPHKNKNKNALISALFLKSITQKEIENLEDFFANNKISGNQTFKGFFERLSELKKRYQNRFFHILEHEPTKELEGILKNYKKVMEKIVEHNSNFSFKAPFDDSTISTNFNYLTQLGDIIFDEKSRGFAKTCKFHTLENLIRSSAKSAIASRLASNSARLINGKIEMYLDRLAHEIIKKIDFTDIYNVQINVEMNKFNFESNLSKLGLAKERQKDEESFICPYSGAKISQTNCEYDHILPRSKGLYNSLANLIPTSSTSNQIKSNTKYLLSNLDENYLKYIFAKTQTTDLNSFKAFIDENISKIDENDFTNFKNLSFFEQIAFRHALFLDTDDNSFKKALRLLKLDTIKTHSNGTQKRFINILIEKISKLTKSGIDLNFIDSKLVSSTRKDLAQNDTSIAKQEIQDSHSHCVDASIVFYLANSKIIKGQIEPDYDYFKDIYPKDSDIILPQSKQYLELNQKSQKSKKLFDNSVYSLVYEGKFDEKQKKILTQYELLKENGFVDTHKVFELIFKSFKDKDTIVLKDLKFLDNHLKSYIRKDIFSIFFNEKGELKEAKELKSATKNIDKFYTILSQNQDKIYTIKLDEKAKEKKTLQRNKVIELYKEIFYTKNAKPRARGKNRVTFSLPVYAKDAKYAIKRNSGFAGLKNKRIATKTYIDIDSREILKIPYYSTNVLPIRISDILEILSLQSKNAKQIYKIKIQDNLPKQIVSLDFILSQARRHEVLVSFDKSKLEIQNINDDNGENTFIQKYLCDDFKEFLGKPRDNKIEIIKNNDDILAIKYCVESTSKANKEIIVKALSDETPSA

SEQ ID NO: 42 - protein, 1247 aa, synthetic construct
KSLSINIDMGAINNGIFIATCQDDKIIDKNAFDIKFRKGKLNFSKIDRTLRRHTRRSFDRLRFVLRLLGEILPLENLSNNQKEKLFGLFKNRGFNYLNVNFNAEIDSDNLEILNALDRYYFKDCRVLSDFENSISKIFNELENNEILAFLDDQAQILNQAKEHKNKILNKNINAILEFLESIKNESFKNNKHRKSYLKDIKNEIENSFKDIILKLKIFKNSQELYYFIGNIANFQTRILRRYFNAKFDLVFDDAKLKKNILRNINYLDFISTDEKANKNKILENLNAFSTLEFLKNTDPIVTIPPYENAKNKKPQSCQALVINDEKITPSLKDIAHKILSNSNFECLKTDENGVLADNIKDNEIAKYLQRILDISKGILDDKELYPRLLEKDENAKIFAQEIRLNSVELKEFKDFAKKYYDEVNLAKKGIIKNELLKPCCLHTPHKNKNKNALISALFLKSITQKEIENLEDFFANNKISGNQTFKGFFERLSELKKRYQNRFFHILEHEPTKELEGILKNYKKVMEKIVEHNSNFSFKAPFDDSTISTNFNYLTQLGDIIFDEKSRGFAKTCKFHTLENLIRSSAKSAIASRLASNSARLINGKIEMYLDRLAHEIIKKIDFTDIYNVQINVEMNKFNFESNLSKLGLAKERQKDEESFICPYSGAKISQTNCEYDHILPRSKGLYNSLANLIPTSSTSNQIKSNTKYLLSNLDENYLKYIFAKTQTTDLNSFKAFIDENISKIDENDFTNFKNLSFFEQIAFRHALFLDTDDNSFKKALRLLKLDTIKTHSNGTQKRFINILIEKISKLTKSGIDLNFIDSKLVSSTRKDLAQNDTSIAKQEIQDSHSHCVDASIVFYLANSKIIKGQIEPDYDYFKDIYPKDSDIILPQSKQYLELNQKSQKSKKLFDRSVYSLVYEGKFDEKQKKILTQYELLKENGFVDTHKVFELIFKSFKDKDTIVLKDLKFLDNHLKSYIRKDIFSIFFNEKGELKEAKELKSATKNIDKFYTILSQNQDKIYTIKLDEKAKEKKTLQRNKVIELYKEIFYTKNAKPRARGKNRVTFSLPVYAKDAKYAIKRNSGFAGLKNKDIATKTYIDIDSREILKIPYYSTNVLPIRISDILEILSLQSKNAKQIYKIKIQDNLPKQIVSLDFILSQANRHEVLVSFDKSKLEIQNINDDNGENTFIQKYLCDDFKEFLGKPRDNKIEIIKNNDDILAIKYCVESTSKANKEIIVKALSDETPSA

SEQ ID NO: 43 - protein, 1247 aa, synthetic construct
KSLSINIDMGAINNGIFIATCQDDKIIDKNAFDIKFRKGKLNFSKIDRTLRRHTRRSFDRDRFVLRLLGEILPLENLSNNQKEKLFGLFKNRGFNYLNVNFNAEIDSDNLEILNALDRYYFKDCRVLSDFENSISKIFNELENNEILAFLDDQAQILNQAKEHKNKILNKNINAILEFLESIKNESFKNNKHRKSYLKDIKNEIENSFKDIILKLKIFKNSQELYYFIGNIANFQTRILRRYFNAKFDLVFDDAKLKKNILRNINYLDFISTDEKANKNKILENLNAFSTLEFLKNTDPIVTIPPYENAKNKKPQSCQALVINDEKITPSLKDIAHKILSNSNFECLKTDENGVLADNIKDNEIAKYLQRILDISKGILDDKELYPRLLEKDENAKIFAQEIRLNSVELKEFKDFAKKYYDEVNLAKKGIIKNELLKPCCLHTPHKNKNKNALISALFLKSITQKEIENLEDFFANNKISGNQTFKGFFERLSELKKRYQNRFFHILEHEPTKELEGILKNYKKVMEKIVEHNSNFSFKAPFDDSTISTNFNYLTQLGDIIFDEKSRGFAKTCKFHTLENLIRSSAKSAIASRLASNSARLINGKIEMYLDRLAHEIIKKIDFTDIYNVQINVEMNKFNFESNLSKLGLAKERQKDEESFICPYSGAKISQTNCEYDHILPRSKGLYNSLANLIPTSSTSNQIKSNTKYLLSNLDENYLKYIFAKTQTTDLNSFKAFIDENISKIDENDFTNFKNLSFFEQIAFRHALFLDTDDNSFKKALRLLKLDTIKTHSNGTQKRFINILIEKISKLTKSGIDLNFIDSKLVSSTRKDLAQNDTSIAKQEIQDSHSHCVDASIVFYLANSKIIKGQIEPDYDYFKDIYPKDSDIILPQSKQYLELNQKSQKSKKLFGRSVYSLVYEGKFDEKQKKILTQYELLKENGFVDTHKVFELIFKSFKDKDTIVLKDLKFLDNHLKSYIRKDIFSIFFNEKGELKEAKELKSATKNIDKFYTILSQNQDKIYTIKLDEKAKEKKTLQRNKVIELYKEIFYTKNAKPRARGKNRVTFSLPVYAKDAKYAIKRNSGFAGLKNKDIATKTYIDIDSREILKIPYYSTNVLPIRISDILEILSLQSKNAKQIYKIKIQDNLPKQIVSLDFILSQANRHEVLVSFDKSKLEIQNINDDNGENTFIQKYLCDDFKEFLGKPRDNKIEIIKNNDDILAIKYCVESTSKANKEIIVKALSDETPSA

SEQ ID NO: 44 - protein, 1247 aa, synthetic construct
KSLSINIDMGAINNGIFIATCQDDKIIDKNAFDIKFRKGKLNFSKIDRTLRRHTRRSFDRDRFVLRLLGEILPLENLSNNQKEKLFGLFKNRGFNYLNVNFNAEIDSDNLEILNALDRYYFKDCRVLSDFENSISKIFNELENNEILAFLDDQAQILNQAKEHKNKILNKNINAILEFLESIKNESFKNNKHRKSYLKDIKNEIENSFKDIILKLKIFKNSQELYYFIGNIANFQTRILRRYFNAKFDLVFDDAKLKKNILRNINYLDFISTDEKANKNKILENLNAFSTLEFLKNTDPIVTIPPYENAKNKKPQSCQALVINDEKITPSLKDIAHKILSNSNFECLKTDENGVLADNIKDNEIAKYLQRILDISKGILDDKELYPRLLEKDENAKIFAQEIRLNSVELKEFKDFAKKYYDEVNLAKKGIIKNELLKPCCLHTPHKNKNKNALISALFLKSITQKEIENLEDFFANNKISGNQTFKGFFERLSELKKRYQNRFFHILEHEPTKELEGILKNYKKVMEKIVEHNSNFSFKAPFDDSTISTNFNYLTQLGDIIFDEKSRGFAKTCKFHTLENLIRSSAKSAIASRLASNSARLINGKIEMYLDRLAHEIIKKIDFTDIYNVQINVEMNKFNFESNLSKLGLAKERQKDEESFICPYSGAKISQTNCEYDHILPRSKGLYNSLANLIPTSSTSNQIKSNTKYLLSNLDENYLKYIFAKTQTTDLNSFKAFIDENISKIDENDFTNFKNLSFFEQIAFRHALFLDTDDNSFKKALRLLKLDTIKTHSNGTQKRFINILIEKISKLTKSGIDLNFIDSKLVSSTRKDLAQNDTSIAKQEIQDSHSHCVDASIVFYLANSKIIKGQIEPDYDYFKDIYPKDSDIILPQSKQYLELNQKSQKSKKLFSRSVYSLVYEGKFDEKQKKILTQYELLKENGFVDTHKVFELIFKSFKDKDTIVLKDLKFLDNHLKSYIRKDIFSIFFNEKGELKEAKELKSATKNIDKFYTILSQNQDKIYTIKLDEKAKEKKTLQRNKVIELYKEIFYTKNAKPRARGKNRVTFSLPVYAKDAKYAIKRNSGFAGLKNKDIATKTYIDIDSREILKIPYYSTNVLPIRISDILEILSLQSKNAKQIYKIKIQDNLPKQIVSLDFILSQANRHEVLVSFDKSKLEIQNINDDNGENTFIQKYLCDDFKEFLGKPRDNKIEIIKNNDDILAIKYCVESTSKANKEIIVKALSDETPSA

SEQ ID NO: 45 - protein, 1247 aa, synthetic construct
KSLSINIDMGAINNGIFIATCQDDKIIDKNAFDIKFRKGKLNFSKIDRTLRRHTRRSFDRDRFVLRLLGEILPLENLSNNQKEKLFGLFKNRGFNYLNVNFNAEIDSDNLEILNALDRYYFKDCRVLSDFENSISKIFNELENNEILAFLDDQAQILNQAKEHKNKILNKNINAILEFLESIKNESFKNNKHRKSYLKDIKNEIENSFKDIILKLKIFKNSQELYYFIGNIANFQTRILRRYFNAKFDLVFDDAKLKKNILRNINYLDFISTDEKANKNKILENLNAFSTLEFLKNTDPIVTIPPYENAKNKKPQSCQALVINDEKITPSLKDIAHKILSNSNFECLKTDENGVLADNIKDNEIAKYLQRILDISKGILDDKELYPRLLEKDENAKIFAQEIRLNSVELKEFKDFAKKYYDEVNLAKKGIIKNELLKPCCLHTPHKNKNKNALISALFLKSITQKEIENLEDFFANNKISGNQTFKGFFERLSELKKRYQNRFFHILEHEPTKELEGILKNYKKVMEKIVEHNSNFSFKAPFDDSTISTNFNYLTQLGDIIFDEKSRGFAKTCKFHTLENLIRSSAKSAIASRLASNSARLINGKIEMYLDRLAHEIIKKIDFTDIYNVQINVEMNKFNFESNLSKLGLAKERQKDEESFICPYSGAKISQTNCEYDHILPRSKGLYNSLANLIPTSSTSNQIKSNTKYLLSNLDENYLKYIFAKTQTTDLNSFKAFIDENISKIDENDFTNFKNLSFFEQIAFRHALFLDTDDNSFKKALRLLKLDTIKTHSNGTQKRFINILIEKISKLTKSGIDLNFIDSKLVSSTRKDLAQNDTSIAKQEIQDSHSHCVDASIVFYLANSKIIKGQIEPDYDYFKDIYPKDSDIILPQSKQYLELNQKSQKSKKLFDRSVYSLVYEGKFDEKQKKILTQYELLKENGFVDTHKVFELIFKSFKDKDTIVLKDLKFLDNHLKSYIRKDIFSIFFNEKGELKEAKELKSATKNIDKFYTILSQNQDKIYTIKLDEKAKEKKTLQRNKVIELYKEIFYTKNAKPRARGKNRVTFSLPVYAKGAKYAIKRNSGFAGLKNKDIATKTYIDIDSREILKIPYYSTNVLPIRISDILEILSLQSKNAKQIYKIKIQDNLPKQIVSLDFILSQANRHEVLVSFDKSKLEIQNINDDNGENTFIQKYLCDDFKEFLGKPRDNKIEIIKNNDDILAIKYCVESTSKANKEIIVKALSDETPSA

SEQ ID NO: 46 - protein, 1247 aa, synthetic construct
KSLSINIDMGAINNGIFIATCQDDKIIDKNAFDIKFRKGKLNFSKIDRTLRRHTRRSFDRDRFVLRLLGEILPLENLSNNQKEKLFGLFKNRGFNYLNVNFNAEIDSDNLEILNALDRYYFKDCRVLSDFENSISKIFNELENNEILAFLDDQAQILNQAKEHKNKILNKNINAILEFLESIKNESFKNNKHRKSYLKDIKNEIENSFKDIILKLKIFKNSQELYYFIGNIANFQTRILRRYFNAKFDLVFDDAKLKKNILRNINYLDFISTDEKANKNKILENLNAFSTLEFLKNTDPIVTIPPYENAKNKKPQSCQALVINDEKITPSLKDIAHKILSNSNFECLKTDENGVLADNIKDNEIAKYLQRILDISKGILDDKELYPRLLEKDENAKIFAQEIRLNSVELKEFKDFAKKYYDEVNLAKKGIIKNELLKPCCLHTPHKNKNKNALISALFLKSITQKEIENLEDFFANNKISGNQTFKGFFERLSELKKRYQNRFFHILEHEPTKELEGILKNYKKVMEKIVEHNSNFSFKAPFDDSTISTNFNYLTQLGDIIFDEKSRGFAKTCKFHTLENLIRSSAKSAIASRLASNSARLINGKIEMYLDRLAHEIIKKIDFTDIYNVQINVEMNKFNFESNLSKLGLAKERQKDEESFICPYSGAKISQTNCEYDHILPRSKGLYNSLANLIPTSSTSNQIKSNTKYLLSNLDENYLKYIFAKTQTTDLNSFKAFIDENISKIDENDFTNFKNLSFFEQIAFRHALFLDTDDNSFKKALRLLKLDTIKTHSNGTQKRFINILIEKISKLTKSGIDLNFIDSKLVSSTRKDLAQNDTSIAKQEIQDSHSHCVDASIVFYLANSKIIKGQIEPDYDYFKDIYPKDSDIILPQSKQYLELNQKSQKSKKLFDRSVYSLVYEGKFDEKQKKILTQYELLKENGFVDTHKVFELIFKSFKDKDTIVLKDLKFLDNHLKSYIRKDIFSIFFNEKGELKEAKELKSATKNIDKFYTILSQNQDKIYTIKLDEKAKEKKTLQRNKVIELYKEIFYTKNAKPRARGKNRVTFSLPVYAKAAKYAIKRNSGFAGLKNKDIATKTYIDIDSREILKIPYYSTNVLPIRISDILEILSLQSKNAKQIYKIKIQDNLPKQIVSLDFILSQANRHEVLVSFDKSKLEIQNINDDNGENTFIQKYLCDDFKEFLGKPRDNKIEIIKNNDDILAIKYCVESTSKANKEIIVKALSDETPSA

SEQ ID NO: 47 - protein, 1247 aa, synthetic construct
KSLSINIDMGAINNGIFIATCQDDKIIDKNAFDIKFRKGKLNFSKIDRTLRRHTRRSFDRDRFVLRLLGEILPLENLSNNQKEKLFGLFKNRGFNYLNVNFNAEIDSDNLEILNALDRYYFKDCRVLSDFENSISKIFNELENNEILAFLDDQAQILNQAKEHKNKILNKNINAILEFLESIKNESFKNNKHRKSYLKDIKNEIENSFKDIILKLKIFKNSQELYYFIGNIANFQTRILRRYFNAKFDLVFDDAKLKKNILRNINYLDFISTDEKANKNKILENLNAFSTLEFLKNTDPIVTIPPYENAKNKKPQSCQALVINDEKITPSLKDIAHKILSNSNFECLKTDENGVLADNIKDNEIAKYLQRILDISKGILDDKELYPRLLEKDENAKIFAQEIRLNSVELKEFKDFAKKYYDEVNLAKKGIIKNELLKPCCLHTPHKNKNKNALISALFLKSITQKEIENLEDFFANNKISGNQTFKGFFERLSELKKRYQNRFFHILGHEPTKELEGILKNYKKVMEKIVEHNSNFSFKAPFDDSTISTNFNYLTQLGDIIFDEKSRGFAKTCKFHTLENLIRSSAKSAIASRLASNSARLINGKIEMYLDRLAHEIIKKIDFTDIYNVQINVEMNKFNFESNLSKLGLAKERQKDEESFICPYSGAKISQTNCEYDHILPRSKGLYNSLANLIPTSSTSNQIKSNTKYLLSNLDENYLKYIFAKTQTTDLNSFKAFIDENISKIDENDFTNFKNLSFFEQIAFRHALFLDTDDNSFKKALRLLKLDTIKTHSNGTQKRFINILIEKISKLTKSGIDLNFIDSKLVSSTRKDLAQNDTSIAKQEIQDSHSHCVDASIVFYLANSKIIKGQIEPDYDYFKDIYPKDSDIILPQSKQYLELNQKSQKSKKLFDRSVYSLVYEGKFDEKQKKILTQYELLKENGFVDTHKVFELIFKSFKDKDTIVLKDLKFLDNHLKSYIRKDIFSIFFNEKGELKEAKELKSATKNIDKFYTILSQNQDKIYTIKLDEKAKEKKTLQRNKVIELYKEIFYTKNAKPRARGKNRVTFSLPVYAKDAKYAIKRNSGFAGLKNKDIATKTYIDIDSREILKIPYYSTNVLPIRISDILEILSLQSKNAKQIYKIKIQDNLPKQIVSLDFILSQANRHEVLVSFDKSKLEIQNINDDNGENTFIQKYLCDDFKEFLGKPRDNKIEIIKNNDDILAIKYCVESTSKANKEIIVKALSDETPSA

SEQ ID NO: 48 - protein, 1247 aa, synthetic construct
KSLSINIDMGAINNGIFIATCQDDKIIDKNAFDIKFRKGKLNFSKIDRTLRRHTRRSFDRDRFVLRLLGEILPLENLSNNQKEKLFGLFKNRGFNYLNVNFNAEIDSDNLEILNALDRYYFKDCRVLSDFENSISKIFNELENNEILAFLDDQAQILNQAKEHKNKILNKNINAILEFLESIKNESFKNNKHRKSYLKDIKNEIENSFKDIILKLKIFKNSQELYYFIGNIANFQTRILRRYFNAKFDLVFDDAKLKKNILRNINYLDFISTDEKANKNKILENLNAFSTLEFLKNTDPIVTIPPYENAKNKKPQSCQALVINDEKITPSLKDIAHKILSNSNFECLKTDENGVLADNIKDNEIAKYLQRILDISKGILDDKELYPRLLEKDENAKIFAQEIRLNSVELKEFKDFAKKYYDEVNLAKKGIIKNELLKPCCLHTPHKNKNKNALISALFLKSITQKEIENLEDFFANNKISGNQTFKGFFERLSELKKRYQNRFFHILEHEPTKELEGILKNYKKVMEKIVEHNSNFSFKAPFDDSTISTNFNYLTQLGDIIFDEKSRGFAKTCKFHTLENLIRSSAKSAIASRLASNSARLINGKIEMYLDRLAHEIIKKIDFTDIYNVQINVEMNKFNFESNLSKLGLAKERQKDEESFICPYSGAKISQTNCEYDHILPRSKGLYNSLANLIPTSSTSNQIKSNTKYLLSNLDENYLKYIFAKTQTTDLNSFKAFIDENISKIDENDFTNFKNLSFFEQIAFRHALFLDTDDNSFKKALRLLKLDTIKTHSNGTQKRFINILIEKISKLTKSGIDLNFIDSKLVSSTRKDLAQNDTSIAKQEIQDSHSHCVDASIVFYLANSKIIKGQIEPDYDYFKDIYPKDSDIILPQSKQYLELNQKSQKSKKLFDRSVYSLVYEGKFDEKQKKILTQYELLKENGFVDTHKVFELIFKSFKDKDTIVLKDLKFLDNHLKSYIRKDIFSIFFNEKGELKEAKELKSATKNIDKFYTILSQNQDKIYTIKLDEKAKEKKTLQRNKVIELYKEIFYTKNAKPRARGKNRVTFSLPVYAKDAKYAIKRNSGFAGLKNKDIATKTYIDIDSREILKIPYYSTNVLPIRISDILEILSLQSKNAKQIYKIKIQDNLPKQIVSLDFILSQANRHRVLVSFDKSKLEIQNINDDNGENTFIQKYLCDDFKEFLGKPRDNKIEIIKNNDDILAIKYCVESTSKANKEIIVKALSDETPSA

SEQ ID NO: 49 - protein, 1247 aa, synthetic construct
KSLSINIDMGAINNGIFIATCQDDKIIDKNAFDIKFRKGKLNFSKIDRTLRRHTRRSFDRDRFVLRLLGEILPLENLSNNQKEKLFGLFKNRGFNYLNVNFNAEIDSDNLEILNALDRYYFKDCRVLSDFENSISKIFNELENNEILAFLDDQAQILNQAKEHKNKILNKNINAILEFLESIKNESFKNNKHRKSYLKDIKNEIENSFKDIILKLKIFKNSQELYYFIGNIANFQTRILRRYFNAKFDLVFDDAKLKKNILRNINYLDFISTDEKANKNKILENLNAFSTLEFLKNTDPIVTIPPYENAKNKKPQSCQALVINDEKITPSLKDIAHKILSNSNFECLKTDENGVLADNIKDNEIAKYLQRILDISKGILDDKELYPRLLEKDENAKIFAQEIRLNSVELKEFKDFAKKYYDEVNLAKKGIIKNELLKPCCLHTPHKNKNKNALISALFLKSITQKEIENLEDFFANNKISGNQTFKGFFERLSELKKRYQNRFFHILEHEPTKELEGILKNYKKVMEKIVEHNSNFSFKAPFDDSTISTNFNYLTQLGDIIFDEKSRGFAKTCKFHTLENLIRSSAKSAIASRLASNSARLINGKIEMYLDRLAHEIIKKIDFTDIYNVQINVEMNKFNFESNLSKLGLAKERQKDEESFICPYSGAKISQTNCEYDHILPRSKGLYNSLANLIPTSSTSNQIKSNTKYLLSNLDENYLKYIFAKTQTTDLNSFKAFIDENISKIDENDFTNFKNLSFFEQIAFRHALFLDTDDNSFKKALRLLKLDTIKTHSNGTQKRFINILIEKISKLTKSGIDLNFIDSKLVSSTRKDLAQNDTSIAKQEIQDSHSHCVDASIVFYLANSKIIKGQIEPDYDYFKDIYPKDSDIILPQSKQYLELNQKSQKSKKLFDRSVYSLVYEGKFDEKQKKILTQYELLKENGFVDTHKVFELIFKSFKDKDTIVLKDLKFLDNHLKSYIRKDIFSIFFNEKGELKEAKELKSATKNIDKFYTILSQNQDKIYTIKLDEKAKEKKTLQRNKVIELYKEIFYTKNAKPRARGKNRVTFSLPVYAKDAKYAIKRNSGFAGLKNKDIATKTYIDIDSREILKIPYYSTNVLPIRISDILEILSLQSKNAKQIYKIKIQDNLPKQIVSLDFILNQANRHRVLVSFDKSKLEIQNINDDNGENTFIQKYLCDDFKEFLGKPRDNKIEIIKNNDDILAIKYCVESTSKANKEIIVKALSDETPSA

SEQ ID NO: 50 - protein, 1247 aa, synthetic construct
KSLSINIDMGAINNGIFIATCQDDKIIDKNAFDIKFRKGKLNFSKIDRTLRRHTRRSFDRDRFVLRLLGEILPLENLSNNQKEKLFGLFKNRGFNYLNVNFNAEIDSDNLEILNALDRYYFKDCRVLSDFENSISKIFNELENNEILAFLDDQAQILNQAKEHKNKILNKNINAILEFLESIKNESFKNNKHRKSYLKDIKNEIENSFKDIILKLKIFKNSQELYYFIGNIANFQTRILRRYFNAKFDLVFDDAKLKKNILRNINYLDFISTDEKANKNKILENLNAFSTLEFLKNTDPIVTIPPYENAKNKKPQSCQALVINDEKITPSLKDIAHKILSNSNFECLKTDENGVLADNIKDNEIAKYLQRILDISKGILDDKELYPRLLEKDENAKIFAQEIRLNSVELKEFKDFAKKYYDEVNLAKKGIIKNELLKPCCLHTPHKNKNKNALISALFLKSITQKEIENLEDFFANNKISGNQTFKGFFERLSELKKRYQNRFFHILEHEPTKELEGILKNYKKVMEKIVEHNSNFSFKAPFDDSTISTNFNYLTQLGDIIFDEKSRGFAKTCKFHTLENLIRSSAKSAIASRLASNSARLINGKIEMYLDRLAHEIIKKIDFTDIYNVQINVEMNKFNFESNLSKLGLAKERQKDEESFICPYSGAKISQTNCEYDHILPRSKGLYNSLANLIPTSSTSNQIKSNTKYLLSNLDENYLKYIFAKTQTTDLNSFKAFIDENISKIDENDFTNFKNLSFFEQIAFRHALFLDTDDNSFKKALRLLKLDTIKTHSNGTQKRFINILIEKISKLTKSGIDLNFIDSKLVSSTRKDLAQNDTSIAKQEIQDSHSHCVDASIVFYLANSKIIKGQIEPDYDYFKDIYPKDSDIILPQSKQYLELNQKSQKSKKLFDRSVYSLVYEGKFDEKQKKILTQYELLKENGFVDTHKVFELIFKSFKDKDTIVLKDLKFLDNHLKSYIRKDIFSIFFNEKGELKEAKELKSATKNIDKFYTILSQNQDKIYTIKLDEKAKEKKTLQRNKVIELYKEIFYTKNAKPRARGKNRVTFSLPVYAKDAKYAIKRNSGFAGLKNKDIATKTYIDIDSREILKIPYYSTNVLPIRISDILEILSLQSKNAKQIYKIKIQDNLPKQIVSLDFILSQANRHEVLVSFDKSKLEIQNINDDNGENTFIQKYLCDDFKEFLGKPRRNKIEIIKNNDDILAIKYCVESTSKANKEIIVKALSDETPSA

SEQ ID NO: 51 - protein, 1247 aa, synthetic construct
KSLSINIDMGAINNGIFIATCQDDKIIDKNAFDIKFRKGKLNFSKIDRTLRRHTRRSFDRDRFVLRLLGEILPLENLSNNQKEKLFGLFKNRGFNYLNVNFNAEIDSDNLEILNALDRYYFKDCRVLSDFENSISKIFNELENNEILAFLDDQAQILNQAKEHKNKILNKNINAILEFLESIKNESFKNNKHRKSYLKDIKNEIENSFKDIILKLKIFKNSQELYYFIGNIANFQTRILRRYFNAKFDLVFDDAKLKKNILRNINYLDFISTDEKANKNKILENLNAFSTLEFLKNTDPIVTIPPYENAKNKKPQSCQALVINDEKITPSLKDIAHKILSNSNFECLKTDENGVLADNIKDNEIAKYLQRILDISKGILDDKELYPRLLEKDENAKIFAQEIRLNSVELKEFKDFAKKYYDEVNLAKKGIIKNELLKPCCLHTPHKNKNKNALISALFLKSITQKEIENLEDFFANNKISGNQTFKGFFERLSELKKRYQWRFFHILEHEPTKELEGILKNYKKVMEKIVEHNSNFSFKAPFDDSTISTNFNYLTQLGDIIFDEKSRGFAKTCKFHTLENLIRSSAKSAIASRLASNSARLINGKIEMYLDRLAHEIIKKIDFTDIYNVQINVEMNKFNFESNLSKLGLAKERQKDEESFICPYSGAKISQTNCEYDHILPRSKGLYNSLANLIPTSSTSNQIKSNTKYLLSNLDENYLKYIFAKTQTTDLNSFKAFIDENISKIDENDFTNFKNLSFFEQIAFRHALFLDTDDNSFKKALRLLKLDTIKTHSNGTQKRFINILIEKISKLTKSGIDLNFIDSKLVSSTRKDLAQNDTSIAKQEIQDSHSHCVDASIVFYLANSKIIKGQIEPDYDYFKDIYPKDSDIILPQSKQYLELNQKSQKSKKLFDRSVYSLVYEGKFDEKQKKILTQYELLKENGFVDTHKVFELIFKSFKDKDTIVLKDLKFLDNHLKSYIRKDIFSIFFNEKGELKEAKELKSATKNIDKFYTILSQNQDKIYTIKLDEKAKEKKTLQRNKVIELYKEIFYTKNAKPRARGKNRVTFSLPVYAKDAKYAIKRNSGFAGLKNKDIATKTYIDIDSREILKIPYYSTNVLPIRISDILEILSLQSKNAKQIYKIKIQDNLPKQIVSLDFILSQANRHEVLVSFDKSKLEIQNINDDNGENTFIQKYLCDDFKEFLGKPRDNKIEIIKNNDDILAIKYCVESTSKANKEIIVKALSDETPSA

SEQ ID NO: 52 - protein, 1247 aa, synthetic construct
KSLSINIDMGAINNGIFIATCQDDKIIDKNAFDIKFRKGKLNFSKIDRTLRRHTRRSFDRDRFVLRLLGEILPLENLSNNQKEKLFGLFKNRGGNYLNVNFNAEIDSDNLEILNALDRYYFKDCRVLSDFENSISKIFNELENNEILAFLDDQAQILNQAKEHKNKILNKNINAILEFLESIKNESFKNNKHRKSYLKDIKNEIENSFKDIILKLKIFKNSQELYYFIGNIANFQTRILRRYFNAKFDLVFDDAKLKKNILRNINYLDFISTDEKANKNKILENLNAFSTLEFLKNTDPIVTIPPYENAKNKKPQSCQALVINDEKITPSLKDIAHKILSNSNFECLKTDENGVLADNIKDNEIAKYLQRILDISKGILDDKELYPRLLEKDENAKIFAQEIRLNSVELKEFKDFAKKYYDEVNLAKKGIIKNELLKPCCLHTPHKNKNKNALISALFLKSITQKEIENLEDFFANNKISGNQTFKGFFERLSELKKRYQNRFFHILEHEPTKELEGILKNYKKVMEKIVEHNSNFSFKAPFDDSTISTNFNYLTQLGDIIFDEKSRGFAKTCKFHTLENLIRSSAKSAIASRLASNSARLINGKIEMYLDRLAHEIIKKIDFTDIYNVQINVEMNKFNFESNLSKLGLAKERQKDEESFICPYSGAKISQTNCEYDHILPRSKGLYNSLANLIPTSSTSNQIKSNTKYLLSNLDENYLKYIFAKTQTTDLNSFKAFIDENISKIDENDFTNFKNLSFFEQIAFRHALFLDTDDNSFKKALRLLKLDTIKTHSNGTQKRFINILIEKISKLTKSGIDLNFIDSKLVSSTRKDLAQNDTSIAKQEIQDSHSHCVDASIVFYLANSKIIKGQIEPDYDYFKDIYPKDSDIILPQSKQYLELNQKSQKSKKLFDRSVYSLVYEGKFDEKQKKILTQYELLKENGFVDTHKVFELIFKSFKDKDTIVLKDLKFLDNHLKSYIRKDIFSIFFNEKGELKEAKELKSATKNIDKFYTILSQNQDKIYTIKLDEKAKEKKTLQRNKVIELYKEIFYTKNAKPRARGKNRVTFSLPVYAKDAKYAIKRNSGFAGLKNKDIATKTYIDIDSREILKIPYYSTNVLPIRISDILEILSLQSKNAKQIYKIKIQDNLPKQIVSLDFILSQANRHEVLVSFDKSKLEIQNINDDNGENTFIQKYLCDDFKEFLGKPRDNKIEIIKNNDDILAIKYCVESTSKANKEIIVKALSDETPSA

SEQ ID NO: 53 - protein, 1247 aa, synthetic construct
KSLSINIDMGAINNGIFIATCQDDKIIDKNAFDIKFRKGKLNFSKIDRTLRRHTRRSFDRDRFVLRLLGEILPLENLSNNQKEKLFGLFKNRGFNYLNVNFNAEIDSDNLEILNALDRYYFKDCRVLSDFENSISKIFNELENNEILAFLDDQAQILNQAKEHKNKILNKNINAILEFLESIKNESFKNNKHRKSYLKDIKNEIENSFKDIILKLKIFKNSQELYYFIGNIANFQTRILRRYFNAKFDLVFDDAKLKKNILRNINYLDFISTDEKANKNKILENLNAFSTLEFLKNTDPIVTIPPYENAKNKKPQSCQALVINDEKITPSLKDIAHKILSNSNFECLKTDENGVLADNIKDNEIAKYLQRILDISKGILDDKELYPRLLEKDENAKIFAQEIRLNSVELKEFKDFAKKYYDEVNLAKKGIIKNELLKPCCLHTPHKNKNKNALISALFLKSITQKEIENLEDFFANNKISGNQTFKGFFERLSELKKRYQNRFFHILEHEPTKELEGILKNYKKVMEKIVEHNSNFSFKAPFDDSTISTNFNYLTQLGDIIFDEKSRGFAKTCKFHTLENLIRSSAKSAIASRLASNSARLINGKIEMYLDRLAHEIIKKIDFTDIYNVQINVEMNKFNFESNLSKLGLAKERQKDEESFICPYSGAKISQTNCEYDHILPRSKGLYNSLANLIPTSSTSNQIKSNTKYLLSNLDENYLKYIFAKTQTTDLNSFKAFIDENISKIDENDFTNFKNLSFFEQIAFRHALFLDTDDNSFKKALRLLKLDTIKTHSNGTQKRFINILIEKISKLTKSGIDLNFIDSKLVSSTRKDLAQNDTSIAKQEIQDSHSHCVDASIVFYLANSKIIKGQIEPDYDYFKDIYPKDSDIILPQSKQYLELNQKSQKSKKLFDSSVYSLVYEGKFDEKQKKILTQYELLKENGFVDTHKVFELIFKSFKDKDTIVLKDLKFLDNHLKSYIRKDIFSIFFNEKGELKEAKELKSATKNIDKFYTILSQNQDKIYTIKLDEKAKEKKTLQRNKVIELYKEIFYTKNAKPRARGKNRVTFSLPVYAKDAKYAIKRNSGFAGLKNKSIATKTYIDIDSREILKIPYYSTNVLPIRISDILEILSLQSKNAKQIYKIKIQDNLPKQIVSLDFILSQARRHEVLVSFDKSKLEIQNINDDNGENTFIQKYLCDDFKEFLGKPRDNKIEIIKNNDDILAIKYCVESTRKANKEIIVKALSDETPSA

SEQ ID NO: 54 - protein, 1247 aa, synthetic construct
KSLSINIDMGAINNGIFIATCQDDKIIDKNAFDIKFRKGKLNFSKIDRTLRRHTRRSFDRDRFVLRLLGEILPLENLSNNQKEKLFGLFKNRGFNYLNVNFNAEIDSDNLEILNALDRYYFKDCRVLSDFENSISKIFNELENNEILAFLDDQAQILNQAKEHKNKILNKNINAILEFLESIKNESFKNNKHRKSYLKDIKNEIENSFKDIILKLKIFKNSQELYYFIGNIANFQTRILRRYFNAKFDLVFDDAKLKKNILRNINYLDFISTDEKANKNKILENLNAFSTLEFLKNTDPIVTIPPYENAKNKKPQSCQALVINDEKITPSLKDIAHKILSNSNFECLKTDENGVLADNIKDNEIAKYLQRILDISKGILDDKELYPRLLEKDENAKIFAQEIRLNSVELKEFKDFAKKYYDEVNLAKKGIIKNELLKPCCLHTPHKNKNKNALISALFLKSITQKEIENLEDFFANNKISGNQTFKGFFERLSELKKRYQNRFFHILEHEPTKELEGILKNYKKVMEKIVEHNSNFSFKAPFDDSTISTNFNYLTQLGDIIFDEKSRGFAKTCKFHTLENLIRSSAKSAIASRLASNSARLINGKIEMYLDRLAHEIIKKIDFTDIYNVQINVEMNKFNFESNLSKLGLAKERQKDEESFICPYSGAKISQTNCEYDHILPRSKGLYNSLANLIPTSSTSNQIKSNTKYLLSNLDENYLKYIFAKTQTTDLNSFKAFIDENISKIDENDFTNFKNLSFFEQIAFRHALFLDTDDNSFKKALRLLKLDTIKTHSNGTQKRFINILIEKISKLTKSGIDLNFIDSKLVSSTRKDLAQNDTSIAKQEIQDSHSHCVDASIVFYLANSKIIKGQIEPDYDYFKDIYPKDSDIILPQSKQYLELNQKSQKSKKLFDNSVYSLVYEGKFDEKQKKILTQYELLKENGFVDTHKVFELIFKSFKDKDTIVLKDLKFLDNHLKSYIRKDIFSIFFNEKGELKEAKELKSATKNIDKFYTILSQNQDKIYTIKLDEKAKEKKTLQRNKVIELYKEIFYTKNAKPRARGKNRVTFSLPVYAKDAKYAIKRNSGFAGLKNKSIATKTYIDIDSREILKIPYYSTNVLPIRISDILEILSLQSKNAKQIYKIKIQDNLPKQIVSLDFILSQARRHEVLVSFDKSKLEIQNINDDNGENTFIQKYLCDDFKEFLGKPRDNKIEIIKNNDDILAIKYCVESTRKANKEIIVKALSDETPSA

SEQ ID NO: 55 - protein, 1247 aa, synthetic construct
KSLSINIDMGAINNGIFIATCQDDKIIDKNAFDIKFRKGKLNFSKIDRTLRRHTRRSFDRDRFVLRLLGEILPLENLSNNQKEKLFGLFKNRGFNYLNVNFNAEIDSDNLEILNALDRYYFKDCRVLSDFENSISKIFNELENNEILAFLDDQAQILNQAKEHKNKILNKNINAILEFLESIKNESFKNNKHRKSYLKDIKNEIENSFKDIILKLKIFKNSQELYYFIGNIANFQTRILRRYFNAKFDLVFDDAKLKKNILRNINYLDFISTDEKANKNKILENLNAFSTLEFLKNTDPIVTIPPYENAKNKKPQSCQALVINDEKITPSLKDIAHKILSNSNFECLKTDENGVLADNIKDNEIAKYLQRILDISKGILDDKELYPRLLEKDENAKIFAQEIRLNSVELKEFKDFAKKYYDEVNLAKKGIIKNELLKPCCLHTPHKNKNKNALISALFLKSITQKEIENLEDFFANNKISGNQTFKGFFERLSELKKRYQNRFFHILEHEPTKELEGILKNYKKVMEKIVEHNSNFSFKAPFDDSTISTNFNYLTQLGDIIFDEKSRGFAKTCKFHTLENLIRSSAKSAIASRLASNSARLINGKIEMYLDRLAHEIIKKIDFTDIYNVQINVEMNKFNFESNLSKLGLAKERQKDEESFICPYSGAKISQTNCEYDHILPRSKGLYNSLANLIPTSSTSNQIKSNTKYLLSNLDENYLKYIFAKTQTTDLNSFKAFIDENISKIDENDFTNFKNLSFFEQIAFRHALFLDTDDNSFKKALRLLKLDTIKTHSNGTQKRFINILIEKISKLTKSGIDLNFIDSKLVSSTRKDLAQNDTSIAKQEIQDSHSHCVDASIVFYLANSKIIKGQIEPDYDYFKDIYPKDSDIILPQSKQYLELNQKSQKSKKLFDRSVYSLVYEGKFDEKQKKILTQYELLKENGFVDTHKVFELIFKSFKDKDTIVLKDLKFLDNHLKSYIRKDIFSIFFNEKGELKEAKELKSATKNIDKFYTILSQNQDKIYTIKLDEKAKEKKTLQRNKVIELYKEIFYTKNAKPRARGKNRVTFSLPVYAKDAKYAIKRNSGFAGLKNKSIATKTYIDIDSREILKIPYYSTNVLPIRISDILEILSLQSKNAKQIYKIKIQDNLPKQIVSLDFILSQARRHEVLVSFDKSKLEIQNINDDNGENTFIQKYLCDDFKEFLGKPRSNKIEIIKNNDDILAIKYCVESTSKANKEIIVKALSDETPSA

SEQ ID NO: 56 - protein, 1247 aa, synthetic construct
KSLSINIDMGAINNGIFIATCQDDKIIDKNAFDIKFRKGKLNFSKIDRTLRRHTRRSFDRDRFVLRLLGEILPLENLSNNQKEKLFGLFKNRGFNYLNVNFNAEIDSDNLEILNALDRYYFKDCRVLSDFENSISKIFNELENNEILAFLDDQAQILNQAKEHKNKILNKNINAILEFLESIKNESFKNNKHRKSYLKDIKNEIENSFKDIILKLKIFKNSQELYYFIGNIANFQTRILRRYFNAKFDLVFDDAKLKKNILRNINYLDFISTDEKANKNKILENLNAFSTLEFLKNTDPIVTIPPYENAKNKKPQSCQALVINDEKITPSLKDIAHKILSNSNFECLKTDENGVLADNIKDNEIAKYLQRILDISKGILDDKELYPRLLEKDENAKIFAQEIRLNSVELKEFKDFAKKYYDEVNLAKKGIIKNELLKPCCLHTPHKNKNKNALISALFLKSITQKEIENLEDFFANNKISGNQTFKGFFERLSELKKRYQNRFFHILEHEPTKELEGILKNYKKVMEKIVEHNSNFSFKAPFDDSTISTNFNYLTQLGDIIFDEKSRGFAKTCKFHTLENLIRSSAKSAIASRLASNSARLINGKIEMYLDRLAHEIIKKIDFTDIYNVQINVEMNKFNFESNLSKLGLAKERQKDEESFICPYSGAKISQTNCEYDHILPRSKGLYNSLANLIPTSSTSNQIKSNTKYLLSNLDENYLKYIFAKTQTTDLNSFKAFIDENISKIDENDFTNFKNLSFFEQIAFRHALFLDTDDNSFKKALRLLKLDTIKTHSNGTQKRFINILIEKISKLTKSGIDLNFIDSKLVSSTRKDLAQNDTSIAKQEIQDSHSHCVDASIVFYLANSKIIKGQIEPDYDYFKDIYPKDSDIILPQSKQYLELNQKSQKSKKLFDDSVYSLVYEGKFDEKQKKILTQYELLKENGFVDTHKVFELIFKSFKDKDTIVLKDLKFLDNHLKSYIRKDIFSIFFNEKGELKEAKELKSATKNIDKFYTILSQNQDKIYTIKLDEKAKEKKTLQRNKVIELYKEIFYTKNAKPRARGKNRVTFSLPVYAKDAKYAIKRNSGFAGLKNKSIATKTYIDIDSREILKIPYYSTNVLPIRISDILEILSLQSKNAKQIYKIKIQDNLPKQIVSLDFILSQARRHEVLVSFDKSKLEIQNINDDNGENTFIQKYLCDDFKEFLGKPRSNKIEIIKNNDDILAIKYCVGSTSKANKEIIVKALSDETPSA

SEQ ID NO: 57 - protein, 1247 aa, synthetic construct
KSLSINIDMGAINNGIFIATCQDDKIIDKNAFDIKFRKGKLNFSKIDRTLRRHTRRSFDRDRFVLRLLGEILPLENLSNNQKEKLFGLFKNRGFNYLNVNFNAEIDSDNLEILNALDRYYFKDCRVLSDFENSISKIFNELENNEILAFLDDQAQILNQAKEHKNKILNKNINAILEFLESIKNESFKNNKHRKSYLKDIKNEIENSFKDIILKLKIFKNSQELYYFIGNIANFQTRILRRYFNAKFDLVFDDAKLKKNILRNINYLDFISTDEKANKNKILENLNAFSTLEFLKNTDPIVTIPPYENAKNKKPQSCQALVINDEKITPSLKDIAHKILSNSNFECLKTDENGVLADNIKDNEIAKYLQRILDISKGILDDKELYPRLLEKDENAKIFAQEIRLNSVELKEFKDFAKKYYDEVNLAKKGIIKNELLKPCCLHTPHKNKNKNALISALFLKSITQKEIENLEDFFANNKISGNQTFKGFFERLSELKKRYQNRFFHILEHEPTKELEGILKNYKKVMEKIVEHNSNFSFKAPFDDSTISTNFNYLTQLGDIIFDEKSRGFAKTCKFHTLENLIRSSAKSAIASRLASNSARLINGKIEMYLDRLAHEIIKKIDFTDIYNVQINVEMNKFNFESNLSKLGLAKERQKDEESFICPYSGAKISQTNCEYDHILPRSKGLYNSLANLIPTSSTSNQIKSNTKYLLSNLDENYLKYIFAKTQTTDLNSFKAFIDENISKIDENDFTNFKNLSFFEQIAFRHALFLDTDDNSFKKALRLLKLDTIKTHSNGTQKRFINILIEKISKLTKSGIDLNFIDSKLVSSTRKDLAQNDTSIAKQEIQDSHSHCVDASIVFYLANSKIIKGQIEPDYDYFKDIYPKDSDIILPQSKQYLELNQKSQKSKKLFDDSVYSLVYEGKFDEKQKKILTQYELLKENGFVDTHKVFELIFKSFKDKDTIVLKDLKFLDNHLKSYIRKDIFSIFFNEKGELKEAKELKSATKNIDKFYTILSQNQDKIYTIKLDEKAKEKKTLQRNKVIELYKEIFYTKNAKPRARGKNRVTFSLPVYAKDAKYAIKRNSGFAGLKNKSIATKTYIDIDSREILKIPYYSTNVLPIRISDILEILSLQSKNAKQIYKIKIQDNLPKQIVSLDFILSQARRHEVLVSFDKSKLEIQNINDDNGENTFIQKYLCDDFKEFLGKPRSNKIEIIKNNDDILAIKYCVESTRKANKEIIVKALSDETPSA

SEQ ID NO: 58 - protein, 1247 aa, synthetic construct
KSLSINIDMGAINNGIFIATCQDDKIIDKNAFDIKFRKGKLNFSKIDRTLRRHTRRSFDRDRFVLRLLGEILPLENLSNNQKEKLFGLFKNRGFNYLNVNFNAEIDSDNLEILNALDRYYFKDCRVLSDFENSISKIFNELENNEILAFLDDQAQILNQAKEHKNKILNKNINAILEFLESIKNESFKNNKHRKSYLKDIKNEIENSFKDIILKLKIFKNSQELYYFIGNIANFQTRILRRYFNAKFDLVFDDAKLKKNILRNINYLDFISTDEKANKNKILENLNAFSTLEFLKNTDPIVTIPPYENAKNKKPQSCQALVINDEKITPSLKDIAHKILSNSNFECLKTDENGVLADNIKDNEIAKYLQRILDISKGILDDKELYPRLLEKDENAKIFAQEIRLNSVELKEFKDFAKKYYDEVNLAKKGIIKNELLKPCCLHTPHKNKNKNALISALFLKSITQKEIENLEDFFANNKISGNQTFKGFFERLSELKKRYQNRFFHILEHEPTKELEGILKNYKKVMEKIVEHNSNFSFKAPFDDSTISTNFNYLTQLGDIIFDEKSRGFAKTCKFHTLENLIRSSAKSAIASRLASNSARLINGKIEMYLDRLAHEIIKKIDFTDIYNVQINVEMNKFNFESNLSKLGLAKERQKDEESFICPYSGAKISQTNCEYDHILPRSKGLYNSLANLIPTSSTSNQIKSNTKYLLSNLDENYLKYIFAKTQTTDLNSFKAFIDENISKIDENDFTNFKNLSFFEQIAFRHALFLDTDDNSFKKALRLLKLDTIKTHSNGTQKRFINILIEKISKLTKSGIDLNFIDSKLVSSTRKDLAQNDTSIAKQEIQDSHSHCVDASIVFYLANSKIIKGQIEPDYDYFKDIYPKDSDIILPQSKQYLELNQKSQKSKKLFDRSVYSLVYEGKFDEKQKKILTQYELLKENGFVDTHKVFELIFKSFKDKDTIVLKDLKFLDNHLKSYIRKDIFSIFFNEKGELKEAKELKSATKNIDKFYTILSQNQDKIYTIKLDEKAKEKKTLQRNKVIELYKEIFYTKNAKPRARGKNRVTFSLPVYAKDAKYAIKRNSGFAGLKNKSIATKTYIDIDSREILKIPYYSTNVLPIRISDILEILSLQSKNAKQIYKIKIQDNLPKQIVSLDFILSQANRHEVLVSFDKSKLEIQNINDDNGENTFIQKYLCDDFKEFLGKPRSNKIEIIKNNDDILAIKYCVESTSKANKEIIVKALSDETPSA

SEQ ID NO: 59 - protein, 1247 aa, synthetic construct
KSLSINIDMGAINNGIFIATCQDDKIIDKNAFDIKFRKGKLNFSKIDRTLRRHTRRSFDRDRFVLRLLGEILPLENLSNNQKEKLFGLFKNRGFNYLNVNFNAEIDSDNLEILNALDRYYFKDCRVLSDFENSISKIFNELENNEILAFLDDQAQILNQAKEHKNKILNKNINAILEFLESIKNESFKNNKHRKSYLKDIKNEIENSFKDIILKLKIFKNSQELYYFIGNIANFQTRILRRYFNAKFDLVFDDAKLKKNILRNINYLDFISTDEKANKNKILENLNAFSTLEFLKNTDPIVTIPPYENAKNKKPQSCQALVINDEKITPSLKDIAHKILSNSNFECLKTDENGVLADNIKDNEIAKYLQRILDISKGILDDKELYPRLLEKDENAKIFAQEIRLNSVELKEFKDFAKKYYDEVNLAKKGIIKNELLKPCCLHTPHKNKNKNALISALFLKSITQKEIENLEDFFANNKISGNQTFKGFFERLSELKKRYQNRFFHILEHEPTKELEGILKNYKKVMEKIVEHNSNFSFKAPFDDSTISTNFNYLTQLGDIIFDEKRRGFAKTCKFHTLENLIRSSAKSAIASRLASNSARLINGKIEMYLDRLAHEIIKKIDFTDIYNVQINVEMNKFNFESNLSKLGLAKERQKDEESFICPYSGAKISQTNCEYDHILPRSKGLYNSLANLIPTSSTSNQIKSNTKYLLSNLDENYLKYIFAKTQTTDLNSFKAFIDENISKIDENDFTNFKNLSFFEQIAFRHALFLDTDDNSFKKALRLLKLDTIKTHSNGTQKRFINILIEKISKLTKSGIDLNFIDSKLVSSTRKDLAQNDTSIAKQEIQDSHSHCVDASIVFYLANSKIIKGQIEPDYDYFKDIYPKDSDIILPQSKQYLELNQKSQKSKKLFDRSVYSLVYEGKFDEKQKKILTQYELLKENGFVDTHKVFELIFKSFKDKDTIVLKDLKFLDNHLKSYIRKDIFSIFFNEKGELKEAKELKSATKNIDKFYTILSQNQDKIYTIKLDEKAKEKKTLQRNKVIELYKEIFYTKNAKPRARGKNRVTFSLPVYAKDAKYAIKRNSGFAGLKNKSIATKTYIDIDSREILKIPYYSTNVLPIRISDILEILSLQSKNAKQIYKIKIQDNLPKQIVSLDFILSQANRHEVLVSFDKSKLEIQNINDDNGENTFIQKYLCDDFKEFLGKPRDNKIEIIKNNDDILAIKYCVESTSKANKEIIVKALSDETPSA

SEQ ID NO: 60 - protein, 1247 aa, synthetic construct
KSLSINIDMGAINNGIFIATCQDDKIIDKNAFDIKFRKGKLNFSKIDRTLRRHTRRSFDRDRFVLRLLGEILPLENLSNNQKEKLFGLFKNRGFNYLNVNFNAEIDSDNLEILNALDRYYFKDCRVLSDFENSISKIFNELENNEILAFLDDQAQILNQAKEHKNKILNKNINAILEFLESIKNESFKNNKHRKSYLKDIKNEIENSFKDIILKLKIFKNSQELYYFIGNIANFQTRILRRYFNAKFDLVFDDAKLKKNILRNINYLDFISTDEKANKNKILENLNAFSTLEFLKNTDPIVTIPPYENAKNKKPQSCQALVINDEKITPSLKDIAHKILSNSNFECLKTDENGVLADNIKDNEIAKYLQRILDISKGILDDKELYPRLLEKDENAKIFAQEIRLNSVELKEFKDFAKKYYDEVNLAKKGIIKNELLKPCCLHTPHKNKNKNALISALFLKSITQKEIENLEDFFANNKISGNQTFKGFFERLSELKKRYQNRFFHILEHEPTKELEGILKNYKKVMEKIVEHNSNFSFKAPFDDSTISTNFNYLTQLGDIIFDEKSRGFAKTCKFHTLENLIRSSAKSAIASRLASNSARLINGKIEMYLDRLAHEIIKKIDFTDIYNVQINVEMNKFNFESNLSKLGLAKERQKDEESFICPYSGAKISQTNCEYDHILPRSKGLYNSLANLIPTSSTSNQIKSNTKYLLSNLDENYLKYIFAKTQTTDLNSFKAFIDENISKIDENDFTNFKNLSFFEQIAFRHALFLDTDDNSFKKALRLLKLDTIKTHSNGTQKRFINILIEKISKLTKSGIDLNFIDSKLVSSTRKDLAQNDTSIAKQEIQDSHSHCVDASIVFYLANSKIIKGQIEPDYDYFKDIYPKDSDIILPQSKQYLELNQKSQKSKKLFDDSVYSLVYEGKFDEKQKKILTQYELLKENGFVDTHKVFELIFKSFKDKDTIVLKDLKFLDNHLKSYIRKDIFSIFFNEKGELKEAKELKSATKNIDKFYTILSQNQDKIYTIKLDEKAKEKKTLQRNKVIELYKEIFYTKNAKPRARGKNRVTFSLPVYAKDAKYAIKRNSGFAGLKNKDIATKTYIDIDSREILKIPYYSTNVLPIRISDILEILSLQSKNAKQIYKIKIQDNLPKQIVSLDFILSQARRHEVLVSFDKSKLEIQNINDDNGENTFIQKYLCDDFKEFLGKPRDNKIEIIKNNDDILAIKYCVESTSKANKEIIVKALSDETPSA

SEQ ID NO: 61 - protein, 1247 aa, synthetic construct
KSLSINIDMGAINNGIFIATCQDDKIIDKNAFDIKFRKGKLNFSKIDRTLRRHTRRSFDRDRFVLRLLGEILPLENLSNNQKEKLFGLFKNRGFNYLNVNFNAEIDSDNLEILNALDRYYFKDCRVLSDFENSISKIFNELENNEILAFLDDQAQILNQAKEHKNKILNKNINAILEFLESIKNESFKNNKHRKSYLKDIKNEIENSFKDIILKLKIFKNSQELYYFIGNIANFQTRILRRYFNAKFDLVFDDAKLKKNILRNINYLDFISTDEKANKNKILENLNAFSTLEFLKNTDPIVTIPPYENAKNKKPQSCQALVINDEKITPSLKDIAHKILSNSNFECLKTDENGVLADNIKDNEIAKYLQRILDISKGILDDKELYPRLLEKDENAKIFAQEIRLNSVELKEFKDFAKKYYDEVNLAKKGIIKNELLKPCCLHTPHKNKNKNALISALFLKSITQKEIENLEDFFANNKISGNQTFKGFFERLSELKKRYQNRFFHILEHEPTKELEGILKNYKKVMEKIVEHNSNFSFKAPFDDSTISTNFNYLTQLGDIIFDEKSRGFAKTCKFHTLENLIRSSAKSAIASRLASNSARLINGKIEMYLDRLAHEIIKKIDFTDIYNVQINVEMNKFNFESNLSKLGLAKERQKDEESFICPYSGAKISQTNCEYDHILPRSKGLYNSLANLIPTSSTSNQIKSNTKYLLSNLDENYLKYIFAKTQTTDLNSFKAFIDENISKIDENDFTNFKNLSFFEQIAFRHALFLDTDDNSFKKALRLLKLDTIKTHSNGTQKRFINILIEKISKLTKSGIDLNFIDSKLVSSTRKDLAQNDTSIAKQEIQDSHSHCVDASIVFYLANSKIIKGQIEPDYDYFKDIYPKDSDIILPQSKQYLELNQKSQKSKKLFDRSVYSLVYEGKFDEKQKKILTQYELLKENGFVDTHKVFELIFKSFKDKDTIVLKDLKFLDNHLKSYIRKDIFSIFFNEKGELKEAKELKSATKNIDKFYTILSQNQDKIYTIKLDEKAKEKKTLQRNKVIELYKEIFYTKNAKPRARGKNRVTFSLPVYAKDAKYAIKRNSGFAGLKNKDIATKTYIDIDSREILKIPYYSTNVLPIRISDILEILSLQSKNAKQIYKIKIQDNLPKQIVSLDFILSQANRHEVLVSFDKSKLEIQNINDDNGENTFIQKYLCDDFKEFLGKPRDNKIEIIKNNDDILAIKYCVESTSKANKEIIVKALSDETPSA

SEQ ID NO: 62 - protein, 1247 aa, synthetic construct
KSLSINIDMGAINNGIFIATCQDDKIIDKNAFDIKFRKGKLNFSKIDRTLRRHTRRSFDRDRFVLRLLGEILPLENLSNNQKEKLFGLFKNRGFNYLNVNFNAEIDSDNLEILNALDRYYFKDCRVLSDFENSISKIFNELENNEILAFLDDQAQILNQAKEHKNKILNKNINAILEFLESIKNESFKNNKHRKSYLKDIKNEIENSFKDIILKLKIFKNSQELYYFIGNIANFQTRILRRYFNAKFDLVFDDAKLKKNILRNINYLDFISTDEKANKNKILENLNAFSTLEFLKNTDPIVTIPPYENAKNKKPQSCQALVINDEKITPSLKDIAHKILSNSNFECLKTDENGVLADNIKDNEIAKYLQRILDISKGILDDKELYPRLLEKDENAKIFAQEIRLNSVELKEFKDFAKKYYDEVNLAKKGIIKNELLKPCCLHTPHKNKNKNALISALFLKSITQKEIENLEDFFANNKISGNQTFKGFFERLSELKKRYQNRFFHILEHEPTKELEGILKNYKKVMEKIVEHNSNFSFKAPFDDSTISTNFNYLTQLGDIIFDEKSRGFAKTCKFHTLENLIRSSAKSAIASRLASNSARLINGKIEMYLDRLAHEIIKKIDFTDIYNVQINVEMNKFNFESNLSKLGLAKERQKDEESFICPYSGAKISQTNCEYDHILPRSKGLYNSLANLIPTSSTSNQIKSNTKYLLSNLDENYLKYIFAKTQTTDLNSFKAFIDENISKIDENDFTNFKNLSFFEQIAFRHALFLDTDDNSFKKALRLLKLDTIKTHSNGTQKRFINILIEKISKLTKSGIDLNFIDSKLVSSTRKDLAQNDTSIAKQEIQDSHSHCVDASIVFYLANSKIIKGQIEPDYDYFKDIYPKDSDIILPQSKQYLELNQKSQKSKKLFDDSVYSLVYEGKFDEKQKKILTQYELLKENGFVDTHKVFELIFKSFKDKDTIVLKDLKFLDNHLKSYIRKDIFSIFFNEKGELKEAKELKSATKNIDKFYTILSQNQDKIYTIKLDEKAKEKKTLQRNKVIELYKEIFYTKNAKPRARGKNRVTFSLPVYAKDAKYAIKRNSGFAGLKNKDIATKTYIDIDSREILKIPYYSTNVLPIRISDILEILSLQSKNAKQIYKIKIQDNLPKQIVSLDFILSQANRHEVLVSFDKSKLEIQNINDDNGENTFIQKYLCDDFKEFLGKPRDNKIEIIKNNDDILAIKYCVESTRKANKEIIVKALSDETPSA

SEQ ID NO: 63 - protein, 1247 aa, synthetic construct
KSLSINIDMGAINNGIFIATCQDDKIIDKNAFDIKFRKRKLNFSKIDRTLRRHTRRSFDRDRFVLRLLGEILPLENLSNNQKEKLFGLFKNRGFNYLNVNFNAEIDSDNLEILNALDRYYFKDCRVLSDFENSISKIFNELENNEILAFLDDQAQILNQAKEHKNKILNKNINAILEFLESIKNESFKNNKHRKSYLKDIKNEIENSFKDIILKLKIFKNSQELYYFIGNIANFQTRILRRYFNAKFDLVFDDAKLKKNILRNINYLDFISTDEKANKNKILENLNAFSTLEFLKNTDPIVTIPPYENAKNKKPQSCQALVINDEKITPSLKDIAHKILSNSNFECLKTDENGVLADNIKDNEIAKYLQRILDISKGILDDKELYPRLLEKDENAKIFAQEIRLNSVELKEFKDFAKKYYDEVNLAKKGIIKNELLKPCCLHTPHKNKNKNALISALFLKSITQKEIENLEDFFANNKISGNQTFKGFFERLSELKKRYQNRFFHILEHEPTKELEGILKNYKKVMEKIVEHNSNFSFKAPFDDSTISTNFNYLTQLGDIIFDEKSRGFAKTCKFHTLENLIRSSAKSAIASRLASNSARLINGKIEMYLDRLAHEIIKKIDFTDIYNVQINVEMNKFNFESNLSKLGLAKERQKDEESFICPYSGAKISQTNCEYDHILPRSKGLYNSLANLIPTSSTSNQIKSNTKYLLSNLDENYLKYIFAKTQTTDLNSFKAFIDENISKIDENDFTNFKNLSFFEQIAFRHALFLDTDDNSFKKALRLLKLDTIKTHSNGTQKRFINILIEKISKLTKSGIDLNFIDSKLVSSTRKDLAQNDTSIAKQEIQDSHSHCVDASIVFYLANSKIIKGQIEPDYDYFKDIYPKDSDIILPQSKQYLELNQKSQKSKKLFDDSVYSLVYEGKFDEKQKKILTQYELLKENGFVDTHKVFELIFKSFKDKDTIVLKDLKFLDNHLKSYIRKDIFSIFFNEKGELKEAKELKSATKNIDKFYTILSQNQDKIYTIKLDEKAKEKKTLQRNKVIELYKEIFYTKNAKPRARGKNRVTFSLPVYAKDAKYAIKRNSGFAGLKNKDIATKTYIDIDSREILKIPYYSTNVLPIRISDILEILSLQSKNAKQIYKIKIQDNLPKQIVSLDFILSQANRHEVLVSFDKSKLEIQNINDDNGENTFIQKYLCDDFKEFLGKPRDNKIEIIKNNDDILAIKYCVESTSKANKEIIVKALSDETPSA

SEQ ID NO: 64 - protein, 1247 aa, synthetic construct
KSLSINIDMGAINNGIFIATCQDDKIIDKNAFDIKFDKGKLNFSKIDRTLRRHTRRSFDRDRFVLRLLGEILPLENLSNNQKEKLFGLFKNRGFNYLNVNFNAEIDSDNLEILNALDRYYFKDCRVLSDFENSISKIFNELENNEILAFLDDQAQILNQAKEHKNKILNKNINAILEFLESIKNESFKNNKHRKSYLKDIKNEIENSFKDIILKLKIFKNSQELYYFIGNIANFQTRILRRYFNAKFDLVFDDAKLKKNILRNINYLDFISTDEKANKNKILENLNAFSTLEFLKNTDPIVTIPPYENAKNKKPQSCQALVINDEKITPSLKDIAHKILSNSNFECLKTDENGVLADNIKDNEIAKYLQRILDISKGILDDKELYPRLLEKDENAKIFAQEIRLNSVELKEFKDFAKKYYDEVNLAKKGIIKNELLKPCCLHTPHKNKNKNALISALFLKSITQKEIENLEDFFANNKISGNQTFKGFFERLSELKKRYQNRFFHILEHEPTKELEGILKNYKKVMEKIVEHNSNFSFKAPFDDSTISTNFNYLTQLGDIIFDEKSRGFAKTCKFHTLENLIRSSAKSAIASRLASNSARLINGKIEMYLDRLAHEIIKKIDFTDIYNVQINVEMNKFNFESNLSKLGLAKERQKDEESFICPYSGAKISQTNCEYDHILPRSKGLYNSLANLIPTSSTSNQIKSNTKYLLSNLDENYLKYIFAKTQTTDLNSFKAFIDENISKIDENDFTNFKNLSFFEQIAFRHALFLDTDDNSFKKALRLLKLDTIKTHSNGTQKRFINILIEKISKLTKSGIDLNFIDSKLVSSTRKDLAQNDTSIAKQEIQDSHSHCVDASIVFYLANSKIIKGQIEPDYDYFKDIYPKDSDIILPQSKQYLELNQKSQKSKKLFDDSVYSLVYEGKFDEKQKKILTQYELLKENGFVDTHKVFELIFKSFKDKDTIVLKDLKFLDNHLKSYIRKDIFSIFFNEKGELKEAKELKSATKNIDKFYTILSQNQDKIYTIKLDEKAKEKKTLQRNKVIELYKEIFYTKNAKPRARGKNRVTFSLPVYAKDAKYAIKRNSGFAGLKNKRIATKTYIDIDSREILKIPYYSTNVLPIRISDILEILSLQSKNAKQIYKIKIQDNLPKQIVSLDFILSQARRHEVLVSFDKSKLEIQNINDDNGENTFIQKYLCDDFKEFLGKPRDNKIEIIKNNDDILAIKYCVESTSKANKEIIVKALSDETPSA

SEQ ID NO: 65 - protein, 1247 aa, synthetic construct
KSLSINIDMGAINNGIFIATCQDDKIIDKNAFDIKFDKGKLNFSKIDRTLRRHTRRSFDRDRFVLRLLGEILPLENLSNNQKEKLFGLFKNRGFNYLNVNFNAEIDSDNLEILNALDRYYFKDCRVLSDFENSISKIFNELENNEILAFLDDQAQILNQAKEHKNKILNKNINAILEFLESIKNESFKNNKHRKSYLKDIKNEIENSFKDIILKLKIFKNSQELYYFIGNIANFQTRILRRYFNAKFDLVFDDAKLKKNILRNINYLDFISTDEKANKNKILENLNAFSTLEFLKNTDPIVTIPPYENAKNKKPQSCQALVINDEKITPSLKDIAHKILSNSNFECLKTDENGVLADNIKDNEIAKYLQRILDISKGILDDKELYPRLLEKDENAKIFAQEIRLNSVELKEFKDFAKKYYDEVNLAKKGIIKNELLKPCCLHTPHKNKNKNALISALFLKSITQKEIENLEDFFANNKISGNQTFKGFFERLSELKKRYQNRFFHILEHEPTKELEGILKNYKKVMEKIVEHNSNFSFKAPFDDSTISTNFNYLTQLGDIIFDEKSRGFAKTCKFHTLENLIRSSAKSAIASRLASNSARLINGKIEMYLDRLAHEIIKKIDFTDIYNVQINVEMNKFNFESNLSKLGLAKERQKDEESFICPYSGAKISQTNCEYDHILPRSKGLYNSLANLIPTSSTSNQIKSNTKYLLSNLDENYLKYIFAKTQTTDLNSFKAFIDENISKIDENDFTNFKNLSFFEQIAFRHALFLDTDDNSFKKALRLLKLDTIKTHSNGTQKRFINILIEKISKLTKSGIDLNFIDSKLVSSTRKDLAQNDTSIAKQEIQDSHSHCVDASIVFYLANSKIIKGQIEPDYDYFKDIYPKDSDIILPQSKQYLELNQKSQKSKKLFDDSVYSLVYEGKFDEKQKKILTQYELLKENGFVDTHKVFELIFKSFKDKDTIVLKDLKFLDNHLKSYIRKDIFSIFFNEKGELKEAKELKSATKNIDKFYTILSQNQDKIYTIKLDEKAKEKKTLQRNKVIELYKEIFYTKNAKPRARGKNRVTFSLPVYAKDAKYAIKRNSGFAGLKNKRIATKTYIDIDSREILKIPYYSTNVLPIRISDILEILSLQSKNAKQIYKIKIQDNLPKQIVSLDFILSQANRHEVLVSFDKSKLEIQNINDDNGENTFIQKYLCDDFKEFLGKPRDNKIEIIKNNDDILAIKYCVESTRKANKEIIVKALSDETPSA

SEQ ID NO: 66 - protein, 1247 aa, synthetic construct
KSLSINIDMGAINNGIFIATCQDDKIIDKNAFDIKFRKGKLNFSKIDRTLRRHTRRSFDRDRFVLRLLGEILPLENLSNNQKEKLFGLFKNRGFNYLNVNFNAEIDSDNLEILNALDRYYFKDCRVLSDFENSISKIFNELENNEILAFLDDQAQILNQAKEHKNKILNKNINAILEFLESIKNESFKNNKHRKSYLKDIKNEIENSFKDIILKLKIFKNSQELYYFIGNIANFQTRILRRYFNAKFDLVFDDAKLKKNILRNINYLDFISTDEKANKNKILENLNAFSTLEFLKNTDPIVTIPPYENAKNKKPQSCQALVINDEKITPSLKDIAHKILSNSNFECLKTDENGVLADNIKDNEIAKYLQRILDISKGILDDKELYPRLLEKDENAKIFAQEIRLNSVELKEFKDFAKKYYDEVNLAKKGIIKNELLKPCCLHTPHKNKNKNALISALFLKSITQKEIENLEDFFANNKISGNQTFKGFFERLSELKKRYQNRFFHILEHEPTKELEGILKNYKKVMEKIVEHNSNFSFKAPFDDSTISTNFNYLTQLGDIIFDEKSRGFAKTCKFHTLENLIRSSAKSAIASRLASNSARLINGKIEMYLDRLAHEIIKKIDFTDIYNVQINVEMNKFNFESNLSKLGLAKERQKDEESFICPYSGAKISQTNCEYDHILPRSKGLYNSLANLIPTSSTSNQIKSNTKYLLSNLDENYLKYIFAKTQTTDLNSFKAFIDENISKIDENDFTNFKNLSFFEQIAFRHALFLDTDDNSFKKALRLLKLDTIKTHSNGTQKRFINILIEKISKLTKSGIDLNFIDSKLVSSTRKDLAQNDTSIAKQEIQDSHSHCVDASIVFYLANSKIIKGQIEPDYDYFKDIYPKDSDIILPQSKQYLELNQKSQKSKKLFDGSVYSLVYEGKFDEKQKKILTQYELLKENGFVDTHKVFELIFKSFKDKDTIVLKDLKFLDNHLKSYIRKDIFSIFFNEKGELKEAKELKSATKNIDKFYTILSQNQDKIYTIKLDEKAKEKKTLQRNKVIELYKEIFYTKNAKPRARGKNRVTFSLPVYAKDAKYAIKRNSGFAGLKNKDIATKTYIDIDSREILKIPYYSTNVLPIRISDILEILSLQSKNAKQIYKIKIQDNLPKQIVSLDFILSQARRHEVLVSFDKSKLEIQNINDDNGENTFIQKYLCDDFKEFLGKPRDNKIEIIKNNDDILAIKYCVESTSKANKEIIVKALSDETPSA

SEQ ID NO: 67 - protein, 1247 aa, synthetic construct
KSLSINIDMGAINNGIFIATCQDDKIIDKNAFDIKFRKGKLNFSKIDRTLRRHTRRSFDRDRFVLRLLGEILPLENLSNNQKEKLFGLFKNRGFNYLNVNFNAEIDSDNLEILNALDRYYFKDCRVLSDFENSISKIFNELENNEILAFLDDQAQILNQAKEHKNKILNKNINAILEFLESIKNESFKNNKHRKSYLKDIKNEIENSFKDIILKLKIFKNSQELYYFIGNIANFQTRILRRYFNAKFDLVFDDAKLKKNILRNINYLDFISTDEKANKNKILENLNAFSTLEFLKNTDPIVTIPPYENAKNKKPQSCQALVINDEKITPSLKDIAHKILSNSNFECLKTDENGVLADNIKDNEIAKYLQRILDISKGILDDKELYPRLLEKDENAKIFAQEIRLNSVELKEFKDFAKKYYDEVNLAKKGIIKNELLKPCCLHTPHKNKNKNALISALFLKSITQKEIENLEDFFANNKISGNQTFKGFFERLSELKKRYQNRFFHILEHEPTKELEGILKNYKKVMEKIVEHNSNFSFKAPFDDSTISTNFNYLTQLGDIIFDEKSRGFAKTCKFHTLENLIRSSAKSAIASRLASNSARLINGKIEMYLDRLAHEIIKKIDFTDIYNVQINVEMNKFNFESNLSKLGLAKERQKDEESFICPYSGAKISQTNCEYDHILPRSKGLYNSLANLIPTSSTSNQIKSNTKYLLSNLDENYLKYIFAKTQTTDLNSFKAFIDENISKIDENDFTNFKNLSFFEQIAFRHALFLDTDDNSFKKALRLLKLDTIKTHSNGTQKRFINILIEKISKLTKSGIDLNFIDSKLVSSTRKDLAQNDTSIAKQEIQDSHSHCVDASIVFYLANSKIIKGQIEPDYDYFKDIYPKDSDIILPQSKQYLELNQKSQKSKKLFDRSVYSLVYEGKFDEKQKKILTQYELLKENGFVDTHKVFELIFKSFKDKDTIVLKDLKFLDNHLKSYIRKDIFSIFFNEKGELKEAKELKSATKNIDKFYTILSQNQDKIYTIKLDEKAKEKKTLQRNKVIELYKEIFYTKNAKPRARGKNRVTFSLPVYAKDAKYAIKRNSGFAGLKNKDIATKTYIDIDSREILKIPYYSTNVLPIRISDILEILSLQSKNAKQIYKIKIQDNLPKQIVSLDFILSQANRHEVLVSFDKSKLEIQNINDDNGENTFIQKYLCDDFKEFLGKPRDNKIEIIKNNDDILAIKYCVESTRKANKEIIVKALSDETPSA

SEQ ID NO: 68 - protein, 1247 aa, synthetic construct
KSLSINIDMGAINNGIFIATCQDDKIIDKNAFDIKFRKGKLNFSKIDRTLRRHTRRSFDRDRFVLRLLGEILPLENLSNNQKEKLFGLFKNRGFNYLNVNFNAEIDSDNLEILNALDRYYFKDCRVLSDFENSISKIFNELENNEILAFLDDQAQILNQAKEHKNKILNKNINAILEFLESIKNESFKNNKHRKSYLKDIKNEIENSFKDIILKLKIFKNSQELYYFIGNIANFQTRILRRYFNAKFDLVFDDAKLKKNILRNINYLDFISTDEKANKNKILENLNAFSTLEFLKNTDPIVTIPPYENAKNKKPQSCQALVINDEKITPSLKDIAHKILSNSNFECLKTDENGVLADNIKDNEIAKYLQRILDISKGILDDKELYPRLLEKDENAKIFAQEIRLNSVELKEFKDFAKKYYDEVNLAKKGIIKNELLKPCCLHTPHKNKNKNALISALFLKSITQKEIENLEDFFANNKISGNQTFKGFFERLSELKKRYQNRFFHILEHEPTKELEGILKNYKKVMEKIVEHNSNFSFKAPFDDSTISTNFNYLTQLGDIIFDEKSRGFAKTCKFHTLENLIRSSAKSAIASRLASNSARLINGKIEMYLDRLAHEIIKKIDFTDIYNVQINVEMNKFNFESNLSKLGLAKERQKDEESFICPYSGAKISQTNCEYDHILPRSKGLYNSLANLIPTSSTSNQIKSNTKYLLSNLDENYLKYIFAKTQTTDLNSFKAFIDENISKIDENDFTNFKNLSFFEQIAFRHALFLDTDDNSFKKALRLLKLDTIKTHSNGTQKRFINILIEKISKLTKSGIDLNFIDSKLVSSTRKDLAQNDTSIAKQEIQDSHSHCVDASIVFYLANSKIIKGQIEPDYDYFKDIYPKDSDIILPQSKQYLELNQKSQKSKKLFDRSVYSLVYEGKFDEKQKKILTQYELLKENGFVDTHKVFELIFKSFKDKDTIVLKDLKFLDNHLKSYIRKDIFSIFFNEKGELKEAKELKSATKNIDKFYTILSQNQDKIYTIKLDEKAKEKKTLQRNKVIELYKEIFYTKNAKPRARGKNRVTFSLPVYAKDAKYAIKRNSGFAGLKNKGIATKTYIDIDSREILKIPYYSTNVLPIRISDILEILSLQSKNAKQIYKIKIQDNLPKQIVSLDFILSQANRHEVLVSFDKSKLEIQNINDDNGENTFIQKYLCDDFKEFLGKPRDNKIEIIKNNDDILAIKYCVESTSKANKEIIVKALSDETPSA

SEQ ID NO: 69 - protein, 1247 aa, synthetic construct
KSLSINIDMGAINNGIFIATCQDDKIIDKNAFDIKFRKGKLNFSKIDRTLRRHTRRSFDRDRFVLRLLGEILPLENLSNNQKEKLFGLFKNRGFNYLNVNFNAEIDSDNLEILNALDRYYFKDCRVLSDFENSISKIFNELENNEILAFLDDQAQILNQAKEHKNKILNKNINAILEFLESIKNESFKNNKHRKSYLKDIKNEIENSFKDIILKLKIFKNSQELYYFIGNIANFQTRILRRYFNAKFDLVFDDAKLKKNILRNINYLDFISTDEKANKNKILENLNAFSTLEFLKNTDPIVTIPPYENAKNKKPQSCQALVINDEKITPSLKDIAHKILSNSNFECLKTDENGVLADNIKDNEIAKYLQRILDISKGILDDKELYPRLLEKDENAKIFAQEIRLNSVELKEFKDFAKKYYDEVNLAKKGIIKNELLKPCCLHTPHKNKNKNALISALFLKSITQKEIENLEDFFANNKISGNQTFKGFFERLSELKKRYQNRFFHILEHEPTKELEGILKNYKKVMEKIVEHNSNFSFKAPFDDSTISTNFNYLTQLGDIIFDEKSRGFAKTCKFHTLENLIRSSAKSAIASRLASNSARLINGKIEMYLDRLAHEIIKKIDFTDIYNVQINVEMNKFNFESNLSKLGLAKERQKDEESFICPYSGAKISQTNCEYDHILPRSKGLYNSLANLIPTSSTSNQIKSNTKYLLSNLDENYLKYIFAKTQTTDLNSFKAFIDENISKIDENDFTNFKNLSFFEQIAFRHALFLDTDDNSFKKALRLLKLDTIKTHSNGTQKRFINILIEKISKLTKSGIDLNFIDSKLVSSTRKDLAQNDTSIAKQEIQDSHSHCVDASIVFYLANSKIIKGQIEPDYDYFKDIYPKDSDIILPQSKQYLELNQKSQKSKKLFDRSVYSLVYEGKFDEKQKKILTQYELLKENGFVDTHKVFELIFKSFKDKDTIVLKDLKFLDNHLKSYIRKDIFSIFFNEKGELKEAKELKSATKNIDKFYTILSQNQDKIYTIKLDEKAKEKKTLQRNKVIELYKEIFYTKNAKPRARGKNRVTFSLPVYAKDAKYAIKRNSGFAGLKNKSIATKTYIDIDSREILKIPYYSTNVLPIRISDILEILSLQSKNAKQIYKIKIQDNLPKQIVSLDFILSQANRHEVLVSFDKSKLEIQNINDDNGENTFIQKYLCDDFKEFLGKPRDNKIEIIKNNDDILAIKYCVESTSKANKEIIVKALSDETPSA

SEQ ID NO: 70 - protein, 1247 aa, synthetic construct
KSLSINIDMGAINNGIFIATCQDDKIIDKNAFDIKFRKGKLNFSKIDRTLRRHTRRSFDRDRFVLRLLGEILPLENLSNNQKEKLFGLFKNRGFNYLNVNFNAEIDSDNLEILNALDRYYFKDCRVLSDFENSISKIFNELENNEILAFLDDQAQILNQAKEHKNKILNKNINAILEFLESIKNESFKNNKHRKSYLKDIKNEIENSFKDIILKLKIFKNSQELYYFIGNIANFQTRILRRYFNAKFDLVFDDAKLKKNILRNINYLDFISTDEKANKNKILENLNAFSTLEFLKNTDPIVTIPPYENAKNKKPQSCQALVINDEKITPSLKDIAHKILSNSNFECLKTDENGVLADNIKDNEIAKYLQRILDISKGILDDKELYPRLLEKDENAKIFAQEIRLNSVELKEFKDFAKKYYDEVNLAKKGIIKNELLKPCCLHTPHKNKNKNALISALFLKSITQKEIENLEDFFANNKISGNQTFKGFFERLSELKKRYQNRFFHILEHEPTKELEGILKNYKKVMEKIVEHNSNFSFKAPFDDSTISTNFNYLTQLGDIIFDEKSRGFAKTCKFHTLENLIRSSAKSAIASRLASNSARLINGKIEMYLDRLAHEIIKKIDFTDIYNVQINVEMNKFNFESNLSKLGLAKERQKDEESFICPYSGAKISQTNCEYDHILPRSKGLYNSLANLIPTSSTSNQIKSNTKYLLSNLDENYLKYIFAKTQTTDLNSFKAFIDENISKIDENDFTNFKNLSFFEQIAFRHALFLDTDDNSFKKALRLLKLDTIKTHSNGTQKRFINILIEKISKLTKSGIDLNFIDSKLVSSTRKDLAQNDTSIAKQEIQDSHSHCVDASIVFYLANSKIIKGQIEPDYDYFKDIYPKDSDIILPQSKQYLELNQKSQKSKKLFDRSVYSLVYEGKFDEKQKKILTQYELLKENGFVDTHKVFELIFKSFKDKDTIVLKDLKFLDNHLKSYIRKDIFSIFFNEKGELKEAKELKSATKNIDKFYTILSQNQDKIYTIKLDEKAKEKKTLQRNKVIELYKEIFYTKNAKPRARGKNRVTFSLPVYAKDAKYAIKRNSGFAGLKNKNIATKTYIDIDSREILKIPYYSTNVLPIRISDILEILSLQSKNAKQIYKIKIQDNLPKQIVSLDFILSQANRHEVLVSFDKSKLEIQNINDDNGENTFIQKYLCDDFKEFLGKPRDNKIEIIKNNDDILAIKYCVESTSKANKEIIVKALSDETPSA

SEQ ID NO: 71 - protein, 1247 aa, synthetic construct
KSLSINIDMGAINNGIFIATCQDDKIIDKNAFDIKFRKGKLNFSKIDRTLRRHTRRSFDRDRFVLRLLGEILPLENLSNNQKEKLFGLFKNRGFNYLNVNFNAEIDSDNLEILNALDRYYFKDCRVLSDFENSISKIFNELENNEILAFLDDQAQILNQAKEHKNKILNKNINAILEFLESIKNESFKNNKHRKSYLKDIKNEIENSFKDIILKLKIFKNSQELYYFIGNIANFQTRILRRYFNAKFDLVFDDAKLKKNILRNINYLDFISTDEKANKNKILENLNAFSTLEFLKNTDPIVTIPPYENAKNKKPQSCQALVINDEKITPSLKDIAHKILSNSNFECLKTDENGVLADNIKDNEIAKYLQRILDISKGILDDKELYPRLLEKDENAKIFAQEIRLNSVELKEFKDFAKKYYDEVNLAKKGIIKNELLKPCCLHTPHKNKNKNALISALFLKSITQKEIENLEDFFANNKISGNQTFKGFFERLSELKKRYQNRFFHILEHEPTKELEGILKNYKKVMEKIVEHNSNFSFKAPFDDSTISTNFNYLTQLGDIIFDEKSRGFAKTCKFHTLENLIRSSAKSAIASRLASNSARLINGKIEMYLDRLAHEIIKKIDFTDIYNVQINVEMNKFNFESNLSKLGLAKERQKDEESFICPYSGAKISQTNCEYDHILPRSKGLYNSLANLIPTSSTSNQIKSNTKYLLSNLDENYLKYIFAKTQTTDLNSFKAFIDENISKIDENDFTNFKNLSFFEQIAFRHALFLDTDDNSFKKALRLLKLDTIKTHSNGTQKRFINILIEKISKLTKSGIDLNFIDSKLVSSTRKDLAQNDTSIAKQEIQDSHSHCVDASIVFYLANSKIIKGQIEPDYDYFKDIYPKDSDIILPQSKQYLELNQKSQKSKKLFDGSVYSLVYEGKFDEKQKKILTQYELLKENGFVDTHKVFELIFKSFKDKDTIVLKDLKFLDNHLKSYIRKDIFSIFFNEKGELKEAKELKSATKNIDKFYTILSQNQDKIYTIKLDEKAKEKKTLQRNKVIELYKEIFYTKNAKPRARGKNRVTFSLPVYAKDAKYAIKRNSGFAGLKNKDIATKTYIDIDSREILKIPYYSTNVLPIRISDILEILSLQSKNAKQIYKIKIQDNLPKQIVSLDFILSQANRHEVLVSFDKSKLEIQNINDDNGENTFIQKYLCDDFKEFLGKPRDNKIEIIKNNDDILAIKYCVESTRKANKEIIVKALSDETPSA

SEQ ID NO: 72 - protein, 1247 aa, synthetic construct
KSLSINIDMGAINNGIFIATCQDDKIIDKNAFDIKFRKGKLNFSKIDRTLRRHTRRSFDRDRFVLRLLGEILPLENLSNNQKEKLFGLFKNRGFNYLNVNFNAEIDSDNLEILNALDRYYFKDCRVLSDFENSISKIFNELENNEILAFLDDQAQILNQAKEHKNKILNKNINAILEFLESIKNESFKNNKHRKSYLKDIKNEIENSFKDIILKLKIFKNSQELYYFIGNIANFQTRILRRYFNAKFDLVFDDAKLKKNILRNINYLDFISTDEKANKNKILENLNAFSTLEFLKNTDPIVTIPPYENAKNKKPQSCQALVINDEKITPSLKDIAHKILSNSNFECLKTDENGVLADNIKDNEIAKYLQRILDISKGILDDKELYPRLLEKDENAKIFAQEIRLNSVELKEFKDFAKKYYDEVNLAKKGIIKNELLKPCCLHTPHKNKNKNALISALFLKSITQKEIENLEDFFANNKISGNQTFKGFFERLSELKKRYQNRFFHILEHEPTKELEGILKNYKKVMEKIVEHNSNFSFKAPFDDSTISTNFNYLTQLGDIIFDEKSRGFAKTCKFHTLENLIRSSAKSAIASRLASNSARLINGKIEMYLDRLAHEIIKKIDFTDIYNVQINVEMNKFNFESNLSKLGLAKERQKDEESFICPYSGAKISQTNCEYDHILPRSKGLYNSLANLIPTSSTSNQIKSNTKYLLSNLDENYLKYIFAKTQTTDLNSFKAFIDENISKIDENDFTNFKNLSFFEQIAFRHALFLDTDDNSFKKALRLLKLDTIKTHSNGTQKRFINILIEKISKLTKSGIDLNFIDSKLVSSTRKDLAQNDTSIAKQEIQDSHSHCVDASIVFYLANSKIIKGQIEPDYDYFKDIYPKDSDIILPQSKQYLELNQKSQKSKKLFDSSVYSLVYEGKFDEKQKKILTQYELLKENGFVDTHKVFELIFKSFKDKDTIVLKDLKFLDNHLKSYIRKDIFSIFFNEKGELKEAKELKSATKNIDKFYTILSQNQDKIYTIKLDEKAKEKKTLQRNKVIELYKEIFYTKNAKPRARGKNRVTFSLPVYAKDAKYAIKRNSGFAGLKNKDIATKTYIDIDSREILKIPYYSTNVLPIRISDILEILSLQSKNAKQIYKIKIQDNLPKQIVSLDFILSQANRHEVLVSFDKSKLEIQNINDDNGENTFIQKYLCDDFKEFLGKPRDNKIEIIKNNDDILAIKYCVESTRKANKEIIVKALSDETPSA

SEQ ID NO: 73 - protein, 1247 aa, synthetic construct
KSLSINIDMGAINNGIFIATCQDDKIIDKNAFDIKFRKGKLNFSKIDRTLRRHTRRSFDRDRFVLRLLGEILPLENLSNNQKEKLFGLFKNRGFNYLNVNFNAEIDSDNLEILNALDRYYFKDCRVLSDFENSISKIFNELENNEILAFLDDQAQILNQAKEHKNKILNKNINAILEFLESIKNESFKNNKHRKSYLKDIKNEIENSFKDIILKLKIFKNSQELYYFIGNIANFQTRILRRYFNAKFDLVFDDAKLKKNILRNINYLDFISTDEKANKNKILENLNAFSTLEFLKNTDPIVTIPPYENAKNKKPQSCQALVINDEKITPSLKDIAHKILSNSNFECLKTDENGVLADNIKDNEIAKYLQRILDISKGILDDKELYPRLLEKDENAKIFAQEIRLNSVELKEFKDFAKKYYDEVNLAKKGIIKNELLKPCCLHTPHKNKNKNALISALFLKSITQKEIENLEDFFANNKISGNQTFKGFFERLSELKKRYQNRFFHILEHEPTKELEGILKNYKKVMEKIVEHNSNFSFKAPFDDSTISTNFNYLTQLGDIIFDEKSRGFAKTCKFHTLENLIRSSAKSAIASRLASNSARLINGKIEMYLDRLAHEIIKKIDFTDIYNVQINVEMNKFNFESNLSKLGLAKERQKDEESFICPYSGAKISQTNCEYDHILPRSKGLYNSLANLIPTSSTSNQIKSNTKYLLSNLDENYLKYIFAKTQTTDLNSFKAFIDENISKIDENDFTNFKNLSFFEQIAFRHALFLDTDDNSFKKALRLLKLDTIKTHSNGTQKRFINILIEKISKLTKSGIDLNFIDSKLVSSTRKDLAQNDTSIAKQEIQDSHSHCVDASIVFYLANSKIIKGQIEPDYDYFKDIYPKDSDIILPQSKQYLELNQKSQKSKKLFDNSVYSLVYEGKFDEKQKKILTQYELLKENGFVDTHKVFELIFKSFKDKDTIVLKDLKFLDNHLKSYIRKDIFSIFFNEKGELKEAKELKSATKNIDKFYTILSQNQDKIYTIKLDEKAKEKKTLQRNKVIELYKEIFYTKNAKPRARGKNRVTFSLPVYAKDAKYAIKRNSGFAGLKNKDIATKTYIDIDSREILKIPYYSTNVLPIRISDILEILSLQSKNAKQIYKIKIQDNLPKQIVSLDFILSQANRHEVLVSFDKSKLEIQNINDDNGENTFIQKYLCDDFKEFLGKPRDNKIEIIKNNDDILAIKYCVESTRKANKEIIVKALSDETPSA

SEQ ID NO: 74 - protein, 1247 aa, synthetic construct
KSLSINIDMGAINNGIFIATCQDDKIIDKNAFDIKFRKGKLNFSKIDRTLRRHTRRSFDRDRFVLRLLGEILPLENLSNNQKEKLFGLFKNRGFNYLNVNFNAEIDSDNLEILNALDRYYFKDCRVLSDFENSISKIFNELENNEILAFLDDQAQILNQAKEHKNKILNKNINAILEFLESIKNESFKNNKHRKSYLKDIKNEIENSFKDIILKLKIFKNSQELYYFIGNIANFQTRILRRYFNAKFDLVFDDAKLKKNILRNINYLDFISTDEKANKNKILENLNAFSTLEFLKNTDPIVTIPPYENAKNKKPQSCQALVINDEKITPSLKDIAHKILSNSNFECLKTDENGVLADNIKDNEIAKYLQRILDISKGILDDKELYPRLLEKDENAKIFAQEIRLNSVELKEFKDFAKKYYDEVNLAKKGIIKNELLKPCCLHTPHKNKNKNALISALFLKSITQKEIENLEDFFANNKISGNQTFKGFFERLSELKKRYQNRFFHILEHEPTKELEGILKNYKKVMEKIVEHNSNFSFKAPFDDSTISTNFNYLTQLGDIIFDEKSRGFAKTCKFHTLENLIRSSAKSAIASRLASNSARLINGKIEMYLDRLAHEIIKKIDFTDIYNVQINVEMNKFNFESNLSKLGLAKERQKDEESFICPYSGAKISQTNCEYDHILPRSKGLYNSLANLIPTSSTSNQIKSNTKYLLSNLDENYLKYIFAKTQTTDLNSFKAFIDENISKIDENDFTNFKNLSFFEQIAFRHALFLDTDDNSFKKALRLLKLDTIKTHSNGTQKRFINILIEKISKLTKSGIDLNFIDSKLVSSTRKDLAQNDTSIAKQEIQDSHSHCVDASIVFYLANSKIIKGQIEPDYDYFKDIYPKDSDIILPQSKQYLELNQKSQKSKKLFDDSVYSLVYEGKFDEKQKKILTQYELLKENGFVDTHKVFELIFKSFKDKDTIVLKDLKFLDNHLKSYIRKDIFSIFFNEKGELKEAKELKSATKNIDKFYTILSQNQDKIYTIKLDEKAKEKKTLQRNKVIELYKEIFYTKNAKPRARGKNRVTFSLPVYAKDAKYAIKRNSGFAGLKNKGIATKTYIDIDSREILKIPYYSTNVLPIRISDILEILSLQSKNAKQIYKIKIQDNLPKQIVSLDFILSQANRHEVLVSFDKSKLEIQNINDDNGENTFIQKYLCDDFKEFLGKPRDNKIEIIKNNDDILAIKYCVESTRKANKEIIVKALSDETPSA

SEQ ID NO: 75 - protein, 1247 aa, synthetic construct
KSLSINIDMGAINNGIFIATCQDDKIIDKNAFDIKFRKGKLNFSKIDRTLRRHTRRSFDRDRFVLRLLGEILPLENLSNNQKEKLFGLFKNRGFNYLNVNFNAEIDSDNLEILNALDRYYFKDCRVLSDFENSISKIFNELENNEILAFLDDQAQILNQAKEHKNKILNKNINAILEFLESIKNESFKNNKHRKSYLKDIKNEIENSFKDIILKLKIFKNSQELYYFIGNIANFQTRILRRYFNAKFDLVFDDAKLKKNILRNINYLDFISTDEKANKNKILENLNAFSTLEFLKNTDPIVTIPPYENAKNKKPQSCQALVINDEKITPSLKDIAHKILSNSNFECLKTDENGVLADNIKDNEIAKYLQRILDISKGILDDKELYPRLLEKDENAKIFAQEIRLNSVELKEFKDFAKKYYDEVNLAKKGIIKNELLKPCCLHTPHKNKNKNALISALFLKSITQKEIENLEDFFANNKISGNQTFKGFFERLSELKKRYQNRFFHILEHEPTKELEGILKNYKKVMEKIVEHNSNFSFKAPFDDSTISTNFNYLTQLGDIIFDEKSRGFAKTCKFHTLENLIRSSAKSAIASRLASNSARLINGKIEMYLDRLAHEIIKKIDFTDIYNVQINVEMNKFNFESNLSKLGLAKERQKDEESFICPYSGAKISQTNCEYDHILPRSKGLYNSLANLIPTSSTSNQIKSNTKYLLSNLDENYLKYIFAKTQTTDLNSFKAFIDENISKIDENDFTNFKNLSFFEQIAFRHALFLDTDDNSFKKALRLLKLDTIKTHSNGTQKRFINILIEKISKLTKSGIDLNFIDSKLVSSTRKDLAQNDTSIAKQEIQDSHSHCVDASIVFYLANSKIIKGQIEPDYDYFKDIYPKDSDIILPQSKQYLELNQKSQKSKKLFDDSVYSLVYEGKFDEKQKKILTQYELLKENGFVDTHKVFELIFKSFKDKDTIVLKDLKFLDNHLKSYIRKDIFSIFFNEKGELKEAKELKSATKNIDKFYTILSQNQDKIYTIKLDEKAKEKKTLQRNKVIELYKEIFYTKNAKPRARGKNRVTFSLPVYAKDAKYAIKRNSGFAGLKNKNIATKTYIDIDSREILKIPYYSTNVLPIRISDILEILSLQSKNAKQIYKIKIQDNLPKQIVSLDFILSQANRHEVLVSFDKSKLEIQNINDDNGENTFIQKYLCDDFKEFLGKPRDNKIEIIKNNDDILAIKYCVESTRKANKEIIVKALSDETPSA

SEQ ID NO: 76 - protein, 1247 aa, synthetic construct
KSLSINIDMGAINNGIFIATCQDDKIIDKNAFDIKFRKRKLNFSKIDRTLRRHTRRSFDRDRFVLRLLGEILPLENLSNNQKEKLFGLFKNRGFNYLNVNFNAEIDSDNLEILNALDRYYFKDCRVLSDFENSISKIFNELENNEILAFLDDQAQILNQAKEHKNKILNKNINAILEFLESIKNESFKNNKHRKSYLKDIKNEIENSFKDIILKLKIFKNSQELYYFIGNIANFQTRILRRYFNAKFDLVFDDAKLKKNILRNINYLDFISTDEKANKNKILENLNAFSTLEFLKNTDPIVTIPPYENAKNKKPQSCQALVINDEKITPSLKDIAHKILSNSNFECLKTDENGVLADNIKDNEIAKYLQRILDISKGILDDKELYPRLLEKDENAKIFAQEIRLNSVELKEFKDFAKKYYDEVNLAKKGIIKNELLKPCCLHTPHKNKNKNALISALFLKSITQKEIENLEDFFANNKISGNQTFKGFFERLSELKKRYQNRFFHILEHEPTKELEGILKNYKKVMEKIVEHNSNFSFKAPFDDSTISTNFNYLTQLGDIIFDEKSRGFAKTCKFHTLENLIRSSAKSAIASRLASNSARLINGKIEMYLDRLAHEIIKKIDFTDIYNVQINVEMNKFNFESNLSKLGLAKERQKDEESFICPYSGAKISQTNCEYDHILPRSKGLYNSLANLIPTSSTSNQIKSNTKYLLSNLDENYLKYIFAKTQTTDLNSFKAFIDENISKIDENDFTNFKNLSFFEQIAFRHALFLDTDDNSFKKALRLLKLDTIKTHSNGTQKRFINILIEKISKLTKSGIDLNFIDSKLVSSTRKDLAQNDTSIAKQEIQDSHSHCVDASIVFYLANSKIIKGQIEPDYDYFKDIYPKDSDIILPQSKQYLELNQKSQKSKKLFDDSVYSLVYEGKFDEKQKKILTQYELLKENGFVDTHKVFELIFKSFKDKDTIVLKDLKFLDNHLKSYIRKDIFSIFFNEKGELKEAKELKSATKNIDKFYTILSQNQDKIYTIKLDEKAKEKKTLQRNKVIELYKEIFYTKNAKPRARGKNRVTFSLPVYAKDAKYAIKRNSGFAGLKNKDIATKTYIDIDSREILKIPYYSTNVLPIRISDILEILSLQSKNAKQIYKIKIQDNLPKQIVSLDFILSQARRHEVLVSFDKSKLEIQNINDDNGENTFIQKYLCDDFKEFLGKPRDNKIEIIKNNDDILAIKYCVESTSKANKEIIVKALSDETPSA

SEQ ID NO: 77 - protein, 1247 aa, synthetic construct
KSLSINIDMGAINNGIFIATCQDDKIIDKNAFDIKFRKRKLNFSKIDRTLRRHTRRSFDRDRFVLRLLGEILPLENLSNNQKEKLFGLFKNRGFNYLNVNFNAEIDSDNLEILNALDRYYFKDCRVLSDFENSISKIFNELENNEILAFLDDQAQILNQAKEHKNKILNKNINAILEFLESIKNESFKNNKHRKSYLKDIKNEIENSFKDIILKLKIFKNSQELYYFIGNIANFQTRILRRYFNAKFDLVFDDAKLKKNILRNINYLDFISTDEKANKNKILENLNAFSTLEFLKNTDPIVTIPPYENAKNKKPQSCQALVINDEKITPSLKDIAHKILSNSNFECLKTDENGVLADNIKDNEIAKYLQRILDISKGILDDKELYPRLLEKDENAKIFAQEIRLNSVELKEFKDFAKKYYDEVNLAKKGIIKNELLKPCCLHTPHKNKNKNALISALFLKSITQKEIENLEDFFANNKISGNQTFKGFFERLSELKKRYQNRFFHILEHEPTKELEGILKNYKKVMEKIVEHNSNFSFKAPFDDSTISTNFNYLTQLGDIIFDEKSRGFAKTCKFHTLENLIRSSAKSAIASRLASNSARLINGKIEMYLDRLAHEIIKKIDFTDIYNVQINVEMNKFNFESNLSKLGLAKERQKDEESFICPYSGAKISQTNCEYDHILPRSKGLYNSLANLIPTSSTSNQIKSNTKYLLSNLDENYLKYIFAKTQTTDLNSFKAFIDENISKIDENDFTNFKNLSFFEQIAFRHALFLDTDDNSFKKALRLLKLDTIKTHSNGTQKRFINILIEKISKLTKSGIDLNFIDSKLVSSTRKDLAQNDTSIAKQEIQDSHSHCVDASIVFYLANSKIIKGQIEPDYDYFKDIYPKDSDIILPQSKQYLELNQKSQKSKKLFDDSVYSLVYEGKFDEKQKKILTQYELLKENGFVDTHKVFELIFKSFKDKDTIVLKDLKFLDNHLKSYIRKDIFSIFFNEKGELKEAKELKSATKNIDKFYTILSQNQDKIYTIKLDEKAKEKKTLQRNKVIELYKEIFYTKNAKPRARGKNRVTFSLPVYAKDAKYAIKRNSGFAGLKNKDIATKTYIDIDSREILKIPYYSTNVLPIRISDILEILSLQSKNAKQIYKIKIQDNLPKQIVSLDFILSQANRHEVLVSFDKSKLEIQNINDDNGENTFIQKYLCDDFKEFLGKPRDNKIEIIKNNDDILAIKYCVESTRKANKEIIVKALSDETPSA

SEQ ID NO: 78 - protein, 1247 aa, synthetic construct
KSLSINIDMGAINNGIFIATCQDDKIIDKNAFDIKFRKRKLNFSKIDRTLRRHTRRSFDRDRFVLRLLGEILPLENLSNNQKEKLFGLFKNRGFNYLNVNFNAEIDSDNLEILNALDRYYFKDCRVLSDFENSISKIFNELENNEILAFLDDQAQILNQAKEHKNKILNKNINAILEFLESIKNESFKNNKHRKSYLKDIKNEIENSFKDIILKLKIFKNSQELYYFIGNIANFQTRILRRYFNAKFDLVFDDAKLKKNILRNINYLDFISTDEKANKNKILENLNAFSTLEFLKNTDPIVTIPPYENAKNKKPQSCQALVINDEKITPSLKDIAHKILSNSNFECLKTDENGVLADNIKDNEIAKYLQRILDISKGILDDKELYPRLLEKDENAKIFAQEIRLNSVELKEFKDFAKKYYDEVNLAKKGIIKNELLKPCCLHTPHKNKNKNALISALFLKSITQKEIENLEDFFANNKISGNQTFKGFFERLSELKKRYQNRFFHILEHEPTKELEGILKNYKKVMEKIVEHNSNFSFKAPFDDSTISTNFNYLTQLGDIIFDEKSRGFAKTCKFHTLENLIRSSAKSAIASRLASNSARLINGKIEMYLDRLAHEIIKKIDFTDIYNVQINVEMNKFNFESNLSKLGLAKERQKDEESFICPYSGAKISQTNCEYDHILPRSKGLYNSLANLIPTSSTSNQIKSNTKYLLSNLDENYLKYIFAKTQTTDLNSFKAFIDENISKIDENDFTNFKNLSFFEQIAFRHALFLDTDDNSFKKALRLLKLDTIKTHSNGTQKRFINILIEKISKLTKSGIDLNFIDSKLVSSTRKDLAQNDTSIAKQEIQDSHSHCVDASIVFYLANSKIIKGQIEPDYDYFKDIYPKDSDIILPQSKQYLELNQKSQKSKKLFDDSVYSLVYEGKFDEKQKKILTQYELLKENGFVDTHKVFELIFKSFKDKDTIVLKDLKFLDNHLKSYIRKDIFSIFFNEKGELKEAKELKSATKNIDKFYTILSQNQDKIYTIKLDEKAKEKKTLQRNKVIELYKEIFYTKNAKPRARGKNRVTFSLPVYAKDAKYAIKRNSGFAGLKNKGIATKTYIDIDSREILKIPYYSTNVLPIRISDILEILSLQSKNAKQIYKIKIQDNLPKQIVSLDFILSQANRHEVLVSFDKSKLEIQNINDDNGENTFIQKYLCDDFKEFLGKPRDNKIEIIKNNDDILAIKYCVESTSKANKEIIVKALSDETPSA

SEQ ID NO: 79 - protein, 1247 aa, synthetic construct
KSLSINIDMGAINNGIFIATCQDDKIIDKNAFDIKFRKRKLNFSKIDRTLRRHTRRSFDRDRFVLRLLGEILPLENLSNNQKEKLFGLFKNRGFNYLNVNFNAEIDSDNLEILNALDRYYFKDCRVLSDFENSISKIFNELENNEILAFLDDQAQILNQAKEHKNKILNKNINAILEFLESIKNESFKNNKHRKSYLKDIKNEIENSFKDIILKLKIFKNSQELYYFIGNIANFQTRILRRYFNAKFDLVFDDAKLKKNILRNINYLDFISTDEKANKNKILENLNAFSTLEFLKNTDPIVTIPPYENAKNKKPQSCQALVINDEKITPSLKDIAHKILSNSNFECLKTDENGVLADNIKDNEIAKYLQRILDISKGILDDKELYPRLLEKDENAKIFAQEIRLNSVELKEFKDFAKKYYDEVNLAKKGIIKNELLKPCCLHTPHKNKNKNALISALFLKSITQKEIENLEDFFANNKISGNQTFKGFFERLSELKKRYQNRFFHILEHEPTKELEGILKNYKKVMEKIVEHNSNFSFKAPFDDSTISTNFNYLTQLGDIIFDEKSRGFAKTCKFHTLENLIRSSAKSAIASRLASNSARLINGKIEMYLDRLAHEIIKKIDFTDIYNVQINVEMNKFNFESNLSKLGLAKERQKDEESFICPYSGAKISQTNCEYDHILPRSKGLYNSLANLIPTSSTSNQIKSNTKYLLSNLDENYLKYIFAKTQTTDLNSFKAFIDENISKIDENDFTNFKNLSFFEQIAFRHALFLDTDDNSFKKALRLLKLDTIKTHSNGTQKRFINILIEKISKLTKSGIDLNFIDSKLVSSTRKDLAQNDTSIAKQEIQDSHSHCVDASIVFYLANSKIIKGQIEPDYDYFKDIYPKDSDIILPQSKQYLELNQKSQKSKKLFDDSVYSLVYEGKFDEKQKKILTQYELLKENGFVDTHKVFELIFKSFKDKDTIVLKDLKFLDNHLKSYIRKDIFSIFFNEKGELKEAKELKSATKNIDKFYTILSQNQDKIYTIKLDEKAKEKKTLQRNKVIELYKEIFYTKNAKPRARGKNRVTFSLPVYAKDAKYAIKRNSGFAGLKNKSIATKTYIDIDSREILKIPYYSTNVLPIRISDILEILSLQSKNAKQIYKIKIQDNLPKQIVSLDFILSQANRHEVLVSFDKSKLEIQNINDDNGENTFIQKYLCDDFKEFLGKPRDNKIEIIKNNDDILAIKYCVESTSKANKEIIVKALSDETPSA

SEQ ID NO: 80 - protein, 1247 aa, synthetic construct
KSLSINIDMGAINNGIFIATCQDDKIIDKNAFDIKFRKRKLNFSKIDRTLRRHTRRSFDRDRFVLRLLGEILPLENLSNNQKEKLFGLFKNRGFNYLNVNFNAEIDSDNLEILNALDRYYFKDCRVLSDFENSISKIFNELENNEILAFLDDQAQILNQAKEHKNKILNKNINAILEFLESIKNESFKNNKHRKSYLKDIKNEIENSFKDIILKLKIFKNSQELYYFIGNIANFQTRILRRYFNAKFDLVFDDAKLKKNILRNINYLDFISTDEKANKNKILENLNAFSTLEFLKNTDPIVTIPPYENAKNKKPQSCQALVINDEKITPSLKDIAHKILSNSNFECLKTDENGVLADNIKDNEIAKYLQRILDISKGILDDKELYPRLLEKDENAKIFAQEIRLNSVELKEFKDFAKKYYDEVNLAKKGIIKNELLKPCCLHTPHKNKNKNALISALFLKSITQKEIENLEDFFANNKISGNQTFKGFFERLSELKKRYQNRFFHILEHEPTKELEGILKNYKKVMEKIVEHNSNFSFKAPFDDSTISTNFNYLTQLGDIIFDEKSRGFAKTCKFHTLENLIRSSAKSAIASRLASNSARLINGKIEMYLDRLAHEIIKKIDFTDIYNVQINVEMNKFNFESNLSKLGLAKERQKDEESFICPYSGAKISQTNCEYDHILPRSKGLYNSLANLIPTSSTSNQIKSNTKYLLSNLDENYLKYIFAKTQTTDLNSFKAFIDENISKIDENDFTNFKNLSFFEQIAFRHALFLDTDDNSFKKALRLLKLDTIKTHSNGTQKRFINILIEKISKLTKSGIDLNFIDSKLVSSTRKDLAQNDTSIAKQEIQDSHSHCVDASIVFYLANSKIIKGQIEPDYDYFKDIYPKDSDIILPQSKQYLELNQKSQKSKKLFDDSVYSLVYEGKFDEKQKKILTQYELLKENGFVDTHKVFELIFKSFKDKDTIVLKDLKFLDNHLKSYIRKDIFSIFFNEKGELKEAKELKSATKNIDKFYTILSQNQDKIYTIKLDEKAKEKKTLQRNKVIELYKEIFYTKNAKPRARGKNRVTFSLPVYAKDAKYAIKRNSGFAGLKNKNIATKTYIDIDSREILKIPYYSTNVLPIRISDILEILSLQSKNAKQIYKIKIQDNLPKQIVSLDFILSQANRHEVLVSFDKSKLEIQNINDDNGENTFIQKYLCDDFKEFLGKPRDNKIEIIKNNDDILAIKYCVESTSKANKEIIVKALSDETPSA

SEQ ID NO: 81 - protein, 1247 aa, synthetic construct
KSLSINIDMGAINNGIFIATCQDDKIIDKNAFDIKFGKGKLNFSKIDRTLRRHTRRSFDRDRFVLRLLGEILPLENLSNNQKEKLFGLFKNRGFNYLNVNFNAEIDSDNLEILNALDRYYFKDCRVLSDFENSISKIFNELENNEILAFLDDQAQILNQAKEHKNKILNKNINAILEFLESIKNESFKNNKHRKSYLKDIKNEIENSFKDIILKLKIFKNSQELYYFIGNIANFQTRILRRYFNAKFDLVFDDAKLKKNILRNINYLDFISTDEKANKNKILENLNAFSTLEFLKNTDPIVTIPPYENAKNKKPQSCQALVINDEKITPSLKDIAHKILSNSNFECLKTDENGVLADNIKDNEIAKYLQRILDISKGILDDKELYPRLLEKDENAKIFAQEIRLNSVELKEFKDFAKKYYDEVNLAKKGIIKNELLKPCCLHTPHKNKNKNALISALFLKSITQKEIENLEDFFANNKISGNQTFKGFFERLSELKKRYQNRFFHILEHEPTKELEGILKNYKKVMEKIVEHNSNFSFKAPFDDSTISTNFNYLTQLGDIIFDEKSRGFAKTCKFHTLENLIRSSAKSAIASRLASNSARLINGKIEMYLDRLAHEIIKKIDFTDIYNVQINVEMNKFNFESNLSKLGLAKERQKDEESFICPYSGAKISQTNCEYDHILPRSKGLYNSLANLIPTSSTSNQIKSNTKYLLSNLDENYLKYIFAKTQTTDLNSFKAFIDENISKIDENDFTNFKNLSFFEQIAFRHALFLDTDDNSFKKALRLLKLDTIKTHSNGTQKRFINILIEKISKLTKSGIDLNFIDSKLVSSTRKDLAQNDTSIAKQEIQDSHSHCVDASIVFYLANSKIIKGQIEPDYDYFKDIYPKDSDIILPQSKQYLELNQKSQKSKKLFDDSVYSLVYEGKFDEKQKKILTQYELLKENGFVDTHKVFELIFKSFKDKDTIVLKDLKFLDNHLKSYIRKDIFSIFFNEKGELKEAKELKSATKNIDKFYTILSQNQDKIYTIKLDEKAKEKKTLQRNKVIELYKEIFYTKNAKPRARGKNRVTFSLPVYAKDAKYAIKRNSGFAGLKNKRIATKTYIDIDSREILKIPYYSTNVLPIRISDILEILSLQSKNAKQIYKIKIQDNLPKQIVSLDFILSQARRHEVLVSFDKSKLEIQNINDDNGENTFIQKYLCDDFKEFLGKPRDNKIEIIKNNDDILAIKYCVESTSKANKEIIVKALSDETPSA

SEQ ID NO: 82 - protein, 1247 aa, synthetic construct
KSLSINIDMGAINNGIFIATCQDDKIIDKNAFDIKFNKGKLNFSKIDRTLRRHTRRSFDRDRFVLRLLGEILPLENLSNNQKEKLFGLFKNRGFNYLNVNFNAEIDSDNLEILNALDRYYFKDCRVLSDFENSISKIFNELENNEILAFLDDQAQILNQAKEHKNKILNKNINAILEFLESIKNESFKNNKHRKSYLKDIKNEIENSFKDIILKLKIFKNSQELYYFIGNIANFQTRILRRYFNAKFDLVFDDAKLKKNILRNINYLDFISTDEKANKNKILENLNAFSTLEFLKNTDPIVTIPPYENAKNKKPQSCQALVINDEKITPSLKDIAHKILSNSNFECLKTDENGVLADNIKDNEIAKYLQRILDISKGILDDKELYPRLLEKDENAKIFAQEIRLNSVELKEFKDFAKKYYDEVNLAKKGIIKNELLKPCCLHTPHKNKNKNALISALFLKSITQKEIENLEDFFANNKISGNQTFKGFFERLSELKKRYQNRFFHILEHEPTKELEGILKNYKKVMEKIVEHNSNFSFKAPFDDSTISTNFNYLTQLGDIIFDEKSRGFAKTCKFHTLENLIRSSAKSAIASRLASNSARLINGKIEMYLDRLAHEIIKKIDFTDIYNVQINVEMNKFNFESNLSKLGLAKERQKDEESFICPYSGAKISQTNCEYDHILPRSKGLYNSLANLIPTSSTSNQIKSNTKYLLSNLDENYLKYIFAKTQTTDLNSFKAFIDENISKIDENDFTNFKNLSFFEQIAFRHALFLDTDDNSFKKALRLLKLDTIKTHSNGTQKRFINILIEKISKLTKSGIDLNFIDSKLVSSTRKDLAQNDTSIAKQEIQDSHSHCVDASIVFYLANSKIIKGQIEPDYDYFKDIYPKDSDIILPQSKQYLELNQKSQKSKKLFDDSVYSLVYEGKFDEKQKKILTQYELLKENGFVDTHKVFELIFKSFKDKDTIVLKDLKFLDNHLKSYIRKDIFSIFFNEKGELKEAKELKSATKNIDKFYTILSQNQDKIYTIKLDEKAKEKKTLQRNKVIELYKEIFYTKNAKPRARGKNRVTFSLPVYAKDAKYAIKRNSGFAGLKNKRIATKTYIDIDSREILKIPYYSTNVLPIRISDILEILSLQSKNAKQIYKIKIQDNLPKQIVSLDFILSQARRHEVLVSFDKSKLEIQNINDDNGENTFIQKYLCDDFKEFLGKPRDNKIEIIKNNDDILAIKYCVESTSKANKEIIVKALSDETPSA

SEQ ID NO: 83 - protein, 1247 aa, synthetic construct
KSLSINIDMGAINNGIFIATCQDDKIIDKNAFDIKFDKGKLNFSKIDRTLRRHTRRSFDRDRFVLRLLGEILPLENLSNNQKEKLFGLFKNRGFNYLNVNFNAEIDSDNLEILNALDRYYFKDCRVLSDFENSISKIFNELENNEILAFLDDQAQILNQAKEHKNKILNKNINAILEFLESIKNESFKNNKHRKSYLKDIKNEIENSFKDIILKLKIFKNSQELYYFIGNIANFQTRILRRYFNAKFDLVFDDAKLKKNILRNINYLDFISTDEKANKNKILENLNAFSTLEFLKNTDPIVTIPPYENAKNKKPQSCQALVINDEKITPSLKDIAHKILSNSNFECLKTDENGVLADNIKDNEIAKYLQRILDISKGILDDKELYPRLLEKDENAKIFAQEIRLNSVELKEFKDFAKKYYDEVNLAKKGIIKNELLKPCCLHTPHKNKNKNALISALFLKSITQKEIENLEDFFANNKISGNQTFKGFFERLSELKKRYQNRFFHILEHEPTKELEGILKNYKKVMEKIVEHNSNFSFKAPFDDSTISTNFNYLTQLGDIIFDEKSRGFAKTCKFHTLENLIRSSAKSAIASRLASNSARLINGKIEMYLDRLAHEIIKKIDFTDIYNVQINVEMNKFNFESNLSKLGLAKERQKDEESFICPYSGAKISQTNCEYDHILPRSKGLYNSLANLIPTSSTSNQIKSNTKYLLSNLDENYLKYIFAKTQTTDLNSFKAFIDENISKIDENDFTNFKNLSFFEQIAFRHALFLDTDDNSFKKALRLLKLDTIKTHSNGTQKRFINILIEKISKLTKSGIDLNFIDSKLVSSTRKDLAQNDTSIAKQEIQDSHSHCVDASIVFYLANSKIIKGQIEPDYDYFKDIYPKDSDIILPQSKQYLELNQKSQKSKKLFDSSVYSLVYEGKFDEKQKKILTQYELLKENGFVDTHKVFELIFKSFKDKDTIVLKDLKFLDNHLKSYIRKDIFSIFFNEKGELKEAKELKSATKNIDKFYTILSQNQDKIYTIKLDEKAKEKKTLQRNKVIELYKEIFYTKNAKPRARGKNRVTFSLPVYAKDAKYAIKRNSGFAGLKNKRIATKTYIDIDSREILKIPYYSTNVLPIRISDILEILSLQSKNAKQIYKIKIQDNLPKQIVSLDFILSQARRHEVLVSFDKSKLEIQNINDDNGENTFIQKYLCDDFKEFLGKPRDNKIEIIKNNDDILAIKYCVESTSKANKEIIVKALSDETPSA

SEQ ID NO: 84 - protein, 1247 aa, synthetic construct
KSLSINIDMGAINNGIFIATCQDDKIIDKNAFDIKFRKGKLNFSKIGRTLRRHTRRSFDRDRFVLRLLGEILPLENLSNNQKEKLFGLFKNRGFNYLNVNFNAEIDSDNLEILNALDRYYFKDCRVLSDFENSISKIFNELENNEILAFLDDQAQILNQAKEHKNKILNKNINAILEFLESIKNESFKNNKHRKSYLKDIKNEIENSFKDIILKLKIFKNSQELYYFIGNIANFQTRILRRYFNAKFDLVFDDAKLKKNILRNINYLDFISTDEKANKNKILENLNAFSTLEFLKNTDPIVTIPPYENAKNKKPQSCQALVINDEKITPSLKDIAHKILSNSNFECLKTDENGVLADNIKDNEIAKYLQRILDISKGILDDKELYPRLLEKDENAKIFAQEIRLNSVELKEFKDFAKKYYDEVNLAKKGIIKNELLKPCCLHTPHKNKNKNALISALFLKSITQKEIENLEDFFANNKISGNQTFKGFFERLSELKKRYQNRFFHILEHEPTKELEGILKNYKKVMEKIVEHNSNFSFKAPFDDSTISTNFNYLTQLGDIIFDEKSRGFAKTCKFHTLENLIRSSAKSAIASRLASNSARLINGKIEMYLDRLAHEIIKKIDFTDIYNVQINVEMNKFNFESNLSKLGLAKERQKDEESFICPYSGAKISQTNCEYDHILPRSKGLYNSLANLIPTSSTSNQIKSNTKYLLSNLDENYLKYIFAKTQTTDLNSFKAFIDENISKIDENDFTNFKNLSFFEQIAFRHALFLDTDDNSFKKALRLLKLDTIKTHSNGTQKRFINILIEKISKLTKSGIDLNFIDSKLVSSTRKDLAQNDTSIAKQEIQDSHSHCVDASIVFYLANSKIIKGQIEPDYDYFKDIYPKDSDIILPQSKQYLELNQKSQKSKKLFDRSVYSLVYEGKFDEKQKKILTQYELLKENGFVDTHKVFELIFKSFKDKDTIVLKDLKFLDNHLKSYIRKDIFSIFFNEKGELKEAKELKSATKNIDKFYTILSQNQDKIYTIKLDEKAKEKKTLQRNKVIELYKEIFYTKNAKPRARGKNRVTFSLPVYAKDAKYAIKRNSGFAGLKNKDIATKTYIDIDSREILKIPYYSTNVLPIRISDILEILSLQSKNAKQIYKIKIQDNLPKQIVSLDFILSQANRHEVLVSFDKSKLEIQNINDDNGENTFIQKYLCDDFKEFLGKPRDNKIEIIKNNDDILAIKYCVESTSKANKEIIVKALSDETPSA

SEQ ID NO: 85 - protein, 1247 aa, synthetic construct
KSLSINIDMGAINNGIFIATCQDDKIIDKNAFDIKFRKGKLNFSKILRTLRRHTRRSFDRDRFVLRLLGEILPLENLSNNQKEKLFGLFKNRGFNYLNVNFNAEIDSDNLEILNALDRYYFKDCRVLSDFENSISKIFNELENNEILAFLDDQAQILNQAKEHKNKILNKNINAILEFLESIKNESFKNNKHRKSYLKDIKNEIENSFKDIILKLKIFKNSQELYYFIGNIANFQTRILRRYFNAKFDLVFDDAKLKKNILRNINYLDFISTDEKANKNKILENLNAFSTLEFLKNTDPIVTIPPYENAKNKKPQSCQALVINDEKITPSLKDIAHKILSNSNFECLKTDENGVLADNIKDNEIAKYLQRILDISKGILDDKELYPRLLEKDENAKIFAQEIRLNSVELKEFKDFAKKYYDEVNLAKKGIIKNELLKPCCLHTPHKNKNKNALISALFLKSITQKEIENLEDFFANNKISGNQTFKGFFERLSELKKRYQNRFFHILEHEPTKELEGILKNYKKVMEKIVEHNSNFSFKAPFDDSTISTNFNYLTQLGDIIFDEKSRGFAKTCKFHTLENLIRSSAKSAIASRLASNSARLINGKIEMYLDRLAHEIIKKIDFTDIYNVQINVEMNKFNFESNLSKLGLAKERQKDEESFICPYSGAKISQTNCEYDHILPRSKGLYNSLANLIPTSSTSNQIKSNTKYLLSNLDENYLKYIFAKTQTTDLNSFKAFIDENISKIDENDFTNFKNLSFFEQIAFRHALFLDTDDNSFKKALRLLKLDTIKTHSNGTQKRFINILIEKISKLTKSGIDLNFIDSKLVSSTRKDLAQNDTSIAKQEIQDSHSHCVDASIVFYLANSKIIKGQIEPDYDYFKDIYPKDSDIILPQSKQYLELNQKSQKSKKLFDRSVYSLVYEGKFDEKQKKILTQYELLKENGFVDTHKVFELIFKSFKDKDTIVLKDLKFLDNHLKSYIRKDIFSIFFNEKGELKEAKELKSATKNIDKFYTILSQNQDKIYTIKLDEKAKEKKTLQRNKVIELYKEIFYTKNAKPRARGKNRVTFSLPVYAKDAKYAIKRNSGFAGLKNKDIATKTYIDIDSREILKIPYYSTNVLPIRISDILEILSLQSKNAKQIYKIKIQDNLPKQIVSLDFILSQANRHEVLVSFDKSKLEIQNINDDNGENTFIQKYLCDDFKEFLGKPRDNKIEIIKNNDDILAIKYCVESTSKANKEIIVKALSDETPSA

SEQ ID NO: 86 - protein, 1247 aa, synthetic construct
KSLSINIDMGAINNGIFIATCQDDKIIDKNAFDIKFRKGKLNFSKIDRTLRRHRRRSFDRDRFVLRLLGEILPLENLSNNQKEKLFGLFKNRGFNYLNVNFNAEIDSDNLEILNALDRYYFKDCRVLSDFENSISKIFNELENNEILAFLDDQAQILNQAKEHKNKILNKNINAILEFLESIKNESFKNNKHRKSYLKDIKNEIENSFKDIILKLKIFKNSQELYYFIGNIANFQTRILRRYFNAKFDLVFDDAKLKKNILRNINYLDFISTDEKANKNKILENLNAFSTLEFLKNTDPIVTIPPYENAKNKKPQSCQALVINDEKITPSLKDIAHKILSNSNFECLKTDENGVLADNIKDNEIAKYLQRILDISKGILDDKELYPRLLEKDENAKIFAQEIRLNSVELKEFKDFAKKYYDEVNLAKKGIIKNELLKPCCLHTPHKNKNKNALISALFLKSITQKEIENLEDFFANNKISGNQTFKGFFERLSELKKRYQNRFFHILEHEPTKELEGILKNYKKVMEKIVEHNSNFSFKAPFDDSTISTNFNYLTQLGDIIFDEKSRGFAKTCKFHTLENLIRSSAKSAIASRLASNSARLINGKIEMYLDRLAHEIIKKIDFTDIYNVQINVEMNKFNFESNLSKLGLAKERQKDEESFICPYSGAKISQTNCEYDHILPRSKGLYNSLANLIPTSSTSNQIKSNTKYLLSNLDENYLKYIFAKTQTTDLNSFKAFIDENISKIDENDFTNFKNLSFFEQIAFRHALFLDTDDNSFKKALRLLKLDTIKTHSNGTQKRFINILIEKISKLTKSGIDLNFIDSKLVSSTRKDLAQNDTSIAKQEIQDSHSHCVDASIVFYLANSKIIKGQIEPDYDYFKDIYPKDSDIILPQSKQYLELNQKSQKSKKLFDRSVYSLVYEGKFDEKQKKILTQYELLKENGFVDTHKVFELIFKSFKDKDTIVLKDLKFLDNHLKSYIRKDIFSIFFNEKGELKEAKELKSATKNIDKFYTILSQNQDKIYTIKLDEKAKEKKTLQRNKVIELYKEIFYTKNAKPRARGKNRVTFSLPVYAKDAKYAIKRNSGFAGLKNKDIATKTYIDIDSREILKIPYYSTNVLPIRISDILEILSLQSKNAKQIYKIKIQDNLPKQIVSLDFILSQANRHEVLVSFDKSKLEIQNINDDNGENTFIQKYLCDDFKEFLGKPRDNKIEIIKNNDDILAIKYCVESTSKANKEIIVKALSDETPSA

SEQ ID NO: 87 - protein, 1247 aa, synthetic construct
KSLSINIDMGAINNGIFIATCQDDKIIDKNAFDIKFRKGKLNFSKIDRTLRRHTRRAFDRDRFVLRLLGEILPLENLSNNQKEKLFGLFKNRGFNYLNVNFNAEIDSDNLEILNALDRYYFKDCRVLSDFENSISKIFNELENNEILAFLDDQAQILNQAKEHKNKILNKNINAILEFLESIKNESFKNNKHRKSYLKDIKNEIENSFKDIILKLKIFKNSQELYYFIGNIANFQTRILRRYFNAKFDLVFDDAKLKKNILRNINYLDFISTDEKANKNKILENLNAFSTLEFLKNTDPIVTIPPYENAKNKKPQSCQALVINDEKITPSLKDIAHKILSNSNFECLKTDENGVLADNIKDNEIAKYLQRILDISKGILDDKELYPRLLEKDENAKIFAQEIRLNSVELKEFKDFAKKYYDEVNLAKKGIIKNELLKPCCLHTPHKNKNKNALISALFLKSITQKEIENLEDFFANNKISGNQTFKGFFERLSELKKRYQNRFFHILEHEPTKELEGILKNYKKVMEKIVEHNSNFSFKAPFDDSTISTNFNYLTQLGDIIFDEKSRGFAKTCKFHTLENLIRSSAKSAIASRLASNSARLINGKIEMYLDRLAHEIIKKIDFTDIYNVQINVEMNKFNFESNLSKLGLAKERQKDEESFICPYSGAKISQTNCEYDHILPRSKGLYNSLANLIPTSSTSNQIKSNTKYLLSNLDENYLKYIFAKTQTTDLNSFKAFIDENISKIDENDFTNFKNLSFFEQIAFRHALFLDTDDNSFKKALRLLKLDTIKTHSNGTQKRFINILIEKISKLTKSGIDLNFIDSKLVSSTRKDLAQNDTSIAKQEIQDSHSHCVDASIVFYLANSKIIKGQIEPDYDYFKDIYPKDSDIILPQSKQYLELNQKSQKSKKLFDRSVYSLVYEGKFDEKQKKILTQYELLKENGFVDTHKVFELIFKSFKDKDTIVLKDLKFLDNHLKSYIRKDIFSIFFNEKGELKEAKELKSATKNIDKFYTILSQNQDKIYTIKLDEKAKEKKTLQRNKVIELYKEIFYTKNAKPRARGKNRVTFSLPVYAKDAKYAIKRNSGFAGLKNKDIATKTYIDIDSREILKIPYYSTNVLPIRISDILEILSLQSKNAKQIYKIKIQDNLPKQIVSLDFILSQANRHEVLVSFDKSKLEIQNINDDNGENTFIQKYLCDDFKEFLGKPRDNKIEIIKNNDDILAIKYCVESTSKANKEIIVKALSDETPSA

SEQ ID NO: 88 - protein, 1247 aa, synthetic construct
KSLSINIDMGAINNGIFIATCQDDKIIDKNAFDIKFRKGKLNFSKIDRTLRRHTRRSFGRDRFVLRLLGEILPLENLSNNQKEKLFGLFKNRGFNYLNVNFNAEIDSDNLEILNALDRYYFKDCRVLSDFENSISKIFNELENNEILAFLDDQAQILNQAKEHKNKILNKNINAILEFLESIKNESFKNNKHRKSYLKDIKNEIENSFKDIILKLKIFKNSQELYYFIGNIANFQTRILRRYFNAKFDLVFDDAKLKKNILRNINYLDFISTDEKANKNKILENLNAFSTLEFLKNTDPIVTIPPYENAKNKKPQSCQALVINDEKITPSLKDIAHKILSNSNFECLKTDENGVLADNIKDNEIAKYLQRILDISKGILDDKELYPRLLEKDENAKIFAQEIRLNSVELKEFKDFAKKYYDEVNLAKKGIIKNELLKPCCLHTPHKNKNKNALISALFLKSITQKEIENLEDFFANNKISGNQTFKGFFERLSELKKRYQNRFFHILEHEPTKELEGILKNYKKVMEKIVEHNSNFSFKAPFDDSTISTNFNYLTQLGDIIFDEKSRGFAKTCKFHTLENLIRSSAKSAIASRLASNSARLINGKIEMYLDRLAHEIIKKIDFTDIYNVQINVEMNKFNFESNLSKLGLAKERQKDEESFICPYSGAKISQTNCEYDHILPRSKGLYNSLANLIPTSSTSNQIKSNTKYLLSNLDENYLKYIFAKTQTTDLNSFKAFIDENISKIDENDFTNFKNLSFFEQIAFRHALFLDTDDNSFKKALRLLKLDTIKTHSNGTQKRFINILIEKISKLTKSGIDLNFIDSKLVSSTRKDLAQNDTSIAKQEIQDSHSHCVDASIVFYLANSKIIKGQIEPDYDYFKDIYPKDSDIILPQSKQYLELNQKSQKSKKLFDRSVYSLVYEGKFDEKQKKILTQYELLKENGFVDTHKVFELIFKSFKDKDTIVLKDLKFLDNHLKSYIRKDIFSIFFNEKGELKEAKELKSATKNIDKFYTILSQNQDKIYTIKLDEKAKEKKTLQRNKVIELYKEIFYTKNAKPRARGKNRVTFSLPVYAKDAKYAIKRNSGFAGLKNKDIATKTYIDIDSREILKIPYYSTNVLPIRISDILEILSLQSKNAKQIYKIKIQDNLPKQIVSLDFILSQANRHEVLVSFDKSKLEIQNINDDNGENTFIQKYLCDDFKEFLGKPRDNKIEIIKNNDDILAIKYCVESTSKANKEIIVKALSDETPSA

SEQ ID NO: 89 - protein, 1247 aa, synthetic construct
KSLSINIDMGAINNGIFIATCQDDKIIDKNAFDIKFRKGKLNFSKIDRTLRRHTRRSFSRDRFVLRLLGEILPLENLSNNQKEKLFGLFKNRGFNYLNVNFNAEIDSDNLEILNALDRYYFKDCRVLSDFENSISKIFNELENNEILAFLDDQAQILNQAKEHKNKILNKNINAILEFLESIKNESFKNNKHRKSYLKDIKNEIENSFKDIILKLKIFKNSQELYYFIGNIANFQTRILRRYFNAKFDLVFDDAKLKKNILRNINYLDFISTDEKANKNKILENLNAFSTLEFLKNTDPIVTIPPYENAKNKKPQSCQALVINDEKITPSLKDIAHKILSNSNFECLKTDENGVLADNIKDNEIAKYLQRILDISKGILDDKELYPRLLEKDENAKIFAQEIRLNSVELKEFKDFAKKYYDEVNLAKKGIIKNELLKPCCLHTPHKNKNKNALISALFLKSITQKEIENLEDFFANNKISGNQTFKGFFERLSELKKRYQNRFFHILEHEPTKELEGILKNYKKVMEKIVEHNSNFSFKAPFDDSTISTNFNYLTQLGDIIFDEKSRGFAKTCKFHTLENLIRSSAKSAIASRLASNSARLINGKIEMYLDRLAHEIIKKIDFTDIYNVQINVEMNKFNFESNLSKLGLAKERQKDEESFICPYSGAKISQTNCEYDHILPRSKGLYNSLANLIPTSSTSNQIKSNTKYLLSNLDENYLKYIFAKTQTTDLNSFKAFIDENISKIDENDFTNFKNLSFFEQIAFRHALFLDTDDNSFKKALRLLKLDTIKTHSNGTQKRFINILIEKISKLTKSGIDLNFIDSKLVSSTRKDLAQNDTSIAKQEIQDSHSHCVDASIVFYLANSKIIKGQIEPDYDYFKDIYPKDSDIILPQSKQYLELNQKSQKSKKLFDRSVYSLVYEGKFDEKQKKILTQYELLKENGFVDTHKVFELIFKSFKDKDTIVLKDLKFLDNHLKSYIRKDIFSIFFNEKGELKEAKELKSATKNIDKFYTILSQNQDKIYTIKLDEKAKEKKTLQRNKVIELYKEIFYTKNAKPRARGKNRVTFSLPVYAKDAKYAIKRNSGFAGLKNKDIATKTYIDIDSREILKIPYYSTNVLPIRISDILEILSLQSKNAKQIYKIKIQDNLPKQIVSLDFILSQANRHEVLVSFDKSKLEIQNINDDNGENTFIQKYLCDDFKEFLGKPRDNKIEIIKNNDDILAIKYCVESTSKANKEIIVKALSDETPSA

SEQ ID NO: 90 - protein, 1247 aa, synthetic construct
KSLSINIDMGAINNGIFIATCQDDKIIDKNAFDIKFRKGKLNFSKIDRTLRRHTRRSFDRDRFVLRLLGEILPLENLSNNQKEKLFGLFKNRGFNYLNVNFNAEIDSDNLEILNALDRYYFKDCRVLSDFENSISKIFNELENNEILAFLDDQAQILNQAKEHKNKILNKNINAILEFLESIKNESFKNNKHRKSYLKDIKNEIENSFKDIILKLKIFKNSQELYYFIGNIANFQTRILRRYFNAKFDLVFDDAKLKKNILRNINYLDFISTDEKANKNKILENLNAFSTLEFLKNTDPIVTIPPYENAKNKKPKSCQALVINDEKITPSLKDIAHKILSNSNFECLKTDENGVLADNIKDNEIAKYLQRILDISKGILDDKELYPRLLEKDENAKIFAQEIRLNSVELKEFKDFAKKYYDEVNLAKKGIIKNELLKPCCLHTPHKNKNKNALISALFLKSITQKEIENLEDFFANNKISGNQTFKGFFERLSELKKRYQNRFFHILEHEPTKELEGILKNYKKVMEKIVEHNSNFSFKAPFDDSTISTNFNYLTQLGDIIFDEKSRGFAKTCKFHTLENLIRSSAKSAIASRLASNSARLINGKIEMYLDRLAHEIIKKIDFTDIYNVQINVEMNKFNFESNLSKLGLAKERQKDEESFICPYSGAKISQTNCEYDHILPRSKGLYNSLANLIPTSSTSNQIKSNTKYLLSNLDENYLKYIFAKTQTTDLNSFKAFIDENISKIDENDFTNFKNLSFFEQIAFRHALFLDTDDNSFKKALRLLKLDTIKTHSNGTQKRFINILIEKISKLTKSGIDLNFIDSKLVSSTRKDLAQNDTSIAKQEIQDSHSHCVDASIVFYLANSKIIKGQIEPDYDYFKDIYPKDSDIILPQSKQYLELNQKSQKSKKLFDRSVYSLVYEGKFDEKQKKILTQYELLKENGFVDTHKVFELIFKSFKDKDTIVLKDLKFLDNHLKSYIRKDIFSIFFNEKGELKEAKELKSATKNIDKFYTILSQNQDKIYTIKLDEKAKEKKTLQRNKVIELYKEIFYTKNAKPRARGKNRVTFSLPVYAKDAKYAIKRNSGFAGLKNKDIATKTYIDIDSREILKIPYYSTNVLPIRISDILEILSLQSKNAKQIYKIKIQDNLPKQIVSLDFILSQANRHEVLVSFDKSKLEIQNINDDNGENTFIQKYLCDDFKEFLGKPRDNKIEIIKNNDDILAIKYCVESTSKANKEIIVKALSDETPSA

SEQ ID NO: 91 - protein, 1247 aa, synthetic construct
KSLSINIDMGAINNGIFIATCQDDKIIDKNAFDIKFRKGKLNFSKIDRTLRRHTRRSFDRDRFVLRLLGEILPLENLSNNQKEKLFGLFKNRGFNYLNVNFNAEIDSDNLEILNALDRYYFKDCRVLSDFENSISKIFNELENNEILAFLDDQAQILNQAKEHKNKILNKNINAILEFLESIKNESFKNNKHRKSYLKDIKNEIENSFKDIILKLKIFKNSQELYYFIGNIANFQTRILRRYFNAKFDLVFDDAKLKKNILRNINYLDFISTDEKANKNKILENLNAFSTLEFLKNTDPIVTIPPYENAKNKKPRSCQALVINDEKITPSLKDIAHKILSNSNFECLKTDENGVLADNIKDNEIAKYLQRILDISKGILDDKELYPRLLEKDENAKIFAQEIRLNSVELKEFKDFAKKYYDEVNLAKKGIIKNELLKPCCLHTPHKNKNKNALISALFLKSITQKEIENLEDFFANNKISGNQTFKGFFERLSELKKRYQNRFFHILEHEPTKELEGILKNYKKVMEKIVEHNSNFSFKAPFDDSTISTNFNYLTQLGDIIFDEKSRGFAKTCKFHTLENLIRSSAKSAIASRLASNSARLINGKIEMYLDRLAHEIIKKIDFTDIYNVQINVEMNKFNFESNLSKLGLAKERQKDEESFICPYSGAKISQTNCEYDHILPRSKGLYNSLANLIPTSSTSNQIKSNTKYLLSNLDENYLKYIFAKTQTTDLNSFKAFIDENISKIDENDFTNFKNLSFFEQIAFRHALFLDTDDNSFKKALRLLKLDTIKTHSNGTQKRFINILIEKISKLTKSGIDLNFIDSKLVSSTRKDLAQNDTSIAKQEIQDSHSHCVDASIVFYLANSKIIKGQIEPDYDYFKDIYPKDSDIILPQSKQYLELNQKSQKSKKLFDRSVYSLVYEGKFDEKQKKILTQYELLKENGFVDTHKVFELIFKSFKDKDTIVLKDLKFLDNHLKSYIRKDIFSIFFNEKGELKEAKELKSATKNIDKFYTILSQNQDKIYTIKLDEKAKEKKTLQRNKVIELYKEIFYTKNAKPRARGKNRVTFSLPVYAKDAKYAIKRNSGFAGLKNKDIATKTYIDIDSREILKIPYYSTNVLPIRISDILEILSLQSKNAKQIYKIKIQDNLPKQIVSLDFILSQANRHEVLVSFDKSKLEIQNINDDNGENTFIQKYLCDDFKEFLGKPRDNKIEIIKNNDDILAIKYCVESTSKANKEIIVKALSDETPSA

SEQ ID NO: 92 - protein, 1247 aa, synthetic construct
KSLSINIDMGAINNGIFIATCQDDKIIDKNAFDIKFRKGKLNFSKIDRTLRRHTRRSFDRDRFVLRLLGEILPLENLSNNQKEKLFGLFKNRGFNYLNVNFNAEIDSDNLEILNALDRYYFKDCRVLSDFENSISKIFNELENNEILAFLDDQAQILNQAKEHKNKILNKNINAILEFLESIKNESFKNNKHRKSYLKDIKNEIENSFKDIILKLKIFKNSQELYYFIGNIANFQTRILRRYFNAKFDLVFDDAKLKKNILRNINYLDFISTDEKANKNKILENLNAFSTLEFLKNTDPIVTIPPYENAKNKKPQSCQALVINDEKITPSLKDIAHKILSNSNFECLKTDENGVLADNIKDNEIAKYLQRILDISKGILDDKELYPRLLEKDENAKIFAQEIRLNSVELKEFKDFAKKYYDEVNLAKKGIIKNELLKPCCLHTPHKNKNKNALISALFLKSITQKEIENLEDFFANNKISGNQTFKGFFERLSELKKRYQNRFFHILEHEPTKELEGILKNYKKVMEKIVEHNSNFSFKAPFDDSTISTNFNYLTQLGDIIFDEKKRGFAKTCKFHTLENLIRSSAKSAIASRLASNSARLINGKIEMYLDRLAHEIIKKIDFTDIYNVQINVEMNKFNFESNLSKLGLAKERQKDEESFICPYSGAKISQTNCEYDHILPRSKGLYNSLANLIPTSSTSNQIKSNTKYLLSNLDENYLKYIFAKTQTTDLNSFKAFIDENISKIDENDFTNFKNLSFFEQIAFRHALFLDTDDNSFKKALRLLKLDTIKTHSNGTQKRFINILIEKISKLTKSGIDLNFIDSKLVSSTRKDLAQNDTSIAKQEIQDSHSHCVDASIVFYLANSKIIKGQIEPDYDYFKDIYPKDSDIILPQSKQYLELNQKSQKSKKLFDRSVYSLVYEGKFDEKQKKILTQYELLKENGFVDTHKVFELIFKSFKDKDTIVLKDLKFLDNHLKSYIRKDIFSIFFNEKGELKEAKELKSATKNIDKFYTILSQNQDKIYTIKLDEKAKEKKTLQRNKVIELYKEIFYTKNAKPRARGKNRVTFSLPVYAKDAKYAIKRNSGFAGLKNKDIATKTYIDIDSREILKIPYYSTNVLPIRISDILEILSLQSKNAKQIYKIKIQDNLPKQIVSLDFILSQANRHEVLVSFDKSKLEIQNINDDNGENTFIQKYLCDDFKEFLGKPRDNKIEIIKNNDDILAIKYCVESTSKANKEIIVKALSDETPSA

SEQ ID NO: 93 - protein, 1247 aa, synthetic construct
KSLSINIDMGAINNGIFIATCQDDKIIDKNAFDIKFRKGKLNFSKIDRTLRRHTRRSFDRDRFVLRLLGEILPLENLSNNQKEKLFGLFKNRGFNYLNVNFNAEIDSDNLEILNALDRYYFKDCRVLSDFENSISKIFNELENNEILAFLDDQAQILNQAKEHKNKILNKNINAILEFLESIKNESFKNNKHRKSYLKDIKNEIENSFKDIILKLKIFKNSQELYYFIGNIANFQTRILRRYFNAKFDLVFDDAKLKKNILRNINYLDFISTDEKANKNKILENLNAFSTLEFLKNTDPIVTIPPYENAKNKKPQSCQALVINDEKITPSLKDIAHKILSNSNFECLKTDENGVLADNIKDNEIAKYLQRILDISKGILDDKELYPRLLEKDENAKIFAQEIRLNSVELKEFKDFAKKYYDEVNLAKKGIIKNELLKPCCLHTPHKNKNKNALISALFLKSITQKEIENLEDFFANNKISGNQTFKGFFERLSELKKRYQNRFFHILEHEPTKELEGILKNYKKVMEKIVEHNSNFSFKAPFDDSTISTNFNYLTQLGDIIFDEKRRGFAKTCKFHTLENLIRSSAKSAIASRLASNSARLINGKIEMYLDRLAHEIIKKIDFTDIYNVQINVEMNKFNFESNLSKLGLAKERQKDEESFICPYSGAKISQTNCEYDHILPRSKGLYNSLANLIPTSSTSNQIKSNTKYLLSNLDENYLKYIFAKTQTTDLNSFKAFIDENISKIDENDFTNFKNLSFFEQIAFRHALFLDTDDNSFKKALRLLKLDTIKTHSNGTQKRFINILIEKISKLTKSGIDLNFIDSKLVSSTRKDLAQNDTSIAKQEIQDSHSHCVDASIVFYLANSKIIKGQIEPDYDYFKDIYPKDSDIILPQSKQYLELNQKSQKSKKLFDRSVYSLVYEGKFDEKQKKILTQYELLKENGFVDTHKVFELIFKSFKDKDTIVLKDLKFLDNHLKSYIRKDIFSIFFNEKGELKEAKELKSATKNIDKFYTILSQNQDKIYTIKLDEKAKEKKTLQRNKVIELYKEIFYTKNAKPRARGKNRVTFSLPVYAKDAKYAIKRNSGFAGLKNKDIATKTYIDIDSREILKIPYYSTNVLPIRISDILEILSLQSKNAKQIYKIKIQDNLPKQIVSLDFILSQANRHEVLVSFDKSKLEIQNINDDNGENTFIQKYLCDDFKEFLGKPRDNKIEIIKNNDDILAIKYCVESTSKANKEIIVKALSDETPSA

SEQ ID NO: 94 - protein, 1247 aa, synthetic construct
KSLSINIDMGAINNGIFIATCQDDKIIDKNAFDIKFRKGKLNFSKIDRTLRRHTRRSFDRDRFVLRLLGEILPLENLSNNQKEKLFGLFKNRGFNYLNVNFNAEIDSDNLEILNALDRYYFKDCRVLSDFENSISKIFNELENNEILAFLDDQAQILNQAKEHKNKILNKNINAILEFLESIKNESFKNNKHRKSYLKDIKNEIENSFKDIILKLKIFKNSQELYYFIGNIANFQTRILRRYFNAKFDLVFDDAKLKKNILRNINYLDFISTDEKANKNKILENLNAFSTLEFLKNTDPIVTIPPYENAKNKKPQSCQALVINDEKITPSLKDIAHKILSNSNFECLKTDENGVLADNIKDNEIAKYLQRILDISKGILDDKELYPRLLEKDENAKIFAQEIRLNSVELKEFKDFAKKYYDEVNLAKKGIIKNELLKPCCLHTPHKNKNKNALISALFLKSITQKEIENLEDFFANNKISGNQTFKGFFERLSELKKRYQNRFFHILEHEPTKELEGILKNYKKVMEKIVEHNSNFSFKAPFDDSTISTNFNYLTQLGDIIFDEKSRGFAKTCKFHTLENLIRSSAKSAIASRLASNSARLINGKIEMYLDRLAHEIIKKIDFTDIYNVQINVEMNKFNFESNLSKLGLAKERQKDEESFICPYSGAKISQTNCEYDHILPRSKGLYNSLANLIPTSSTSNQIKSNTKYLLSNLDENYLKYIFAKTQTTDLNSFKAFIDENISKIDENDFTNFKNLSFFEQIAFRHALFLDTDDNSFKKALRLLKLDTIKTHSNGTQKRFINILIEKISKLTKSGIDLNFIDSKLVSSTRKDLAQNDTSIAKQEIQDSHSHCVDASIVFYLANSKIIKGQIEPDYDYFKDIYPKDSDIILPQSKQYLELNQKSQKSKKLFDRSVYSLVYEGKFDEKQKKILTQYELLKENGFVDTHKVFELIFKSFKDKDTIVLKDLKFLDNHLKSYIRRDIFSIFFNEKGELKEAKELKSATKNIDKFYTILSQNQDKIYTIKLDEKAKEKKTLQRNKVIELYKEIFYTKNAKPRARGKNRVTFSLPVYAKDAKYAIKRNSGFAGLKNKDIATKTYIDIDSREILKIPYYSTNVLPIRISDILEILSLQSKNAKQIYKIKIQDNLPKQIVSLDFILSQANRHEVLVSFDKSKLEIQNINDDNGENTFIQKYLCDDFKEFLGKPRDNKIEIIKNNDDILAIKYCVESTSKANKEIIVKALSDETPSA

SEQ ID NO: 95 - protein, 1247 aa, synthetic construct
KSLSINIDMGAINNGIFIATCQDDKIIDKNAFDIKFRKGKLNFSKIDRTLRRHTRRSFDRDRFVLRLLGEILPLENLSNNQKEKLFGLFKNRGFNYLNVNFNAEIDSDNLEILNALDRYYFKDCRVLSDFENSISKIFNELENNEILAFLDDQAQILNQAKEHKNKILNKNINAILEFLESIKNESFKNNKHRKSYLKDIKNEIENSFKDIILKLKIFKNSQELYYFIGNIANFQTRILRRYFNAKFDLVFDDAKLKKNILRNINYLDFISTDEKANKNKILENLNAFSTLEFLKNTDPIVTIPPYENAKNKKPQSCQALVINDEKITPSLKDIAHKILSNSNFECLKTDENGVLADNIKDNEIAKYLQRILDISKGILDDKELYPRLLEKDENAKIFAQEIRLNSVELKEFKDFAKKYYDEVNLAKKGIIKNELLKPCCLHTPHKNKNKNALISALFLKSITQKEIENLEDFFANNKISGNQTFKGFFERLSELKKRYQNRFFHILRHEPTKELEGILKNYKKVMEKIVEHNSNFSFKAPFDDSTISTNFNYLTQLGDIIFDEKSRGFAKTCKFHTLENLIRSSAKSAIASRLASNSARLINGKIEMYLDRLAHEIIKKIDFTDIYNVQINVEMNKFNFESNLSKLGLAKERQKDEESFICPYSGAKISQTNCEYDHILPRSKGLYNSLANLIPTSSTSNQIKSNTKYLLSNLDENYLKYIFAKTQTTDLNSFKAFIDENISKIDENDFTNFKNLSFFEQIAFRHALFLDTDDNSFKKALRLLKLDTIKTHSNGTQKRFINILIEKISKLTKSGIDLNFIDSKLVSSTRKDLAQNDTSIAKQEIQDSHSHCVDASIVFYLANSKIIKGQIEPDYDYFKDIYPKDSDIILPQSKQYLELNQKSQKSKKLFDRSVYSLVYEGKFDEKQKKILTQYELLKENGFVDTHKVFELIFKSFKDKDTIVLKDLKFLDNHLKSYIRKDIFSIFFNEKGELKEAKELKSATKNIDKFYTILSQNQDKIYTIKLDEKAKEKKTLQRNKVIELYKEIFYTKNAKPRARGKNRVTFSLPVYAKDAKYAIKRNSGFAGLKNKDIATKTYIDIDSREILKIPYYSTNVLPIRISDILEILSLQSKNAKQIYKIKIQDNLPKQIVSLDFILSQANRHEVLVSFDKSKLEIQNINDDNGENTFIQKYLCDDFKEFLGKPRDNKIEIIKNNDDILAIKYCVESTSKANKEIIVKALSDETPSA

SEQ ID NO: 96 - protein, 1247 aa, synthetic construct
KSLSINIDMGAINNGIFIATCQDDKIIDKNAFDIKFRKGKLNFSKIDRTLRRHTRRSFDRDRFVLRLLGEILPLENLSNNQKEKLFGLFKNRGFNYLNVNFNAEIDSDNLEILNALDRYYFKDCRVLSDFENSISKIFNELENNEILAFLDDQAQILNQAKEHKNKILNKNINAILEFLESIKNESFKNNKHRKSYLKDIKNEIENSFKDIILKLKIFKNSQELYYFIGNIANFQTRILRRYFNAKFDLVFDDAKLKKNILRNINYLDFISTDEKANKNKILENLNAFSTLEFLKNTDPIVTIPPYENAKNKKPQSCQALVINDEKITPSLKDIAHKILSNSNFECLKTDENGVLADNIKDNEIAKYLQRILDISKGILDDKELYPRLLEKDENAKIFAQEIRLNSVELKEFKDFAKKYYDEVNLAKKGIIKNELLKPCCLHTPHKNKNKNALISALFLKSITQKEIENLEDFFANNKISGNQTFKGFFERLSELKKRYQNRFFHILEHEPTKELEGILKNYKKVMEKIVEHNSNFSFKAPFDDSTISTNFNYLTQLGDIIFDEKSRGFAKTCKFHTLENLIRSSAKSAIASRLASNSARLINGKIEMYLDRLAHEIIKKIDFTDIYNVQINVEMNKFNFESNLSKLGLAKERQKDEESFICPYSGAKISQTNCEYDHILPRSKGLYNSLANLIPTSSTSNQIKSNTKYLLSNLDENYLKYIFAKTQTTDLNSFKAFIDENISKIDENDFTNFKNLSFFEQIAFRHALFLDTDDNSFKKALRLLKLDTIKTHSNGTQKRFINILIEKISKLTKSGIDLNFIDSKLVSSTRKDLAQNDTSIAKQEIQDSHSHCVDASIVFYLANSKIIKGQIEPDYDYFKDIYPKDSDIILPQSKQYLELNQKSQKSKKLFDRSVYSLVYEGKFDEKQKKILTQYELLKENGFVDTHKVFELIFKSFKDKDTIVLKDLKFLDNHLKSYIRKDIFSIFFNEKGELKEAKELKSATKNIDKFYTILSQNQDKIYTIKLDEKAKEKKTLQRNKVIELYKEIFYTKNAKPRARGKNRVTFSLPVYAKDAKYAIKRNSGFAGLKNKDIATKTYIDIDSREILKIPYYSTNVLPIRISRILEILSLQSKNAKQIYKIKIQDNLPKQIVSLDFILSQANRHEVLVSFDKSKLEIQNINDDNGENTFIQKYLCDDFKEFLGKPRDNKIEIIKNNDDILAIKYCVESTSKANKEIIVKALSDETPSA

SEQ ID NO: 97 - protein, 1247 aa, synthetic construct
KSLSINIDMGAINNGIFIATCQDDKIIDKNAFDIKFRKGKLNFSKIDRTLRRHTRRSFDRDRFVLRLLGEILPLENLSNNQKEKLFGLFKNRGFNYLNVNFNAEIDSDNLEILNALDRYYFKDCRVLSDFENSISKIFNELENNEILAFLDDQAQILNQAKEHKNKILNKNINAILEFLESIKNESFKNNKHRKSYLKDIKNEIENSFKDIILKLKIFKNSQELYYFIGNIANFQTRILRRYFNAKFDLVFDDAKLKKNILRNINYLDFISTDEKANKNKILENLNAFSTLEFLKNTDPIVTIPPYENAKNKKPQSCQALVINDEKITPSLKDIAHKILSNSNFECLKTDENGVLADNIKDNEIAKYLQRILDISKGILDDKELYPRLLEKDENAKIFAQEIRLNSVELKEFKDFAKKYYDEVNLAKKGIIKNELLKPCCLHTPHKNKNKNALISALFLKSITQKEIENLEDFFANNKISGNQTFKGFFERLSELKKRYQNRFFHILEHEPTKELEGILKNYKKVMEKIVEHNSNFSFKAPFDDSTISTNFNYLTQLGDIIFDEKSRGFAKTCKFHTLENLIRSSAKSAIASRLASNSARLINGKIEMYLDRLAHEIIKKIDFTDIYNVQINVEMNKFNFESNLSKLGLAKERQKDEESFICPYSGAKISQTNCEYDHILPRSKGLYNSLANLIPTSSTSNQIKSNTKYLLSNLDENYLKYIFAKTQTTDLNSFKAFIDENISKIDENDFTNFKNLSFFEQIAFRHALFLDTDDNSFKKALRLLKLDTIKTHSNGTQKRFINILIEKISKLTKSGIDLNFIDSKLVSSTRKDLAQNDTSIAKQEIQDSHSHCVDASIVFYLANSKIIKGQIEPDYDYFKDIYPKDSDIILPQSKQYLELNQKSQKSKKLFDRSVYSLVYEGKFDEKQKKILTQYELLKENGFVDTHKVFELIFKSFKDKDTIVLKDLKFLDNHLKSYIRKDIFSIFFNEKGELKEAKELKSATKNIDKFYTILSQNQDKIYTIKLDEKAKEKKTLQRNKVIELYKEIFYTKNAKPRARGKNRVTFSLPVYAKDAKYAIKRNSGFAGLKNKDIATKTYIDIDSREILKIPYYSTNVLPIRISDILEILSLQSKNAKQIYKIKIQDNLPKQIVSLDFILSQANRHEVLVSFDKSKLEIQNINDDNGENTFIQKYLCDDFKEFLGKPRDNKIEIIKNNDDILAIKYCVGSTSKANKEIIVKALSDETPSA

SEQ ID NO: 98 - protein, 1247 aa, synthetic construct
KSLSINIDMGAINNGIFIATCQDDKIIDKNAFDIKFRKGKLNFSKIDRTLRRHTRRSFDRDRFVLRLLGEILPLENLSNNQKEKLFGLFKNRGFNYLNVNFNAEIDSDNLEILNALDRYYFKDCRVLSDFENSISKIFNELENNEILAFLDDQAQILNQAKEHKNKILNKNINAILEFLESIKNESFKNNKHRKSYLKDIKNEIENSFKDIILKLKIFKNSQELYYFIGNIANFQTRILRRYFNAKFDLVFDDAKLKKNILRNINYLDFISTDEKANKNKILENLNAFSTLEFLKNTDPIVTIPPYENAKNKKPQSCQALVINDEKITPSLKDIAHKILSNSNFECLKTDENGVLADNIKDNEIAKYLQRILDISKGILDDKELYPRLLEKDENAKIFAQEIRLNSVELKEFKDFAKKYYDEVNLAKKGIIKNELLKPCCLHTPHKNKNKNALISALFLKSITQKEIENLEDFFANNKISGNQTFKGFFERLSELKKRYQNRFFHILEHEPTKELEGILKNYKKVMEKIVEHNSNFSFKAPFDDSTISTNFNYLTQLGDIIFDEKSRGFAKTCKFHTLENLIRSSAKSAIASRLASNSARLINGKIEMYLDRLAHEIIKKIDFTDIYNVQINVEMNKFNFESNLSKLGLAKERQKDEESFICPYSGAKISQTNCEYDHILPRSKGLYNSLANLIPTSSTSNQIKSNTKYLLSNLDENYLKYIFAKTQTTDLNSFKAFIDENISKIDENDFTNFKNLSFFEQIAFRHALFLDTDDNSFKKALRLLKLDTIKTHSNGTQKRFINILIEKISKLTKSGIDLNFIDSKLVSSTRKDLAQNDTSIAKQEIQDSHSHCVDASIVFYLANSKIIKGQIEPDYDYFKDIYPKDSDIILPQSKQYLELNQKSQKSKKLFDRSVYSLVYEGKFDEKQKKILTQYELLKENGFVDTHKVFELIFKSFKDKDTIVLKDLKFLDNHLKSYIRKDIFSIFFNEKGELKEAKELKSATKNIDKFYTILSQNQDKIYTIKLDEKAKEKKTLQRNKVIELYKEIFYTKNAKPRARGKNRVTFSLPVYAKDAKYAIKRNSGFAGLKNKDIATKTYIDIDSREILKIPYYSTNVLPIRISDILEILSLQSKNAKQIYKIKIQDNLPKQIVSLDFILSQANRHEVLVSFDKSKLEIQNINDDNGENTFIQKYLCDDFKEFLGKPRDNKIEIIKNNDDILAIKYCVRSTSKANKEIIVKALSDETPSA

SEQ ID NO: 99 - protein, 1247 aa, synthetic construct
KSLSINIDMGAINNGIFIATCQDDKIIDKNAFDIKFRKGKLNFSKIDRTLRRHTRRSFDRDRFVLRLLGEILPLENLSNNQKEKLFGLFKNRGFNYLNVNFNAEIDSDNLEILNALDRYYFKDCRVLSDFENSISKIFNELENNEILAFLDDQAQILNQAKEHKNKILNKNINAILEFLESIKNESFKNNKHRKSYLKDIKNEIENSFKDIILKLKIFKNSQELYYFIGNIANFQTRILRRYFNAKFDLVFDDAKLKKNILRNINYLDFISTDEKANKNKILENLNAFSTLEFLKNTDPIVTIPPYENAKNKKPQSCQALVINDEKITPSLKDIAHKILSNSNFECLKTDENGVLADNIKDNEIAKYLQRILDISKGILDDKELYPRLLEKDENAKIFAQEIRLNSVELKEFKDFAKKYYDEVNLAKKGIIKNELLKPCCLHTPHKNKNKNALISALFLKSITQKEIENLEDFFANNKISGNQTFKGFFERLSELKKRYQNRFFHILEHEPTKELEGILKNYKKVMEKIVEHNSNFSFKAPFDDSTISTNFNYLTQLGDIIFDEKSRGFAKTCKFHTLENLIRSSAKSAIASRLASNSARLINGKIEMYLDRLAHEIIKKIDFTDIYNVQINVEMNKFNFESNLSKLGLAKERQKDEESFICPYSGAKISQTNCEYDHILPRSKGLYNSLANLIPTSSTSNQIKSNTKYLLSNLDENYLKYIFAKTQTTDLNSFKAFIDENISKIDENDFTNFKNLSFFEQIAFRHALFLDTDDNSFKKALRLLKLDTIKTHSNGTQKRFINILIEKISKLTKSGIDLNFIDSKLVSSTRKDLAQNDTSIAKQEIQDSHSHCVDASIVFYLANSKIIKGQIEPDYDYFKDIYPKDSDIILPQSKQYLELNQKSQKSKKLFDRSVYSLVYEGKFDEKQKKILTQYELLKENGFVDTHKVFELIFKSFKDKDTIVLKDLKFLDNHLKSYRRKDIFSIFFNEKGELKEAKELKSATKNIDKFYTILSQNQDKIYTIKLDEKAKEKKTLQRNKVIELYKEIFYTKNAKPRARGKNRVTFSLPVYAKDAKYAIKRNSGFAGLKNKDIATKTYIDIDSREILKIPYYSTNVLPIRISDILEILSLQSKNAKQIYKIKIQDNLPKQIVSLDFILSQANRHEVLVSFDKSKLEIQNINDDNGENTFIQKYLCDDFKEFLGKPRDNKIEIIKNNDDILAIKYCVESTSKANKEIIVKALSDETPSA

SEQ ID NO: 100 - protein, 1247 aa, synthetic construct
KSLSINIDMGAINNGIFIATCQDDKIIDKNAFDIKFRKGKLNFSKIDRTLRRHTRRSFDRDRFVLRLLGEILPLENLSNNQKEKLFGLFKNRGFNYLNVNFNAEIDSDNLEILNALDRYYFKDCRVLSDFENSISKIFNELENNEILAFLDDQAQILNQAKEHKNKILNKNINAILEFLESIKNESFKNNKHRKSYLKDIKNEIENSFKDIILKLKIFKNSQELYYFIGNIANFQTRILRRYFNAKFDLVFDDAKLKKNILRNINYLDFISTDEKANKNKILENLNAFSTLEFLKNTDPIVTIPPYENAKNKKPQSCQALVINDEKITPSLKDIAHKILSNSNFECLKTDENGVLADNIKDNEIAKYLQRILDISKGILDDKELYPRLLEKDENAKIFAQEIRLNSVELKEFKDFAKKYYDEVNLAKKGIIKNELLKPCCLHTPHKNKNKNALISALFLKSITQKEIENLEDFFANNKISGNQTFKGFFERLSELKKRYQNRFFHILEHEPTKELEGILKNYKKVMEKIVEHNSNFSFKAPFDDSTISTNFNYLTQLGDIIFDEKSRGFAKTCKFHTLENLIRSSAKSAIASRLASNSARLINGKIEMYLDRLAHEIIKKIDFTDIYNVQINVEMNKFNFESNLSKLGLAKERQKDEESFICPYSGAKISQTNCEYDHILPRSKGLYNSLANLIPTSSTSNQIKSNTKYLLSNLDENYLKYIFAKTQTTDLNSFKAFIDENISKIDENDFTNFKNLSFFEQIAFRHALFLDTDDNSFKKALRLLKLDTIKTHSNGTQKRFINILIEKISKLTKSGIDLNFIDSKLVSSTRKDLAQNDTSIAKQEIQDSHSHCVDASIVFYLANSKIIKGQIEPDYDYFKDIYPKDSDIILPQSKQYLELNQKSQKSKKLFDRSVYSLVYEGKFDEKQKKILTQYELLKENGFVDTHKVFELIFKSFKDKDTIVLKDLKFLDNHLKSYIRKDIFSIFFNEKGELKEAKELKSATKNIDKFYTILSQNQDKIYTIKLDEKAKEKKTLQRNKVIELYKEIFYTKNAKPRARGKNRVTFSLPVYAKDAKYAIKRNSGFAGLKNKDIATKTYIDIDSREILKIPYYSTNVLPIRISDILEILSLQSKNAKQIYKIKIQDNLPKQIVSLDFILSQRNRHEVLVSFDKSKLEIQNINDDNGENTFIQKYLCDDFKEFLGKPRDNKIEIIKNNDDILAIKYCVESTSKANKEIIVKALSDETPSA

SEQ ID NO: 101 - protein, 1247 aa, synthetic construct
KSLSINIDMGAINNGIFIATCQDDKIIDKNAFDIKFRKGKLNFSKIDRTLRRHTRRSFDRDRFVLRLLGEILPLENLSNNQKEKLFGLFKNRGFNYLNVNFNAEIDSDNLEILNALDRYYFKDCRVLSDFENSISKIFNELENNEILAFLDDQAQILNQAKEHKNKILNKNINAILEFLESIKNESFKNNKHRKSYLKDIKNEIENSFKDIILKLKIFKNSQELYYFIGNIANFQTRILRRYFNAKFDLVFDDAKLKKNILRNINYLDFISTDEKANKNKILENLNAFSTLEFLKNTDPIVTIPPYENAKNKKPQSCQALVINDEKITPSLKDIAHKILSNSNFECLKTDENGVLADNIKDNEIAKYLQRILDISKGILDDKELYPRLLEKDENAKIFAQEIRLNSVELKEFKDFAKKYYDEVNLAKKGIIKNELLKPCCLHTPHKNKNKNALISALFLKSITQKEIENLEDFFANNKISGNQTFKGFFERLSELKKRYQNRFFHILEHEPTKELEGILKNYKKVMEKIVEHNSNFSFKAPFDDSTISTNFNYLTQLGDIIFDEKSRGFAKTCKFHTLENLIRSSAKSAIASRLASNSARLINGKIEMYLDRLAHEIIKKIDFTDIYNVQINVEMNKFNFESNLSKLGLAKERQKDEESFICPYSGAKISQTNCEYDHILPRSKGLYNSLANLIPTSSTSNQIKSNTKYLLSNLDENYLKYIFAKTQTTDLNSFKAFIDENISKIDENDFTNFKNLSFFEQIAFRHALFLDTDDNSFKKALRLLKLDTIKTHSNGTQKRFINILIEKISKLTKSGIDLNFIDSKLVSSTRKDLAQNDTSIAKQEIQDSHSHCVDASIVFYLANSKIIKGQIEPDYDYFKDIYPKDSDIILPQSKQYLELNQKSQKSKKLFDRSVYSLVYEGKFDEKQKKILTQYELLKENGFVDTHKVFELIFKSFKDKDTIVLKDLKFLDNHLKSYIRKDIFSIFFNEKGELKEAKELKSATKNIDKFYTILSQNQDKIYTIKLDEKAKEKKTLQRNKVIELYKEIFYTKNAKPRARGKNRVTFSLPVYAKDAKYAIKRNSGFAGLKNKSIATKTYIDIDSREILKIPYYSTNVLPIRISDILEILSLQSKNAKQIYKIKIQDNLPKQIVSLDFILSQARRHEVLVSFDKSKLEIQNINDDNGENTFIQKYLCDDFKEFLGKPRDNKIEIIKNNDDILAIKYCVESTSKANKEIIVKALSDETPSA

SEQ ID NO: 102 - protein, 1247 aa, synthetic construct
KSLSINIDMGAINNGIFIATCQDDKIIDKNAFDIKFRKGKLNFSKIDRTLRRHTRRSFDRDRFVLRLLGEILPLENLSNNQKEKLFGLFKNRGFNYLNVNFNAEIDSDNLEILNALDRYYFKDCRVLSDFENSISKIFNELENNEILAFLDDQAQILNQAKEHKNKILNKNINAILEFLESIKNESFKNNKHRKSYLKDIKNEIENSFKDIILKLKIFKNSQELYYFIGNIANFQTRILRRYFNAKFDLVFDDAKLKKNILRNINYLDFISTDEKANKNKILENLNAFSTLEFLKNTDPIVTIPPYENAKNKKPQSCQALVINDEKITPSLKDIAHKILSNSNFECLKTDENGVLADNIKDNEIAKYLQRILDISKGILDDKELYPRLLEKDENAKIFAQEIRLNSVELKEFKDFAKKYYDEVNLAKKGIIKNELLKPCCLHTPHKNKNKNALISALFLKSITQKEIENLEDFFANNKISGNQTFKGFFERLSELKKRYQNRFFHILEHEPTKELEGILKNYKKVMEKIVEHNSNFSFKAPFDDSTISTNFNYLTQLGDIIFDEKSRGFAKTCKFHTLENLIRSSAKSAIASRLASNSARLINGKIEMYLDRLAHEIIKKIDFTDIYNVQINVEMNKFNFESNLSKLGLAKERQKDEESFICPYSGAKISQTNCEYDHILPRSKGLYNSLANLIPTSSTSNQIKSNTKYLLSNLDENYLKYIFAKTQTTDLNSFKAFIDENISKIDENDFTNFKNLSFFEQIAFRHALFLDTDDNSFKKALRLLKLDTIKTHSNGTQKRFINILIEKISKLTKSGIDLNFIDSKLVSSTRKDLAQNDTSIAKQEIQDSHSHCVDASIVFYLANSKIIKGQIEPDYDYFKDIYPKDSDIILPQSKQYLELNQKSQKSKKLFDDSVYSLVYEGKFDEKQKKILTQYELLKENGFVDTHKVFELIFKSFKDKDTIVLKDLKFLDNHLKSYIRKDIFSIFFNEKGELKEAKELKSATKNIDKFYTILSQNQDKIYTIKLDEKAKEKKTLQRNKVIELYKEIFYTKNAKPRARGKNRVTFSLPVYAKDAKYAIKRNSGFAGLKNKSIATKTYIDIDSREILKIPYYSTNVLPIRISDILEILSLQSKNAKQIYKIKIQDNLPKQIVSLDFILSQARRHEVLVSFDKSKLEIQNINDDNGENTFIQKYLCDDFKEFLGKPRDNKIEIIKNNDDILAIKYCVESTRKANKEIIVKALSDETPSA

SEQ ID NO: 103 - protein, 1247 aa, synthetic construct
KSLSINIDMGAINNGIFIATCQDDKIIDKNAFDIKFRKGKLNFSKIDRTLRRHTRRSFDRDRFVLRLLGEILPLENLSNNQKEKLFGLFKNRGFNYLNVNFNAEIDSDNLEILNALDRYYFKDCRVLSDFENSISKIFNELENNEILAFLDDQAQILNQAKEHKNKILNKNINAILEFLESIKNESFKNNKHRKSYLKDIKNEIENSFKDIILKLKIFKNSQELYYFIGNIANFQTRILRRYFNAKFDLVFDDAKLKKNILRNINYLDFISTDEKANKNKILENLNAFSTLEFLKNTDPIVTIPPYENAKNKKPQSCQALVINDEKITPSLKDIAHKILSNSNFECLKTDENGVLADNIKDNEIAKYLQRILDISKGILDDKELYPRLLEKDENAKIFAQEIRLNSVELKEFKDFAKKYYDEVNLAKKGIIKNELLKPCCLHTPHKNKNKNALISALFLKSITQKEIENLEDFFANNKISGNQTFKGFFERLSELKKRYQNRFFHILEHEPTKELEGILKNYKKVMEKIVEHNSNFSFKAPFDDSTISTNFNYLTQLGDIIFDEKSRGFAKTCKFHTLENLIRSSAKSAIASRLASNSARLINGKIEMYLDRLAHEIIKKIDFTDIYNVQINVEMNKFNFESNLSKLGLAKERQKDEESFICPYSGAKISQTNCEYDHILPRSKGLYNSLANLIPTSSTSNQIKSNTKYLLSNLDENYLKYIFAKTQTTDLNSFKAFIDENISKIDENDFTNFKNLSFFEQIAFRHALFLDTDDNSFKKALRLLKLDTIKTHSNGTQKRFINILIEKISKLTKSGIDLNFIDSKLVSSTRKDLAQNDTSIAKQEIQDSHSHCVDASIVFYLANSKIIKGQIEPDYDYFKDIYPKDSDIILPQSKQYLELNQKSQKSKKLFDNSVYSLVYEGKFDEKQKKILTQYELLKENGFVDTHKVFELIFKSFKDKDTIVLKDLKFLDNHLKSYIRKDIFSIFFNEKGELKEAKELKSATKNIDKFYTILSQNQDKIYTIKLDEKAKEKKTLQRNKVIELYKEIFYTKNAKPRARGKNRVTFSLPVYAKDAKYAIKRNSGFAGLKNKSIATKTYIDIDSREILKIPYYSTNVLPIRISDILEILSLQSKNAKQIYKIKIQDNLPKQIVSLDFILSQARRHEVLVSFDKSKLEIQNINDDNGENTFIQKYLCDDFKEFLGKPRSNKIEIIKNNDDILAIKYCVESTSKANKEIIVKALSDETPSA

SEQ ID NO: 104 - protein, 1247 aa, synthetic construct; identical to SEQ ID NO: 57

SEQ ID NO: 105 - protein, 1247 aa, synthetic construct
KSLSINIDMGAINNGIFIATCQDDKIIDKNAFDIKFRKGKLNFSKIDRTLRRHTRRSFDRDRFVLRLLGEILPLENLSNNQKEKLFGLFKNRGFNYLNVNFNAEIDSDNLEILNALDRYYFKDCRVLSDFENSISKIFNELENNEILAFLDDQAQILNQAKEHKNKILNKNINAILEFLESIKNESFKNNKHRKSYLKDIKNEIENSFKDIILKLKIFKNSQELYYFIGNIANFQTRILRRYFNAKFDLVFDDAKLKKNILRNINYLDFISTDEKANKNKILENLNAFSTLEFLKNTDPIVTIPPYENAKNKKPQSCQALVINDEKITPSLKDIAHKILSNSNFECLKTDENGVLADNIKDNEIAKYLQRILDISKGILDDKELYPRLLEKDENAKIFAQEIRLNSVELKEFKDFAKKYYDEVNLAKKGIIKNELLKPCCLHTPHKNKNKNALISALFLKSITQKEIENLEDFFANNKISGNQTFKGFFERLSELKKRYQNRFFHILEHEPTKELEGILKNYKKVMEKIVEHNSNFSFKAPFDDSTISTNFNYLTQLGDIIFDEKSRGFAKTCKFHTLENLIRSSAKSAIASRLASNSARLINGKIEMYLDRLAHEIIKKIDFTDIYNVQINVEMNKFNFESNLSKLGLAKERQKDEESFICPYSGAKISQTNCEYDHILPRSKGLYNSLANLIPTSSTSNQIKSNTKYLLSNLDENYLKYIFAKTQTTDLNSFKAFIDENISKIDENDFTNFKNLSFFEQIAFRHALFLDTDDNSFKKALRLLKLDTIKTHSNGTQKRFINILIEKISKLTKSGIDLNFIDSKLVSSTRKDLAQNDTSIAKQEIQDSHSHCVDASIVFYLANSKIIKGQIEPDYDYFKDIYPKDSDIILPQSKQYLELNQKSQKSKKLFDDSVYSLVYEGKFDEKQKKILTQYELLKENGFVDTHKVFELIFKSFKDKDTIVLKDLKFLDNHLKSYIRKDIFSIFFNEKGELKEAKELKSATKNIDKFYTILSQNQDKIYTIKLDEKAKEKKTLQRNKVIELYKEIFYTKNAKPRARGKNRVTFSLPVYAKDAKYAIKRNSGFAGLKNKSIATKTYIDIDSREILKIPYYSTNVLPIRISDILEILSLQSKNAKQIYKIKIQDNLPKQIVSLDFILSQARRHEVLVSFDKSKLEIQNINDDNGENTFIQKYLCDDFKEFLGKPRDNKIEIIKNNDDILAIKYCVGSTSKANKEIIVKALSDETPSA

SEQ ID NO: 106 - protein, 1247 aa, synthetic construct
KSLSINIDMGAINNGIFIATCQDDKIIDKNAFDIKFRKGKLNFSKIDRTLRRHTRRSFDRDRFVLRLLGEILPLENLSNNQKEKLFGLFKNRGFNYLNVNFNAEIDSDNLEILNALDRYYFKDCRVLSDFENSISKIFNELENNEILAFLDDQAQILNQAKEHKNKILNKNINAILEFLESIKNESFKNNKHRKSYLKDIKNEIENSFKDIILKLKIFKNSQELYYFIGNIANFQTRILRRYFNAKFDLVFDDAKLKKNILRNINYLDFISTDEKANKNKILENLNAFSTLEFLKNTDPIVTIPPYENAKNKKPQSCQALVINDEKITPSLKDIAHKILSNSNFECLKTDENGVLADNIKDNEIAKYLQRILDISKGILDDKELYPRLLEKDENAKIFAQEIRLNSVELKEFKDFAKKYYDEVNLAKKGIIKNELLKPCCLHTPHKNKNKNALISALFLKSITQKEIENLEDFFANNKISGNQTFKGFFERLSELKKRYQNRFFHILEHEPTKELEGILKNYKKVMEKIVEHNSNFSFKAPFDDSTISTNFNYLTQLGDIIFDEKSRGFAKTCKFHTLENLIRSSAKSAIASRLASNSARLINGKIEMYLDRLAHEIIKKIDFTDIYNVQINVEMNKFNFESNLSKLGLAKERQKDEESFICPYSGAKISQTNCEYDHILPRSKGLYNSLANLIPTSSTSNQIKSNTKYLLSNLDENYLKYIFAKTQTTDLNSFKAFIDENISKIDENDFTNFKNLSFFEQIAFRHALFLDTDDNSFKKALRLLKLDTIKTHSNGTQKRFINILIEKISKLTKSGIDLNFIDSKLVSSTRKDLAQNDTSIAKQEIQDSHSHCVDASIVFYLANSKIIKGQIEPDYDYFKDIYPKDSDIILPQSKQYLELNQKSQKSKKLFDDSVYSLVYEGKFDEKQKKILTQYELLKENGFVDTHKVFELIFKSFKDKDTIVLKDLKFLDNHLKSYIRKDIFSIFFNEKGELKEAKELKSATKNIDKFYTILSQNQDKIYTIKLDEKAKEKKTLQRNKVIELYKEIFYTKNAKPRARGKNRVTFSLPVYAKDAKYAIKRNSGFAGLKNKSIATKTYIDIDSREILKIPYYSTNVLPIRISDILEILSLQSKNAKQIYKIKIQDNLPKQIVSLDFILSQARRHEVLVSFDKSKLEIQNINDDNGENTFIQKYLCDDFKEFLGKPRDNKIEIIKNNDDILAIKYCVSSTSKANKEIIVKALSDETPSA

SEQ ID NO: 107 - protein, 1247 aa, synthetic construct
KSLSINIDMGAINNGIFIATCQDDKIIDKNAFDIKFRKGKLNFSKRDRTLRRHTRRSFDRDRFVLRLLGEILPLENLSNNQKEKLFGLFKNRGFNYLNVNFNAEIDSDNLEILNALDRYYFKDCRVLSDFENSISKIFNELENNEILAFLDDQAQILNQAKEHKNKILNKNINAILEFLESIKNESFKNNKHRKSYLKDIKNEIENSFKDIILKLKIFKNSQELYYFIGNIANFQTRILRRYFNAKFDLVFDDAKLKKNILRNINYLDFISTDEKANKNKILENLNAFSTLEFLKNTDPIVTIPPYENAKNKKPQSCQALVINDEKITPSLKDIAHKILSNSNFECLKTDENGVLADNIKDNEIAKYLQRILDISKGILDDKELYPRLLEKDENAKIFAQEIRLNSVELKEFKDFAKKYYDEVNLAKKGIIKNELLKPCCLHTPHKNKNKNALISALFLKSITQKEIENLEDFFANNKISGNQTFKGFFERLSELKKRYQNRFFHILEHEPTKELEGILKNYKKVMEKIVEHNSNFSFKAPFDDSTISTNFNYLTQLGDIIFDEKSRGFAKTCKFHTLENLIRSSAKSAIASRLASNSARLINGKIEMYLDRLAHEIIKKIDFTDIYNVQINVEMNKFNFESNLSKLGLAKERQKDEESFICPYSGAKISQTNCEYDHILPRSKGLYNSLANLIPTSSTSNQIKSNTKYLLSNLDENYLKYIFAKTQTTDLNSFKAFIDENISKIDENDFTNFKNLSFFEQIAFRHALFLDTDDNSFKKALRLLKLDTIKTHSNGTQKRFINILIEKISKLTKSGIDLNFIDSKLVSSTRKDLAQNDTSIAKQEIQDSHSHCVDASIVFYLANSKIIKGQIEPDYDYFKDIYPKDSDIILPQSKQYLELNQKSQKSKKLFDDSVYSLVYEGKFDEKQKKILTQYELLKENGFVDTHKVFELIFKSFKDKDTIVLKDLKFLDNHLKSYIRKDIFSIFFNEKGELKEAKELKSATKNIDKFYTILSQNQDKIYTIKLDEKAKEKKTLQRNKVIELYKEIFYTKNAKPRARGKNRVTFSLPVYAKDAKYAIKRNSGFAGLKNKSIATKTYIDIDSREILKIPYYSTNVLPIRISDILEILSLQSKNAKQIYKIKIQDNLPKQIVSLDFILSQARRHEVLVSFDKSKLEIQNINDDNGENTFIQKYLCDDFKEFLGKPRDNKIEIIKNNDDILAIKYCVESTRKANKEIIVKALSDETPSA

SEQ ID NO: 108 - protein, 1247 aa, synthetic construct
KSLSINIDMGAINNGIFIATCQDDKIIDKNAFDIKFRKRKLNFSKRDRTLRRHTRRSFDRDRFVLRLLGEILPLENLSNNQKEKLFGLFKNRGFNYLNVNFNAEIDSDNLEILNALDRYYFKDCRVLSDFENSISKIFNELENNEILAFLDDQAQILNQAKEHKNKILNKNINAILEFLESIKNESFKNNKHRKSYLKDIKNEIENSFKDIILKLKIFKNSQELYYFIGNIANFQTRILRRYFNAKFDLVFDDAKLKKNILRNINYLDFISTDEKANKNKILENLNAFSTLEFLKNTDPIVTIPPYENAKNKKPQSCQALVINDEKITPSLKDIAHKILSNSNFECLKTDENGVLADNIKDNEIAKYLQRILDISKGILDDKELYPRLLEKDENAKIFAQEIRLNSVELKEFKDFAKKYYDEVNLAKKGIIKNELLKPCCLHTPHKNKNKNALISALFLKSITQKEIENLEDFFANNKISGNQTFKGFFERLSELKKRYQNRFFHILEHEPTKELEGILKNYKKVMEKIVEHNSNFSFKAPFDDSTISTNFNYLTQLGDIIFDEKSRGFAKTCKFHTLENLIRSSAKSAIASRLASNSARLINGKIEMYLDRLAHEIIKKIDFTDIYNVQINVEMNKFNFESNLSKLGLAKERQKDEESFICPYSGAKISQTNCEYDHILPRSKGLYNSLANLIPTSSTSNQIKSNTKYLLSNLDENYLKYIFAKTQTTDLNSFKAFIDENISKIDENDFTNFKNLSFFEQIAFRHALFLDTDDNSFKKALRLLKLDTIKTHSNGTQKRFINILIEKISKLTKSGIDLNFIDSKLVSSTRKDLAQNDTSIAKQEIQDSHSHCVDASIVFYLANSKIIKGQIEPDYDYFKDIYPKDSDIILPQSKQYLELNQKSQKSKKLFDDSVYSLVYEGKFDEKQKKILTQYELLKENGFVDTHKVFELIFKSFKDKDTIVLKDLKFLDNHLKSYIRKDIFSIFFNEKGELKEAKELKSATKNIDKFYTILSQNQDKIYTIKLDEKAKEKKTLQRNKVIELYKEIFYTKNAKPRARGKNRVTFSLPVYAKDAKYAIKRNSGFAGLKNKSIATKTYIDIDSREILKIPYYSTNVLPIRISDILEILSLQSKNAKQIYKIKIQDNLPKQIVSLDFILSQARRHEVLVSFDKSKLEIQNINDDNGENTFIQKYLCDDFKEFLGKPRDNKIEIIKNNDDILAIKYCVESTSKANKEIIVKALSDETPSA

SEQ ID NO: 109 - protein, 1247 aa, synthetic construct
KSLSINIDMGAINNGIFIATCQDDKIIDKNAFDIKFRKRKLNFSKIDRTLRRHTRRSFDRDRFVLRLLGEILPLENLSNNQKEKLFGLFKNRGFNYLNVNFNAEIDSDNLEILNALDRYYFKDCRVLSDFENSISKIFNELENNEILAFLDDQAQILNQAKEHKNKILNKNINAILEFLESIKNESFKNNKHRKSYLKDIKNEIENSFKDIILKLKIFKNSQELYYFIGNIANFQTRILRRYFNAKFDLVFDDAKLKKNILRNINYLDFISTDEKANKNKILENLNAFSTLEFLKNTDPIVTIPPYENAKNKKPQSCQALVINDEKITPSLKDIAHKILSNSNFECLKTDENGVLADNIKDNEIAKYLQRILDISKGILDDKELYPRLLEKDENAKIFAQEIRLNSVELKEFKDFAKKYYDEVNLAKKGIIKNELLKPCCLHTPHKNKNKNALISALFLKSITQKEIENLEDFFANNKISGNQTFKGFFERLSELKKRYQNRFFHILEHEPTKELEGILKNYKKVMEKIVEHNSNFSFKAPFDDSTISTNFNYLTQLGDIIFDEKSRGFAKTCKFHTLENLIRSSAKSAIASRLASNSARLINGKIEMYLDRLAHEIIKKIDFTDIYNVQINVEMNKFNFESNLSKLGLAKERQKDEESFICPYSGAKISQTNCEYDHILPRSKGLYNSLANLIPTSSTSNQIKSNTKYLLSNLDENYLKYIFAKTQTTDLNSFKAFIDENISKIDENDFTNFKNLSFFEQIAFRHALFLDTDDNSFKKALRLLKLDTIKTHSNGTQKRFINILIEKISKLTKSGIDLNFIDSKLVSSTRKDLAQNDTSIAKQEIQDSHSHCVDASIVFYLANSKIIKGQIEPDYDYFKDIYPKDSDIILPQSKQYLELNQKSQKSKKLFDDSVYSLVYEGKFDEKQKKILTQYELLKENGFVDTHKVFELIFKSFKDKDTIVLKDLKFLDNHLKSYIRKDIFSIFFNEKGELKEAKELKSATKNIDKFYTILSQNQDKIYTIKLDEKAKEKKTLQRNKVIELYKEIFYTKNAKPRARGKNRVTFSLPVYAKDAKYAIKRNSGFAGLKNKSIATKTYIDIDSREILKIPYYSTNVLPIRISDILEILSLQSKNAKQIYKIKIQDNLPKQIVSLDFILSQARRHEVLVSFDKSKLEIQNINDDNGENTFIQKYLCDDFKEFLGKPRSNKIEIIKNNDDILAIKYCVESTSKANKEIIVKALSDETPSA

SEQ ID NO: 110 - protein, 1247 aa, synthetic construct
KSLSINIDMGAINNGIFIATCQDDKIIDKNAFDIKFRKGKLNFSKRDRTLRRHTRRSFDRDRFVLRLLGEILPLENLSNNQKEKLFGLFKNRGFNYLNVNFNAEIDSDNLEILNALDRYYFKDCRVLSDFENSISKIFNELENNEILAFLDDQAQILNQAKEHKNKILNKNINAILEFLESIKNESFKNNKHRKSYLKDIKNEIENSFKDIILKLKIFKNSQELYYFIGNIANFQTRILRRYFNAKFDLVFDDAKLKKNILRNINYLDFISTDEKANKNKILENLNAFSTLEFLKNTDPIVTIPPYENAKNKKPQSCQALVINDEKITPSLKDIAHKILSNSNFECLKTDENGVLADNIKDNEIAKYLQRILDISKGILDDKELYPRLLEKDENAKIFAQEIRLNSVELKEFKDFAKKYYDEVNLAKKGIIKNELLKPCCLHTPHKNKNKNALISALFLKSITQKEIENLEDFFANNKISGNQTFKGFFERLSELKKRYQNRFFHILEHEPTKELEGILKNYKKVMEKIVEHNSNFSFKAPFDDSTISTNFNYLTQLGDIIFDEKSRGFAKTCKFHTLENLIRSSAKSAIASRLASNSARLINGKIEMYLDRLAHEIIKKIDFTDIYNVQINVEMNKFNFESNLSKLGLAKERQKDEESFICPYSGAKISQTNCEYDHILPRSKGLYNSLANLIPTSSTSNQIKSNTKYLLSNLDENYLKYIFAKTQTTDLNSFKAFIDENISKIDENDFTNFKNLSFFEQIAFRHALFLDTDDNSFKKALRLLKLDTIKTHSNGTQKRFINILIEKISKLTKSGIDLNFIDSKLVSSTRKDLAQNDTSIAKQEIQDSHSHCVDASIVFYLANSKIIKGQIEPDYDYFKDIYPKDSDIILPQSKQYLELNQKSQKSKKLFDDSVYSLVYEGKFDEKQKKILTQYELLKENGFVDTHKVFELIFKSFKDKDTIVLKDLKFLDNHLKSYIRKDIFSIFFNEKGELKEAKELKSATKNIDKFYTILSQNQDKIYTIKLDEKAKEKKTLQRNKVIELYKEIFYTKNAKPRARGKNRVTFSLPVYAKDAKYAIKRNSGFAGLKNKSIATKTYIDIDSREILKIPYYSTNVLPIRISDILEILSLQSKNAKQIYKIKIQDNLPKQIVSLDFILSQARRHEVLVSFDKSKLEIQNINDDNGENTFIQKYLCDDFKEFLGKPRNNKIEIIKNNDDILAIKYCVESTRKANKEIIVKALSDETPSA

SEQ ID NO: 111 - protein, 1247 aa, synthetic construct
KSLSINIDMGAINNGIFIATCQDDKIIDKNAFDIKFRKGKLNFSKRDRTLRRHTRRSFDRDRFVLRLLGEILPLENLSNNQKEKLFGLFKNRGFNYLNVNFNAEIDSDNLEILNALDRYYFKDCRVLSDFENSISKIFNELENNEILAFLDDQAQILNQAKEHKNKILNKNINAILEFLESIKNESFKNNKHRKSYLKDIKNEIENSFKDIILKLKIFKNSQELYYFIGNIANFQTRILRRYFNAKFDLVFDDAKLKKNILRNINYLDFISTDEKANKNKILENLNAFSTLEFLKNTDPIVTIPPYENAKNKKPQSCQALVINDEKITPSLKDIAHKILSNSNFECLKTDENGVLADNIKDNEIAKYLQRILDISKGILDDKELYPRLLEKDENAKIFAQEIRLNSVELKEFKDFAKKYYDEVNLAKKGIIKNELLKPCCLHTPHKNKNKNALISALFLKSITQKEIENLEDFFANNKISGNQTFKGFFERLSELKKRYQNRFFHILEHEPTKELEGILKNYKKVMEKIVEHNSNFSFKAPFDDSTISTNFNYLTQLGDIIFDEKRRGFAKTCKFHTLENLIRSSAKSAIASRLASNSARLINGKIEMYLDRLAHEIIKKIDFTDIYNVQINVEMNKFNFESNLSKLGLAKERQKDEESFICPYSGAKISQTNCEYDHILPRSKGLYNSLANLIPTSSTSNQIKSNTKYLLSNLDENYLKYIFAKTQTTDLNSFKAFIDENISKIDENDFTNFKNLSFFEQIAFRHALFLDTDDNSFKKALRLLKLDTIKTHSNGTQKRFINILIEKISKLTKSGIDLNFIDSKLVSSTRKDLAQNDTSIAKQEIQDSHSHCVDASIVFYLANSKIIKGQIEPDYDYFKDIYPKDSDIILPQSKQYLELNQKSQKSKKLFDNSVYSLVYEGKFDEKQKKILTQYELLKENGFVDTHKVFELIFKSFKDKDTIVLKDLKFLDNHLKSYIRKDIFSIFFNEKGELKEAKELKSATKNIDKFYTILSQNQDKIYTIKLDEKAKEKKTLQRNKVIELYKEIFYTKNAKPRARGKNRVTFSLPVYAKDAKYAIKRNSGFAGLKNKSIATKTYIDIDSREILKIPYYSTNVLPIRISDILEILSLQSKNAKQIYKIKIQDNLPKQIVSLDFILSQARRHEVLVSFDKSKLEIQNINDDNGENTFIQKYLCDDFKEFLGKPRNNKIEIIKNNDDILAIKYCVESTSKANKEIIVKALSDETPSA

SEQ ID NO: 112 - protein, 1247 aa, synthetic construct
KSLSINIDMGAINNGIFIATCQDDKIIDKNAFDIKFRKGKLNFSKIDRTLRRHTRRSFDRDRFVLRLLGEILPLENLSNNQKEKLFGLFKNRGFNYLNVNFNAEIDSDNLEILNALDRYYFKDCRVLSDFENSISKIFNELENNEILAFLDDQAQILNQAKEHKNKILNKNINAILEFLESIKNESFKNNKHRKSYLKDIKNEIENSFKDIILKLKIFKNSQELYYFIGNIANFQTRILRRYFNAKFDLVFDDAKLKKNILRNINYLDFISTDEKANKNKILENLNAFSTLEFLKNTDPIVTIPPYENAKNKKPQSCQALVINDEKITPSLKDIAHKILSNSNFECLKTDENGVLADNIKDNEIAKYLQRILDISKGILDDKELYPRLLEKDENAKIFAQEIRLNSVELKEFKDFAKKYYDEVNLAKKGIIKNELLKPCCLHTPHKNKNKNALISALFLKSITQKEIENLEDFFANNKISGNQTFKGFFERLSELKKRYQNRFFHILEHEPTKELEGILKNYKKVMEKIVEHNSNFSFKAPFDDSTISTNFNYLTQLGDIIFDEKSRGFAKTCKFHTLENLIRSSAKSAIASRLASNSARLINGKIEMYLDRLAHEIIKKIDFTDIYNVQINVEMNKFNFESNLSKLGLAKERQKDEESFICPYSGAKISQTNCEYDHILPRSKGLYNSLANLIPTSSTSNQIKSNTKYLLSNLDENYLKYIFAKTQTTDLNSFKAFIDENISKIDENDFTNFKNLSFFEQIAFRHALFLDTDDNSFKKALRLLKLDTIKTHSNGTQKRFINILIEKISKLTKSGIDLNFIDSKLVSSTRKDLAQNDTSIAKQEIQDSHSHCVDASIVFYLANSKIIKGQIEPDYDYFKDIYPKDSDIILPQSKQYLELNQKSQKSKKLFDDSVYSLVYEGKFDEKQKKILTQYELLKENGFVDTHKVFELIFKSFKDKDTIVLKDLKFLDNHLKSYIRKDIFSIFFNEKGELKEAKELKSATKNIDKFYTILSQNQDKIYTIKLDEKAKEKKTLQRNKVIELYKEIFYTKNAKPRARGKNRVTFSLPVYAKDAKYAIKRNSGFAGLKNKDIATKTYIDIDSREILKIPYYSTNVLPIRISDILEILSLQSKNAKQIYKIKIQDNLPKQIVSLDFILSQARRHEVLVSFDKSKLEIQNINDDNGENTFIQKYLCDDFKEFLGKPRDNKIEIIKNNDDILAIKYCVESTRKANKEIIVKALSDETPSA

SEQ ID NO: 113 - protein, 1247 aa, synthetic construct
KSLSINIDMGAINNGIFIATCQDDKIIDKNAFDIKFRKGKLNFSKIDRTLRRHTRRSFDRDRFVLRLLGEILPLENLSNNQKEKLFGLFKNRGFNYLNVNFNAEIDSDNLEILNALDRYYFKDCRVLSDFENSISKIFNELENNEILAFLDDQAQILNQAKEHKNKILNKNINAILEFLESIKNESFKNNKHRKSYLKDIKNEIENSFKDIILKLKIFKNSQELYYFIGNIANFQTRILRRYFNAKFDLVFDDAKLKKNILRNINYLDFISTDEKANKNKILENLNAFSTLEFLKNTDPIVTIPPYENAKNKKPQSCQALVINDEKITPSLKDIAHKILSNSNFECLKTDENGVLADNIKDNEIAKYLQRILDISKGILDDKELYPRLLEKDENAKIFAQEIRLNSVELKEFKDFAKKYYDEVNLAKKGIIKNELLKPCCLHTPHKNKNKNALISALFLKSITQKEIENLEDFFANNKISGNQTFKGFFERLSELKKRYQNRFFHILEHEPTKELEGILKNYKKVMEKIVEHNSNFSFKAPFDDSTISTNFNYLTQLGDIIFDEKSRGFAKTCKFHTLENLIRSSAKSAIASRLASNSARLINGKIEMYLDRLAHEIIKKIDFTDIYNVQINVEMNKFNFESNLSKLGLAKERQKDEESFICPYSGAKISQTNCEYDHILPRSKGLYNSLANLIPTSSTSNQIKSNTKYLLSNLDENYLKYIFAKTQTTDLNSFKAFIDENISKIDENDFTNFKNLSFFEQIAFRHALFLDTDDNSFKKALRLLKLDTIKTHSNGTQKRFINILIEKISKLTKSGIDLNFIDSKLVSSTRKDLAQNDTSIAKQEIQDSHSHCVDASIVFYLANSKIIKGQIEPDYDYFKDIYPKDSDIILPQSKQYLELNQKSQKSKKLFDSSVYSLVYEGKFDEKQKKILTQYELLKENGFVDTHKVFELIFKSFKDKDTIVLKDLKFLDNHLKSYIRKDIFSIFFNEKGELKEAKELKSATKNIDKFYTILSQNQDKIYTIKLDEKAKEKKTLQRNKVIELYKEIFYTKNAKPRARGKNRVTFSLPVYAKDAKYAIKRNSGFAGLKNKDIATKTYIDIDSREILKIPYYSTNVLPIRISDILEILSLQSKNAKQIYKIKIQDNLPKQIVSLDFILSQARRHEVLVSFDKSKLEIQNINDDNGENTFIQKYLCDDFKEFLGKPRDNKIEIIKNNDDILAIKYCVESTSKANKEIIVKALSDETPSA

SEQ ID NO: 114 - protein, 1247 aa, synthetic construct
KSLSINIDMGAINNGIFIATCQDDKIIDKNAFDIKFRKGKLNFSKIDRTLRRHTRRSFDRDRFVLRLLGEILPLENLSNNQKEKLFGLFKNRGFNYLNVNFNAEIDSDNLEILNALDRYYFKDCRVLSDFENSISKIFNELENNEILAFLDDQAQILNQAKEHKNKILNKNINAILEFLESIKNESFKNNKHRKSYLKDIKNEIENSFKDIILKLKIFKNSQELYYFIGNIANFQTRILRRYFNAKFDLVFDDAKLKKNILRNINYLDFISTDEKANKNKILENLNAFSTLEFLKNTDPIVTIPPYENAKNKKPQSCQALVINDEKITPSLKDIAHKILSNSNFECLKTDENGVLADNIKDNEIAKYLQRILDISKGILDDKELYPRLLEKDENAKIFAQEIRLNSVELKEFKDFAKKYYDEVNLAKKGIIKNELLKPCCLHTPHKNKNKNALISALFLKSITQKEIENLEDFFANNKISGNQTFKGFFERLSELKKRYQNRFFHILEHEPTKELEGILKNYKKVMEKIVEHNSNFSFKAPFDDSTISTNFNYLTQLGDIIFDEKSRGFAKTCKFHTLENLIRSSAKSAIASRLASNSARLINGKIEMYLDRLAHEIIKKIDFTDIYNVQINVEMNKFNFESNLSKLGLAKERQKDEESFICPYSGAKISQTNCEYDHILPRSKGLYNSLANLIPTSSTSNQIKSNTKYLLSNLDENYLKYIFAKTQTTDLNSFKAFIDENISKIDENDFTNFKNLSFFEQIAFRHALFLDTDDNSFKKALRLLKLDTIKTHSNGTQKRFINILIEKISKLTKSGIDLNFIDSKLVSSTRKDLAQNDTSIAKQEIQDSHSHCVDASIVFYLANSKIIKGQIEPDYDYFKDIYPKDSDIILPQSKQYLELNQKSQKSKKLFDNSVYSLVYEGKFDEKQKKILTQYELLKENGFVDTHKVFELIFKSFKDKDTIVLKDLKFLDNHLKSYIRKDIFSIFFNEKGELKEAKELKSATKNIDKFYTILSQNQDKIYTIKLDEKAKEKKTLQRNKVIELYKEIFYTKNAKPRARGKNRVTFSLPVYAKDAKYAIKRNSGFAGLKNKDIATKTYIDIDSREILKIPYYSTNVLPIRISDILEILSLQSKNAKQIYKIKIQDNLPKQIVSLDFILSQARRHEVLVSFDKSKLEIQNINDDNGENTFIQKYLCDDFKEFLGKPRDNKIEIIKNNDDILAIKYCVESTSKANKEIIVKALSDETPSA

SEQ ID NO: 115 - protein, 1247 aa, synthetic construct
KSLSINIDMGAINNGIFIATCQDDKIIDKNAFDIKFRKGKLNFSKIDRTLRRHTRRSFDRDRFVLRLLGEILPLENLSNNQKEKLFGLFKNRGFNYLNVNFNAEIDSDNLEILNALDRYYFKDCRVLSDFENSISKIFNELENNEILAFLDDQAQILNQAKEHKNKILNKNINAILEFLESIKNESFKNNKHRKSYLKDIKNEIENSFKDIILKLKIFKNSQELYYFIGNIANFQTRILRRYFNAKFDLVFDDAKLKKNILRNINYLDFISTDEKANKNKILENLNAFSTLEFLKNTDPIVTIPPYENAKNKKPQSCQALVINDEKITPSLKDIAHKILSNSNFECLKTDENGVLADNIKDNEIAKYLQRILDISKGILDDKELYPRLLEKDENAKIFAQEIRLNSVELKEFKDFAKKYYDEVNLAKKGIIKNELLKPCCLHTPHKNKNKNALISALFLKSITQKEIENLEDFFANNKISGNQTFKGFFERLSELKKRYQNRFFHILEHEPTKELEGILKNYKKVMEKIVEHNSNFSFKAPFDDSTISTNFNYLTQLGDIIFDEKSRGFAKTCKFHTLENLIRSSAKSAIASRLASNSARLINGKIEMYLDRLAHEIIKKIDFTDIYNVQINVEMNKFNFESNLSKLGLAKERQKDEESFICPYSGAKISQTNCEYDHILPRSKGLYNSLANLIPTSSTSNQIKSNTKYLLSNLDENYLKYIFAKTQTTDLNSFKAFIDENISKIDENDFTNFKNLSFFEQIAFRHALFLDTDDNSFKKALRLLKLDTIKTHSNGTQKRFINILIEKISKLTKSGIDLNFIDSKLVSSTRKDLAQNDTSIAKQEIQDSHSHCVDASIVFYLANSKIIKGQIEPDYDYFKDIYPKDSDIILPQSKQYLELNQKSQKSKKLFDRSVYSLVYEGKFDEKQKKILTQYELLKENGFVDTHKVFELIFKSFKDKDTIVLKDLKFLDNHLKSYIRKDIFSIFFNEKGELKEAKELKSATKNIDKFYTILSQNQDKIYTIKLDEKAKEKKTLQRNKVIELYKEIFYTKNAKPRARGKNRVTFSLPVYAKDAKYAIKRNSGFAGLKNKDIATKTYIDIDSREILKIPYYSTNVLPIRISDILEILSLQSKNAKQIYKIKIQDNLPKQIVSLDFILSQARRHEVLVSFDKSKLEIQNINDDNGENTFIQKYLCDDFKEFLGKPRDNKIEIIKNNDDILAIKYCVESTSKANKEIIVKALSDETPSA

SEQ ID NO: 116 - protein, 1247 aa, synthetic construct
KSLSINIDMGAINNGIFIATCQDDKIIDKNAFDIKFRKGKLNFSKIDRTLRRHTRRSFDRDRFVLRLLGEILPLENLSNNQKEKLFGLFKNRGFNYLNVNFNAEIDSDNLEILNALDRYYFKDCRVLSDFENSISKIFNELENNEILAFLDDQAQILNQAKEHKNKILNKNINAILEFLESIKNESFKNNKHRKSYLKDIKNEIENSFKDIILKLKIFKNSQELYYFIGNIANFQTRILRRYFNAKFDLVFDDAKLKKNILRNINYLDFISTDEKANKNKILENLNAFSTLEFLKNTDPIVTIPPYENAKNKKPQSCQALVINDEKITPSLKDIAHKILSNSNFECLKTDENGVLADNIKDNEIAKYLQRILDISKGILDDKELYPRLLEKDENAKIFAQEIRLNSVELKEFKDFAKKYYDEVNLAKKGIIKNELLKPCCLHTPHKNKNKNALISALFLKSITQKEIENLEDFFANNKISGNQTFKGFFERLSELKKRYQNRFFHILEHEPTKELEGILKNYKKVMEKIVEHNSNFSFKAPFDDSTISTNFNYLTQLGDIIFDEKSRGFAKTCKFHTLENLIRSSAKSAIASRLASNSARLINGKIEMYLDRLAHEIIKKIDFTDIYNVQINVEMNKFNFESNLSKLGLAKERQKDEESFICPYSGAKISQTNCEYDHILPRSKGLYNSLANLIPTSSTSNQIKSNTKYLLSNLDENYLKYIFAKTQTTDLNSFKAFIDENISKIDENDFTNFKNLSFFEQIAFRHALFLDTDDNSFKKALRLLKLDTIKTHSNGTQKRFINILIEKISKLTKSGIDLNFIDSKLVSSTRKDLAQNDTSIAKQEIQDSHSHCVDASIVFYLANSKIIKGQIEPDYDYFKDIYPKDSDIILPQSKQYLELNQKSQKSKKLFDDSVYSLVYEGKFDEKQKKILTQYELLKENGFVDTHKVFELIFKSFKDKDTIVLKDLKFLDNHLKSYIRKDIFSIFFNEKGELKEAKELKSATKNIDKFYTILSQNQDKIYTIKLDEKAKEKKTLQRNKVIELYKEIFYTKNAKPRARGKNRVTFSLPVYAKDAKYAIKRNSGFAGLKNKGIATKTYIDIDSREILKIPYYSTNVLPIRISDILEILSLQSKNAKQIYKIKIQDNLPKQIVSLDFILSQARRHEVLVSFDKSKLEIQNINDDNGENTFIQKYLCDDFKEFLGKPRDNKIEIIKNNDDILAIKYCVESTSKANKEIIVKALSDETPSA

SEQ ID NO: 117 - protein, 1247 aa, synthetic construct
KSLSINIDMGAINNGIFIATCQDDKIIDKNAFDIKFRKGKLNFSKIDRTLRRHTRRSFDRDRFVLRLLGEILPLENLSNNQKEKLFGLFKNRGFNYLNVNFNAEIDSDNLEILNALDRYYFKDCRVLSDFENSISKIFNELENNEILAFLDDQAQILNQAKEHKNKILNKNINAILEFLESIKNESFKNNKHRKSYLKDIKNEIENSFKDIILKLKIFKNSQELYYFIGNIANFQTRILRRYFNAKFDLVFDDAKLKKNILRNINYLDFISTDEKANKNKILENLNAFSTLEFLKNTDPIVTIPPYENAKNKKPQSCQALVINDEKITPSLKDIAHKILSNSNFECLKTDENGVLADNIKDNEIAKYLQRILDISKGILDDKELYPRLLEKDENAKIFAQEIRLNSVELKEFKDFAKKYYDEVNLAKKGIIKNELLKPCCLHTPHKNKNKNALISALFLKSITQKEIENLEDFFANNKISGNQTFKGFFERLSELKKRYQNRFFHILEHEPTKELEGILKNYKKVMEKIVEHNSNFSFKAPFDDSTISTNFNYLTQLGDIIFDEKSRGFAKTCKFHTLENLIRSSAKSAIASRLASNSARLINGKIEMYLDRLAHEIIKKIDFTDIYNVQINVEMNKFNFESNLSKLGLAKERQKDEESFICPYSGAKISQTNCEYDHILPRSKGLYNSLANLIPTSSTSNQIKSNTKYLLSNLDENYLKYIFAKTQTTDLNSFKAFIDENISKIDENDFTNFKNLSFFEQIAFRHALFLDTDDNSFKKALRLLKLDTIKTHSNGTQKRFINILIEKISKLTKSGIDLNFIDSKLVSSTRKDLAQNDTSIAKQEIQDSHSHCVDASIVFYLANSKIIKGQIEPDYDYFKDIYPKDSDIILPQSKQYLELNQKSQKSKKLFDDSVYSLVYEGKFDEKQKKILTQYELLKENGFVDTHKVFELIFKSFKDKDTIVLKDLKFLDNHLKSYIRKDIFSIFFNEKGELKEAKELKSATKNIDKFYTILSQNQDKIYTIKLDEKAKEKKTLQRNKVIELYKEIFYTKNAKPRARGKNRVTFSLPVYAKDAKYAIKRNSGFAGLKNKSIATKTYIDIDSREILKIPYYSTNVLPIRISDILEILSLQSKNAKQIYKIKIQDNLPKQIVSLDFILSQARRHEVLVSFDKSKLEIQNINDDNGENTFIQKYLCDDFKEFLGKPRDNKIEIIKNNDDILAIKYCVESTSKANKEIIVKALSDETPSA

SEQ ID NO: 118 - protein, 1247 aa, synthetic construct
KSLSINIDMGAINNGIFIATCQDDKIIDKNAFDIKFRKGKLNFSKIDRTLRRHTRRSFDRDRFVLRLLGEILPLENLSNNQKEKLFGLFKNRGFNYLNVNFNAEIDSDNLEILNALDRYYFKDCRVLSDFENSISKIFNELENNEILAFLDDQAQILNQAKEHKNKILNKNINAILEFLESIKNESFKNNKHRKSYLKDIKNEIENSFKDIILKLKIFKNSQELYYFIGNIANFQTRILRRYFNAKFDLVFDDAKLKKNILRNINYLDFISTDEKANKNKILENLNAFSTLEFLKNTDPIVTIPPYENAKNKKPQSCQALVINDEKITPSLKDIAHKILSNSNFECLKTDENGVLADNIKDNEIAKYLQRILDISKGILDDKELYPRLLEKDENAKIFAQEIRLNSVELKEFKDFAKKYYDEVNLAKKGIIKNELLKPCCLHTPHKNKNKNALISALFLKSITQKEIENLEDFFANNKISGNQTFKGFFERLSELKKRYQNRFFHILEHEPTKELEGILKNYKKVMEKIVEHNSNFSFKAPFDDSTISTNFNYLTQLGDIIFDEKSRGFAKTCKFHTLENLIRSSAKSAIASRLASNSARLINGKIEMYLDRLAHEIIKKIDFTDIYNVQINVEMNKFNFESNLSKLGLAKERQKDEESFICPYSGAKISQTNCEYDHILPRSKGLYNSLANLIPTSSTSNQIKSNTKYLLSNLDENYLKYIFAKTQTTDLNSFKAFIDENISKIDENDFTNFKNLSFFEQIAFRHALFLDTDDNSFKKALRLLKLDTIKTHSNGTQKRFINILIEKISKLTKSGIDLNFIDSKLVSSTRKDLAQNDTSIAKQEIQDSHSHCVDASIVFYLANSKIIKGQIEPDYDYFKDIYPKDSDIILPQSKQYLELNQKSQKSKKLFDDSVYSLVYEGKFDEKQKKILTQYELLKENGFVDTHKVFELIFKSFKDKDTIVLKDLKFLDNHLKSYIRKDIFSIFFNEKGELKEAKELKSATKNIDKFYTILSQNQDKIYTIKLDEKAKEKKTLQRNKVIELYKEIFYTKNAKPRARGKNRVTFSLPVYAKDAKYAIKRNSGFAGLKNKNIATKTYIDIDSREILKIPYYSTNVLPIRISDILEILSLQSKNAKQIYKIKIQDNLPKQIVSLDFILSQARRHEVLVSFDKSKLEIQNINDDNGENTFIQKYLCDDFKEFLGKPRDNKIEIIKNNDDILAIKYCVESTSKANKEIIVKALSDETPSA

SEQ ID NO: 119 - protein, 1247 aa, synthetic construct
KSLSINIDMGAINNGIFIATCQDDKIIDKNAFDIKFRKGKLNFSKIDRTLRRHTRRSFDRDRFVLRLLGEILPLENLSNNQKEKLFGLFKNRGFNYLNVNFNAEIDSDNLEILNALDRYYFKDCRVLSDFENSISKIFNELENNEILAFLDDQAQILNQAKEHKNKILNKNINAILEFLESIKNESFKNNKHRKSYLKDIKNEIENSFKDIILKLKIFKNSQELYYFIGNIANFQTRILRRYFNAKFDLVFDDAKLKKNILRNINYLDFISTDEKANKNKILENLNAFSTLEFLKNTDPIVTIPPYENAKNKKPQSCQALVINDEKITPSLKDIAHKILSNSNFECLKTDENGVLADNIKDNEIAKYLQRILDISKGILDDKELYPRLLEKDENAKIFAQEIRLNSVELKEFKDFAKKYYDEVNLAKKGIIKNELLKPCCLHTPHKNKNKNALISALFLKSITQKEIENLEDFFANNKISGNQTFKGFFERLSELKKRYQNRFFHILEHEPTKELEGILKNYKKVMEKIVEHNSNFSFKAPFDDSTISTNFNYLTQLGDIIFDEKSRGFAKTCKFHTLENLIRSSAKSAIASRLASNSARLINGKIEMYLDRLAHEIIKKIDFTDIYNVQINVEMNKFNFESNLSKLGLAKERQKDEESFICPYSGAKISQTNCEYDHILPRSKGLYNSLANLIPTSSTSNQIKSNTKYLLSNLDENYLKYIFAKTQTTDLNSFKAFIDENISKIDENDFTNFKNLSFFEQIAFRHALFLDTDDNSFKKALRLLKLDTIKTHSNGTQKRFINILIEKISKLTKSGIDLNFIDSKLVSSTRKDLAQNDTSIAKQEIQDSHSHCVDASIVFYLANSKIIKGQIEPDYDYFKDIYPKDSDIILPQSKQYLELNQKSQKSKKLFDDSVYSLVYEGKFDEKQKKILTQYELLKENGFVDTHKVFELIFKSFKDKDTIVLKDLKFLDNHLKSYIRKDIFSIFFNEKGELKEAKELKSATKNIDKFYTILSQNQDKIYTIKLDEKAKEKKTLQRNKVIELYKEIFYTKNAKPRARGKNRVTFSLPVYAKDAKYAIKRNSGFAGLKNKSIATKTYIDIDSREILKIPYYSTNVLPIRISDILEILSLQSKNAKQIYKIKIQDNLPKQIVSLDFILSQANRHEVLVSFDKSKLEIQNINDDNGENTFIQKYLCDDFKEFLGKPRDNKIEIIKNNDDILAIKYCVESTRKANKEIIVKALSDETPSA

SEQ ID NO: 120 - protein, 1247 aa, synthetic construct
KSLSINIDMGAINNGIFIATCQDDKIIDKNAFDIKFRKGKLNFSKADRTLRRHTRRSFDRDRFVLRLLGEILPLENLSNNQKEKLFGLFKNRGFNYLNVNFNAEIDSDNLEILNALDRYYFKDCRVLSDFENSISKIFNELENNEILAFLDDQAQILNQAKEHKNKILNKNINAILEFLESIKNESFKNNKHRKSYLKDIKNEIENSFKDIILKLKIFKNSQELYYFIGNIANFQTRILRRYFNAKFDLVFDDAKLKKNILRNINYLDFISTDEKANKNKILENLNAFSTLEFLKNTDPIVTIPPYENAKNKKPQSCQALVINDEKITPSLKDIAHKILSNSNFECLKTDENGVLADNIKDNEIAKYLQRILDISKGILDDKELYPRLLEKDENAKIFAQEIRLNSVELKEFKDFAKKYYDEVNLAKKGIIKNELLKPCCLHTPHKNKNKNALISALFLKSITQKEIENLEDFFANNKISGNQTFKGFFERLSELKKRYQNRFFHILEHEPTKELEGILKNYKKVMEKIVEHNSNFSFKAPFDDSTISTNFNYLTQLGDIIFDEKSRGFAKTCKFHTLENLIRSSAKSAIASRLASNSARLINGKIEMYLDRLAHEIIKKIDFTDIYNVQINVEMNKFNFESNLSKLGLAKERQKDEESFICPYSGAKISQTNCEYDHILPRSKGLYNSLANLIPTSSTSNQIKSNTKYLLSNLDENYLKYIFAKTQTTDLNSFKAFIDENISKIDENDFTNFKNLSFFEQIAFRHALFLDTDDNSFKKALRLLKLDTIKTHSNGTQKRFINILIEKISKLTKSGIDLNFIDSKLVSSTRKDLAQNDTSIAKQEIQDSHSHCVDASIVFYLANSKIIKGQIEPDYDYFKDIYPKDSDIILPQSKQYLELNQKSQKSKKLFDRSVYSLVYEGKFDEKQKKILTQYELLKENGFVDTHKVFELIFKSFKDKDTIVLKDLKFLDNHLKSYIRKDIFSIFFNEKGELKEAKELKSATKNIDKFYTILSQNQDKIYTIKLDEKAKEKKTLQRNKVIELYKEIFYTKNAKPRARGKNRVTFSLPVYAKDAKYAIKRNSGFAGLKNKDIATKTYIDIDSREILKIPYYSTNVLPIRISDILEILSLQSKNAKQIYKIKIQDNLPKQIVSLDFILSQANRHEVLVSFDKSKLEIQNINDDNGENTFIQKYLCDDFKEFLGKPRDNKIEIIKNNDDILAIKYCVESTSKANKEIIVKALSDETPSA

SEQ ID NO: 121 - protein, 1247 aa, synthetic construct
KSLSINIDMGAINNGIFIATCQDDKIIDKNAFDIKFRKGKLNFSKRDRTLRRHTRRSFDRDRFVLRLLGEILPLENLSNNQKEKLFGLFKNRGFNYLNVNFNAEIDSDNLEILNALDRYYFKDCRVLSDFENSISKIFNELENNEILAFLDDQAQILNQAKEHKNKILNKNINAILEFLESIKNESFKNNKHRKSYLKDIKNEIENSFKDIILKLKIFKNSQELYYFIGNIANFQTRILRRYFNAKFDLVFDDAKLKKNILRNINYLDFISTDEKANKNKILENLNAFSTLEFLKNTDPIVTIPPYENAKNKKPQSCQALVINDEKITPSLKDIAHKILSNSNFECLKTDENGVLADNIKDNEIAKYLQRILDISKGILDDKELYPRLLEKDENAKIFAQEIRLNSVELKEFKDFAKKYYDEVNLAKKGIIKNELLKPCCLHTPHKNKNKNALISALFLKSITQKEIENLEDFFANNKISGNQTFKGFFERLSELKKRYQNRFFHILEHEPTKELEGILKNYKKVMEKIVEHNSNFSFKAPFDDSTISTNFNYLTQLGDIIFDEKSRGFAKTCKFHTLENLIRSSAKSAIASRLASNSARLINGKIEMYLDRLAHEIIKKIDFTDIYNVQINVEMNKFNFESNLSKLGLAKERQKDEESFICPYSGAKISQTNCEYDHILPRSKGLYNSLANLIPTSSTSNQIKSNTKYLLSNLDENYLKYIFAKTQTTDLNSFKAFIDENISKIDENDFTNFKNLSFFEQIAFRHALFLDTDDNSFKKALRLLKLDTIKTHSNGTQKRFINILIEKISKLTKSGIDLNFIDSKLVSSTRKDLAQNDTSIAKQEIQDSHSHCVDASIVFYLANSKIIKGQIEPDYDYFKDIYPKDSDIILPQSKQYLELNQKSQKSKKLFDRSVYSLVYEGKFDEKQKKILTQYELLKENGFVDTHKVFELIFKSFKDKDTIVLKDLKFLDNHLKSYIRKDIFSIFFNEKGELKEAKELKSATKNIDKFYTILSQNQDKIYTIKLDEKAKEKKTLQRNKVIELYKEIFYTKNAKPRARGKNRVTFSLPVYAKDAKYAIKRNSGFAGLKNKDIATKTYIDIDSREILKIPYYSTNVLPIRISDILEILSLQSKNAKQIYKIKIQDNLPKQIVSLDFILSQANRHEVLVSFDKSKLEIQNINDDNGENTFIQKYLCDDFKEFLGKPRDNKIEIIKNNDDILAIKYCVESTSKANKEIIVKALSDETPSA

SEQ ID NO: 122 - protein, 1247 aa, synthetic construct
KSLSINIDMGAINNGIFIATCQDDKIIDKNAFDIKFRKGKLNFSKIDRTLRRHTRRRFDRDRFVLRLLGEILPLENLSNNQKEKLFGLFKNRGFNYLNVNFNAEIDSDNLEILNALDRYYFKDCRVLSDFENSISKIFNELENNEILAFLDDQAQILNQAKEHKNKILNKNINAILEFLESIKNESFKNNKHRKSYLKDIKNEIENSFKDIILKLKIFKNSQELYYFIGNIANFQTRILRRYFNAKFDLVFDDAKLKKNILRNINYLDFISTDEKANKNKILENLNAFSTLEFLKNTDPIVTIPPYENAKNKKPQSCQALVINDEKITPSLKDIAHKILSNSNFECLKTDENGVLADNIKDNEIAKYLQRILDISKGILDDKELYPRLLEKDENAKIFAQEIRLNSVELKEFKDFAKKYYDEVNLAKKGIIKNELLKPCCLHTPHKNKNKNALISALFLKSITQKEIENLEDFFANNKISGNQTFKGFFERLSELKKRYQNRFFHILEHEPTKELEGILKNYKKVMEKIVEHNSNFSFKAPFDDSTISTNFNYLTQLGDIIFDEKSRGFAKTCKFHTLENLIRSSAKSAIASRLASNSARLINGKIEMYLDRLAHEIIKKIDFTDIYNVQINVEMNKFNFESNLSKLGLAKERQKDEESFICPYSGAKISQTNCEYDHILPRSKGLYNSLANLIPTSSTSNQIKSNTKYLLSNLDENYLKYIFAKTQTTDLNSFKAFIDENISKIDENDFTNFKNLSFFEQIAFRHALFLDTDDNSFKKALRLLKLDTIKTHSNGTQKRFINILIEKISKLTKSGIDLNFIDSKLVSSTRKDLAQNDTSIAKQEIQDSHSHCVDASIVFYLANSKIIKGQIEPDYDYFKDIYPKDSDIILPQSKQYLELNQKSQKSKKLFDRSVYSLVYEGKFDEKQKKILTQYELLKENGFVDTHKVFELIFKSFKDKDTIVLKDLKFLDNHLKSYIRKDIFSIFFNEKGELKEAKELKSATKNIDKFYTILSQNQDKIYTIKLDEKAKEKKTLQRNKVIELYKEIFYTKNAKPRARGKNRVTFSLPVYAKDAKYAIKRNSGFAGLKNKDIATKTYIDIDSREILKIPYYSTNVLPIRISDILEILSLQSKNAKQIYKIKIQDNLPKQIVSLDFILSQANRHEVLVSFDKSKLEIQNINDDNGENTFIQKYLCDDFKEFLGKPRDNKIEIIKNNDDILAIKYCVESTSKANKEIIVKALSDETPSA

SEQ ID NO: 123 - protein, 1247 aa, synthetic construct
KSLSINIDMGAINNGIFIATCQDDKIIDKNAFDIKFRKGKLNFSKIDRTLRRHTRRSFRRDRFVLRLLGEILPLENLSNNQKEKLFGLFKNRGFNYLNVNFNAEIDSDNLEILNALDRYYFKDCRVLSDFENSISKIFNELENNEILAFLDDQAQILNQAKEHKNKILNKNINAILEFLESIKNESFKNNKHRKSYLKDIKNEIENSFKDIILKLKIFKNSQELYYFIGNIANFQTRILRRYFNAKFDLVFDDAKLKKNILRNINYLDFISTDEKANKNKILENLNAFSTLEFLKNTDPIVTIPPYENAKNKKPQSCQALVINDEKITPSLKDIAHKILSNSNFECLKTDENGVLADNIKDNEIAKYLQRILDISKGILDDKELYPRLLEKDENAKIFAQEIRLNSVELKEFKDFAKKYYDEVNLAKKGIIKNELLKPCCLHTPHKNKNKNALISALFLKSITQKEIENLEDFFANNKISGNQTFKGFFERLSELKKRYQNRFFHILEHEPTKELEGILKNYKKVMEKIVEHNSNFSFKAPFDDSTISTNFNYLTQLGDIIFDEKSRGFAKTCKFHTLENLIRSSAKSAIASRLASNSARLINGKIEMYLDRLAHEIIKKIDFTDIYNVQINVEMNKFNFESNLSKLGLAKERQKDEESFICPYSGAKISQTNCEYDHILPRSKGLYNSLANLIPTSSTSNQIKSNTKYLLSNLDENYLKYIFAKTQTTDLNSFKAFIDENISKIDENDFTNFKNLSFFEQIAFRHALFLDTDDNSFKKALRLLKLDTIKTHSNGTQKRFINILIEKISKLTKSGIDLNFIDSKLVSSTRKDLAQNDTSIAKQEIQDSHSHCVDASIVFYLANSKIIKGQIEPDYDYFKDIYPKDSDIILPQSKQYLELNQKSQKSKKLFDRSVYSLVYEGKFDEKQKKILTQYELLKENGFVDTHKVFELIFKSFKDKDTIVLKDLKFLDNHLKSYIRKDIFSIFFNEKGELKEAKELKSATKNIDKFYTILSQNQDKIYTIKLDEKAKEKKTLQRNKVIELYKEIFYTKNAKPRARGKNRVTFSLPVYAKDAKYAIKRNSGFAGLKNKDIATKTYIDIDSREILKIPYYSTNVLPIRISDILEILSLQSKNAKQIYKIKIQDNLPKQIVSLDFILSQANRHEVLVSFDKSKLEIQNINDDNGENTFIQKYLCDDFKEFLGKPRDNKIEIIKNNDDILAIKYCVESTSKANKEIIVKALSDETPSA

SEQ ID NO: 124 - protein, 1247 aa, synthetic construct
KSLSINIDMGAINNGIFIATCQDDKIIDKNAFDIKFRKGKLNFSKIDRTLRRHTRRSFDRGRFVLRLLGEILPLENLSNNQKEKLFGLFKNRGFNYLNVNFNAEIDSDNLEILNALDRYYFKDCRVLSDFENSISKIFNELENNEILAFLDDQAQILNQAKEHKNKILNKNINAILEFLESIKNESFKNNKHRKSYLKDIKNEIENSFKDIILKLKIFKNSQELYYFIGNIANFQTRILRRYFNAKFDLVFDDAKLKKNILRNINYLDFISTDEKANKNKILENLNAFSTLEFLKNTDPIVTIPPYENAKNKKPQSCQALVINDEKITPSLKDIAHKILSNSNFECLKTDENGVLADNIKDNEIAKYLQRILDISKGILDDKELYPRLLEKDENAKIFAQEIRLNSVELKEFKDFAKKYYDEVNLAKKGIIKNELLKPCCLHTPHKNKNKNALISALFLKSITQKEIENLEDFFANNKISGNQTFKGFFERLSELKKRYQNRFFHILEHEPTKELEGILKNYKKVMEKIVEHNSNFSFKAPFDDSTISTNFNYLTQLGDIIFDEKSRGFAKTCKFHTLENLIRSSAKSAIASRLASNSARLINGKIEMYLDRLAHEIIKKIDFTDIYNVQINVEMNKFNFESNLSKLGLAKERQKDEESFICPYSGAKISQTNCEYDHILPRSKGLYNSLANLIPTSSTSNQIKSNTKYLLSNLDENYLKYIFAKTQTTDLNSFKAFIDENISKIDENDFTNFKNLSFFEQIAFRHALFLDTDDNSFKKALRLLKLDTIKTHSNGTQKRFINILIEKISKLTKSGIDLNFIDSKLVSSTRKDLAQNDTSIAKQEIQDSHSHCVDASIVFYLANSKIIKGQIEPDYDYFKDIYPKDSDIILPQSKQYLELNQKSQKSKKLFDRSVYSLVYEGKFDEKQKKILTQYELLKENGFVDTHKVFELIFKSFKDKDTIVLKDLKFLDNHLKSYIRKDIFSIFFNEKGELKEAKELKSATKNIDKFYTILSQNQDKIYTIKLDEKAKEKKTLQRNKVIELYKEIFYTKNAKPRARGKNRVTFSLPVYAKDAKYAIKRNSGFAGLKNKDIATKTYIDIDSREILKIPYYSTNVLPIRISDILEILSLQSKNAKQIYKIKIQDNLPKQIVSLDFILSQANRHEVLVSFDKSKLEIQNINDDNGENTFIQKYLCDDFKEFLGKPRDNKIEIIKNNDDILAIKYCVESTSKANKEIIVKALSDETPSA

SEQ ID NO: 125 - protein, 1247 aa, synthetic construct
KSLSINIDMGAINNGIFIATCQDDKIIDKNAFDIKFRKGKLNFSKIDRTLRRHTRRSFDRRRFVLRLLGEILPLENLSNNQKEKLFGLFKNRGFNYLNVNFNAEIDSDNLEILNALDRYYFKDCRVLSDFENSISKIFNELENNEILAFLDDQAQILNQAKEHKNKILNKNINAILEFLESIKNESFKNNKHRKSYLKDIKNEIENSFKDIILKLKIFKNSQELYYFIGNIANFQTRILRRYFNAKFDLVFDDAKLKKNILRNINYLDFISTDEKANKNKILENLNAFSTLEFLKNTDPIVTIPPYENAKNKKPQSCQALVINDEKITPSLKDIAHKILSNSNFECLKTDENGVLADNIKDNEIAKYLQRILDISKGILDDKELYPRLLEKDENAKIFAQEIRLNSVELKEFKDFAKKYYDEVNLAKKGIIKNELLKPCCLHTPHKNKNKNALISALFLKSITQKEIENLEDFFANNKISGNQTFKGFFERLSELKKRYQNRFFHILEHEPTKELEGILKNYKKVMEKIVEHNSNFSFKAPFDDSTISTNFNYLTQLGDIIFDEKSRGFAKTCKFHTLENLIRSSAKSAIASRLASNSARLINGKIEMYLDRLAHEIIKKIDFTDIYNVQINVEMNKFNFESNLSKLGLAKERQKDEESFICPYSGAKISQTNCEYDHILPRSKGLYNSLANLIPTSSTSNQIKSNTKYLLSNLDENYLKYIFAKTQTTDLNSFKAFIDENISKIDENDFTNFKNLSFFEQIAFRHALFLDTDDNSFKKALRLLKLDTIKTHSNGTQKRFINILIEKISKLTKSGIDLNFIDSKLVSSTRKDLAQNDTSIAKQEIQDSHSHCVDASIVFYLANSKIIKGQIEPDYDYFKDIYPKDSDIILPQSKQYLELNQKSQKSKKLFDRSVYSLVYEGKFDEKQKKILTQYELLKENGFVDTHKVFELIFKSFKDKDTIVLKDLKFLDNHLKSYIRKDIFSIFFNEKGELKEAKELKSATKNIDKFYTILSQNQDKIYTIKLDEKAKEKKTLQRNKVIELYKEIFYTKNAKPRARGKNRVTFSLPVYAKDAKYAIKRNSGFAGLKNKDIATKTYIDIDSREILKIPYYSTNVLPIRISDILEILSLQSKNAKQIYKIKIQDNLPKQIVSLDFILSQANRHEVLVSFDKSKLEIQNINDDNGENTFIQKYLCDDFKEFLGKPRDNKIEIIKNNDDILAIKYCVESTSKANKEIIVKALSDETPSA

SEQ ID NO: 126 - protein, 1247 aa, synthetic construct
KSLSINIDMGAINNGIFIATCQDDKIIDKNAFDIKFRKGKLNFSKIDRTLRRHTRRSFDRDRFVLRLLGEILPLENLSNNQKEKLFGLFKNRGFNYLNVNFNAEIDSDNLEILNALDRYYFKDCRVLSDFENSISKIFNELENNEILAFLDDQAQILNQAKEHKNKILNKNINAILEFLESIKNESFKNNKHRKSYLKDIKNEIENSFKDIILKLKIFKNSQELYYFIGNIANFQTRILRRYFNAKFDLVFDDAKLKKNILRNINYLDFISTDEKANKNKILENLNAFSTLEFLKNTDPIVTIPPYENAKNKKPQSCQALVINDEKITPSLKDIAHKILSNSNFECLKTDENGVLADNIKDNEIAKYLQRILDISKGILDDKELYPRLLEKDENAKIFAQEIRLNSVELKEFKDFAKKYYDEVNLAKKGIIKNELLKPCCLHTPHKNKNKNALISALFLKSITQKEIENLEDFFANNKISGNQTFKGFFERLSELKKRYQNRFFHILEHEPTKELEGILKNYKKVMEKIVEHNSNFSFKAPFDDSTISTNFNYLTQLGDIIFDEKSRGFAKTCKFHTLENLIRSSAKSAIASRLASNSARLINGKIEMYLDRLAHEIIKKIDFTDIYNVQINVEMNKFNFESNLSKLGLAKERQKDEESFICPYSGAKISQTNCEYDHILPRSKGLYNSLANLIPTSSTSNQIKSNTKYLLSNLDENYLKYIFAKTQTTDLNSFKAFIDENISKIDENDFTNFKNLSFFEQIAFRHALFLDTDDNSFKKALRLLKLDTIKTHSNGTQKRFINILIEKISKLTKSGIDLNFIDSKLVSSTRKDLAQNDTSIAKQEIQDSHSHCVDASIVFYLANSKIIKGQIEPDYDYFKDIYPKDSDIILPQSKQYLELNQKSQKSKKLFDRSVYSLVYEGKFDEKQKKILTQYELLKENGFVDTHKVFELIFKSFKDKDTIVLKDLKFLDNHLKSYIRKDIFSIFFNEKGELKEAKELKSATKNIDKFYTILSQNQDKIYTIKLDEKAKEKKTLQRNKVIELYKEIFYTKNAKPRARGKNRVTFSLPVYAKDAKYAIKRNSGFAGLKNKDIATKTYIDIDSREILKIPYYSTNVLPIRISDILEILSLQSKNAKQIYKIKIQDNLPKQIVSLDFILSQANRHEVLVSFDKSKLEIQNINDDNGENTFIQKYLCDDFKEFLGKPRGNKIEIIKNNDDILAIKYCVESTSKANKEIIVKALSDETPSA

SEQ ID NO: 127 - protein, 1247 aa, synthetic construct
KSLSINIDMGAINNGIFIATCQDDKIIDKNAFDIKFRKGKLNFSKIDRTLRRHTRRSFDRDRFVLRLLGEILPLENLSNNQKEKLFGLFKNRGFNYLNVNFNAEIDSDNLEILNALDRYYFKDCRVLSDFENSISKIFNELENNEILAFLDDQAQILNQAKEHKNKILNKNINAILEFLESIKNESFKNNKHRKSYLKDIKNEIENSFKDIILKLKIFKNSQELYYFIGNIANFQTRILRRYFNAKFDLVFDDAKLKKNILRNINYLDFISTDEKANKNKILENLNAFSTLEFLKNTDPIVTIPPYENAKNKKPQSCQALVINDEKITPSLKDIAHKILSNSNFECLKTDENGVLADNIKDNEIAKYLQRILDISKGILDDKELYPRLLEKDENAKIFAQEIRLNSVELKEFKDFAKKYYDEVNLAKKGIIKNELLKPCCLHTPHKNKNKNALISALFLKSITQKEIENLEDFFANNKISGNQTFKGFFERLSELKKRYQNRFFHILEHEPTKELEGILKNYKKVMEKIVEHNSNFSFKAPFDDSTISTNFNYLTQLGDIIFDEKSRGFAKTCKFHTLENLIRSSAKSAIASRLASNSARLINGKIEMYLDRLAHEIIKKIDFTDIYNVQINVEMNKFNFESNLSKLGLAKERQKDEESFICPYSGAKISQTNCEYDHILPRSKGLYNSLANLIPTSSTSNQIKSNTKYLLSNLDENYLKYIFAKTQTTDLNSFKAFIDENISKIDENDFTNFKNLSFFEQIAFRHALFLDTDDNSFKKALRLLKLDTIKTHSNGTQKRFINILIEKISKLTKSGIDLNFIDSKLVSSTRKDLAQNDTSIAKQEIQDSHSHCVDASIVFYLANSKIIKGQIEPDYDYFKDIYPKDSDIILPQSKQYLELNQKSQKSKKLFDRSVYSLVYEGKFDEKQKKILTQYELLKENGFVDTHKVFELIFKSFKDKDTIVLKDLKFLDNHLKSYIRKDIFSIFFNEKGELKEAKELKSATKNIDKFYTILSQNQDKIYTIKLDEKAKEKKTLQRNKVIELYKEIFYTKNAKPRARGKNRVTFSLPVYAKDAKYAIKRNSGFAGLKNKDIATKTYIDIDSREILKIPYYSTNVLPIRISDILEILSLQSKNAKQIYKIKIQDNLPKQIVSLDFILSQANRHEVLVSFDKSKLEIQNINDDNGENTFIQKYLCDDFKEFLGKPRSNKIEIIKNNDDILAIKYCVESTSKANKEIIVKALSDETPSA

SEQ ID NO: 128 - protein, 1247 aa, synthetic construct
KSLSINIDMGAINNGIFIATCQDDKIIDKNAFDIKFRKGKLNFSKIDRTLRRHTRRSFDRDRFVLRLLGEILPLENLSNNQKEKLFGLFKNRGFNYLNVNFNAEIDSDNLEILNALDRYYFKDCRVLSDFENSISKIFNELENNEILAFLDDQAQILNQAKEHKNKILNKNINAILEFLESIKNESFKNNKHRKSYLKDIKNEIENSFKDIILKLKIFKNSQELYYFIGNIANFQTRILRRYFNAKFDLVFDDAKLKKNILRNINYLDFISTDEKANKNKILENLNAFSTLEFLKNTDPIVTIPPYENAKNKKPQSCQALVINDEKITPSLKDIAHKILSNSNFECLKTDENGVLADNIKDNEIAKYLQRILDISKGILDDKELYPRLLEKDENAKIFAQEIRLNSVELKEFKDFAKKYYDEVNLAKKGIIKNELLKPCCLHTPHKNKNKNALISALFLKSITQKEIENLEDFFANNKISGNQTFKGFFERLSELKKRYQNRFFHILEHEPTKELEGILKNYKKVMEKIVEHNSNFSFKAPFDDSTISTNFNYLTQLGDIIFDEKSRGFAKTCKFHTLENLIRSSAKSAIASRLASNSARLINGKIEMYLDRLAHEIIKKIDFTDIYNVQINVEMNKFNFESNLSKLGLAKERQKDEESFICPYSGAKISQTNCEYDHILPRSKGLYNSLANLIPTSSTSNQIKSNTKYLLSNLDENYLKYIFAKTQTTDLNSFKAFIDENISKIDENDFTNFKNLSFFEQIAFRHALFLDTDDNSFKKALRLLKLDTIKTHSNGTQKRFINILIEKISKLTKSGIDLNFIDSKLVSSTRKDLAQNDTSIAKQEIQDSHSHCVDASIVFYLANSKIIKGQIEPDYDYFKDIYPKDSDIILPQSKQYLELNQKSQKSKKLFDRSVYSLVYEGKFDEKQKKILTQYELLKENGFVDTHKVFELIFKSFKDKDTIVLKDLKFLDNHLKSYIRKDIFSIFFNEKGELKEAKELKSATKNIDKFYTILSQNQDKIYTIKLDEKAKEKKTLQRNKVIELYKEIFYTKNAKPRARGKNRVTFSLPVYAKDAKYAIKRNSGFAGLKNKDIATKTYIDIDSREILKIPYYSTNVLPIRISDILEILSLQSKNAKQIYKIKIQDNLPKQIVSLDFILSQANRHEVLVSFDKSKLEIQNINDDNGENTFIQKYLCDDFKEFLGKPRDNKIEIIKNNDDILAIKYCVSSTSKANKEIIVKALSDETPSA

SEQ ID NO: 129 - protein, 1247 aa, synthetic construct
KSLSINIDMGAINNGIFIATCQDDKIIDKNAFDIKFRKGKLNFSKIDRTLRRHTRRSFDRDRFVLRLLGEILPLENLSNNQKEKLFGLFKNRGYNYLNVNFNAEIDSDNLEILNALDRYYFKDCRVLSDFENSISKIFNELENNEILAFLDDQAQILNQAKEHKNKILNKNINAILEFLESIKNESFKNNKHRKSYLKDIKNEIENSFKDIILKLKIFKNSQELYYFIGNIANFQTRILRRYFNAKFDLVFDDAKLKKNILRNINYLDFISTDEKANKNKILENLNAFSTLEFLKNTDPIVTIPPYENAKNKKPQSCQALVINDEKITPSLKDIAHKILSNSNFECLKTDENGVLADNIKDNEIAKYLQRILDISKGILDDKELYPRLLEKDENAKIFAQEIRLNSVELKEFKDFAKKYYDEVNLAKKGIIKNELLKPCCLHTPHKNKNKNALISALFLKSITQKEIENLEDFFANNKISGNQTFKGFFERLSELKKRYQNRFFHILEHEPTKELEGILKNYKKVMEKIVEHNSNFSFKAPFDDSTISTNFNYLTQLGDIIFDEKSRGFAKTCKFHTLENLIRSSAKSAIASRLASNSARLINGKIEMYLDRLAHEIIKKIDFTDIYNVQINVEMNKFNFESNLSKLGLAKERQKDEESFICPYSGAKISQTNCEYDHILPRSKGLYNSLANLIPTSSTSNQIKSNTKYLLSNLDENYLKYIFAKTQTTDLNSFKAFIDENISKIDENDFTNFKNLSFFEQIAFRHALFLDTDDNSFKKALRLLKLDTIKTHSNGTQKRFINILIEKISKLTKSGIDLNFIDSKLVSSTRKDLAQNDTSIAKQEIQDSHSHCVDASIVFYLANSKIIKGQIEPDYDYFKDIYPKDSDIILPQSKQYLELNQKSQKSKKLFDRSVYSLVYEGKFDEKQKKILTQYELLKENGFVDTHKVFELIFKSFKDKDTIVLKDLKFLDNHLKSYIRKDIFSIFFNEKGELKEAKELKSATKNIDKFYTILSQNQDKIYTIKLDEKAKEKKTLQRNKVIELYKEIFYTKNAKPRARGKNRVTFSLPVYAKDAKYAIKRNSGFAGLKNKDIATKTYIDIDSREILKIPYYSTNVLPIRISDILEILSLQSKNAKQIYKIKIQDNLPKQIVSLDFILSQANRHEVLVSFDKSKLEIQNINDDNGENTFIQKYLCDDFKEFLGKPRDNKIEIIKNNDDILAIKYCVESTSKANKEIIVKALSDETPSA

SEQ ID NO: 130 - protein, 1247 aa, synthetic construct
KSLSINIDMGAINNGIFIATCQDDKIIDKNAFDIKFRKGKLNFSKIDRTLRRHTRRSFDRDRFVLRLLGEILPLENLSNNQKEKLFGLFKNRGFNYLNVNFNAEIDSDNLEILNALDRYYFKDCRVLSDFENSISKIFNELENNEILAFLDDQAQILNQAKEHKNKILNKNINAILEFLESIKNESFKNNKHRKSYLKDIKNEIENSFKDIILKLKIFKNSQELYYFIGNIANFQTRILRRYFNAKFDLVFDDAKLKKNILRNINYLDFISTDEKANKNKILENLNAFSTLEFLKNTDPIVTIPPYENAKNKKPQSCQALVINDEKITPSLKDIAHKILSNSNFECLKTDENGVLADNIKDNEIAKYLQRILDISKGILDDKELYPRLLEKDENAKIFAQEIRLNSVELKEFKDFAKKYYDEVNLAKKGIIKNELLKPCCLHTPHKNKNKNALISALFLKSITQKEIENLEDFFANNKISGNQTFKGFFERLSELKKRYQNRFFHILEHEPTKELEGILKNYKKVMEKIVEHNSNFSFKAPFDDSTISTNFNYLTQLGDIIFDEKSRGFAKTCKFHTLENLIRSSAKSAIASRLASNSARLINGKIEMYLDRLAHEIIKKIDFTDIYNVQINVEMNKFNFESNLSKLGLAKERQKDEESFICPYSGAKISQTNCEYDHILPRSKGLYNSLANLIPTSSTSNQIKSNTKYLLSNLDENYLKYIFAKTQTTDLNSFKAFIDENISKIDENDFTNFKNLSFFEQIAFRHALFLDTDDNSFKKALRLLKLDTIKTHSNGTQKRFINILIEKISKLTKSGIDLNFIDSKLVSSTRKDLAQNDTSIAKQEIQDSHSHCVDASIVFYLANSKIIKGQIEPDYDYFKDIYPKDSDIILPQSKQYLELNQKSQKSKKLFDSSVYSLVYEGKFDEKQKKILTQYELLKENGFVDTHKVFELIFKSFKDKDTIVLKDLKFLDNHLKSYIRKDIFSIFFNEKGELKEAKELKSATKNIDKFYTILSQNQDKIYTIKLDEKAKEKKTLQRNKVIELYKEIFYTKNAKPRARGKNRVTFSLPVYAKDAKYAIKRNSGFAGLKNKSIATKTYIDIDSREILKIPYYSTNVLPIRISDILEILSLQSKNAKQIYKIKIQDNLPKQIVSLDFILSQARRHEVLVSFDKSKLEIQNINDDNGENTFIQKYLCDDFKEFLGKPRDNKIEIIKNNDDILAIKYCVESTSKANKEIIVKALSDETPSA

SEQ ID NO: 131 - protein, 1247 aa, synthetic construct
KSLSINIDMGAINNGIFIATCQDDKIIDKNAFDIKFRKGKLNFSKIDRTLRRHTRRSFDRDRFVLRLLGEILPLENLSNNQKEKLFGLFKNRGFNYLNVNFNAEIDSDNLEILNALDRYYFKDCRVLSDFENSISKIFNELENNEILAFLDDQAQILNQAKEHKNKILNKNINAILEFLESIKNESFKNNKHRKSYLKDIKNEIENSFKDIILKLKIFKNSQELYYFIGNIANFQTRILRRYFNAKFDLVFDDAKLKKNILRNINYLDFISTDEKANKNKILENLNAFSTLEFLKNTDPIVTIPPYENAKNKKPQSCQALVINDEKITPSLKDIAHKILSNSNFECLKTDENGVLADNIKDNEIAKYLQRILDISKGILDDKELYPRLLEKDENAKIFAQEIRLNSVELKEFKDFAKKYYDEVNLAKKGIIKNELLKPCCLHTPHKNKNKNALISALFLKSITQKEIENLEDFFANNKISGNQTFKGFFERLSELKKRYQNRFFHILEHEPTKELEGILKNYKKVMEKIVEHNSNFSFKAPFDDSTISTNFNYLTQLGDIIFDEKSRGFAKTCKFHTLENLIRSSAKSAIASRLASNSARLINGKIEMYLDRLAHEIIKKIDFTDIYNVQINVEMNKFNFESNLSKLGLAKERQKDEESFICPYSGAKISQTNCEYDHILPRSKGLYNSLANLIPTSSTSNQIKSNTKYLLSNLDENYLKYIFAKTQTTDLNSFKAFIDENISKIDENDFTNFKNLSFFEQIAFRHALFLDTDDNSFKKALRLLKLDTIKTHSNGTQKRFINILIEKISKLTKSGIDLNFIDSKLVSSTRKDLAQNDTSIAKQEIQDSHSHCVDASIVFYLANSKIIKGQIEPDYDYFKDIYPKDSDIILPQSKQYLELNQKSQKSKKLFDNSVYSLVYEGKFDEKQKKILTQYELLKENGFVDTHKVFELIFKSFKDKDTIVLKDLKFLDNHLKSYIRKDIFSIFFNEKGELKEAKELKSATKNIDKFYTILSQNQDKIYTIKLDEKAKEKKTLQRNKVIELYKEIFYTKNAKPRARGKNRVTFSLPVYAKDAKYAIKRNSGFAGLKNKSIATKTYIDIDSREILKIPYYSTNVLPIRISDILEILSLQSKNAKQIYKIKIQDNLPKQIVSLDFILSQARRHEVLVSFDKSKLEIQNINDDNGENTFIQKYLCDDFKEFLGKPRDNKIEIIKNNDDILAIKYCVESTSKANKEIIVKALSDETPSA

SEQ ID NO: 132 - protein, 1247 aa, synthetic construct
KSLSINIDMGAINNGIFIATCQDDKIIDKNAFDIKFRKGKLNFSKRDRTLRRHTRRSFDRDRFVLRLLGEILPLENLSNNQKEKLFGLFKNRGFNYLNVNFNAEIDSDNLEILNALDRYYFKDCRVLSDFENSISKIFNELENNEILAFLDDQAQILNQAKEHKNKILNKNINAILEFLESIKNESFKNNKHRKSYLKDIKNEIENSFKDIILKLKIFKNSQELYYFIGNIANFQTRILRRYFNAKFDLVFDDAKLKKNILRNINYLDFISTDEKANKNKILENLNAFSTLEFLKNTDPIVTIPPYENAKNKKPQSCQALVINDEKITPSLKDIAHKILSNSNFECLKTDENGVLADNIKDNEIAKYLQRILDISKGILDDKELYPRLLEKDENAKIFAQEIRLNSVELKEFKDFAKKYYDEVNLAKKGIIKNELLKPCCLHTPHKNKNKNALISALFLKSITQKEIENLEDFFANNKISGNQTFKGFFERLSELKKRYQNRFFHILEHEPTKELEGILKNYKKVMEKIVEHNSNFSFKAPFDDSTISTNFNYLTQLGDIIFDEKSRGFAKTCKFHTLENLIRSSAKSAIASRLASNSARLINGKIEMYLDRLAHEIIKKIDFTDIYNVQINVEMNKFNFESNLSKLGLAKERQKDEESFICPYSGAKISQTNCEYDHILPRSKGLYNSLANLIPTSSTSNQIKSNTKYLLSNLDENYLKYIFAKTQTTDLNSFKAFIDENISKIDENDFTNFKNLSFFEQIAFRHALFLDTDDNSFKKALRLLKLDTIKTHSNGTQKRFINILIEKISKLTKSGIDLNFIDSKLVSSTRKDLAQNDTSIAKQEIQDSHSHCVDASIVFYLANSKIIKGQIEPDYDYFKDIYPKDSDIILPQSKQYLELNQKSQKSKKLFDDSVYSLVYEGKFDEKQKKILTQYELLKENGFVDTHKVFELIFKSFKDKDTIVLKDLKFLDNHLKSYIRKDIFSIFFNEKGELKEAKELKSATKNIDKFYTILSQNQDKIYTIKLDEKAKEKKTLQRNKVIELYKEIFYTKNAKPRARGKNRVTFSLPVYAKDAKYAIKRNSGFAGLKNKSIATKTYIDIDSREILKIPYYSTNVLPIRISDILEILSLQSKNAKQIYKIKIQDNLPKQIVSLDFILSQARRHEVLVSFDKSKLEIQNINDDNGENTFIQKYLCDDFKEFLGKPRDNKIEIIKNNDDILAIKYCVESTSKANKEIIVKALSDETPSA

SEQ ID NO: 133 - protein, 1247 aa, synthetic construct
KSLSINIDMGAINNGIFIATCQDDKIIDKNAFDIKFRKGKLNFSKIDRTLRRHTRRRFDRDRFVLRLLGEILPLENLSNNQKEKLFGLFKNRGFNYLNVNFNAEIDSDNLEILNALDRYYFKDCRVLSDFENSISKIFNELENNEILAFLDDQAQILNQAKEHKNKILNKNINAILEFLESIKNESFKNNKHRKSYLKDIKNEIENSFKDIILKLKIFKNSQELYYFIGNIANFQTRILRRYFNAKFDLVFDDAKLKKNILRNINYLDFISTDEKANKNKILENLNAFSTLEFLKNTDPIVTIPPYENAKNKKPQSCQALVINDEKITPSLKDIAHKILSNSNFECLKTDENGVLADNIKDNEIAKYLQRILDISKGILDDKELYPRLLEKDENAKIFAQEIRLNSVELKEFKDFAKKYYDEVNLAKKGIIKNELLKPCCLHTPHKNKNKNALISALFLKSITQKEIENLEDFFANNKISGNQTFKGFFERLSELKKRYQNRFFHILEHEPTKELEGILKNYKKVMEKIVEHNSNFSFKAPFDDSTISTNFNYLTQLGDIIFDEKSRGFAKTCKFHTLENLIRSSAKSAIASRLASNSARLINGKIEMYLDRLAHEIIKKIDFTDIYNVQINVEMNKFNFESNLSKLGLAKERQKDEESFICPYSGAKISQTNCEYDHILPRSKGLYNSLANLIPTSSTSNQIKSNTKYLLSNLDENYLKYIFAKTQTTDLNSFKAFIDENISKIDENDFTNFKNLSFFEQIAFRHALFLDTDDNSFKKALRLLKLDTIKTHSNGTQKRFINILIEKISKLTKSGIDLNFIDSKLVSSTRKDLAQNDTSIAKQEIQDSHSHCVDASIVFYLANSKIIKGQIEPDYDYFKDIYPKDSDIILPQSKQYLELNQKSQKSKKLFDDSVYSLVYEGKFDEKQKKILTQYELLKENGFVDTHKVFELIFKSFKDKDTIVLKDLKFLDNHLKSYIRKDIFSIFFNEKGELKEAKELKSATKNIDKFYTILSQNQDKIYTIKLDEKAKEKKTLQRNKVIELYKEIFYTKNAKPRARGKNRVTFSLPVYAKDAKYAIKRNSGFAGLKNKSIATKTYIDIDSREILKIPYYSTNVLPIRISDILEILSLQSKNAKQIYKIKIQDNLPKQIVSLDFILSQARRHEVLVSFDKSKLEIQNINDDNGENTFIQKYLCDDFKEFLGKPRDNKIEIIKNNDDILAIKYCVESTSKANKEIIVKALSDETPSA

SEQ ID NO: 134 - protein, 1247 aa, synthetic construct
KSLSINIDMGAINNGIFIATCQDDKIIDKNAFDIKFRKGKLNFSKIDRTLRRHTRRSFSRDRFVLRLLGEILPLENLSNNQKEKLFGLFKNRGFNYLNVNFNAEIDSDNLEILNALDRYYFKDCRVLSDFENSISKIFNELENNEILAFLDDQAQILNQAKEHKNKILNKNINAILEFLESIKNESFKNNKHRKSYLKDIKNEIENSFKDIILKLKIFKNSQELYYFIGNIANFQTRILRRYFNAKFDLVFDDAKLKKNILRNINYLDFISTDEKANKNKILENLNAFSTLEFLKNTDPIVTIPPYENAKNKKPQSCQALVINDEKITPSLKDIAHKILSNSNFECLKTDENGVLADNIKDNEIAKYLQRILDISKGILDDKELYPRLLEKDENAKIFAQEIRLNSVELKEFKDFAKKYYDEVNLAKKGIIKNELLKPCCLHTPHKNKNKNALISALFLKSITQKEIENLEDFFANNKISGNQTFKGFFERLSELKKRYQNRFFHILEHEPTKELEGILKNYKKVMEKIVEHNSNFSFKAPFDDSTISTNFNYLTQLGDIIFDEKSRGFAKTCKFHTLENLIRSSAKSAIASRLASNSARLINGKIEMYLDRLAHEIIKKIDFTDIYNVQINVEMNKFNFESNLSKLGLAKERQKDEESFICPYSGAKISQTNCEYDHILPRSKGLYNSLANLIPTSSTSNQIKSNTKYLLSNLDENYLKYIFAKTQTTDLNSFKAFIDENISKIDENDFTNFKNLSFFEQIAFRHALFLDTDDNSFKKALRLLKLDTIKTHSNGTQKRFINILIEKISKLTKSGIDLNFIDSKLVSSTRKDLAQNDTSIAKQEIQDSHSHCVDASIVFYLANSKIIKGQIEPDYDYFKDIYPKDSDIILPQSKQYLELNQKSQKSKKLFDDSVYSLVYEGKFDEKQKKILTQYELLKENGFVDTHKVFELIFKSFKDKDTIVLKDLKFLDNHLKSYIRKDIFSIFFNEKGELKEAKELKSATKNIDKFYTILSQNQDKIYTIKLDEKAKEKKTLQRNKVIELYKEIFYTKNAKPRARGKNRVTFSLPVYAKDAKYAIKRNSGFAGLKNKSIATKTYIDIDSREILKIPYYSTNVLPIRISDILEILSLQSKNAKQIYKIKIQDNLPKQIVSLDFILSQARRHEVLVSFDKSKLEIQNINDDNGENTFIQKYLCDDFKEFLGKPRDNKIEIIKNNDDILAIKYCVESTSKANKEIIVKALSDETPSA

SEQ ID NO: 135 - protein, 1247 aa, synthetic construct
KSLSINIDMGAINNGIFIATCQDDKIIDKNAFDIKFRKGKLNFSKIDRTLRRHTRRSFDRDRFVLRLLGEILPLENLSNNQKEKLFGLFKNRGFNYLNVNFNAEIDSDNLEILNALDRYYFKDCRVLSDFENSISKIFNELENNEILAFLDDQAQILNQAKEHKNKILNKNINAILEFLESIKNESFKNNKHRKSYLKDIKNEIENSFKDIILKLKIFKNSQELYYFIGNIANFQTRILRRYFNAKFDLVFDDAKLKKNILRNINYLDFISTDEKANKNKILENLNAFSTLEFLKNTDPIVTIPPYENAKNKKPQSCQALVINDEKITPSLKDIAHKILSNSNFECLKTDENGVLADNIKDNEIAKYLQRILDISKGILDDKELYPRLLEKDENAKIFAQEIRLNSVELKEFKDFAKKYYDEVNLAKKGIIKNELLKPCCLHTPHKNKNKNALISALFLKSITQKEIENLEDFFANNKISGNQTFKGFFERLSELKKRYQNRFFHILEHEPTKELEGILKNYKKVMEKIVEHNSNFSFKAPFDDSTISTNFNYLTQLGDIIFDEKRRGFAKTCKFHTLENLIRSSAKSAIASRLASNSARLINGKIEMYLDRLAHEIIKKIDFTDIYNVQINVEMNKFNFESNLSKLGLAKERQKDEESFICPYSGAKISQTNCEYDHILPRSKGLYNSLANLIPTSSTSNQIKSNTKYLLSNLDENYLKYIFAKTQTTDLNSFKAFIDENISKIDENDFTNFKNLSFFEQIAFRHALFLDTDDNSFKKALRLLKLDTIKTHSNGTQKRFINILIEKISKLTKSGIDLNFIDSKLVSSTRKDLAQNDTSIAKQEIQDSHSHCVDASIVFYLANSKIIKGQIEPDYDYFKDIYPKDSDIILPQSKQYLELNQKSQKSKKLFDDSVYSLVYEGKFDEKQKKILTQYELLKENGFVDTHKVFELIFKSFKDKDTIVLKDLKFLDNHLKSYIRKDIFSIFFNEKGELKEAKELKSATKNIDKFYTILSQNQDKIYTIKLDEKAKEKKTLQRNKVIELYKEIFYTKNAKPRARGKNRVTFSLPVYAKDAKYAIKRNSGFAGLKNKSIATKTYIDIDSREILKIPYYSTNVLPIRISDILEILSLQSKNAKQIYKIKIQDNLPKQIVSLDFILSQARRHEVLVSFDKSKLEIQNINDDNGENTFIQKYLCDDFKEFLGKPRDNKIEIIKNNDDILAIKYCVESTSKANKEIIVKALSDETPSA

SEQ ID NO: 136 - protein, 1247 aa, synthetic construct
KSLSINIDMGAINNGIFIATCQDDKIIDKNAFDIKFRKGKLNFSKIDRTLRRHTRRSFDRDRFVLRLLGEILPLENLSNNQKEKLFGLFKNRGFNYLNVNFNAEIDSDNLEILNALDRYYFKDCRVLSDFENSISKIFNELENNEILAFLDDQAQILNQAKEHKNKILNKNINAILEFLESIKNESFKNNKHRKSYLKDIKNEIENSFKDIILKLKIFKNSQELYYFIGNIANFQTRILRRYFNAKFDLVFDDAKLKKNILRNINYLDFISTDEKANKNKILENLNAFSTLEFLKNTDPIVTIPPYENAKNKKPQSCQALVINDEKITPSLKDIAHKILSNSNFECLKTDENGVLADNIKDNEIAKYLQRILDISKGILDDKELYPRLLEKDENAKIFAQEIRLNSVELKEFKDFAKKYYDEVNLAKKGIIKNELLKPCCLHTPHKNKNKNALISALFLKSITQKEIENLEDFFANNKISGNQTFKGFFERLSELKKRYQNRFFHILEHEPTKELEGILKNYKKVMEKIVEHNSNFSFKAPFDDSTISTNFNYLTQLGDIIFDEKSRGFAKTCKFHTLENLIRSSAKSAIASRLASNSARLINGKIEMYLDRLAHEIIKKIDFTDIYNVQINVEMNKFNFESNLSKLGLAKERQKDEESFICPYSGAKISQTNCEYDHILPRSKGLYNSLANLIPTSSTSNQIKSNTKYLLSNLDENYLKYIFAKTQTTDLNSFKAFIDENISKIDENDFTNFKNLSFFEQIAFRHALFLDTDDNSFKKALRLLKLDTIKTHSNGTQKRFINILIEKISKLTKSGIDLNFIDSKLVSSTRKDLAQNDTSIAKQEIQDSHSHCVDASIVFYLANSKIIKGQIEPDYDYFKDIYPKDSDIILPQSKQYLELNQKSQKSKKLFDDSVYSLVYEGKFDEKQKKILTQYELLKENGFVDTHKVFELIFKSFKDKDTIVLKDLKFLDNHLKSYIRKDIFSIFFNEKGELKEAKELKSATKNIDKFYTILSQNQDKIYTIKLDEKAKEKKTLQRNKVIELYKEIFYTKNAKPRARGKNRVTFSLPVYAKDAKYAIKRNSGFAGLKNKSIATKTYIDIDSREILKIPYYSTNVLPIRISDILEILSLQSKNAKQIYKIKIQDNLPKQIVSLDFILSQARRHEVLVSFDKSKLEIQNINDDNGENTFIQKYLCDDFKEFLGKPRSNKIEIIKNNDDILAIKYCVESTSKANKEIIVKALSDETPSA

SEQ ID NO: 137 - protein, 1247 aa, synthetic construct
KSLSINIDMGAINNGIFIATCQDDKIIDKNAFDIKFRKGKLNFSKIDRTLRRHTRRSFDRDRFVLRLLGEILPLENLSNNQKEKLFGLFKNRGFNYLNVNFNAEIDSDNLEILNALDRYYFKDCRVLSDFENSISKIFNELENNEILAFLDDQAQILNQAKEHKNKILNKNINAILEFLESIKNESFKNNKHRKSYLKDIKNEIENSFKDIILKLKIFKNSQELYYFIGNIANFQTRILRRYFNAKFDLVFDDAKLKKNILRNINYLDFISTDEKANKNKILENLNAFSTLEFLKNTDPIVTIPPYENAKNKKPQSCQALVINDEKITPSLKDIAHKILSNSNFECLKTDENGVLADNIKDNEIAKYLQRILDISKGILDDKELYPRLLEKDENAKIFAQEIRLNSVELKEFKDFAKKYYDEVNLAKKGIIKNELLKPCCLHTPHKNKNKNALISALFLKSITQKEIENLEDFFANNKISGNQTFKGFFERLSELKKRYQNRFFHILEHEPTKELEGILKNYKKVMEKIVEHNSNFSFKAPFDDSTISTNFNYLTQLGDIIFDEKSRGFAKTCKFHTLENLIRSSAKSAIASRLASNSARLINGKIEMYLDRLAHEIIKKIDFTDIYNVQINVEMNKFNFESNLSKLGLAKERQKDEESFICPYSGAKISQTNCEYDHILPRSKGLYNSLANLIPTSSTSNQIKSNTKYLLSNLDENYLKYIFAKTQTTDLNSFKAFIDENISKIDENDFTNFKNLSFFEQIAFRHALFLDTDDNSFKKALRLLKLDTIKTHSNGTQKRFINILIEKISKLTKSGIDLNFIDSKLVSSTRKDLAQNDTSIAKQEIQDSHSHCVDASIVFYLANSKIIKGQIEPDYDYFKDIYPKDSDIILPQSKQYLELNQKSQKSKKLFDSSVYSLVYEGKFDEKQKKILTQYELLKENGFVDTHKVFELIFKSFKDKDTIVLKDLKFLDNHLKSYIRKDIFSIFFNEKGELKEAKELKSATKNIDKFYTILSQNQDKIYTIKLDEKAKEKKTLQRNKVIELYKEIFYTKNAKPRARGKNRVTFSLPVYAKDAKYAIKRNSGFAGLKNKSIATKTYIDIDSREILKIPYYSTNVLPIRISDILEILSLQSKNAKQIYKIKIQDNLPKQIVSLDFILSQARRHEVLVSFDKSKLEIQNINDDNGENTFIQKYLCDDFKEFLGKPRSNKIEIIKNNDDILAIKYCVESTSKANKEIIVKALSDETPSA

SEQ ID NO: 138 - protein, 1247 aa, synthetic construct
KSLSINIDMGAINNGIFIATCQDDKIIDKNAFDIKFRKGKLNFSKIDRTLRRHTRRSFDRDRFVLRLLGEILPLENLSNNQKEKLFGLFKNRGYNYLNVNFNAEIDSDNLEILNALDRYYFKDCRVLSDFENSISKIFNELENNEILAFLDDQAQILNQAKEHKNKILNKNINAILEFLESIKNESFKNNKHRKSYLKDIKNEIENSFKDIILKLKIFKNSQELYYFIGNIANFQTRILRRYFNAKFDLVFDDAKLKKNILRNINYLDFISTDEKANKNKILENLNAFSTLEFLKNTDPIVTIPPYENAKNKKPQSCQALVINDEKITPSLKDIAHKILSNSNFECLKTDENGVLADNIKDNEIAKYLQRILDISKGILDDKELYPRLLEKDENAKIFAQEIRLNSVELKEFKDFAKKYYDEVNLAKKGIIKNELLKPCCLHTPHKNKNKNALISALFLKSITQKEIENLEDFFANNKISGNQTFKGFFERLSELKKRYQNRFFHILEHEPTKELEGILKNYKKVMEKIVEHNSNFSFKAPFDDSTISTNFNYLTQLGDIIFDEKSRGFAKTCKFHTLENLIRSSAKSAIASRLASNSARLINGKIEMYLDRLAHEIIKKIDFTDIYNVQINVEMNKFNFESNLSKLGLAKERQKDEESFICPYSGAKISQTNCEYDHILPRSKGLYNSLANLIPTSSTSNQIKSNTKYLLSNLDENYLKYIFAKTQTTDLNSFKAFIDENISKIDENDFTNFKNLSFFEQIAFRHALFLDTDDNSFKKALRLLKLDTIKTHSNGTQKRFINILIEKISKLTKSGIDLNFIDSKLVSSTRKDLAQNDTSIAKQEIQDSHSHCVDASIVFYLANSKIIKGQIEPDYDYFKDIYPKDSDIILPQSKQYLELNQKSQKSKKLFDDSVYSLVYEGKFDEKQKKILTQYELLKENGFVDTHKVFELIFKSFKDKDTIVLKDLKFLDNHLKSYIRKDIFSIFFNEKGELKEAKELKSATKNIDKFYTILSQNQDKIYTIKLDEKAKEKKTLQRNKVIELYKEIFYTKNAKPRARGKNRVTFSLPVYAKDAKYAIKRNSGFAGLKNKSIATKTYIDIDSREILKIPYYSTNVLPIRISDILEILSLQSKNAKQIYKIKIQDNLPKQIVSLDFILSQARRHEVLVSFDKSKLEIQNINDDNGENTFIQKYLCDDFKEFLGKPRDNKIEIIKNNDDILAIKYCVESTSKANKEIIVKALSDETPSA

SEQ ID NO: 139 - protein, 1247 aa, synthetic construct
KSLSINIDMGAINNGIFIATCQDDKIIDKNAFDIKFRKGKLNFSKRDRTLRRHTRRSFDRDRFVLRLLGEILPLENLSNNQKEKLFGLFKNRGFNYLNVNFNAEIDSDNLEILNALDRYYFKDCRVLSDFENSISKIFNELENNEILAFLDDQAQILNQAKEHKNKILNKNINAILEFLESIKNESFKNNKHRKSYLKDIKNEIENSFKDIILKLKIFKNSQELYYFIGNIANFQTRILRRYFNAKFDLVFDDAKLKKNILRNINYLDFISTDEKANKNKILENLNAFSTLEFLKNTDPIVTIPPYENAKNKKPQSCQALVINDEKITPSLKDIAHKILSNSNFECLKTDENGVLADNIKDNEIAKYLQRILDISKGILDDKELYPRLLEKDENAKIFAQEIRLNSVELKEFKDFAKKYYDEVNLAKKGIIKNELLKPCCLHTPHKNKNKNALISALFLKSITQKEIENLEDFFANNKISGNQTFKGFFERLSELKKRYQNRFFHILEHEPTKELEGILKNYKKVMEKIVEHNSNFSFKAPFDDSTISTNFNYLTQLGDIIFDEKSRGFAKTCKFHTLENLIRSSAKSAIASRLASNSARLINGKIEMYLDRLAHEIIKKIDFTDIYNVQINVEMNKFNFESNLSKLGLAKERQKDEESFICPYSGAKISQTNCEYDHILPRSKGLYNSLANLIPTSSTSNQIKSNTKYLLSNLDENYLKYIFAKTQTTDLNSFKAFIDENISKIDENDFTNFKNLSFFEQIAFRHALFLDTDDNSFKKALRLLKLDTIKTHSNGTQKRFINILIEKISKLTKSGIDLNFIDSKLVSSTRKDLAQNDTSIAKQEIQDSHSHCVDASIVFYLANSKIIKGQIEPDYDYFKDIYPKDSDIILPQSKQYLELNQKSQKSKKLFDDSVYSLVYEGKFDEKQKKILTQYELLKENGFVDTHKVFELIFKSFKDKDTIVLKDLKFLDNHLKSYIRKDIFSIFFNEKGELKEAKELKSATKNIDKFYTILSQNQDKIYTIKLDEKAKEKKTLQRNKVIELYKEIFYTKNAKPRARGKNRVTFSLPVYAKDAKYAIKRNSGFAGLKNKSIATKTYIDIDSREILKIPYYSTNVLPIRISDILEILSLQSKNAKQIYKIKIQDNLPKQIVSLDFILSQARRHEVLVSFDKSKLEIQNINDDNGENTFIQKYLCDDFKEFLGKPRSNKIEIIKNNDDILAIKYCVESTSKANKEIIVKALSDETPSA

SEQ ID NO: 140 - protein, 1247 aa, synthetic construct
KSLSINIDMGAINNGIFIATCQDDKIIDKNAFDIKFRKGKLNFSKRDRTLRRHTRRSFDRDRFVLRLLGEILPLENLSNNQKEKLFGLFKNRGFNYLNVNFNAEIDSDNLEILNALDRYYFKDCRVLSDFENSISKIFNELENNEILAFLDDQAQILNQAKEHKNKILNKNINAILEFLESIKNESFKNNKHRKSYLKDIKNEIENSFKDIILKLKIFKNSQELYYFIGNIANFQTRILRRYFNAKFDLVFDDAKLKKNILRNINYLDFISTDEKANKNKILENLNAFSTLEFLKNTDPIVTIPPYENAKNKKPQSCQALVINDEKITPSLKDIAHKILSNSNFECLKTDENGVLADNIKDNEIAKYLQRILDISKGILDDKELYPRLLEKDENAKIFAQEIRLNSVELKEFKDFAKKYYDEVNLAKKGIIKNELLKPCCLHTPHKNKNKNALISALFLKSITQKEIENLEDFFANNKISGNQTFKGFFERLSELKKRYQNRFFHILEHEPTKELEGILKNYKKVMEKIVEHNSNFSFKAPFDDSTISTNFNYLTQLGDIIFDEKSRGFAKTCKFHTLENLIRSSAKSAIASRLASNSARLINGKIEMYLDRLAHEIIKKIDFTDIYNVQINVEMNKFNFESNLSKLGLAKERQKDEESFICPYSGAKISQTNCEYDHILPRSKGLYNSLANLIPTSSTSNQIKSNTKYLLSNLDENYLKYIFAKTQTTDLNSFKAFIDENISKIDENDFTNFKNLSFFEQIAFRHALFLDTDDNSFKKALRLLKLDTIKTHSNGTQKRFINILIEKISKLTKSGIDLNFIDSKLVSSTRKDLAQNDTSIAKQEIQDSHSHCVDASIVFYLANSKIIKGQIEPDYDYFKDIYPKDSDIILPQSKQYLELNQKSQKSKKLFDDSVYSLVYEGKFDEKQKKILTQYELLKENGFVDTHKVFELIFKSFKDKDTIVLKDLKFLDNHLKSYIRKDIFSIFFNEKGELKEAKELKSATKNIDKFYTILSQNQDKIYTIKLDEKAKEKKTLQRNKVIELYKEIFYTKNAKPRARGKNRVTFSLPVYAKDAKYAIKRNSGFAGLKNKSIATKTYIDIDSREILKIPYYSTNVLPIRISDILEILSLQSKNAKQIYKIKIQDNLPKQIVSLDFILSQARRHEVLVSFDKSKLEIQNINDDNGENTFIQKYLCDDFKEFLGKPRNNKIEIIKNNDDILAIKYCVESTSKANKEIIVKALSDETPSA

SEQ ID NO: 141 - protein, 1247 aa, synthetic construct
KSLSINIDMGAINNGIFIATCQDDKIIDKNAFDIKFRKGKLNFSKRDRTLRRHTRRSFDRDRFVLRLLGEILPLENLSNNQKEKLFGLFKNRGFNYLNVNFNAEIDSDNLEILNALDRYYFKDCRVLSDFENSISKIFNELENNEILAFLDDQAQILNQAKEHKNKILNKNINAILEFLESIKNESFKNNKHRKSYLKDIKNEIENSFKDIILKLKIFKNSQELYYFIGNIANFQTRILRRYFNAKFDLVFDDAKLKKNILRNINYLDFISTDEKANKNKILENLNAFSTLEFLKNTDPIVTIPPYENAKNKKPQSCQALVINDEKITPSLKDIAHKILSNSNFECLKTDENGVLADNIKDNEIAKYLQRILDISKGILDDKELYPRLLEKDENAKIFAQEIRLNSVELKEFKDFAKKYYDEVNLAKKGIIKNELLKPCCLHTPHKNKNKNALISALFLKSITQKEIENLEDFFANNKISGNQTFKGFFERLSELKKRYQNRFFHILEHEPTKELEGILKNYKKVMEKIVEHNSNFSFKAPFDDSTISTNFNYLTQLGDIIFDEKRRGFAKTCKFHTLENLIRSSAKSAIASRLASNSARLINGKIEMYLDRLAHEIIKKIDFTDIYNVQINVEMNKFNFESNLSKLGLAKERQKDEESFICPYSGAKISQTNCEYDHILPRSKGLYNSLANLIPTSSTSNQIKSNTKYLLSNLDENYLKYIFAKTQTTDLNSFKAFIDENISKIDENDFTNFKNLSFFEQIAFRHALFLDTDDNSFKKALRLLKLDTIKTHSNGTQKRFINILIEKISKLTKSGIDLNFIDSKLVSSTRKDLAQNDTSIAKQEIQDSHSHCVDASIVFYLANSKIIKGQIEPDYDYFKDIYPKDSDIILPQSKQYLELNQKSQKSKKLFDDSVYSLVYEGKFDEKQKKILTQYELLKENGFVDTHKVFELIFKSFKDKDTIVLKDLKFLDNHLKSYIRKDIFSIFFNEKGELKEAKELKSATKNIDKFYTILSQNQDKIYTIKLDEKAKEKKTLQRNKVIELYKEIFYTKNAKPRARGKNRVTFSLPVYAKDAKYAIKRNSGFAGLKNKSIATKTYIDIDSREILKIPYYSTNVLPIRISDILEILSLQSKNAKQIYKIKIQDNLPKQIVSLDFILSQARRHEVLVSFDKSKLEIQNINDDNGENTFIQKYLCDDFKEFLGKPRDNKIEIIKNNDDILAIKYCVESTSKANKEIIVKALSDETPSA

SEQ ID NO: 142 - protein, 1247 aa, synthetic construct
KSLSINIDMGAINNGIFIATCQDDKIIDKNAFDIKFRKGKLNFSKIDRTLRRHTRRSFDRDRFVLRLLGEILPLENLSNNQKEKLFGLFKNRGFNYLNVNFNAEIDSDNLEILNALDRYYFKDCRVLSDFENSISKIFNELENNEILAFLDDQAQILNQAKEHKNKILNKNINAILEFLESIKNESFKNNKHRKSYLKDIKNEIENSFKDIILKLKIFKNSQELYYFIGNIANFQTRILRRYFNAKFDLVFDDAKLKKNILRNINYLDFISTDEKANKNKILENLNAFSTLEFLKNTDPIVTIPPYENAKNKKPQSCQALVINDEKITPSLKDIAHKILSNSNFECLKTDENGVLADNIKDNEIAKYLQRILDISKGILDDKELYPRLLEKDENAKIFAQEIRLNSVELKEFKDFAKKYYDEVNLAKKGIIKNELLKPCCLHTPHKNKNKNALISALFLKSITQKEIENLEDFFANNKISGNQTFKGFFERLSELKKRYQNRFFHILEHEPTKELEGILKNYKKVMEKIVEHNSNFSFKAPFDDSTISTNFNYLTQLGDIIFDEKRRGFAKTCKFHTLENLIRSSAKSAIASRLASNSARLINGKIEMYLDRLAHEIIKKIDFTDIYNVQINVEMNKFNFESNLSKLGLAKERQKDEESFICPYSGAKISQTNCEYDHILPRSKGLYNSLANLIPTSSTSNQIKSNTKYLLSNLDENYLKYIFAKTQTTDLNSFKAFIDENISKIDENDFTNFKNLSFFEQIAFRHALFLDTDDNSFKKALRLLKLDTIKTHSNGTQKRFINILIEKISKLTKSGIDLNFIDSKLVSSTRKDLAQNDTSIAKQEIQDSHSHCVDASIVFYLANSKIIKGQIEPDYDYFKDIYPKDSDIILPQSKQYLELNQKSQKSKKLFDDSVYSLVYEGKFDEKQKKILTQYELLKENGFVDTHKVFELIFKSFKDKDTIVLKDLKFLDNHLKSYIRKDIFSIFFNEKGELKEAKELKSATKNIDKFYTILSQNQDKIYTIKLDEKAKEKKTLQRNKVIELYKEIFYTKNAKPRARGKNRVTFSLPVYAKDAKYAIKRNSGFAGLKNKSIATKTYIDIDSREILKIPYYSTNVLPIRISDILEILSLQSKNAKQIYKIKIQDNLPKQIVSLDFILSQARRHEVLVSFDKSKLEIQNINDDNGENTFIQKYLCDDFKEFLGKPRSNKIEIIKNNDDILAIKYCVESTSKANKEIIVKALSDETPSA

SEQ ID NO: 143 - protein, 1247 aa, synthetic construct
KSLSINIDMGAINNGIFIATCQDDKIIDKNAFDIKFRKGKLNFSKIDRTLRRHTRRSFDRDRFVLRLLGEILPLENLSNNQKEKLFGLFKNRGFNYLNVNFNAEIDSDNLEILNALDRYYFKDCRVLSDFENSISKIFNELENNEILAFLDDQAQILNQAKEHKNKILNKNINAILEFLESIKNESFKNNKHRKSYLKDIKNEIENSFKDIILKLKIFKNSQELYYFIGNIANFQTRILRRYFNAKFDLVFDDAKLKKNILRNINYLDFISTDEKANKNKILENLNAFSTLEFLKNTDPIVTIPPYENAKNKKPQSCQALVINDEKITPSLKDIAHKILSNSNFECLKTDENGVLADNIKDNEIAKYLQRILDISKGILDDKELYPRLLEKDENAKIFAQEIRLNSVELKEFKDFAKKYYDEVNLAKKGIIKNELLKPCCLHTPHKNKNKNALISALFLKSITQKEIENLEDFFANNKISGNQTFKGFFERLSELKKRYQNRFFHILEHEPTKELEGILKNYKKVMEKIVEHNSNFSFKAPFDDSTISTNFNYLTQLGDIIFDEKRRGFAKTCKFHTLENLIRSSAKSAIASRLASNSARLINGKIEMYLDRLAHEIIKKIDFTDIYNVQINVEMNKFNFESNLSKLGLAKERQKDEESFICPYSGAKISQTNCEYDHILPRSKGLYNSLANLIPTSSTSNQIKSNTKYLLSNLDENYLKYIFAKTQTTDLNSFKAFIDENISKIDENDFTNFKNLSFFEQIAFRHALFLDTDDNSFKKALRLLKLDTIKTHSNGTQKRFINILIEKISKLTKSGIDLNFIDSKLVSSTRKDLAQNDTSIAKQEIQDSHSHCVDASIVFYLANSKIIKGQIEPDYDYFKDIYPKDSDIILPQSKQYLELNQKSQKSKKLFDNSVYSLVYEGKFDEKQKKILTQYELLKENGFVDTHKVFELIFKSFKDKDTIVLKDLKFLDNHLKSYIRKDIFSIFFNEKGELKEAKELKSATKNIDKFYTILSQNQDKIYTIKLDEKAKEKKTLQRNKVIELYKEIFYTKNAKPRARGKNRVTFSLPVYAKDAKYAIKRNSGFAGLKNKSIATKTYIDIDSREILKIPYYSTNVLPIRISDILEILSLQSKNAKQIYKIKIQDNLPKQIVSLDFILSQARRHEVLVSFDKSKLEIQNINDDNGENTFIQKYLCDDFKEFLGKPRDNKIEIIKNNDDILAIKYCVESTSKANKEIIVKALSDETPSA

SEQ ID NO: 144 - protein, 1247 aa, synthetic construct
KSLSINIDMGAINNGIFIATCQDDKIIDKNAFDIKFRKGKLNFSKRDRTLRRHTRRSFDRDRFVLRLLGEILPLENLSNNQKEKLFGLFKNRGFNYLNVNFNAEIDSDNLEILNALDRYYFKDCRVLSDFENSISKIFNELENNEILAFLDDQAQILNQAKEHKNKILNKNINAILEFLESIKNESFKNNKHRKSYLKDIKNEIENSFKDIILKLKIFKNSQELYYFIGNIANFQTRILRRYFNAKFDLVFDDAKLKKNILRNINYLDFISTDEKANKNKILENLNAFSTLEFLKNTDPIVTIPPYENAKNKKPQSCQALVINDEKITPSLKDIAHKILSNSNFECLKTDENGVLADNIKDNEIAKYLQRILDISKGILDDKELYPRLLEKDENAKIFAQEIRLNSVELKEFKDFAKKYYDEVNLAKKGIIKNELLKPCCLHTPHKNKNKNALISALFLKSITQKEIENLEDFFANNKISGNQTFKGFFERLSELKKRYQNRFFHILEHEPTKELEGILKNYKKVMEKIVEHNSNFSFKAPFDDSTISTNFNYLTQLGDIIFDEKRRGFAKTCKFHTLENLIRSSAKSAIASRLASNSARLINGKIEMYLDRLAHEIIKKIDFTDIYNVQINVEMNKFNFESNLSKLGLAKERQKDEESFICPYSGAKISQTNCEYDHILPRSKGLYNSLANLIPTSSTSNQIKSNTKYLLSNLDENYLKYIFAKTQTTDLNSFKAFIDENISKIDENDFTNFKNLSFFEQIAFRHALFLDTDDNSFKKALRLLKLDTIKTHSNGTQKRFINILIEKISKLTKSGIDLNFIDSKLVSSTRKDLAQNDTSIAKQEIQDSHSHCVDASIVFYLANSKIIKGQIEPDYDYFKDIYPKDSDIILPQSKQYLELNQKSQKSKKLFDDSVYSLVYEGKFDEKQKKILTQYELLKENGFVDTHKVFELIFKSFKDKDTIVLKDLKFLDNHLKSYIRKDIFSIFFNEKGELKEAKELKSATKNIDKFYTILSQNQDKIYTIKLDEKAKEKKTLQRNKVIELYKEIFYTKNAKPRARGKNRVTFSLPVYAKDAKYAIKRNSGFAGLKNKSIATKTYIDIDSREILKIPYYSTNVLPIRISDILEILSLQSKNAKQIYKIKIQDNLPKQIVSLDFILSQARRHEVLVSFDKSKLEIQNINDDNGENTFIQKYLCDDFKEFLGKPRNNKIEIIKNNDDILAIKYCVESTSKANKEIIVKALSDETPSA

SEQ ID NO: 145 - protein, 1274 aa, synthetic construct
MPKLKRQSSGSETPGTSESATPESGKSLSINIDMGAINNGIFIATCQDDKIIDKNAFDIKFRKGKLNFSKIDRTLRRHTRRSFDRDRFVLRLLGEILPLENLSNNQKEKLFGLFKNRGFNYLNVNFNAEIDSDNLEILNALDRYYFKDCRVLSDFENSISKIFNELENNEILAFLDDQAQILNQAKEHKNKILNKNINAILEFLESIKNESFKNNKHRKSYLKDIKNEIENSFKDIILKLKIFKNSQELYYFIGNIANFQTRILRRYFNAKFDLVFDDAKLKKNILRNINYLDFISTDEKANKNKILENLNAFSTLEFLKNTDPIVTIPPYENAKNKKPQSCQALVINDEKITPSLKDIAHKILSNSNFECLKTDENGVLADNIKDNEIAKYLQRILDISKGILDDKELYPRLLEKDENAKIFAQEIRLNSVELKEFKDFAKKYYDEVNLAKKGIIKNELLKPCCLHTPHKNKNKNALISALFLKSITQKEIENLEDFFANNKISGNQTFKGFFERLSELKKRYQNRFFHILEHEPTKELEGILKNYKKVMEKIVEHNSNFSFKAPFDDSTISTNFNYLTQLGDIIFDEKSRGFAKTCKFHTLENLIRSSAKSAIASRLASNSARLINGKIEMYLDRLAHEIIKKIDFTDIYNVQINVEMNKFNFESNLSKLGLAKERQKDEESFICPYSGAKISQTNCEYDHILPRSKGLYNSLANLIPTSSTSNQIKSNTKYLLSNLDENYLKYIFAKTQTTDLNSFKAFIDENISKIDENDFTNFKNLSFFEQIAFRHALFLDTDDNSFKKALRLLKLDTIKTHSNGTQKRFINILIEKISKLTKSGIDLNFIDSKLVSSTRKDLAQNDTSIAKQEIQDSHSHCVDASIVFYLANSKIIKGQIEPDYDYFKDIYPKDSDIILPQSKQYLELNQKSQKSKKLFDDSVYSLVYEGKFDEKQKKILTQYELLKENGFVDTHKVFELIFKSFKDKDTIVLKDLKFLDNHLKSYIRKDIFSIFFNEKGELKEAKELKSATKNIDKFYTILSQNQDKIYTIKLDEKAKEKKTLQRNKVIELYKEIFYTKNAKPRARGKNRVTFSLPVYAKDAKYAIKRNSGFAGLKNKDIATKTYIDIDSREILKIPYYSTNVLPIRISDILEILSLQSKNAKQIYKIKIQDNLPKQIVSLDFILSQANRHEVLVSFDKSKLEIQNINDDNGENTFIQKYLCDDFKEFLGKPRDNKIEIIKNNDDILAIKYCVESTSKANKEIIVKALSDETPSAGT

SEQ ID NO: 146 - protein, 1287 aa, synthetic construct
MGPGKMDKGEHRQERRDRPYSSGSETPGTSESATPESGKSLSINIDMGAINNGIFIATCQDDKIIDKNAFDIKFRKGKLNFSKIDRTLRRHTRRSFDRDRFVLRLLGEILPLENLSNNQKEKLFGLFKNRGFNYLNVNFNAEIDSDNLEILNALDRYYFKDCRVLSDFENSISKIFNELENNEILAFLDDQAQILNQAKEHKNKILNKNINAILEFLESIKNESFKNNKHRKSYLKDIKNEIENSFKDIILKLKIFKNSQELYYFIGNIANFQTRILRRYFNAKFDLVFDDAKLKKNILRNINYLDFISTDEKANKNKILENLNAFSTLEFLKNTDPIVTIPPYENAKNKKPQSCQALVINDEKITPSLKDIAHKILSNSNFECLKTDENGVLADNIKDNEIAKYLQRILDISKGILDDKELYPRLLEKDENAKIFAQEIRLNSVELKEFKDFAKKYYDEVNLAKKGIIKNELLKPCCLHTPHKNKNKNALISALFLKSITQKEIENLEDFFANNKISGNQTFKGFFERLSELKKRYQNRFFHILEHEPTKELEGILKNYKKVMEKIVEHNSNFSFKAPFDDSTISTNFNYLTQLGDIIFDEKSRGFAKTCKFHTLENLIRSSAKSAIASRLASNSARLINGKIEMYLDRLAHEIIKKIDFTDIYNVQINVEMNKFNFESNLSKLGLAKERQKDEESFICPYSGAKISQTNCEYDHILPRSKGLYNSLANLIPTSSTSNQIKSNTKYLLSNLDENYLKYIFAKTQTTDLNSFKAFIDENISKIDENDFTNFKNLSFFEQIAFRHALFLDTDDNSFKKALRLLKLDTIKTHSNGTQKRFINILIEKISKLTKSGIDLNFIDSKLVSSTRKDLAQNDTSIAKQEIQDSHSHCVDASIVFYLANSKIIKGQIEPDYDYFKDIYPKDSDIILPQSKQYLELNQKSQKSKKLFDDSVYSLVYEGKFDEKQKKILTQYELLKENGFVDTHKVFELIFKSFKDKDTIVLKDLKFLDNHLKSYIRKDIFSIFFNEKGELKEAKELKSATKNIDKFYTILSQNQDKIYTIKLDEKAKEKKTLQRNKVIELYKEIFYTKNAKPRARGKNRVTFSLPVYAKDAKYAIKRNSGFAGLKNKDIATKTYIDIDSREILKIPYYSTNVLPIRISDILEILSLQSKNAKQIYKIKIQDNLPKQIVSLDFILSQANRHEVLVSFDKSKLEIQNINDDNGENTFIQKYLCDDFKEFLGKPRDNKIEIIKNNDDILAIKYCVESTSKANKEIIVKALSDETPSAGT

SEQ ID NO: 147 - protein, 1283 aa, synthetic construct
MKEKNIKRGGNRFEPYSSGSETPGTSESATPESGKSLSINIDMGAINNGIFIATCQDDKIIDKNAFDIKFRKGKLNFSKIDRTLRRHTRRSFDRDRFVLRLLGEILPLENLSNNQKEKLFGLFKNRGFNYLNVNFNAEIDSDNLEILNALDRYYFKDCRVLSDFENSISKIFNELENNEILAFLDDQAQILNQAKEHKNKILNKNINAILEFLESIKNESFKNNKHRKSYLKDIKNEIENSFKDIILKLKIFKNSQELYYFIGNIANFQTRILRRYFNAKFDLVFDDAKLKKNILRNINYLDFISTDEKANKNKILENLNAFSTLEFLKNTDPIVTIPPYENAKNKKPQSCQALVINDEKITPSLKDIAHKILSNSNFECLKTDENGVLADNIKDNEIAKYLQRILDISKGILDDKELYPRLLEKDENAKIFAQEIRLNSVELKEFKDFAKKYYDEVNLAKKGIIKNELLKPCCLHTPHKNKNKNALISALFLKSITQKEIENLEDFFANNKISGNQTFKGFFERLSELKKRYQNRFFHILEHEPTKELEGILKNYKKVMEKIVEHNSNFSFKAPFDDSTISTNFNYLTQLGDIIFDEKSRGFAKTCKFHTLENLIRSSAKSAIASRLASNSARLINGKIEMYLDRLAHEIIKKIDFTDIYNVQINVEMNKFNFESNLSKLGLAKERQKDEESFICPYSGAKISQTNCEYDHILPRSKGLYNSLANLIPTSSTSNQIKSNTKYLLSNLDENYLKYIFAKTQTTDLNSFKAFIDENISKIDENDFTNFKNLSFFEQIAFRHALFLDTDDNSFKKALRLLKLDTIKTHSNGTQKRFINILIEKISKLTKSGIDLNFIDSKLVSSTRKDLAQNDTSIAKQEIQDSHSHCVDASIVFYLANSKIIKGQIEPDYDYFKDIYPKDSDIILPQSKQYLELNQKSQKSKKLFDDSVYSLVYEGKFDEKQKKILTQYELLKENGFVDTHKVFELIFKSFKDKDTIVLKDLKFLDNHLKSYIRKDIFSIFFNEKGELKEAKELKSATKNIDKFYTILSQNQDKIYTIKLDEKAKEKKTLQRNKVIELYKEIFYTKNAKPRARGKNRVTFSLPVYAKDAKYAIKRNSGFAGLKNKDIATKTYIDIDSREILKIPYYSTNVLPIRISDILEILSLQSKNAKQIYKIKIQDNLPKQIVSLDFILSQANRHEVLVSFDKSKLEIQNINDDNGENTFIQKYLCDDFKEFLGKPRDNKIEIIKNNDDILAIKYCVESTSKANKEIIVKALSDETPSAGT

SEQ ID NO: 148 - protein, 1252 aa, synthetic construct
MTGKSLSINIDMGAINNGIFIATCQDDKIIDKNAFDIKFRKGKLNFSKIDRTLRRHTRRSFDRDRFVLRLLGEILPLENLSNNQKEKLFGLFKNRGFNYLNVNFNAEIDSDNLEILNALDRYYFKDCRVLSDFENSISKIFNELENNEILAFLDDQAQILNQAKEHKNKILNKNINAILEFLESIKNESFKNNKHRKSYLKDIKNEIENSFKDIILKLKIFKNSQELYYFIGNIANFQTRILRRYFNAKFDLVFDDAKLKKNILRNINYLDFISTDEKANKNKILENLNAFSTLEFLKNTDPIVTIPPYENAKNKKPQSCQALVINDEKITPSLKDIAHKILSNSNFECLKTDENGVLADNIKDNEIAKYLQRILDISKGILDDKELYPRLLEKDENAKIFAQEIRLNSVELKEFKDFAKKYYDEVNLAKKGIIKNELLKPCCLHTPHKNKNKNALISALFLKSITQKEIENLEDFFANNKISGNQTFKGFFERLSELKKRYQNRFFHILEHEPTKELEGILKNYKKVMEKIVEHNSNFSFKAPFDDSTISTNFNYLTQLGDIIFDEKSRGFAKTCKFHTLENLIRSSAKSAIASRLASNSARLINGKIEMYLDRLAHEIIKKIDFTDIYNVQINVEMNKFNFESNLSKLGLAKERQKDEESFICPYSGAKISQTNCEYDHILPRSKGLYNSLANLIPTSSTSNQIKSNTKYLLSNLDENYLKYIFAKTQTTDLNSFKAFIDENISKIDENDFTNFKNLSFFEQIAFRHALFLDTDDNSFKKALRLLKLDTIKTHSNGTQKRFINILIEKISKLTKSGIDLNFIDSKLVSSTRKDLAQNDTSIAKQEIQDSHSHCVDASIVFYLANSKIIKGQIEPDYDYFKDIYPKDSDIILPQSKQYLELNQKSQKSKKLFDDSVYSLVYEGKFDEKQKKILTQYELLKENGFVDTHKVFELIFKSFKDKDTIVLKDLKFLDNHLKSYIRKDIFSIFFNEKGELKEAKELKSATKNIDKFYTILSQNQDKIYTIKLDEKAKEKKTLQRNKVIELYKEIFYTKNAKPRARGKNRVTFSLPVYAKDAKYAIKRNSGFAGLKNKDIATKTYIDIDSREILKIPYYSTNVLPIRISDILEILSLQSKNAKQIYKIKIQDNLPKQIVSLDFILSQANRHEVLVSFDKSKLEIQNINDDNGENTFIQKYLCDDFKEFLGKPRDNKIEIIKNNDDILAIKYCVESTSKANKEIIVKALSDETPSAGT

SEQ ID NO: 149 - protein, 1275 aa, synthetic construct
MPKKKRKVSSGSETPGTSESATPESGKSLSINIDMGAINNGIFIATCQDDKIIDKNAFDIKFRKGKLNFSKIDRTLRRHTRRSFDRDRFVLRLLGEILPLENLSNNQKEKLFGLFKNRGFNYLNVNFNAEIDSDNLEILNALDRYYFKDCRVLSDFENSISKIFNELENNEILAFLDDQAQILNQAKEHKNKILNKNINAILEFLESIKNESFKNNKHRKSYLKDIKNEIENSFKDIILKLKIFKNSQELYYFIGNIANFQTRILRRYFNAKFDLVFDDAKLKKNILRNINYLDFISTDEKANKNKILENLNAFSTLEFLKNTDPIVTIPPYENAKNKKPQSCQALVINDEKITPSLKDIAHKILSNSNFECLKTDENGVLADNIKDNEIAKYLQRILDISKGILDDKELYPRLLEKDENAKIFAQEIRLNSVELKEFKDFAKKYYDEVNLAKKGIIKNELLKPCCLHTPHKNKNKNALISALFLKSITQKEIENLEDFFANNKISGNQTFKGFFERLSELKKRYQNRFFHILEHEPTKELEGILKNYKKVMEKIVEHNSNFSFKAPFDDSTISTNFNYLTQLGDIIFDEKSRGFAKTCKFHTLENLIRSSAKSAIASRLASNSARLINGKIEMYLDRLAHEIIKKIDFTDIYNVQINVEMNKFNFESNLSKLGLAKERQKDEESFICPYSGAKISQTNCEYDHILPRSKGLYNSLANLIPTSSTSNQIKSNTKYLLSNLDENYLKYIFAKTQTTDLNSFKAFIDENISKIDENDFTNFKNLSFFEQIAFRHALFLDTDDNSFKKALRLLKLDTIKTHSNGTQKRFINILIEKISKLTKSGIDLNFIDSKLVSSTRKDLAQNDTSIAKQEIQDSHSHCVDASIVFYLANSKIIKGQIEPDYDYFKDIYPKDSDIILPQSKQYLELNQKSQKSKKLFDDSVYSLVYEGKFDEKQKKILTQYELLKENGFVDTHKVFELIFKSFKDKDTIVLKDLKFLDNHLKSYIRKDIFSIFFNEKGELKEAKELKSATKNIDKFYTILSQNQDKIYTIKLDEKAKEKKTLQRNKVIELYKEIFYTKNAKPRARGKNRVTFSLPVYAKDAKYAIKRNSGFAGLKNKDIATKTYIDIDSREILKIPYYSTNVLPIRISDILEILSLQSKNAKQIYKIKIQDNLPKQIVSLDFILSQANRHEVLVSFDKSKLEIQNINDDNGENTFIQKYLCDDFKEFLGKPRDNKIEIIKNNDDILAIKYCVESTSKANKEIIVKALSDETPSAGT

SEQ ID NO: 150 - protein, 1277 aa, synthetic construct
MPAAKRVKLDSSGSETPGTSESATPESGKSLSINIDMGAINNGIFIATCQDDKIIDKNAFDIKFRKGKLNFSKIDRTLRRHTRRSFDRDRFVLRLLGEILPLENLSNNQKEKLFGLFKNRGFNYLNVNFNAEIDSDNLEILNALDRYYFKDCRVLSDFENSISKIFNELENNEILAFLDDQAQILNQAKEHKNKILNKNINAILEFLESIKNESFKNNKHRKSYLKDIKNEIENSFKDIILKLKIFKNSQELYYFIGNIANFQTRILRRYFNAKFDLVFDDAKLKKNILRNINYLDFISTDEKANKNKILENLNAFSTLEFLKNTDPIVTIPPYENAKNKKPQSCQALVINDEKITPSLKDIAHKILSNSNFECLKTDENGVLADNIKDNEIAKYLQRILDISKGILDDKELYPRLLEKDENAKIFAQEIRLNSVELKEFKDFAKKYYDEVNLAKKGIIKNELLKPCCLHTPHKNKNKNALISALFLKSITQKEIENLEDFFANNKISGNQTFKGFFERLSELKKRYQNRFFHILEHEPTKELEGILKNYKKVMEKIVEHNSNFSFKAPFDDSTISTNFNYLTQLGDIIFDEKSRGFAKTCKFHTLENLIRSSAKSAIASRLASNSARLINGKIEMYLDRLAHEIIKKIDFTDIYNVQINVEMNKFNFESNLSKLGLAKERQKDEESFICPYSGAKISQTNCEYDHILPRSKGLYNSLANLIPTSSTSNQIKSNTKYLLSNLDENYLKYIFAKTQTTDLNSFKAFIDENISKIDENDFTNFKNLSFFEQIAFRHALFLDTDDNSFKKALRLLKLDTIKTHSNGTQKRFINILIEKISKLTKSGIDLNFIDSKLVSSTRKDLAQNDTSIAKQEIQDSHSHCVDASIVFYLANSKIIKGQIEPDYDYFKDIYPKDSDIILPQSKQYLELNQKSQKSKKLFDDSVYSLVYEGKFDEKQKKILTQYELLKENGFVDTHKVFELIFKSFKDKDTIVLKDLKFLDNHLKSYIRKDIFSIFFNEKGELKEAKELKSATKNIDKFYTILSQNQDKIYTIKLDEKAKEKKTLQRNKVIELYKEIFYTKNAKPRARGKNRVTFSLPVYAKDAKYAIKRNSGFAGLKNKDIATKTYIDIDSREILKIPYYSTNVLPIRISDILEILSLQSKNAKQIYKIKIQDNLPKQIVSLDFILSQANRHEVLVSFDKSKLEIQNINDDNGENTFIQKYLCDDFKEFLGKPRDNKIEIIKNNDDILAIKYCVESTSKANKEIIVKALSDETPSAGT

SEQ ID NO: 151 - protein, 1274 aa, synthetic construct
MKRKRRPSSGSETPGTSESATPESGKSLSINIDMGAINNGIFIATCQDDKIIDKNAFDIKFRKGKLNFSKIDRTLRRHTRRSFDRDRFVLRLLGEILPLENLSNNQKEKLFGLFKNRGFNYLNVNFNAEIDSDNLEILNALDRYYFKDCRVLSDFENSISKIFNELENNEILAFLDDQAQILNQAKEHKNKILNKNINAILEFLESIKNESFKNNKHRKSYLKDIKNEIENSFKDIILKLKIFKNSQELYYFIGNIANFQTRILRRYFNAKFDLVFDDAKLKKNILRNINYLDFISTDEKANKNKILENLNAFSTLEFLKNTDPIVTIPPYENAKNKKPQSCQALVINDEKITPSLKDIAHKILSNSNFECLKTDENGVLADNIKDNEIAKYLQRILDISKGILDDKELYPRLLEKDENAKIFAQEIRLNSVELKEFKDFAKKYYDEVNLAKKGIIKNELLKPCCLHTPHKNKNKNALISALFLKSITQKEIENLEDFFANNKISGNQTFKGFFERLSELKKRYQNRFFHILEHEPTKELEGILKNYKKVMEKIVEHNSNFSFKAPFDDSTISTNFNYLTQLGDIIFDEKSRGFAKTCKFHTLENLIRSSAKSAIASRLASNSARLINGKIEMYLDRLAHEIIKKIDFTDIYNVQINVEMNKFNFESNLSKLGLAKERQKDEESFICPYSGAKISQTNCEYDHILPRSKGLYNSLANLIPTSSTSNQIKSNTKYLLSNLDENYLKYIFAKTQTTDLNSFKAFIDENISKIDENDFTNFKNLSFFEQIAFRHALFLDTDDNSFKKALRLLKLDTIKTHSNGTQKRFINILIEKISKLTKSGIDLNFIDSKLVSSTRKDLAQNDTSIAKQEIQDSHSHCVDASIVFYLANSKIIKGQIEPDYDYFKDIYPKDSDIILPQSKQYLELNQKSQKSKKLFDDSVYSLVYEGKFDEKQKKILTQYELLKENGFVDTHKVFELIFKSFKDKDTIVLKDLKFLDNHLKSYIRKDIFSIFFNEKGELKEAKELKSATKNIDKFYTILSQNQDKIYTIKLDEKAKEKKTLQRNKVIELYKEIFYTKNAKPRARGKNRVTFSLPVYAKDAKYAIKRNSGFAGLKNKDIATKTYIDIDSREILKIPYYSTNVLPIRISDILEILSLQSKNAKQIYKIKIQDNLPKQIVSLDFILSQANRHEVLVSFDKSKLEIQNINDDNGENTFIQKYLCDDFKEFLGKPRDNKIEIIKNNDDILAIKYCVESTSKANKEIIVKALSDETPSAGT

SEQ ID NO: 152 - protein, 1278 aa, synthetic construct
MPKKNRLRRKSSSGSETPGTSESATPESGKSLSINIDMGAINNGIFIATCQDDKIIDKNAFDIKFRKGKLNFSKIDRTLRRHTRRSFDRDRFVLRLLGEILPLENLSNNQKEKLFGLFKNRGFNYLNVNFNAEIDSDNLEILNALDRYYFKDCRVLSDFENSISKIFNELENNEILAFLDDQAQILNQAKEHKNKILNKNINAILEFLESIKNESFKNNKHRKSYLKDIKNEIENSFKDIILKLKIFKNSQELYYFIGNIANFQTRILRRYFNAKFDLVFDDAKLKKNILRNINYLDFISTDEKANKNKILENLNAFSTLEFLKNTDPIVTIPPYENAKNKKPQSCQALVINDEKITPSLKDIAHKILSNSNFECLKTDENGVLADNIKDNEIAKYLQRILDISKGILDDKELYPRLLEKDENAKIFAQEIRLNSVELKEFKDFAKKYYDEVNLAKKGIIKNELLKPCCLHTPHKNKNKNALISALFLKSITQKEIENLEDFFANNKISGNQTFKGFFERLSELKKRYQNRFFHILEHEPTKELEGILKNYKKVMEKIVEHNSNFSFKAPFDDSTISTNFNYLTQLGDIIFDEKSRGFAKTCKFHTLENLIRSSAKSAIASRLASNSARLINGKIEMYLDRLAHEIIKKIDFTDIYNVQINVEMNKFNFESNLSKLGLAKERQKDEESFICPYSGAKISQTNCEYDHILPRSKGLYNSLANLIPTSSTSNQIKSNTKYLLSNLDENYLKYIFAKTQTTDLNSFKAFIDENISKIDENDFTNFKNLSFFEQIAFRHALFLDTDDNSFKKALRLLKLDTIKTHSNGTQKRFINILIEKISKLTKSGIDLNFIDSKLVSSTRKDLAQNDTSIAKQEIQDSHSHCVDASIVFYLANSKIIKGQIEPDYDYFKDIYPKDSDIILPQSKQYLELNQKSQKSKKLFDDSVYSLVYEGKFDEKQKKILTQYELLKENGFVDTHKVFELIFKSFKDKDTIVLKDLKFLDNHLKSYIRKDIFSIFFNEKGELKEAKELKSATKNIDKFYTILSQNQDKIYTIKLDEKAKEKKTLQRNKVIELYKEIFYTKNAKPRARGKNRVTFSLPVYAKDAKYAIKRNSGFAGLKNKDIATKTYIDIDSREILKIPYYSTNVLPIRISDILEILSLQSKNAKQIYKIKIQDNLPKQIVSLDFILSQANRHEVLVSFDKSKLEIQNINDDNGENTFIQKYLCDDFKEFLGKPRDNKIEIIKNNDDILAIKYCVESTSKANKEIIVKALSDETPSAGT

SEQ ID NO: 153 - protein, 1284 aa, synthetic construct
MKASRGGGNHQNNYQPYSSGSETPGTSESATPESGKSLSINIDMGAINNGIFIATCQDDKIIDKNAFDIKFRKGKLNFSKIDRTLRRHTRRSFDRDRFVLRLLGEILPLENLSNNQKEKLFGLFKNRGFNYLNVNFNAEIDSDNLEILNALDRYYFKDCRVLSDFENSISKIFNELENNEILAFLDDQAQILNQAKEHKNKILNKNINAILEFLESIKNESFKNNKHRKSYLKDIKNEIENSFKDIILKLKIFKNSQELYYFIGNIANFQTRILRRYFNAKFDLVFDDAKLKKNILRNINYLDFISTDEKANKNKILENLNAFSTLEFLKNTDPIVTIPPYENAKNKKPQSCQALVINDEKITPSLKDIAHKILSNSNFECLKTDENGVLADNIKDNEIAKYLQRILDISKGILDDKELYPRLLEKDENAKIFAQEIRLNSVELKEFKDFAKKYYDEVNLAKKGIIKNELLKPCCLHTPHKNKNKNALISALFLKSITQKEIENLEDFFANNKISGNQTFKGFFERLSELKKRYQNRFFHILEHEPTKELEGILKNYKKVMEKIVEHNSNFSFKAPFDDSTISTNFNYLTQLGDIIFDEKSRGFAKTCKFHTLENLIRSSAKSAIASRLASNSARLINGKIEMYLDRLAHEIIKKIDFTDIYNVQINVEMNKFNFESNLSKLGLAKERQKDEESFICPYSGAKISQTNCEYDHILPRSKGLYNSLANLIPTSSTSNQIKSNTKYLLSNLDENYLKYIFAKTQTTDLNSFKAFIDENISKIDENDFTNFKNLSFFEQIAFRHALFLDTDDNSFKKALRLLKLDTIKTHSNGTQKRFINILIEKISKLTKSGIDLNFIDSKLVSSTRKDLAQNDTSIAKQEIQDSHSHCVDASIVFYLANSKIIKGQIEPDYDYFKDIYPKDSDIILPQSKQYLELNQKSQKSKKLFDDSVYSLVYEGKFDEKQKKILTQYELLKENGFVDTHKVFELIFKSFKDKDTIVLKDLKFLDNHLKSYIRKDIFSIFFNEKGELKEAKELKSATKNIDKFYTILSQNQDKIYTIKLDEKAKEKKTLQRNKVIELYKEIFYTKNAKPRARGKNRVTFSLPVYAKDAKYAIKRNSGFAGLKNKDIATKTYIDIDSREILKIPYYSTNVLPIRISDILEILSLQSKNAKQIYKIKIQDNLPKQIVSLDFILSQANRHEVLVSFDKSKLEIQNINDDNGENTFIQKYLCDDFKEFLGKPRDNKIEIIKNNDDILAIKYCVESTSKANKEIIVKALSDETPSAGT

SEQ ID NO: 154 - protein, 1280 aa, synthetic construct
MGRKKRRQRRRAPSSGSETPGTSESATPESGKSLSINIDMGAINNGIFIATCQDDKIIDKNAFDIKFRKGKLNFSKIDRTLRRHTRRSFDRDRFVLRLLGEILPLENLSNNQKEKLFGLFKNRGFNYLNVNFNAEIDSDNLEILNALDRYYFKDCRVLSDFENSISKIFNELENNEILAFLDDQAQILNQAKEHKNKILNKNINAILEFLESIKNESFKNNKHRKSYLKDIKNEIENSFKDIILKLKIFKNSQELYYFIGNIANFQTRILRRYFNAKFDLVFDDAKLKKNILRNINYLDFISTDEKANKNKILENLNAFSTLEFLKNTDPIVTIPPYENAKNKKPQSCQALVINDEKITPSLKDIAHKILSNSNFECLKTDENGVLADNIKDNEIAKYLQRILDISKGILDDKELYPRLLEKDENAKIFAQEIRLNSVELKEFKDFAKKYYDEVNLAKKGIIKNELLKPCCLHTPHKNKNKNALISALFLKSITQKEIENLEDFFANNKISGNQTFKGFFERLSELKKRYQNRFFHILEHEPTKELEGILKNYKKVMEKIVEHNSNFSFKAPFDDSTISTNFNYLTQLGDIIFDEKSRGFAKTCKFHTLENLIRSSAKSAIASRLASNSARLINGKIEMYLDRLAHEIIKKIDFTDIYNVQINVEMNKFNFESNLSKLGLAKERQKDEESFICPYSGAKISQTNCEYDHILPRSKGLYNSLANLIPTSSTSNQIKSNTKYLLSNLDENYLKYIFAKTQTTDLNSFKAFIDENISKIDENDFTNFKNLSFFEQIAFRHALFLDTDDNSFKKALRLLKLDTIKTHSNGTQKRFINILIEKISKLTKSGIDLNFIDSKLVSSTRKDLAQNDTSIAKQEIQDSHSHCVDASIVFYLANSKIIKGQIEPDYDYFKDIYPKDSDIILPQSKQYLELNQKSQKSKKLFDDSVYSLVYEGKFDEKQKKILTQYELLKENGFVDTHKVFELIFKSFKDKDTIVLKDLKFLDNHLKSYIRKDIFSIFFNEKGELKEAKELKSATKNIDKFYTILSQNQDKIYTIKLDEKAKEKKTLQRNKVIELYKEIFYTKNAKPRARGKNRVTFSLPVYAKDAKYAIKRNSGFAGLKNKDIATKTYIDIDSREILKIPYYSTNVLPIRISDILEILSLQSKNAKQIYKIKIQDNLPKQIVSLDFILSQANRHEVLVSFDKSKLEIQNINDDNGENTFIQKYLCDDFKEFLGKPRDNKIEIIKNNDDILAIKYCVESTSKANKEIIVKALSDETPSAGT

SEQ ID NO: 155 - protein, 1286 aa, synthetic construct
MTRQARRNRRRRWRERQRQSSGSETPGTSESATPESGKSLSINIDMGAINNGIFIATCQDDKIIDKNAFDIKFRKGKLNFSKIDRTLRRHTRRSFDRDRFVLRLLGEILPLENLSNNQKEKLFGLFKNRGFNYLNVNFNAEIDSDNLEILNALDRYYFKDCRVLSDFENSISKIFNELENNEILAFLDDQAQILNQAKEHKNKILNKNINAILEFLESIKNESFKNNKHRKSYLKDIKNEIENSFKDIILKLKIFKNSQELYYFIGNIANFQTRILRRYFNAKFDLVFDDAKLKKNILRNINYLDFISTDEKANKNKILENLNAFSTLEFLKNTDPIVTIPPYENAKNKKPQSCQALVINDEKITPSLKDIAHKILSNSNFECLKTDENGVLADNIKDNEIAKYLQRILDISKGILDDKELYPRLLEKDENAKIFAQEIRLNSVELKEFKDFAKKYYDEVNLAKKGIIKNELLKPCCLHTPHKNKNKNALISALFLKSITQKEIENLEDFFANNKISGNQTFKGFFERLSELKKRYQNRFFHILEHEPTKELEGILKNYKKVMEKIVEHNSNFSFKAPFDDSTISTNFNYLTQLGDIIFDEKSRGFAKTCKFHTLENLIRSSAKSAIASRLASNSARLINGKIEMYLDRLAHEIIKKIDFTDIYNVQINVEMNKFNFESNLSKLGLAKERQKDEESFICPYSGAKISQTNCEYDHILPRSKGLYNSLANLIPTSSTSNQIKSNTKYLLSNLDENYLKYIFAKTQTTDLNSFKAFIDENISKIDENDFTNFKNLSFFEQIAFRHALFLDTDDNSFKKALRLLKLDTIKTHSNGTQKRFINILIEKISKLTKSGIDLNFIDSKLVSSTRKDLAQNDTSIAKQEIQDSHSHCVDASIVFYLANSKIIKGQIEPDYDYFKDIYPKDSDIILPQSKQYLELNQKSQKSKKLFDDSVYSLVYEGKFDEKQKKILTQYELLKENGFVDTHKVFELIFKSFKDKDTIVLKDLKFLDNHLKSYIRKDIFSIFFNEKGELKEAKELKSATKNIDKFYTILSQNQDKIYTIKLDEKAKEKKTLQRNKVIELYKEIFYTKNAKPRARGKNRVTFSLPVYAKDAKYAIKRNSGFAGLKNKDIATKTYIDIDSREILKIPYYSTNVLPIRISDILEILSLQSKNAKQIYKIKIQDNLPKQIVSLDFILSQANRHEVLVSFDKSKLEIQNINDDNGENTFIQKYLCDDFKEFLGKPRDNKIEIIKNNDDILAIKYCVESTSKANKEIIVKALSDETPSAGT

SEQ ID NO: 156 - protein, 1287 aa, synthetic construct
MMPKTRRRPRRSQRKRPPTPSSGSETPGTSESATPESGKSLSINIDMGAINNGIFIATCQDDKIIDKNAFDIKFRKGKLNFSKIDRTLRRHTRRSFDRDRFVLRLLGEILPLENLSNNQKEKLFGLFKNRGFNYLNVNFNAEIDSDNLEILNALDRYYFKDCRVLSDFENSISKIFNELENNEILAFLDDQAQILNQAKEHKNKILNKNINAILEFLESIKNESFKNNKHRKSYLKDIKNEIENSFKDIILKLKIFKNSQELYYFIGNIANFQTRILRRYFNAKFDLVFDDAKLKKNILRNINYLDFISTDEKANKNKILENLNAFSTLEFLKNTDPIVTIPPYENAKNKKPQSCQALVINDEKITPSLKDIAHKILSNSNFECLKTDENGVLADNIKDNEIAKYLQRILDISKGILDDKELYPRLLEKDENAKIFAQEIRLNSVELKEFKDFAKKYYDEVNLAKKGIIKNELLKPCCLHTPHKNKNKNALISALFLKSITQKEIENLEDFFANNKISGNQTFKGFFERLSELKKRYQNRFFHILEHEPTKELEGILKNYKKVMEKIVEHNSNFSFKAPFDDSTISTNFNYLTQLGDIIFDEKSRGFAKTCKFHTLENLIRSSAKSAIASRLASNSARLINGKIEMYLDRLAHEIIKKIDFTDIYNVQINVEMNKFNFESNLSKLGLAKERQKDEESFICPYSGAKISQTNCEYDHILPRSKGLYNSLANLIPTSSTSNQIKSNTKYLLSNLDENYLKYIFAKTQTTDLNSFKAFIDENISKIDENDFTNFKNLSFFEQIAFRHALFLDTDDNSFKKALRLLKLDTIKTHSNGTQKRFINILIEKISKLTKSGIDLNFIDSKLVSSTRKDLAQNDTSIAKQEIQDSHSHCVDASIVFYLANSKIIKGQIEPDYDYFKDIYPKDSDIILPQSKQYLELNQKSQKSKKLFDDSVYSLVYEGKFDEKQKKILTQYELLKENGFVDTHKVFELIFKSFKDKDTIVLKDLKFLDNHLKSYIRKDIFSIFFNEKGELKEAKELKSATKNIDKFYTILSQNQDKIYTIKLDEKAKEKKTLQRNKVIELYKEIFYTKNAKPRARGKNRVTFSLPVYAKDAKYAIKRNSGFAGLKNKDIATKTYIDIDSREILKIPYYSTNVLPIRISDILEILSLQSKNAKQIYKIKIQDNLPKQIVSLDFILSQANRHEVLVSFDKSKLEIQNINDDNGENTFIQKYLCDDFKEFLGKPRDNKIEIIKNNDDILAIKYCVESTSKANKEIIVKALSDETPSAGT

SEQ ID NO: 157 - protein, 1284 aa, synthetic construct
MTGKSLSINIDMGAINNGIFIATCQDDKIIDKNAFDIKFRKGKLNFSKIDRTLRRHTRRSFDRDRFVLRLLGEILPLENLSNNQKEKLFGLFKNRGFNYLNVNFNAEIDSDNLEILNALDRYYFKDCRVLSDFENSISKIFNELENNEILAFLDDQAQILNQAKEHKNKILNKNINAILEFLESIKNESFKNNKHRKSYLKDIKNEIENSFKDIILKLKIFKNSQELYYFIGNIANFQTRILRRYFNAKFDLVFDDAKLKKNILRNINYLDFISTDEKANKNKILENLNAFSTLEFLKNTDPIVTIPPYENAKNKKPQSCQALVINDEKITPSLKDIAHKILSNSNFECLKTDENGVLADNIKDNEIAKYLQRILDISKGILDDKELYPRLLEKDENAKIFAQEIRLNSVELKEFKDFAKKYYDEVNLAKKGIIKNELLKPCCLHTPHKNKNKNALISALFLKSITQKEIENLEDFFANNKISGNQTFKGFFERLSELKKRYQNRFFHILEHEPTKELEGILKNYKKVMEKIVEHNSNFSFKAPFDDSTISTNFNYLTQLGDIIFDEKSRGFAKTCKFHTLENLIRSSAKSAIASRLASNSARLINGKIEMYLDRLAHEIIKKIDFTDIYNVQINVEMNKFNFESNLSKLGLAKERQKDEESFICPYSGAKISQTNCEYDHILPRSKGLYNSLANLIPTSSTSNQIKSNTKYLLSNLDENYLKYIFAKTQTTDLNSFKAFIDENISKIDENDFTNFKNLSFFEQIAFRHALFLDTDDNSFKKALRLLKLDTIKTHSNGTQKRFINILIEKISKLTKSGIDLNFIDSKLVSSTRKDLAQNDTSIAKQEIQDSHSHCVDASIVFYLANSKIIKGQIEPDYDYFKDIYPKDSDIILPQSKQYLELNQKSQKSKKLFDDSVYSLVYEGKFDEKQKKILTQYELLKENGFVDTHKVFELIFKSFKDKDTIVLKDLKFLDNHLKSYIRKDIFSIFFNEKGELKEAKELKSATKNIDKFYTILSQNQDKIYTIKLDEKAKEKKTLQRNKVIELYKEIFYTKNAKPRARGKNRVTFSLPVYAKDAKYAIKRNSGFAGLKNKDIATKTYIDIDSREILKIPYYSTNVLPIRISDILEILSLQSKNAKQIYKIKIQDNLPKQIVSLDFILSQANRHEVLVSFDKSKLEIQNINDDNGENTFIQKYLCDDFKEFLGKPRDNKIEIIKNNDDILAIKYCVESTSKANKEIIVKALSDETPSAGSSGSETPGTSESATPESKRLVPQKQASVAKKKK

SEQ ID NO: 158 - protein, 1274 aa, synthetic construct
MTGKSLSINIDMGAINNGIFIATCQDDKIIDKNAFDIKFRKGKLNFSKIDRTLRRHTRRSFDRDRFVLRLLGEILPLENLSNNQKEKLFGLFKNRGFNYLNVNFNAEIDSDNLEILNALDRYYFKDCRVLSDFENSISKIFNELENNEILAFLDDQAQILNQAKEHKNKILNKNINAILEFLESIKNESFKNNKHRKSYLKDIKNEIENSFKDIILKLKIFKNSQELYYFIGNIANFQTRILRRYFNAKFDLVFDDAKLKKNILRNINYLDFISTDEKANKNKILENLNAFSTLEFLKNTDPIVTIPPYENAKNKKPQSCQALVINDEKITPSLKDIAHKILSNSNFECLKTDENGVLADNIKDNEIAKYLQRILDISKGILDDKELYPRLLEKDENAKIFAQEIRLNSVELKEFKDFAKKYYDEVNLAKKGIIKNELLKPCCLHTPHKNKNKNALISALFLKSITQKEIENLEDFFANNKISGNQTFKGFFERLSELKKRYQNRFFHILEHEPTKELEGILKNYKKVMEKIVEHNSNFSFKAPFDDSTISTNFNYLTQLGDIIFDEKSRGFAKTCKFHTLENLIRSSAKSAIASRLASNSARLINGKIEMYLDRLAHEIIKKIDFTDIYNVQINVEMNKFNFESNLSKLGLAKERQKDEESFICPYSGAKISQTNCEYDHILPRSKGLYNSLANLIPTSSTSNQIKSNTKYLLSNLDENYLKYIFAKTQTTDLNSFKAFIDENISKIDENDFTNFKNLSFFEQIAFRHALFLDTDDNSFKKALRLLKLDTIKTHSNGTQKRFINILIEKISKLTKSGIDLNFIDSKLVSSTRKDLAQNDTSIAKQEIQDSHSHCVDASIVFYLANSKIIKGQIEPDYDYFKDIYPKDSDIILPQSKQYLELNQKSQKSKKLFDDSVYSLVYEGKFDEKQKKILTQYELLKENGFVDTHKVFELIFKSFKDKDTIVLKDLKFLDNHLKSYIRKDIFSIFFNEKGELKEAKELKSATKNIDKFYTILSQNQDKIYTIKLDEKAKEKKTLQRNKVIELYKEIFYTKNAKPRARGKNRVTFSLPVYAKDAKYAIKRNSGFAGLKNKDIATKTYIDIDSREILKIPYYSTNVLPIRISDILEILSLQSKNAKQIYKIKIQDNLPKQIVSLDFILSQANRHEVLVSFDKSKLEIQNINDDNGENTFIQKYLCDDFKEFLGKPRDNKIEIIKNNDDILAIKYCVESTSKANKEIIVKALSDETPSAGSSGSETPGTSESATPESPKLKRQ

SEQ ID NO: 159 - protein, 1274 aa, synthetic construct
MTGKSLSINIDMGAINNGIFIATCQDDKIIDKNAFDIKFRKGKLNFSKIDRTLRRHTRRSFDRDRFVLRLLGEILPLENLSNNQKEKLFGLFKNRGFNYLNVNFNAEIDSDNLEILNALDRYYFKDCRVLSDFENSISKIFNELENNEILAFLDDQAQILNQAKEHKNKILNKNINAILEFLESIKNESFKNNKHRKSYLKDIKNEIENSFKDIILKLKIFKNSQELYYFIGNIANFQTRILRRYFNAKFDLVFDDAKLKKNILRNINYLDFISTDEKANKNKILENLNAFSTLEFLKNTDPIVTIPPYENAKNKKPQSCQALVINDEKITPSLKDIAHKILSNSNFECLKTDENGVLADNIKDNEIAKYLQRILDISKGILDDKELYPRLLEKDENAKIFAQEIRLNSVELKEFKDFAKKYYDEVNLAKKGIIKNELLKPCCLHTPHKNKNKNALISALFLKSITQKEIENLEDFFANNKISGNQTFKGFFERLSELKKRYQNRFFHILEHEPTKELEGILKNYKKVMEKIVEHNSNFSFKAPFDDSTISTNFNYLTQLGDIIFDEKSRGFAKTCKFHTLENLIRSSAKSAIASRLASNSARLINGKIEMYLDRLAHEIIKKIDFTDIYNVQINVEMNKFNFESNLSKLGLAKERQKDEESFICPYSGAKISQTNCEYDHILPRSKGLYNSLANLIPTSSTSNQIKSNTKYLLSNLDENYLKYIFAKTQTTDLNSFKAFIDENISKIDENDFTNFKNLSFFEQIAFRHALFLDTDDNSFKKALRLLKLDTIKTHSNGTQKRFINILIEKISKLTKSGIDLNFIDSKLVSSTRKDLAQNDTSIAKQEIQDSHSHCVDASIVFYLANSKIIKGQIEPDYDYFKDIYPKDSDIILPQSKQYLELNQKSQKSKKLFDDSVYSLVYEGKFDEKQKKILTQYELLKENGFVDTHKVFELIFKSFKDKDTIVLKDLKFLDNHLKSYIRKDIFSIFFNEKGELKEAKELKSATKNIDKFYTILSQNQDKIYTIKLDEKAKEKKTLQRNKVIELYKEIFYTKNAKPRARGKNRVTFSLPVYAKDAKYAIKRNSGFAGLKNKDIATKTYIDIDSREILKIPYYSTNVLPIRISDILEILSLQSKNAKQIYKIKIQDNLPKQIVSLDFILSQANRHEVLVSFDKSKLEIQNINDDNGENTFIQKYLCDDFKEFLGKPRDNKIEIIKNNDDILAIKYCVESTSKANKEIIVKALSDETPSAGSSGSETPGTSESATPESKRKRRP

SEQ ID NO: 160 - protein, 1278 aa, synthetic construct
MTGKSLSINIDMGAINNGIFIATCQDDKIIDKNAFDIKFRKGKLNFSKIDRTLRRHTRRSFDRDRFVLRLLGEILPLENLSNNQKEKLFGLFKNRGFNYLNVNFNAEIDSDNLEILNALDRYYFKDCRVLSDFENSISKIFNELENNEILAFLDDQAQILNQAKEHKNKILNKNINAILEFLESIKNESFKNNKHRKSYLKDIKNEIENSFKDIILKLKIFKNSQELYYFIGNIANFQTRILRRYFNAKFDLVFDDAKLKKNILRNINYLDFISTDEKANKNKILENLNAFSTLEFLKNTDPIVTIPPYENAKNKKPQSCQALVINDEKITPSLKDIAHKILSNSNFECLKTDENGVLADNIKDNEIAKYLQRILDISKGILDDKELYPRLLEKDENAKIFAQEIRLNSVELKEFKDFAKKYYDEVNLAKKGIIKNELLKPCCLHTPHKNKNKNALISALFLKSITQKEIENLEDFFANNKISGNQTFKGFFERLSELKKRYQNRFFHILEHEPTKELEGILKNYKKVMEKIVEHNSNFSFKAPFDDSTISTNFNYLTQLGDIIFDEKSRGFAKTCKFHTLENLIRSSAKSAIASRLASNSARLINGKIEMYLDRLAHEIIKKIDFTDIYNVQINVEMNKFNFESNLSKLGLAKERQKDEESFICPYSGAKISQTNCEYDHILPRSKGLYNSLANLIPTSSTSNQIKSNTKYLLSNLDENYLKYIFAKTQTTDLNSFKAFIDENISKIDENDFTNFKNLSFFEQIAFRHALFLDTDDNSFKKALRLLKLDTIKTHSNGTQKRFINILIEKISKLTKSGIDLNFIDSKLVSSTRKDLAQNDTSIAKQEIQDSHSHCVDASIVFYLANSKIIKGQIEPDYDYFKDIYPKDSDIILPQSKQYLELNQKSQKSKKLFDDSVYSLVYEGKFDEKQKKILTQYELLKENGFVDTHKVFELIFKSFKDKDTIVLKDLKFLDNHLKSYIRKDIFSIFFNEKGELKEAKELKSATKNIDKFYTILSQNQDKIYTIKLDEKAKEKKTLQRNKVIELYKEIFYTKNAKPRARGKNRVTFSLPVYAKDAKYAIKRNSGFAGLKNKDIATKTYIDIDSREILKIPYYSTNVLPIRISDILEILSLQSKNAKQIYKIKIQDNLPKQIVSLDFILSQANRHEVLVSFDKSKLEIQNINDDNGENTFIQKYLCDDFKEFLGKPRDNKIEIIKNNDDILAIKYCVESTSKANKEIIVKALSDETPSAGSSGSETPGTSESATPESPKKNRLRRKS

SEQ ID NO: 161 - protein, 1284 aa, synthetic construct
MKRLVPQKQASVAKKKKSSGSETPGTSESATPESGKSLSINIDMGAINNGIFIATCQDDKIIDKNAFDIKFRKGKLNFSKIDRTLRRHTRRSFDRDRFVLRLLGEILPLENLSNNQKEKLFGLFKNRGFNYLNVNFNAEIDSDNLEILNALDRYYFKDCRVLSDFENSISKIFNELENNEILAFLDDQAQILNQAKEHKNKILNKNINAILEFLESIKNESFKNNKHRKSYLKDIKNEIENSFKDIILKLKIFKNSQELYYFIGNIANFQTRILRRYFNAKFDLVFDDAKLKKNILRNINYLDFISTDEKANKNKILENLNAFSTLEFLKNTDPIVTIPPYENAKNKKPQSCQALVINDEKITPSLKDIAHKILSNSNFECLKTDENGVLADNIKDNEIAKYLQRILDISKGILDDKELYPRLLEKDENAKIFAQEIRLNSVELKEFKDFAKKYYDEVNLAKKGIIKNELLKPCCLHTPHKNKNKNALISALFLKSITQKEIENLEDFFANNKISGNQTFKGFFERLSELKKRYQNRFFHILEHEPTKELEGILKNYKKVMEKIVEHNSNFSFKAPFDDSTISTNFNYLTQLGDIIFDEKSRGFAKTCKFHTLENLIRSSAKSAIASRLASNSARLINGKIEMYLDRLAHEIIKKIDFTDIYNVQINVEMNKFNFESNLSKLGLAKERQKDEESFICPYSGAKISQTNCEYDHILPRSKGLYNSLANLIPTSSTSNQIKSNTKYLLSNLDENYLKYIFAKTQTTDLNSFKAFIDENISKIDENDFTNFKNLSFFEQIAFRHALFLDTDDNSFKKALRLLKLDTIKTHSNGTQKRFINILIEKISKLTKSGIDLNFIDSKLVSSTRKDLAQNDTSIAKQEIQDSHSHCVDASIVFYLANSKIIKGQIEPDYDYFKDIYPKDSDIILPQSKQYLELNQKSQKSKKLFDDSVYSLVYEGKFDEKQKKILTQYELLKENGFVDTHKVFELIFKSFKDKDTIVLKDLKFLDNHLKSYIRKDIFSIFFNEKGELKEAKELKSATKNIDKFYTILSQNQDKIYTIKLDEKAKEKKTLQRNKVIELYKEIFYTKNAKPRARGKNRVTFSLPVYAKDAKYAIKRNSGFAGLKNKDIATKTYIDIDSREILKIPYYSTNVLPIRISDILEILSLQSKNAKQIYKIKIQDNLPKQIVSLDFILSQANRHEVLVSFDKSKLEIQNINDDNGENTFIQKYLCDDFKEFLGKPRDNKIEIIKNNDDILAIKYCVESTSKANKEIIVKALSDETPSAGT

SEQ ID NO: 162 - protein, 1288 aa, synthetic construct
MGPGKMDSRGEHRQDRRERPYSSGSETPGTSESATPESGKSLSINIDMGAINNGIFIATCQDDKIIDKNAFDIKFRKGKLNFSKIDRTLRRHTRRSFDRDRFVLRLLGEILPLENLSNNQKEKLFGLFKNRGFNYLNVNFNAEIDSDNLEILNALDRYYFKDCRVLSDFENSISKIFNELENNEILAFLDDQAQILNQAKEHKNKILNKNINAILEFLESIKNESFKNNKHRKSYLKDIKNEIENSFKDIILKLKIFKNSQELYYFIGNIANFQTRILRRYFNAKFDLVFDDAKLKKNILRNINYLDFISTDEKANKNKILENLNAFSTLEFLKNTDPIVTIPPYENAKNKKPQSCQALVINDEKITPSLKDIAHKILSNSNFECLKTDENGVLADNIKDNEIAKYLQRILDISKGILDDKELYPRLLEKDENAKIFAQEIRLNSVELKEFKDFAKKYYDEVNLAKKGIIKNELLKPCCLHTPHKNKNKNALISALFLKSITQKEIENLEDFFANNKISGNQTFKGFFERLSELKKRYQNRFFHILEHEPTKELEGILKNYKKVMEKIVEHNSNFSFKAPFDDSTISTNFNYLTQLGDIIFDEKSRGFAKTCKFHTLENLIRSSAKSAIASRLASNSARLINGKIEMYLDRLAHEIIKKIDFTDIYNVQINVEMNKFNFESNLSKLGLAKERQKDEESFICPYSGAKISQTNCEYDHILPRSKGLYNSLANLIPTSSTSNQIKSNTKYLLSNLDENYLKYIFAKTQTTDLNSFKAFIDENISKIDENDFTNFKNLSFFEQIAFRHALFLDTDDNSFKKALRLLKLDTIKTHSNGTQKRFINILIEKISKLTKSGIDLNFIDSKLVSSTRKDLAQNDTSIAKQEIQDSHSHCVDASIVFYLANSKIIKGQIEPDYDYFKDIYPKDSDIILPQSKQYLELNQKSQKSKKLFDDSVYSLVYEGKFDEKQKKILTQYELLKENGFVDTHKVFELIFKSFKDKDTIVLKDLKFLDNHLKSYIRKDIFSIFFNEKGELKEAKELKSATKNIDKFYTILSQNQDKIYTIKLDEKAKEKKTLQRNKVIELYKEIFYTKNAKPRARGKNRVTFSLPVYAKDAKYAIKRNSGFAGLKNKDIATKTYIDIDSREILKIPYYSTNVLPIRISDILEILSLQSKNAKQIYKIKIQDNLPKQIVSLDFILSQANRHEVLVSFDKSKLEIQNINDDNGENTFIQKYLCDDFKEFLGKPRDNKIEIIKNNDDILAIKYCVESTSKANKEIIVKALSDETPSAGT

SEQ ID NO: 163 - protein, 1289 aa, synthetic construct
MGKKKKGKPGKRREQRKKKRRTSSGSETPGTSESATPESGKSLSINIDMGAINNGIFIATCQDDKIIDKNAFDIKFRKGKLNFSKIDRTLRRHTRRSFDRDRFVLRLLGEILPLENLSNNQKEKLFGLFKNRGFNYLNVNFNAEIDSDNLEILNALDRYYFKDCRVLSDFENSISKIFNELENNEILAFLDDQAQILNQAKEHKNKILNKNINAILEFLESIKNESFKNNKHRKSYLKDIKNEIENSFKDIILKLKIFKNSQELYYFIGNIANFQTRILRRYFNAKFDLVFDDAKLKKNILRNINYLDFISTDEKANKNKILENLNAFSTLEFLKNTDPIVTIPPYENAKNKKPQSCQALVINDEKITPSLKDIAHKILSNSNFECLKTDENGVLADNIKDNEIAKYLQRILDISKGILDDKELYPRLLEKDENAKIFAQEIRLNSVELKEFKDFAKKYYDEVNLAKKGIIKNELLKPCCLHTPHKNKNKNALISALFLKSITQKEIENLEDFFANNKISGNQTFKGFFERLSELKKRYQNRFFHILEHEPTKELEGILKNYKKVMEKIVEHNSNFSFKAPFDDSTISTNFNYLTQLGDIIFDEKSRGFAKTCKFHTLENLIRSSAKSAIASRLASNSARLINGKIEMYLDRLAHEIIKKIDFTDIYNVQINVEMNKFNFESNLSKLGLAKERQKDEESFICPYSGAKISQTNCEYDHILPRSKGLYNSLANLIPTSSTSNQIKSNTKYLLSNLDENYLKYIFAKTQTTDLNSFKAFIDENISKIDENDFTNFKNLSFFEQIAFRHALFLDTDDNSFKKALRLLKLDTIKTHSNGTQKRFINILIEKISKLTKSGIDLNFIDSKLVSSTRKDLAQNDTSIAKQEIQDSHSHCVDASIVFYLANSKIIKGQIEPDYDYFKDIYPKDSDIILPQSKQYLELNQKSQKSKKLFDDSVYSLVYEGKFDEKQKKILTQYELLKENGFVDTHKVFELIFKSFKDKDTIVLKDLKFLDNHLKSYIRKDIFSIFFNEKGELKEAKELKSATKNIDKFYTILSQNQDKIYTIKLDEKAKEKKTLQRNKVIELYKEIFYTKNAKPRARGKNRVTFSLPVYAKDAKYAIKRNSGFAGLKNKDIATKTYIDIDSREILKIPYYSTNVLPIRISDILEILSLQSKNAKQIYKIKIQDNLPKQIVSLDFILSQANRHEVLVSFDKSKLEIQNINDDNGENTFIQKYLCDDFKEFLGKPRDNKIEIIKNNDDILAIKYCVESTSKANKEIIVKALSDETPSAGT

SEQ ID NO: 164 - protein, 1288 aa, synthetic construct
MTGKSLSINIDMGAINNGIFIATCQDDKIIDKNAFDIKFRKGKLNFSKIDRTLRRHTRRSFDRDRFVLRLLGEILPLENLSNNQKEKLFGLFKNRGFNYLNVNFNAEIDSDNLEILNALDRYYFKDCRVLSDFENSISKIFNELENNEILAFLDDQAQILNQAKEHKNKILNKNINAILEFLESIKNESFKNNKHRKSYLKDIKNEIENSFKDIILKLKIFKNSQELYYFIGNIANFQTRILRRYFNAKFDLVFDDAKLKKNILRNINYLDFISTDEKANKNKILENLNAFSTLEFLKNTDPIVTIPPYENAKNKKPQSCQALVINDEKITPSLKDIAHKILSNSNFECLKTDENGVLADNIKDNEIAKYLQRILDISKGILDDKELYPRLLEKDENAKIFAQEIRLNSVELKEFKDFAKKYYDEVNLAKKGIIKNELLKPCCLHTPHKNKNKNALISALFLKSITQKEIENLEDFFANNKISGNQTFKGFFERLSELKKRYQNRFFHILEHEPTKELEGILKNYKKVMEKIVEHNSNFSFKAPFDDSTISTNFNYLTQLGDIIFDEKSRGFAKTCKFHTLENLIRSSAKSAIASRLASNSARLINGKIEMYLDRLAHEIIKKIDFTDIYNVQINVEMNKFNFESNLSKLGLAKERQKDEESFICPYSGAKISQTNCEYDHILPRSKGLYNSLANLIPTSSTSNQIKSNTKYLLSNLDENYLKYIFAKTQTTDLNSFKAFIDENISKIDENDFTNFKNLSFFEQIAFRHALFLDTDDNSFKKALRLLKLDTIKTHSNGTQKRFINILIEKISKLTKSGIDLNFIDSKLVSSTRKDLAQNDTSIAKQEIQDSHSHCVDASIVFYLANSKIIKGQIEPDYDYFKDIYPKDSDIILPQSKQYLELNQKSQKSKKLFDDSVYSLVYEGKFDEKQKKILTQYELLKENGFVDTHKVFELIFKSFKDKDTIVLKDLKFLDNHLKSYIRKDIFSIFFNEKGELKEAKELKSATKNIDKFYTILSQNQDKIYTIKLDEKAKEKKTLQRNKVIELYKEIFYTKNAKPRARGKNRVTFSLPVYAKDAKYAIKRNSGFAGLKNKDIATKTYIDIDSREILKIPYYSTNVLPIRISDILEILSLQSKNAKQIYKIKIQDNLPKQIVSLDFILSQANRHEVLVSFDKSKLEIQNINDDNGENTFIQKYLCDDFKEFLGKPRDNKIEIIKNNDDILAIKYCVESTSKANKEIIVKALSDETPSAGSSGSETPGTSESATPESGPGKMDSRGEHRQDRRERPY

SEQ ID NO: 165 - protein, 1287 aa, synthetic construct
MTGKSLSINIDMGAINNGIFIATCQDDKIIDKNAFDIKFRKGKLNFSKIDRTLRRHTRRSFDRDRFVLRLLGEILPLENLSNNQKEKLFGLFKNRGFNYLNVNFNAEIDSDNLEILNALDRYYFKDCRVLSDFENSISKIFNELENNEILAFLDDQAQILNQAKEHKNKILNKNINAILEFLESIKNESFKNNKHRKSYLKDIKNEIENSFKDIILKLKIFKNSQELYYFIGNIANFQTRILRRYFNAKFDLVFDDAKLKKNILRNINYLDFISTDEKANKNKILENLNAFSTLEFLKNTDPIVTIPPYENAKNKKPQSCQALVINDEKITPSLKDIAHKILSNSNFECLKTDENGVLADNIKDNEIAKYLQRILDISKGILDDKELYPRLLEKDENAKIFAQEIRLNSVELKEFKDFAKKYYDEVNLAKKGIIKNELLKPCCLHTPHKNKNKNALISALFLKSITQKEIENLEDFFANNKISGNQTFKGFFERLSELKKRYQNRFFHILEHEPTKELEGILKNYKKVMEKIVEHNSNFSFKAPFDDSTISTNFNYLTQLGDIIFDEKSRGFAKTCKFHTLENLIRSSAKSAIASRLASNSARLINGKIEMYLDRLAHEIIKKIDFTDIYNVQINVEMNKFNFESNLSKLGLAKERQKDEESFICPYSGAKISQTNCEYDHILPRSKGLYNSLANLIPTSSTSNQIKSNTKYLLSNLDENYLKYIFAKTQTTDLNSFKAFIDENISKIDENDFTNFKNLSFFEQIAFRHALFLDTDDNSFKKALRLLKLDTIKTHSNGTQKRFINILIEKISKLTKSGIDLNFIDSKLVSSTRKDLAQNDTSIAKQEIQDSHSHCVDASIVFYLANSKIIKGQIEPDYDYFKDIYPKDSDIILPQSKQYLELNQKSQKSKKLFDDSVYSLVYEGKFDEKQKKILTQYELLKENGFVDTHKVFELIFKSFKDKDTIVLKDLKFLDNHLKSYIRKDIFSIFFNEKGELKEAKELKSATKNIDKFYTILSQNQDKIYTIKLDEKAKEKKTLQRNKVIELYKEIFYTKNAKPRARGKNRVTFSLPVYAKDAKYAIKRNSGFAGLKNKDIATKTYIDIDSREILKIPYYSTNVLPIRISDILEILSLQSKNAKQIYKIKIQDNLPKQIVSLDFILSQANRHEVLVSFDKSKLEIQNINDDNGENTFIQKYLCDDFKEFLGKPRDNKIEIIKNNDDILAIKYCVESTSKANKEIIVKALSDETPSAGSSGSETPGTSESATPESGPGKMDKGEHRQERRDRPY

SEQ ID NO: 166 - protein, 1283 aa, synthetic construct
MTGKSLSINIDMGAINNGIFIATCQDDKIIDKNAFDIKFRKGKLNFSKIDRTLRRHTRRSFDRDRFVLRLLGEILPLENLSNNQKEKLFGLFKNRGFNYLNVNFNAEIDSDNLEILNALDRYYFKDCRVLSDFENSISKIFNELENNEILAFLDDQAQILNQAKEHKNKILNKNINAILEFLESIKNESFKNNKHRKSYLKDIKNEIENSFKDIILKLKIFKNSQELYYFIGNIANFQTRILRRYFNAKFDLVFDDAKLKKNILRNINYLDFISTDEKANKNKILENLNAFSTLEFLKNTDPIVTIPPYENAKNKKPQSCQALVINDEKITPSLKDIAHKILSNSNFECLKTDENGVLADNIKDNEIAKYLQRILDISKGILDDKELYPRLLEKDENAKIFAQEIRLNSVELKEFKDFAKKYYDEVNLAKKGIIKNELLKPCCLHTPHKNKNKNALISALFLKSITQKEIENLEDFFANNKISGNQTFKGFFERLSELKKRYQNRFFHILEHEPTKELEGILKNYKKVMEKIVEHNSNFSFKAPFDDSTISTNFNYLTQLGDIIFDEKSRGFAKTCKFHTLENLIRSSAKSAIASRLASNSARLINGKIEMYLDRLAHEIIKKIDFTDIYNVQINVEMNKFNFESNLSKLGLAKERQKDEESFICPYSGAKISQTNCEYDHILPRSKGLYNSLANLIPTSSTSNQIKSNTKYLLSNLDENYLKYIFAKTQTTDLNSFKAFIDENISKIDENDFTNFKNLSFFEQIAFRHALFLDTDDNSFKKALRLLKLDTIKTHSNGTQKRFINILIEKISKLTKSGIDLNFIDSKLVSSTRKDLAQNDTSIAKQEIQDSHSHCVDASIVFYLANSKIIKGQIEPDYDYFKDIYPKDSDIILPQSKQYLELNQKSQKSKKLFDDSVYSLVYEGKFDEKQKKILTQYELLKENGFVDTHKVFELIFKSFKDKDTIVLKDLKFLDNHLKSYIRKDIFSIFFNEKGELKEAKELKSATKNIDKFYTILSQNQDKIYTIKLDEKAKEKKTLQRNKVIELYKEIFYTKNAKPRARGKNRVTFSLPVYAKDAKYAIKRNSGFAGLKNKDIATKTYIDIDSREILKIPYYSTNVLPIRISDILEILSLQSKNAKQIYKIKIQDNLPKQIVSLDFILSQANRHEVLVSFDKSKLEIQNINDDNGENTFIQKYLCDDFKEFLGKPRDNKIEIIKNNDDILAIKYCVESTSKANKEIIVKALSDETPSAGSSGSETPGTSESATPESKEKNIKRGGNRFEPY

SEQ ID NO: 167 - protein, 1284 aa, synthetic construct
MTGKSLSINIDMGAINNGIFIATCQDDKIIDKNAFDIKFRKGKLNFSKIDRTLRRHTRRSFDRDRFVLRLLGEILPLENLSNNQKEKLFGLFKNRGFNYLNVNFNAEIDSDNLEILNALDRYYFKDCRVLSDFENSISKIFNELENNEILAFLDDQAQILNQAKEHKNKILNKNINAILEFLESIKNESFKNNKHRKSYLKDIKNEIENSFKDIILKLKIFKNSQELYYFIGNIANFQTRILRRYFNAKFDLVFDDAKLKKNILRNINYLDFISTDEKANKNKILENLNAFSTLEFLKNTDPIVTIPPYENAKNKKPQSCQALVINDEKITPSLKDIAHKILSNSNFECLKTDENGVLADNIKDNEIAKYLQRILDISKGILDDKELYPRLLEKDENAKIFAQEIRLNSVELKEFKDFAKKYYDEVNLAKKGIIKNELLKPCCLHTPHKNKNKNALISALFLKSITQKEIENLEDFFANNKISGNQTFKGFFERLSELKKRYQNRFFHILEHEPTKELEGILKNYKKVMEKIVEHNSNFSFKAPFDDSTISTNFNYLTQLGDIIFDEKSRGFAKTCKFHTLENLIRSSAKSAIASRLASNSARLINGKIEMYLDRLAHEIIKKIDFTDIYNVQINVEMNKFNFESNLSKLGLAKERQKDEESFICPYSGAKISQTNCEYDHILPRSKGLYNSLANLIPTSSTSNQIKSNTKYLLSNLDENYLKYIFAKTQTTDLNSFKAFIDENISKIDENDFTNFKNLSFFEQIAFRHALFLDTDDNSFKKALRLLKLDTIKTHSNGTQKRFINILIEKISKLTKSGIDLNFIDSKLVSSTRKDLAQNDTSIAKQEIQDSHSHCVDASIVFYLANSKIIKGQIEPDYDYFKDIYPKDSDIILPQSKQYLELNQKSQKSKKLFDDSVYSLVYEGKFDEKQKKILTQYELLKENGFVDTHKVFELIFKSFKDKDTIVLKDLKFLDNHLKSYIRKDIFSIFFNEKGELKEAKELKSATKNIDKFYTILSQNQDKIYTIKLDEKAKEKKTLQRNKVIELYKEIFYTKNAKPRARGKNRVTFSLPVYAKDAKYAIKRNSGFAGLKNKDIATKTYIDIDSREILKIPYYSTNVLPIRISDILEILSLQSKNAKQIYKIKIQDNLPKQIVSLDFILSQANRHEVLVSFDKSKLEIQNINDDNGENTFIQKYLCDDFKEFLGKPRDNKIEIIKNNDDILAIKYCVESTSKANKEIIVKALSDETPSAGSSGSETPGTSESATPESKASRGGGNHQNNYQPY

SEQ ID NO: 168 - protein, 1275 aa, synthetic construct
MTGKSLSINIDMGAINNGIFIATCQDDKIIDKNAFDIKFRKGKLNFSKIDRTLRRHTRRSFDRDRFVLRLLGEILPLENLSNNQKEKLFGLFKNRGFNYLNVNFNAEIDSDNLEILNALDRYYFKDCRVLSDFENSISKIFNELENNEILAFLDDQAQILNQAKEHKNKILNKNINAILEFLESIKNESFKNNKHRKSYLKDIKNEIENSFKDIILKLKIFKNSQELYYFIGNIANFQTRILRRYFNAKFDLVFDDAKLKKNILRNINYLDFISTDEKANKNKILENLNAFSTLEFLKNTDPIVTIPPYENAKNKKPQSCQALVINDEKITPSLKDIAHKILSNSNFECLKTDENGVLADNIKDNEIAKYLQRILDISKGILDDKELYPRLLEKDENAKIFAQEIRLNSVELKEFKDFAKKYYDEVNLAKKGIIKNELLKPCCLHTPHKNKNKNALISALFLKSITQKEIENLEDFFANNKISGNQTFKGFFERLSELKKRYQNRFFHILEHEPTKELEGILKNYKKVMEKIVEHNSNFSFKAPFDDSTISTNFNYLTQLGDIIFDEKSRGFAKTCKFHTLENLIRSSAKSAIASRLASNSARLINGKIEMYLDRLAHEIIKKIDFTDIYNVQINVEMNKFNFESNLSKLGLAKERQKDEESFICPYSGAKISQTNCEYDHILPRSKGLYNSLANLIPTSSTSNQIKSNTKYLLSNLDENYLKYIFAKTQTTDLNSFKAFIDENISKIDENDFTNFKNLSFFEQIAFRHALFLDTDDNSFKKALRLLKLDTIKTHSNGTQKRFINILIEKISKLTKSGIDLNFIDSKLVSSTRKDLAQNDTSIAKQEIQDSHSHCVDASIVFYLANSKIIKGQIEPDYDYFKDIYPKDSDIILPQSKQYLELNQKSQKSKKLFDDSVYSLVYEGKFDEKQKKILTQYELLKENGFVDTHKVFELIFKSFKDKDTIVLKDLKFLDNHLKSYIRKDIFSIFFNEKGELKEAKELKSATKNIDKFYTILSQNQDKIYTIKLDEKAKEKKTLQRNKVIELYKEIFYTKNAKPRARGKNRVTFSLPVYAKDAKYAIKRNSGFAGLKNKDIATKTYIDIDSREILKIPYYSTNVLPIRISDILEILSLQSKNAKQIYKIKIQDNLPKQIVSLDFILSQANRHEVLVSFDKSKLEIQNINDDNGENTFIQKYLCDDFKEFLGKPRDNKIEIIKNNDDILAIKYCVESTSKANKEIIVKALSDETPSAGSSGSETPGTSESATPESPKKKRKV

SEQ ID NO: 169 - protein, 1280 aa, synthetic construct
MTGKSLSINIDMGAINNGIFIATCQDDKIIDKNAFDIKFRKGKLNFSKIDRTLRRHTRRSFDRDRFVLRLLGEILPLENLSNNQKEKLFGLFKNRGFNYLNVNFNAEIDSDNLEILNALDRYYFKDCRVLSDFENSISKIFNELENNEILAFLDDQAQILNQAKEHKNKILNKNINAILEFLESIKNESFKNNKHRKSYLKDIKNEIENSFKDIILKLKIFKNSQELYYFIGNIANFQTRILRRYFNAKFDLVFDDAKLKKNILRNINYLDFISTDEKANKNKILENLNAFSTLEFLKNTDPIVTIPPYENAKNKKPQSCQALVINDEKITPSLKDIAHKILSNSNFECLKTDENGVLADNIKDNEIAKYLQRILDISKGILDDKELYPRLLEKDENAKIFAQEIRLNSVELKEFKDFAKKYYDEVNLAKKGIIKNELLKPCCLHTPHKNKNKNALISALFLKSITQKEIENLEDFFANNKISGNQTFKGFFERLSELKKRYQNRFFHILEHEPTKELEGILKNYKKVMEKIVEHNSNFSFKAPFDDSTISTNFNYLTQLGDIIFDEKSRGFAKTCKFHTLENLIRSSAKSAIASRLASNSARLINGKIEMYLDRLAHEIIKKIDFTDIYNVQINVEMNKFNFESNLSKLGLAKERQKDEESFICPYSGAKISQTNCEYDHILPRSKGLYNSLANLIPTSSTSNQIKSNTKYLLSNLDENYLKYIFAKTQTTDLNSFKAFIDENISKIDENDFTNFKNLSFFEQIAFRHALFLDTDDNSFKKALRLLKLDTIKTHSNGTQKRFINILIEKISKLTKSGIDLNFIDSKLVSSTRKDLAQNDTSIAKQEIQDSHSHCVDASIVFYLANSKIIKGQIEPDYDYFKDIYPKDSDIILPQSKQYLELNQKSQKSKKLFDDSVYSLVYEGKFDEKQKKILTQYELLKENGFVDTHKVFELIFKSFKDKDTIVLKDLKFLDNHLKSYIRKDIFSIFFNEKGELKEAKELKSATKNIDKFYTILSQNQDKIYTIKLDEKAKEKKTLQRNKVIELYKEIFYTKNAKPRARGKNRVTFSLPVYAKDAKYAIKRNSGFAGLKNKDIATKTYIDIDSREILKIPYYSTNVLPIRISDILEILSLQSKNAKQIYKIKIQDNLPKQIVSLDFILSQANRHEVLVSFDKSKLEIQNINDDNGENTFIQKYLCDDFKEFLGKPRDNKIEIIKNNDDILAIKYCVESTSKANKEIIVKALSDETPSAGSSGSETPGTSESATPESGRKKRRQRRRAP

SEQ ID NO: 170 - protein, 1286 aa, synthetic construct
MTGKSLSINIDMGAINNGIFIATCQDDKIIDKNAFDIKFRKGKLNFSKIDRTLRRHTRRSFDRDRFVLRLLGEILPLENLSNNQKEKLFGLFKNRGFNYLNVNFNAEIDSDNLEILNALDRYYFKDCRVLSDFENSISKIFNELENNEILAFLDDQAQILNQAKEHKNKILNKNINAILEFLESIKNESFKNNKHRKSYLKDIKNEIENSFKDIILKLKIFKNSQELYYFIGNIANFQTRILRRYFNAKFDLVFDDAKLKKNILRNINYLDFISTDEKANKNKILENLNAFSTLEFLKNTDPIVTIPPYENAKNKKPQSCQALVINDEKITPSLKDIAHKILSNSNFECLKTDENGVLADNIKDNEIAKYLQRILDISKGILDDKELYPRLLEKDENAKIFAQEIRLNSVELKEFKDFAKKYYDEVNLAKKGIIKNELLKPCCLHTPHKNKNKNALISALFLKSITQKEIENLEDFFANNKISGNQTFKGFFERLSELKKRYQNRFFHILEHEPTKELEGILKNYKKVMEKIVEHNSNFSFKAPFDDSTISTNFNYLTQLGDIIFDEKSRGFAKTCKFHTLENLIRSSAKSAIASRLASNSARLINGKIEMYLDRLAHEIIKKIDFTDIYNVQINVEMNKFNFESNLSKLGLAKERQKDEESFICPYSGAKISQTNCEYDHILPRSKGLYNSLANLIPTSSTSNQIKSNTKYLLSNLDENYLKYIFAKTQTTDLNSFKAFIDENISKIDENDFTNFKNLSFFEQIAFRHALFLDTDDNSFKKALRLLKLDTIKTHSNGTQKRFINILIEKISKLTKSGIDLNFIDSKLVSSTRKDLAQNDTSIAKQEIQDSHSHCVDASIVFYLANSKIIKGQIEPDYDYFKDIYPKDSDIILPQSKQYLELNQKSQKSKKLFDDSVYSLVYEGKFDEKQKKILTQYELLKENGFVDTHKVFELIFKSFKDKDTIVLKDLKFLDNHLKSYIRKDIFSIFFNEKGELKEAKELKSATKNIDKFYTILSQNQDKIYTIKLDEKAKEKKTLQRNKVIELYKEIFYTKNAKPRARGKNRVTFSLPVYAKDAKYAIKRNSGFAGLKNKDIATKTYIDIDSREILKIPYYSTNVLPIRISDILEILSLQSKNAKQIYKIKIQDNLPKQIVSLDFILSQANRHEVLVSFDKSKLEIQNINDDNGENTFIQKYLCDDFKEFLGKPRDNKIEIIKNNDDILAIKYCVESTSKANKEIIVKALSDETPSAGSSGSETPGTSESATPESTRQARRNRRRRWRERQRQ

SEQ ID NO: 171 - protein, 1289 aa, synthetic construct
MTGKSLSINIDMGAINNGIFIATCQDDKIIDKNAFDIKFRKGKLNFSKIDRTLRRHTRRSFDRDRFVLRLLGEILPLENLSNNQKEKLFGLFKNRGFNYLNVNFNAEIDSDNLEILNALDRYYFKDCRVLSDFENSISKIFNELENNEILAFLDDQAQILNQAKEHKNKILNKNINAILEFLESIKNESFKNNKHRKSYLKDIKNEIENSFKDIILKLKIFKNSQELYYFIGNIANFQTRILRRYFNAKFDLVFDDAKLKKNILRNINYLDFISTDEKANKNKILENLNAFSTLEFLKNTDPIVTIPPYENAKNKKPQSCQALVINDEKITPSLKDIAHKILSNSNFECLKTDENGVLADNIKDNEIAKYLQRILDISKGILDDKELYPRLLEKDENAKIFAQEIRLNSVELKEFKDFAKKYYDEVNLAKKGIIKNELLKPCCLHTPHKNKNKNALISALFLKSITQKEIENLEDFFANNKISGNQTFKGFFERLSELKKRYQNRFFHILEHEPTKELEGILKNYKKVMEKIVEHNSNFSFKAPFDDSTISTNFNYLTQLGDIIFDEKSRGFAKTCKFHTLENLIRSSAKSAIASRLASNSARLINGKIEMYLDRLAHEIIKKIDFTDIYNVQINVEMNKFNFESNLSKLGLAKERQKDEESFICPYSGAKISQTNCEYDHILPRSKGLYNSLANLIPTSSTSNQIKSNTKYLLSNLDENYLKYIFAKTQTTDLNSFKAFIDENISKIDENDFTNFKNLSFFEQIAFRHALFLDTDDNSFKKALRLLKLDTIKTHSNGTQKRFINILIEKISKLTKSGIDLNFIDSKLVSSTRKDLAQNDTSIAKQEIQDSHSHCVDASIVFYLANSKIIKGQIEPDYDYFKDIYPKDSDIILPQSKQYLELNQKSQKSKKLFDDSVYSLVYEGKFDEKQKKILTQYELLKENGFVDTHKVFELIFKSFKDKDTIVLKDLKFLDNHLKSYIRKDIFSIFFNEKGELKEAKELKSATKNIDKFYTILSQNQDKIYTIKLDEKAKEKKTLQRNKVIELYKEIFYTKNAKPRARGKNRVTFSLPVYAKDAKYAIKRNSGFAGLKNKDIATKTYIDIDSREILKIPYYSTNVLPIRISDILEILSLQSKNAKQIYKIKIQDNLPKQIVSLDFILSQANRHEVLVSFDKSKLEIQNINDDNGENTFIQKYLCDDFKEFLGKPRDNKIEIIKNNDDILAIKYCVESTSKANKEIIVKALSDETPSAGSSGSETPGTSESATPESGKKKKGKPGKRREQRKKKRRT

SEQ ID NO: 172 - protein, 1290 aa, synthetic construct
MKRTADGSEFESPKKKRKVTGKSLSINIDMGAINNGIFIATCQDDKIIDKNAFDIKFRKGKLNFSKIDRTLRRHTRRSFDRDRFVLRLLGEILPLENLSNNQKEKLFGLFKNRGFNYLNVNFNAEIDSDNLEILNALDRYYFKDCRVLSDFENSISKIFNELENNEILAFLDDQAQILNQAKEHKNKILNKNINAILEFLESIKNESFKNNKHRKSYLKDIKNEIENSFKDIILKLKIFKNSQELYYFIGNIANFQTRILRRYFNAKFDLVFDDAKLKKNILRNINYLDFISTDEKANKNKILENLNAFSTLEFLKNTDPIVTIPPYENAKNKKPQSCQALVINDEKITPSLKDIAHKILSNSNFECLKTDENGVLADNIKDNEIAKYLQRILDISKGILDDKELYPRLLEKDENAKIFAQEIRLNSVELKEFKDFAKKYYDEVNLAKKGIIKNELLKPCCLHTPHKNKNKNALISALFLKSITQKEIENLEDFFANNKISGNQTFKGFFERLSELKKRYQNRFFHILEHEPTKELEGILKNYKKVMEKIVEHNSNFSFKAPFDDSTISTNFNYLTQLGDIIFDEKSRGFAKTCKFHTLENLIRSSAKSAIASRLASNSARLINGKIEMYLDRLAHEIIKKIDFTDIYNVQINVEMNKFNFESNLSKLGLAKERQKDEESFICPYSGAKISQTNCEYDHILPRSKGLYNSLANLIPTSSTSNQIKSNTKYLLSNLDENYLKYIFAKTQTTDLNSFKAFIDENISKIDENDFTNFKNLSFFEQIAFRHALFLDTDDNSFKKALRLLKLDTIKTHSNGTQKRFINILIEKISKLTKSGIDLNFIDSKLVSSTRKDLAQNDTSIAKQEIQDSHSHCVDASIVFYLANSKIIKGQIEPDYDYFKDIYPKDSDIILPQSKQYLELNQKSQKSKKLFDDSVYSLVYEGKFDEKQKKILTQYELLKENGFVDTHKVFELIFKSFKDKDTIVLKDLKFLDNHLKSYIRKDIFSIFFNEKGELKEAKELKSATKNIDKFYTILSQNQDKIYTIKLDEKAKEKKTLQRNKVIELYKEIFYTKNAKPRARGKNRVTFSLPVYAKDAKYAIKRNSGFAGLKNKDIATKTYIDIDSREILKIPYYSTNVLPIRISDILEILSLQSKNAKQIYKIKIQDNLPKQIVSLDFILSQANRHEVLVSFDKSKLEIQNINDDNGENTFIQKYLCDDFKEFLGKPRDNKIEIIKNNDDILAIKYCVESTSKANKEIIVKALSDETPSAGTAVKRPAATKKAGQAKKKKLD

SEQ ID NO: 173 - protein, 1277 aa, synthetic construct
MTGKSLSINIDMGAINNGIFIATCQDDKIIDKNAFDIKFRKGKLNFSKIDRTLRRHTRRSFDRDRFVLRLLGEILPLENLSNNQKEKLFGLFKNRGFNYLNVNFNAEIDSDNLEILNALDRYYFKDCRVLSDFENSISKIFNELENNEILAFLDDQAQILNQAKEHKNKILNKNINAILEFLESIKNESFKNNKHRKSYLKDIKNEIENSFKDIILKLKIFKNSQELYYFIGNIANFQTRILRRYFNAKFDLVFDDAKLKKNILRNINYLDFISTDEKANKNKILENLNAFSTLEFLKNTDPIVTIPPYENAKNKKPQSCQALVINDEKITPSLKDIAHKILSNSNFECLKTDENGVLADNIKDNEIAKYLQRILDISKGILDDKELYPRLLEKDENAKIFAQEIRLNSVELKEFKDFAKKYYDEVNLAKKGIIKNELLKPCCLHTPHKNKNKNALISALFLKSITQKEIENLEDFFANNKISGNQTFKGFFERLSELKKRYQNRFFHILEHEPTKELEGILKNYKKVMEKIVEHNSNFSFKAPFDDSTISTNFNYLTQLGDIIFDEKSRGFAKTCKFHTLENLIRSSAKSAIASRLASNSARLINGKIEMYLDRLAHEIIKKIDFTDIYNVQINVEMNKFNFESNLSKLGLAKERQKDEESFICPYSGAKISQTNCEYDHILPRSKGLYNSLANLIPTSSTSNQIKSNTKYLLSNLDENYLKYIFAKTQTTDLNSFKAFIDENISKIDENDFTNFKNLSFFEQIAFRHALFLDTDDNSFKKALRLLKLDTIKTHSNGTQKRFINILIEKISKLTKSGIDLNFIDSKLVSSTRKDLAQNDTSIAKQEIQDSHSHCVDASIVFYLANSKIIKGQIEPDYDYFKDIYPKDSDIILPQSKQYLELNQKSQKSKKLFDDSVYSLVYEGKFDEKQKKILTQYELLKENGFVDTHKVFELIFKSFKDKDTIVLKDLKFLDNHLKSYIRKDIFSIFFNEKGELKEAKELKSATKNIDKFYTILSQNQDKIYTIKLDEKAKEKKTLQRNKVIELYKEIFYTKNAKPRARGKNRVTFSLPVYAKDAKYAIKRNSGFAGLKNKDIATKTYIDIDSREILKIPYYSTNVLPIRISDILEILSLQSKNAKQIYKIKIQDNLPKQIVSLDFILSQANRHEVLVSFDKSKLEIQNINDDNGENTFIQKYLCDDFKEFLGKPRDNKIEIIKNNDDILAIKYCVESTSKANKEIIVKALSDETPSAGSGGSSGGSKRTADGSEFESPKKKRKV

SEQ ID NO: 174 - protein, 1286 aa, synthetic construct
MTGKSLSINIDMGAINNGIFIATCQDDKIIDKNAFDIKFRKGKLNFSKIDRTLRRHTRRSFDRDRFVLRLLGEILPLENLSNNQKEKLFGLFKNRGFNYLNVNFNAEIDSDNLEILNALDRYYFKDCRVLSDFENSISKIFNELENNEILAFLDDQAQILNQAKEHKNKILNKNINAILEFLESIKNESFKNNKHRKSYLKDIKNEIENSFKDIILKLKIFKNSQELYYFIGNIANFQTRILRRYFNAKFDLVFDDAKLKKNILRNINYLDFISTDEKANKNKILENLNAFSTLEFLKNTDPIVTIPPYENAKNKKPQSCQALVINDEKITPSLKDIAHKILSNSNFECLKTDENGVLADNIKDNEIAKYLQRILDISKGILDDKELYPRLLEKDENAKIFAQEIRLNSVELKEFKDFAKKYYDEVNLAKKGIIKNELLKPCCLHTPHKNKNKNALISALFLKSITQKEIENLEDFFANNKISGNQTFKGFFERLSELKKRYQNRFFHILEHEPTKELEGILKNYKKVMEKIVEHNSNFSFKAPFDDSTISTNFNYLTQLGDIIFDEKSRGFAKTCKFHTLENLIRSSAKSAIASRLASNSARLINGKIEMYLDRLAHEIIKKIDFTDIYNVQINVEMNKFNFESNLSKLGLAKERQKDEESFICPYSGAKISQTNCEYDHILPRSKGLYNSLANLIPTSSTSNQIKSNTKYLLSNLDENYLKYIFAKTQTTDLNSFKAFIDENISKIDENDFTNFKNLSFFEQIAFRHALFLDTDDNSFKKALRLLKLDTIKTHSNGTQKRFINILIEKISKLTKSGIDLNFIDSKLVSSTRKDLAQNDTSIAKQEIQDSHSHCVDASIVFYLANSKIIKGQIEPDYDYFKDIYPKDSDIILPQSKQYLELNQKSQKSKKLFDDSVYSLVYEGKFDEKQKKILTQYELLKENGFVDTHKVFELIFKSFKDKDTIVLKDLKFLDNHLKSYIRKDIFSIFFNEKGELKEAKELKSATKNIDKFYTILSQNQDKIYTIKLDEKAKEKKTLQRNKVIELYKEIFYTKNAKPRARGKNRVTFSLPVYAKDAKYAIKRNSGFAGLKNKDIATKTYIDIDSREILKIPYYSTNVLPIRISDILEILSLQSKNAKQIYKIKIQDNLPKQIVSLDFILSQANRHEVLVSFDKSKLEIQNINDDNGENTFIQKYLCDDFKEFLGKPRDNKIEIIKNNDDILAIKYCVESTSKANKEIIVKALSDETPSAGSSGSETPGTSESATPESKRTADGSEFESPKKKRKV

SEQ ID NO: 175 - protein, 1288 aa, synthetic construct
MAVKRPAATKKAGQAKKKKLDSSGSETPGTSESATPESGKSLSINIDMGAINNGIFIATCQDDKIIDKNAFDIKFRKGKLNFSKIDRTLRRHTRRSFDRDRFVLRLLGEILPLENLSNNQKEKLFGLFKNRGFNYLNVNFNAEIDSDNLEILNALDRYYFKDCRVLSDFENSISKIFNELENNEILAFLDDQAQILNQAKEHKNKILNKNINAILEFLESIKNESFKNNKHRKSYLKDIKNEIENSFKDIILKLKIFKNSQELYYFIGNIANFQTRILRRYFNAKFDLVFDDAKLKKNILRNINYLDFISTDEKANKNKILENLNAFSTLEFLKNTDPIVTIPPYENAKNKKPQSCQALVINDEKITPSLKDIAHKILSNSNFECLKTDENGVLADNIKDNEIAKYLQRILDISKGILDDKELYPRLLEKDENAKIFAQEIRLNSVELKEFKDFAKKYYDEVNLAKKGIIKNELLKPCCLHTPHKNKNKNALISALFLKSITQKEIENLEDFFANNKISGNQTFKGFFERLSELKKRYQNRFFHILEHEPTKELEGILKNYKKVMEKIVEHNSNFSFKAPFDDSTISTNFNYLTQLGDIIFDEKSRGFAKTCKFHTLENLIRSSAKSAIASRLASNSARLINGKIEMYLDRLAHEIIKKIDFTDIYNVQINVEMNKFNFESNLSKLGLAKERQKDEESFICPYSGAKISQTNCEYDHILPRSKGLYNSLANLIPTSSTSNQIKSNTKYLLSNLDENYLKYIFAKTQTTDLNSFKAFIDENISKIDENDFTNFKNLSFFEQIAFRHALFLDTDDNSFKKALRLLKLDTIKTHSNGTQKRFINILIEKISKLTKSGIDLNFIDSKLVSSTRKDLAQNDTSIAKQEIQDSHSHCVDASIVFYLANSKIIKGQIEPDYDYFKDIYPKDSDIILPQSKQYLELNQKSQKSKKLFDDSVYSLVYEGKFDEKQKKILTQYELLKENGFVDTHKVFELIFKSFKDKDTIVLKDLKFLDNHLKSYIRKDIFSIFFNEKGELKEAKELKSATKNIDKFYTILSQNQDKIYTIKLDEKAKEKKTLQRNKVIELYKEIFYTKNAKPRARGKNRVTFSLPVYAKDAKYAIKRNSGFAGLKNKDIATKTYIDIDSREILKIPYYSTNVLPIRISDILEILSLQSKNAKQIYKIKIQDNLPKQIVSLDFILSQANRHEVLVSFDKSKLEIQNINDDNGENTFIQKYLCDDFKEFLGKPRDNKIEIIKNNDDILAIKYCVESTSKANKEIIVKALSDETPSAGT

SEQ ID NO: 176 - protein, 1289 aa, synthetic construct
MGKRKLITSEEERSPAKRGRKSSSGSETPGTSESATPESGKSLSINIDMGAINNGIFIATCQDDKIIDKNAFDIKFRKGKLNFSKIDRTLRRHTRRSFDRDRFVLRLLGEILPLENLSNNQKEKLFGLFKNRGFNYLNVNFNAEIDSDNLEILNALDRYYFKDCRVLSDFENSISKIFNELENNEILAFLDDQAQILNQAKEHKNKILNKNINAILEFLESIKNESFKNNKHRKSYLKDIKNEIENSFKDIILKLKIFKNSQELYYFIGNIANFQTRILRRYFNAKFDLVFDDAKLKKNILRNINYLDFISTDEKANKNKILENLNAFSTLEFLKNTDPIVTIPPYENAKNKKPQSCQALVINDEKITPSLKDIAHKILSNSNFECLKTDENGVLADNIKDNEIAKYLQRILDISKGILDDKELYPRLLEKDENAKIFAQEIRLNSVELKEFKDFAKKYYDEVNLAKKGIIKNELLKPCCLHTPHKNKNKNALISALFLKSITQKEIENLEDFFANNKISGNQTFKGFFERLSELKKRYQNRFFHILEHEPTKELEGILKNYKKVMEKIVEHNSNFSFKAPFDDSTISTNFNYLTQLGDIIFDEKSRGFAKTCKFHTLENLIRSSAKSAIASRLASNSARLINGKIEMYLDRLAHEIIKKIDFTDIYNVQINVEMNKFNFESNLSKLGLAKERQKDEESFICPYSGAKISQTNCEYDHILPRSKGLYNSLANLIPTSSTSNQIKSNTKYLLSNLDENYLKYIFAKTQTTDLNSFKAFIDENISKIDENDFTNFKNLSFFEQIAFRHALFLDTDDNSFKKALRLLKLDTIKTHSNGTQKRFINILIEKISKLTKSGIDLNFIDSKLVSSTRKDLAQNDTSIAKQEIQDSHSHCVDASIVFYLANSKIIKGQIEPDYDYFKDIYPKDSDIILPQSKQYLELNQKSQKSKKLFDDSVYSLVYEGKFDEKQKKILTQYELLKENGFVDTHKVFELIFKSFKDKDTIVLKDLKFLDNHLKSYIRKDIFSIFFNEKGELKEAKELKSATKNIDKFYTILSQNQDKIYTIKLDEKAKEKKTLQRNKVIELYKEIFYTKNAKPRARGKNRVTFSLPVYAKDAKYAIKRNSGFAGLKNKDIATKTYIDIDSREILKIPYYSTNVLPIRISDILEILSLQSKNAKQIYKIKIQDNLPKQIVSLDFILSQANRHEVLVSFDKSKLEIQNINDDNGENTFIQKYLCDDFKEFLGKPRDNKIEIIKNNDDILAIKYCVESTSKANKEIIVKALSDETPSAGT

SEQ ID NO: 177 - protein, 1287 aa, synthetic construct
MTGKSLSINIDMGAINNGIFIATCQDDKIIDKNAFDIKFRKGKLNFSKIDRTLRRHTRRSFDRDRFVLRLLGEILPLENLSNNQKEKLFGLFKNRGFNYLNVNFNAEIDSDNLEILNALDRYYFKDCRVLSDFENSISKIFNELENNEILAFLDDQAQILNQAKEHKNKILNKNINAILEFLESIKNESFKNNKHRKSYLKDIKNEIENSFKDIILKLKIFKNSQELYYFIGNIANFQTRILRRYFNAKFDLVFDDAKLKKNILRNINYLDFISTDEKANKNKILENLNAFSTLEFLKNTDPIVTIPPYENAKNKKPQSCQALVINDEKITPSLKDIAHKILSNSNFECLKTDENGVLADNIKDNEIAKYLQRILDISKGILDDKELYPRLLEKDENAKIFAQEIRLNSVELKEFKDFAKKYYDEVNLAKKGIIKNELLKPCCLHTPHKNKNKNALISALFLKSITQKEIENLEDFFANNKISGNQTFKGFFERLSELKKRYQNRFFHILEHEPTKELEGILKNYKKVMEKIVEHNSNFSFKAPFDDSTISTNFNYLTQLGDIIFDEKSRGFAKTCKFHTLENLIRSSAKSAIASRLASNSARLINGKIEMYLDRLAHEIIKKIDFTDIYNVQINVEMNKFNFESNLSKLGLAKERQKDEESFICPYSGAKISQTNCEYDHILPRSKGLYNSLANLIPTSSTSNQIKSNTKYLLSNLDENYLKYIFAKTQTTDLNSFKAFIDENISKIDENDFTNFKNLSFFEQIAFRHALFLDTDDNSFKKALRLLKLDTIKTHSNGTQKRFINILIEKISKLTKSGIDLNFIDSKLVSSTRKDLAQNDTSIAKQEIQDSHSHCVDASIVFYLANSKIIKGQIEPDYDYFKDIYPKDSDIILPQSKQYLELNQKSQKSKKLFDDSVYSLVYEGKFDEKQKKILTQYELLKENGFVDTHKVFELIFKSFKDKDTIVLKDLKFLDNHLKSYIRKDIFSIFFNEKGELKEAKELKSATKNIDKFYTILSQNQDKIYTIKLDEKAKEKKTLQRNKVIELYKEIFYTKNAKPRARGKNRVTFSLPVYAKDAKYAIKRNSGFAGLKNKDIATKTYIDIDSREILKIPYYSTNVLPIRISDILEILSLQSKNAKQIYKIKIQDNLPKQIVSLDFILSQANRHEVLVSFDKSKLEIQNINDDNGENTFIQKYLCDDFKEFLGKPRDNKIEIIKNNDDILAIKYCVESTSKANKEIIVKALSDETPSAGSSGSETPGTSESATPESMPKTRRRPRRSQRKRPPTP

SEQ ID NO: 178 - protein, 1270 aa, synthetic construct
MKRTADGSEFESPKKKRKVTGKSLSINIDMGAINNGIFIATCQDDKIIDKNAFDIKFRKGKLNFSKIDRTLRRHTRRSFDRDRFVLRLLGEILPLENLSNNQKEKLFGLFKNRGFNYLNVNFNAEIDSDNLEILNALDRYYFKDCRVLSDFENSISKIFNELENNEILAFLDDQAQILNQAKEHKNKILNKNINAILEFLESIKNESFKNNKHRKSYLKDIKNEIENSFKDIILKLKIFKNSQELYYFIGNIANFQTRILRRYFNAKFDLVFDDAKLKKNILRNINYLDFISTDEKANKNKILENLNAFSTLEFLKNTDPIVTIPPYENAKNKKPQSCQALVINDEKITPSLKDIAHKILSNSNFECLKTDENGVLADNIKDNEIAKYLQRILDISKGILDDKELYPRLLEKDENAKIFAQEIRLNSVELKEFKDFAKKYYDEVNLAKKGIIKNELLKPCCLHTPHKNKNKNALISALFLKSITQKEIENLEDFFANNKISGNQTFKGFFERLSELKKRYQNRFFHILEHEPTKELEGILKNYKKVMEKIVEHNSNFSFKAPFDDSTISTNFNYLTQLGDIIFDEKSRGFAKTCKFHTLENLIRSSAKSAIASRLASNSARLINGKIEMYLDRLAHEIIKKIDFTDIYNVQINVEMNKFNFESNLSKLGLAKERQKDEESFICPYSGAKISQTNCEYDHILPRSKGLYNSLANLIPTSSTSNQIKSNTKYLLSNLDENYLKYIFAKTQTTDLNSFKAFIDENISKIDENDFTNFKNLSFFEQIAFRHALFLDTDDNSFKKALRLLKLDTIKTHSNGTQKRFINILIEKISKLTKSGIDLNFIDSKLVSSTRKDLAQNDTSIAKQEIQDSHSHCVDASIVFYLANSKIIKGQIEPDYDYFKDIYPKDSDIILPQSKQYLELNQKSQKSKKLFDDSVYSLVYEGKFDEKQKKILTQYELLKENGFVDTHKVFELIFKSFKDKDTIVLKDLKFLDNHLKSYIRKDIFSIFFNEKGELKEAKELKSATKNIDKFYTILSQNQDKIYTIKLDEKAKEKKTLQRNKVIELYKEIFYTKNAKPRARGKNRVTFSLPVYAKDAKYAIKRNSGFAGLKNKDIATKTYIDIDSREILKIPYYSTNVLPIRISDILEILSLQSKNAKQIYKIKIQDNLPKQIVSLDFILSQANRHEVLVSFDKSKLEIQNINDDNGENTFIQKYLCDDFKEFLGKPRDNKIEIIKNNDDILAIKYCVESTSKANKEIIVKALSDETPSAGT

SEQ ID NO: 179 - protein, 1270 aa, synthetic construct
MTGKSLSINIDMGAINNGIFIATCQDDKIIDKNAFDIKFRKGKLNFSKIDRTLRRHTRRSFDRDRFVLRLLGEILPLENLSNNQKEKLFGLFKNRGFNYLNVNFNAEIDSDNLEILNALDRYYFKDCRVLSDFENSISKIFNELENNEILAFLDDQAQILNQAKEHKNKILNKNINAILEFLESIKNESFKNNKHRKSYLKDIKNEIENSFKDIILKLKIFKNSQELYYFIGNIANFQTRILRRYFNAKFDLVFDDAKLKKNILRNINYLDFISTDEKANKNKILENLNAFSTLEFLKNTDPIVTIPPYENAKNKKPQSCQALVINDEKITPSLKDIAHKILSNSNFECLKTDENGVLADNIKDNEIAKYLQRILDISKGILDDKELYPRLLEKDENAKIFAQEIRLNSVELKEFKDFAKKYYDEVNLAKKGIIKNELLKPCCLHTPHKNKNKNALISALFLKSITQKEIENLEDFFANNKISGNQTFKGFFERLSELKKRYQNRFFHILEHEPTKELEGILKNYKKVMEKIVEHNSNFSFKAPFDDSTISTNFNYLTQLGDIIFDEKSRGFAKTCKFHTLENLIRSSAKSAIASRLASNSARLINGKIEMYLDRLAHEIIKKIDFTDIYNVQINVEMNKFNFESNLSKLGLAKERQKDEESFICPYSGAKISQTNCEYDHILPRSKGLYNSLANLIPTSSTSNQIKSNTKYLLSNLDENYLKYIFAKTQTTDLNSFKAFIDENISKIDENDFTNFKNLSFFEQIAFRHALFLDTDDNSFKKALRLLKLDTIKTHSNGTQKRFINILIEKISKLTKSGIDLNFIDSKLVSSTRKDLAQNDTSIAKQEIQDSHSHCVDASIVFYLANSKIIKGQIEPDYDYFKDIYPKDSDIILPQSKQYLELNQKSQKSKKLFDDSVYSLVYEGKFDEKQKKILTQYELLKENGFVDTHKVFELIFKSFKDKDTIVLKDLKFLDNHLKSYIRKDIFSIFFNEKGELKEAKELKSATKNIDKFYTILSQNQDKIYTIKLDEKAKEKKTLQRNKVIELYKEIFYTKNAKPRARGKNRVTFSLPVYAKDAKYAIKRNSGFAGLKNKDIATKTYIDIDSREILKIPYYSTNVLPIRISDILEILSLQSKNAKQIYKIKIQDNLPKQIVSLDFILSQANRHEVLVSFDKSKLEIQNINDDNGENTFIQKYLCDDFKEFLGKPRDNKIEIIKNNDDILAIKYCVESTSKANKEIIVKALSDETPSAGTKRTADGSEFESPKKKRKV

SEQ ID NO: 180 - protein, 1300 aa, synthetic construct
MTGKSLSINIDMGAINNGIFIATCQDDKIIDKNAFDIKFRKGKLNFSKIDRTLRRHTRRSFDRDRFVLRLLGEILPLENLSNNQKEKLFGLFKNRGFNYLNVNFNAEIDSDNLEILNALDRYYFKDCRVLSDFENSISKIFNELENNEILAFLDDQAQILNQAKEHKNKILNKNINAILEFLESIKNESFKNNKHRKSYLKDIKNEIENSFKDIILKLKIFKNSQELYYFIGNIANFQTRILRRYFNAKFDLVFDDAKLKKNILRNINYLDFISTDEKANKNKILENLNAFSTLEFLKNTDPIVTIPPYENAKNKKPQSCQALVINDEKITPSLKDIAHKILSNSNFECLKTDENGVLADNIKDNEIAKYLQRILDISKGILDDKELYPRLLEKDENAKIFAQEIRLNSVELKEFKDFAKKYYDEVNLAKKGIIKNELLKPCCLHTPHKNKNKNALISALFLKSITQKEIENLEDFFANNKISGNQTFKGFFERLSELKKRYQNRFFHILEHEPTKELEGILKNYKKVMEKIVEHNSNFSFKAPFDDSTISTNFNYLTQLGDIIFDEKSRGFAKTCKFHTLENLIRSSAKSAIASRLASNSARLINGKIEMYLDRLAHEIIKKIDFTDIYNVQINVEMNKFNFESNLSKLGLAKERQKDEESFICPYSGAKISQTNCEYDHILPRSKGLYNSLANLIPTSSTSNQIKSNTKYLLSNLDENYLKYIFAKTQTTDLNSFKAFIDENISKIDENDFTNFKNLSFFEQIAFRHALFLDTDDNSFKKALRLLKLDTIKTHSNGTQKRFINILIEKISKLTKSGIDLNFIDSKLVSSTRKDLAQNDTSIAKQEIQDSHSHCVDASIVFYLANSKIIKGQIEPDYDYFKDIYPKDSDIILPQSKQYLELNQKSQKSKKLFDDSVYSLVYEGKFDEKQKKILTQYELLKENGFVDTHKVFELIFKSFKDKDTIVLKDLKFLDNHLKSYIRKDIFSIFFNEKGELKEAKELKSATKNIDKFYTILSQNQDKIYTIKLDEKAKEKKTLQRNKVIELYKEIFYTKNAKPRARGKNRVTFSLPVYAKDAKYAIKRNSGFAGLKNKDIATKTYIDIDSREILKIPYYSTNVLPIRISDILEILSLQSKNAKQIYKIKIQDNLPKQIVSLDFILSQANRHEVLVSFDKSKLEIQNINDDNGENTFIQKYLCDDFKEFLGKPRDNKIEIIKNNDDILAIKYCVESTSKANKEIIVKALSDETPSAGSGGSSGGSSGSETPGTSESATPESSGGSSGTKRTADGSEFESPKKKRKV

SEQ ID NO: 181 - protein, 1286 aa, synthetic construct
MKRLVPQKQASVAKKKKTGKSLSINIDMGAINNGIFIATCQDDKIIDKNAFDIKFRKGKLNFSKIDRTLRRHTRRSFDRDRFVLRLLGEILPLENLSNNQKEKLFGLFKNRGFNYLNVNFNAEIDSDNLEILNALDRYYFKDCRVLSDFENSISKIFNELENNEILAFLDDQAQILNQAKEHKNKILNKNINAILEFLESIKNESFKNNKHRKSYLKDIKNEIENSFKDIILKLKIFKNSQELYYFIGNIANFQTRILRRYFNAKFDLVFDDAKLKKNILRNINYLDFISTDEKANKNKILENLNAFSTLEFLKNTDPIVTIPPYENAKNKKPQSCQALVINDEKITPSLKDIAHKILSNSNFECLKTDENGVLADNIKDNEIAKYLQRILDISKGILDDKELYPRLLEKDENAKIFAQEIRLNSVELKEFKDFAKKYYDEVNLAKKGIIKNELLKPCCLHTPHKNKNKNALISALFLKSITQKEIENLEDFFANNKISGNQTFKGFFERLSELKKRYQNRFFHILEHEPTKELEGILKNYKKVMEKIVEHNSNFSFKAPFDDSTISTNFNYLTQLGDIIFDEKSRGFAKTCKFHTLENLIRSSAKSAIASRLASNSARLINGKIEMYLDRLAHEIIKKIDFTDIYNVQINVEMNKFNFESNLSKLGLAKERQKDEESFICPYSGAKISQTNCEYDHILPRSKGLYNSLANLIPTSSTSNQIKSNTKYLLSNLDENYLKYIFAKTQTTDLNSFKAFIDENISKIDENDFTNFKNLSFFEQIAFRHALFLDTDDNSFKKALRLLKLDTIKTHSNGTQKRFINILIEKISKLTKSGIDLNFIDSKLVSSTRKDLAQNDTSIAKQEIQDSHSHCVDASIVFYLANSKIIKGQIEPDYDYFKDIYPKDSDIILPQSKQYLELNQKSQKSKKLFDDSVYSLVYEGKFDEKQKKILTQYELLKENGFVDTHKVFELIFKSFKDKDTIVLKDLKFLDNHLKSYIRKDIFSIFFNEKGELKEAKELKSATKNIDKFYTILSQNQDKIYTIKLDEKAKEKKTLQRNKVIELYKEIFYTKNAKPRARGKNRVTFSLPVYAKDAKYAIKRNSGFAGLKNKDIATKTYIDIDSREILKIPYYSTNVLPIRISDILEILSLQSKNAKQIYKIKIQDNLPKQIVSLDFILSQANRHEVLVSFDKSKLEIQNINDDNGENTFIQKYLCDDFKEFLGKPRDNKIEIIKNNDDILAIKYCVESTSKANKEIIVKALSDETPSAGTKRTADGSEFESPKKKRKV

SEQ ID NO: 182 - protein, 1277 aa, synthetic construct
MKRTADGSEFESPKKKRKVSGGSSGGSGKSLSINIDMGAINNGIFIATCQDDKIIDKNAFDIKFRKGKLNFSKIDRTLRRHTRRSFDRDRFVLRLLGEILPLENLSNNQKEKLFGLFKNRGFNYLNVNFNAEIDSDNLEILNALDRYYFKDCRVLSDFENSISKIFNELENNEILAFLDDQAQILNQAKEHKNKILNKNINAILEFLESIKNESFKNNKHRKSYLKDIKNEIENSFKDIILKLKIFKNSQELYYFIGNIANFQTRILRRYFNAKFDLVFDDAKLKKNILRNINYLDFISTDEKANKNKILENLNAFSTLEFLKNTDPIVTIPPYENAKNKKPQSCQALVINDEKITPSLKDIAHKILSNSNFECLKTDENGVLADNIKDNEIAKYLQRILDISKGILDDKELYPRLLEKDENAKIFAQEIRLNSVELKEFKDFAKKYYDEVNLAKKGIIKNELLKPCCLHTPHKNKNKNALISALFLKSITQKEIENLEDFFANNKISGNQTFKGFFERLSELKKRYQNRFFHILEHEPTKELEGILKNYKKVMEKIVEHNSNFSFKAPFDDSTISTNFNYLTQLGDIIFDEKSRGFAKTCKFHTLENLIRSSAKSAIASRLASNSARLINGKIEMYLDRLAHEIIKKIDFTDIYNVQINVEMNKFNFESNLSKLGLAKERQKDEESFICPYSGAKISQTNCEYDHILPRSKGLYNSLANLIPTSSTSNQIKSNTKYLLSNLDENYLKYIFAKTQTTDLNSFKAFIDENISKIDENDFTNFKNLSFFEQIAFRHALFLDTDDNSFKKALRLLKLDTIKTHSNGTQKRFINILIEKISKLTKSGIDLNFIDSKLVSSTRKDLAQNDTSIAKQEIQDSHSHCVDASIVFYLANSKIIKGQIEPDYDYFKDIYPKDSDIILPQSKQYLELNQKSQKSKKLFDDSVYSLVYEGKFDEKQKKILTQYELLKENGFVDTHKVFELIFKSFKDKDTIVLKDLKFLDNHLKSYIRKDIFSIFFNEKGELKEAKELKSATKNIDKFYTILSQNQDKIYTIKLDEKAKEKKTLQRNKVIELYKEIFYTKNAKPRARGKNRVTFSLPVYAKDAKYAIKRNSGFAGLKNKDIATKTYIDIDSREILKIPYYSTNVLPIRISDILEILSLQSKNAKQIYKIKIQDNLPKQIVSLDFILSQANRHEVLVSFDKSKLEIQNINDDNGENTFIQKYLCDDFKEFLGKPRDNKIEIIKNNDDILAIKYCVESTSKANKEIIVKALSDETPSAGT

SEQ ID NO: 183 - protein, 1300 aa, synthetic construct
MKRTADGSEFESPKKKRKVSGGSSGGSSGSETPGTSESATPESSGGSSGTGKSLSINIDMGAINNGIFIATCQDDKIIDKNAFDIKFRKGKLNFSKIDRTLRRHTRRSFDRDRFVLRLLGEILPLENLSNNQKEKLFGLFKNRGFNYLNVNFNAEIDSDNLEILNALDRYYFKDCRVLSDFENSISKIFNELENNEILAFLDDQAQILNQAKEHKNKILNKNINAILEFLESIKNESFKNNKHRKSYLKDIKNEIENSFKDIILKLKIFKNSQELYYFIGNIANFQTRILRRYFNAKFDLVFDDAKLKKNILRNINYLDFISTDEKANKNKILENLNAFSTLEFLKNTDPIVTIPPYENAKNKKPQSCQALVINDEKITPSLKDIAHKILSNSNFECLKTDENGVLADNIKDNEIAKYLQRILDISKGILDDKELYPRLLEKDENAKIFAQEIRLNSVELKEFKDFAKKYYDEVNLAKKGIIKNELLKPCCLHTPHKNKNKNALISALFLKSITQKEIENLEDFFANNKISGNQTFKGFFERLSELKKRYQNRFFHILEHEPTKELEGILKNYKKVMEKIVEHNSNFSFKAPFDDSTISTNFNYLTQLGDIIFDEKSRGFAKTCKFHTLENLIRSSAKSAIASRLASNSARLINGKIEMYLDRLAHEIIKKIDFTDIYNVQINVEMNKFNFESNLSKLGLAKERQKDEESFICPYSGAKISQTNCEYDHILPRSKGLYNSLANLIPTSSTSNQIKSNTKYLLSNLDENYLKYIFAKTQTTDLNSFKAFIDENISKIDENDFTNFKNLSFFEQIAFRHALFLDTDDNSFKKALRLLKLDTIKTHSNGTQKRFINILIEKISKLTKSGIDLNFIDSKLVSSTRKDLAQNDTSIAKQEIQDSHSHCVDASIVFYLANSKIIKGQIEPDYDYFKDIYPKDSDIILPQSKQYLELNQKSQKSKKLFDDSVYSLVYEGKFDEKQKKILTQYELLKENGFVDTHKVFELIFKSFKDKDTIVLKDLKFLDNHLKSYIRKDIFSIFFNEKGELKEAKELKSATKNIDKFYTILSQNQDKIYTIKLDEKAKEKKTLQRNKVIELYKEIFYTKNAKPRARGKNRVTFSLPVYAKDAKYAIKRNSGFAGLKNKDIATKTYIDIDSREILKIPYYSTNVLPIRISDILEILSLQSKNAKQIYKIKIQDNLPKQIVSLDFILSQANRHEVLVSFDKSKLEIQNINDDNGENTFIQKYLCDDFKEFLGKPRDNKIEIIKNNDDILAIKYCVESTSKANKEIIVKALSDETPSAGT

SEQ ID NO: 184 - protein, 1291 aa, synthetic construct
MKRTADGSEFESPKKKRKVTGKSLSINIDMGAINNGIFIATCQDDKIIDKNAFDIKFRKGKLNFSKIDRTLRRHTRRSFDRDRFVLRLLGEILPLENLSNNQKEKLFGLFKNRGFNYLNVNFNAEIDSDNLEILNALDRYYFKDCRVLSDFENSISKIFNELENNEILAFLDDQAQILNQAKEHKNKILNKNINAILEFLESIKNESFKNNKHRKSYLKDIKNEIENSFKDIILKLKIFKNSQELYYFIGNIANFQTRILRRYFNAKFDLVFDDAKLKKNILRNINYLDFISTDEKANKNKILENLNAFSTLEFLKNTDPIVTIPPYENAKNKKPQSCQALVINDEKITPSLKDIAHKILSNSNFECLKTDENGVLADNIKDNEIAKYLQRILDISKGILDDKELYPRLLEKDENAKIFAQEIRLNSVELKEFKDFAKKYYDEVNLAKKGIIKNELLKPCCLHTPHKNKNKNALISALFLKSITQKEIENLEDFFANNKISGNQTFKGFFERLSELKKRYQNRFFHILEHEPTKELEGILKNYKKVMEKIVEHNSNFSFKAPFDDSTISTNFNYLTQLGDIIFDEKSRGFAKTCKFHTLENLIRSSAKSAIASRLASNSARLINGKIEMYLDRLAHEIIKKIDFTDIYNVQINVEMNKFNFESNLSKLGLAKERQKDEESFICPYSGAKISQTNCEYDHILPRSKGLYNSLANLIPTSSTSNQIKSNTKYLLSNLDENYLKYIFAKTQTTDLNSFKAFIDENISKIDENDFTNFKNLSFFEQIAFRHALFLDTDDNSFKKALRLLKLDTIKTHSNGTQKRFINILIEKISKLTKSGIDLNFIDSKLVSSTRKDLAQNDTSIAKQEIQDSHSHCVDASIVFYLANSKIIKGQIEPDYDYFKDIYPKDSDIILPQSKQYLELNQKSQKSKKLFDDSVYSLVYEGKFDEKQKKILTQYELLKENGFVDTHKVFELIFKSFKDKDTIVLKDLKFLDNHLKSYIRKDIFSIFFNEKGELKEAKELKSATKNIDKFYTILSQNQDKIYTIKLDEKAKEKKTLQRNKVIELYKEIFYTKNAKPRARGKNRVTFSLPVYAKDAKYAIKRNSGFAGLKNKDIATKTYIDIDSREILKIPYYSTNVLPIRISDILEILSLQSKNAKQIYKIKIQDNLPKQIVSLDFILSQANRHEVLVSFDKSKLEIQNINDDNGENTFIQKYLCDDFKEFLGKPRDNKIEIIKNNDDILAIKYCVESTSKANKEIIVKALSDETPSAGTGKRKLITSEEERSPAKRGRKS

SEQ ID NO: 185 - protein, 1286 aa, synthetic construct
MKRTADGSEFESPKKKRKVSSGSETPGTSESATPESGKSLSINIDMGAINNGIFIATCQDDKIIDKNAFDIKFRKGKLNFSKIDRTLRRHTRRSFDRDRFVLRLLGEILPLENLSNNQKEKLFGLFKNRGFNYLNVNFNAEIDSDNLEILNALDRYYFKDCRVLSDFENSISKIFNELENNEILAFLDDQAQILNQAKEHKNKILNKNINAILEFLESIKNESFKNNKHRKSYLKDIKNEIENSFKDIILKLKIFKNSQELYYFIGNIANFQTRILRRYFNAKFDLVFDDAKLKKNILRNINYLDFISTDEKANKNKILENLNAFSTLEFLKNTDPIVTIPPYENAKNKKPQSCQALVINDEKITPSLKDIAHKILSNSNFECLKTDENGVLADNIKDNEIAKYLQRILDISKGILDDKELYPRLLEKDENAKIFAQEIRLNSVELKEFKDFAKKYYDEVNLAKKGIIKNELLKPCCLHTPHKNKNKNALISALFLKSITQKEIENLEDFFANNKISGNQTFKGFFERLSELKKRYQNRFFHILEHEPTKELEGILKNYKKVMEKIVEHNSNFSFKAPFDDSTISTNFNYLTQLGDIIFDEKSRGFAKTCKFHTLENLIRSSAKSAIASRLASNSARLINGKIEMYLDRLAHEIIKKIDFTDIYNVQINVEMNKFNFESNLSKLGLAKERQKDEESFICPYSGAKISQTNCEYDHILPRSKGLYNSLANLIPTSSTSNQIKSNTKYLLSNLDENYLKYIFAKTQTTDLNSFKAFIDENISKIDENDFTNFKNLSFFEQIAFRHALFLDTDDNSFKKALRLLKLDTIKTHSNGTQKRFINILIEKISKLTKSGIDLNFIDSKLVSSTRKDLAQNDTSIAKQEIQDSHSHCVDASIVFYLANSKIIKGQIEPDYDYFKDIYPKDSDIILPQSKQYLELNQKSQKSKKLFDDSVYSLVYEGKFDEKQKKILTQYELLKENGFVDTHKVFELIFKSFKDKDTIVLKDLKFLDNHLKSYIRKDIFSIFFNEKGELKEAKELKSATKNIDKFYTILSQNQDKIYTIKLDEKAKEKKTLQRNKVIELYKEIFYTKNAKPRARGKNRVTFSLPVYAKDAKYAIKRNSGFAGLKNKDIATKTYIDIDSREILKIPYYSTNVLPIRISDILEILSLQSKNAKQIYKIKIQDNLPKQIVSLDFILSQANRHEVLVSFDKSKLEIQNINDDNGENTFIQKYLCDDFKEFLGKPRDNKIEIIKNNDDILAIKYCVESTSKANKEIIVKALSDETPSAGT

SEQ ID NO: 186 - protein, 1277 aa, synthetic construct
MTGKSLSINIDMGAINNGIFIATCQDDKIIDKNAFDIKFRKGKLNFSKIDRTLRRHTRRSFDRDRFVLRLLGEILPLENLSNNQKEKLFGLFKNRGFNYLNVNFNAEIDSDNLEILNALDRYYFKDCRVLSDFENSISKIFNELENNEILAFLDDQAQILNQAKEHKNKILNKNINAILEFLESIKNESFKNNKHRKSYLKDIKNEIENSFKDIILKLKIFKNSQELYYFIGNIANFQTRILRRYFNAKFDLVFDDAKLKKNILRNINYLDFISTDEKANKNKILENLNAFSTLEFLKNTDPIVTIPPYENAKNKKPQSCQALVINDEKITPSLKDIAHKILSNSNFECLKTDENGVLADNIKDNEIAKYLQRILDISKGILDDKELYPRLLEKDENAKIFAQEIRLNSVELKEFKDFAKKYYDEVNLAKKGIIKNELLKPCCLHTPHKNKNKNALISALFLKSITQKEIENLEDFFANNKISGNQTFKGFFERLSELKKRYQNRFFHILEHEPTKELEGILKNYKKVMEKIVEHNSNFSFKAPFDDSTISTNFNYLTQLGDIIFDEKSRGFAKTCKFHTLENLIRSSAKSAIASRLASNSARLINGKIEMYLDRLAHEIIKKIDFTDIYNVQINVEMNKFNFESNLSKLGLAKERQKDEESFICPYSGAKISQTNCEYDHILPRSKGLYNSLANLIPTSSTSNQIKSNTKYLLSNLDENYLKYIFAKTQTTDLNSFKAFIDENISKIDENDFTNFKNLSFFEQIAFRHALFLDTDDNSFKKALRLLKLDTIKTHSNGTQKRFINILIEKISKLTKSGIDLNFIDSKLVSSTRKDLAQNDTSIAKQEIQDSHSHCVDASIVFYLANSKIIKGQIEPDYDYFKDIYPKDSDIILPQSKQYLELNQKSQKSKKLFDDSVYSLVYEGKFDEKQKKILTQYELLKENGFVDTHKVFELIFKSFKDKDTIVLKDLKFLDNHLKSYIRKDIFSIFFNEKGELKEAKELKSATKNIDKFYTILSQNQDKIYTIKLDEKAKEKKTLQRNKVIELYKEIFYTKNAKPRARGKNRVTFSLPVYAKDAKYAIKRNSGFAGLKNKDIATKTYIDIDSREILKIPYYSTNVLPIRISDILEILSLQSKNAKQIYKIKIQDNLPKQIVSLDFILSQANRHEVLVSFDKSKLEIQNINDDNGENTFIQKYLCDDFKEFLGKPRDNKIEIIKNNDDILAIKYCVESTSKANKEIIVKALSDETPSAGSSGSETPGTSESATPESPAAKRVKLD

SEQ ID NO: 187 - protein, 1288 aa, synthetic construct
MTGKSLSINIDMGAINNGIFIATCQDDKIIDKNAFDIKFRKGKLNFSKIDRTLRRHTRRSFDRDRFVLRLLGEILPLENLSNNQKEKLFGLFKNRGFNYLNVNFNAEIDSDNLEILNALDRYYFKDCRVLSDFENSISKIFNELENNEILAFLDDQAQILNQAKEHKNKILNKNINAILEFLESIKNESFKNNKHRKSYLKDIKNEIENSFKDIILKLKIFKNSQELYYFIGNIANFQTRILRRYFNAKFDLVFDDAKLKKNILRNINYLDFISTDEKANKNKILENLNAFSTLEFLKNTDPIVTIPPYENAKNKKPQSCQALVINDEKITPSLKDIAHKILSNSNFECLKTDENGVLADNIKDNEIAKYLQRILDISKGILDDKELYPRLLEKDENAKIFAQEIRLNSVELKEFKDFAKKYYDEVNLAKKGIIKNELLKPCCLHTPHKNKNKNALISALFLKSITQKEIENLEDFFANNKISGNQTFKGFFERLSELKKRYQNRFFHILEHEPTKELEGILKNYKKVMEKIVEHNSNFSFKAPFDDSTISTNFNYLTQLGDIIFDEKSRGFAKTCKFHTLENLIRSSAKSAIASRLASNSARLINGKIEMYLDRLAHEIIKKIDFTDIYNVQINVEMNKFNFESNLSKLGLAKERQKDEESFICPYSGAKISQTNCEYDHILPRSKGLYNSLANLIPTSSTSNQIKSNTKYLLSNLDENYLKYIFAKTQTTDLNSFKAFIDENISKIDENDFTNFKNLSFFEQIAFRHALFLDTDDNSFKKALRLLKLDTIKTHSNGTQKRFINILIEKISKLTKSGIDLNFIDSKLVSSTRKDLAQNDTSIAKQEIQDSHSHCVDASIVFYLANSKIIKGQIEPDYDYFKDIYPKDSDIILPQSKQYLELNQKSQKSKKLFDDSVYSLVYEGKFDEKQKKILTQYELLKENGFVDTHKVFELIFKSFKDKDTIVLKDLKFLDNHLKSYIRKDIFSIFFNEKGELKEAKELKSATKNIDKFYTILSQNQDKIYTIKLDEKAKEKKTLQRNKVIELYKEIFYTKNAKPRARGKNRVTFSLPVYAKDAKYAIKRNSGFAGLKNKDIATKTYIDIDSREILKIPYYSTNVLPIRISDILEILSLQSKNAKQIYKIKIQDNLPKQIVSLDFILSQANRHEVLVSFDKSKLEIQNINDDNGENTFIQKYLCDDFKEFLGKPRDNKIEIIKNNDDILAIKYCVESTSKANKEIIVKALSDETPSAGSSGSETPGTSESATPESAVKRPAATKKAGQAKKKKLD

SEQ ID NO: 188 - protein, 1290 aa, synthetic construct
MAVKRPAATKKAGQAKKKKLDTGKSLSINIDMGAINNGIFIATCQDDKIIDKNAFDIKFRKGKLNFSKIDRTLRRHTRRSFDRDRFVLRLLGEILPLENLSNNQKEKLFGLFKNRGFNYLNVNFNAEIDSDNLEILNALDRYYFKDCRVLSDFENSISKIFNELENNEILAFLDDQAQILNQAKEHKNKILNKNINAILEFLESIKNESFKNNKHRKSYLKDIKNEIENSFKDIILKLKIFKNSQELYYFIGNIANFQTRILRRYFNAKFDLVFDDAKLKKNILRNINYLDFISTDEKANKNKILENLNAFSTLEFLKNTDPIVTIPPYENAKNKKPQSCQALVINDEKITPSLKDIAHKILSNSNFECLKTDENGVLADNIKDNEIAKYLQRILDISKGILDDKELYPRLLEKDENAKIFAQEIRLNSVELKEFKDFAKKYYDEVNLAKKGIIKNELLKPCCLHTPHKNKNKNALISALFLKSITQKEIENLEDFFANNKISGNQTFKGFFERLSELKKRYQNRFFHILEHEPTKELEGILKNYKKVMEKIVEHNSNFSFKAPFDDSTISTNFNYLTQLGDIIFDEKSRGFAKTCKFHTLENLIRSSAKSAIASRLASNSARLINGKIEMYLDRLAHEIIKKIDFTDIYNVQINVEMNKFNFESNLSKLGLAKERQKDEESFICPYSGAKISQTNCEYDHILPRSKGLYNSLANLIPTSSTSNQIKSNTKYLLSNLDENYLKYIFAKTQTTDLNSFKAFIDENISKIDENDFTNFKNLSFFEQIAFRHALFLDTDDNSFKKALRLLKLDTIKTHSNGTQKRFINILIEKISKLTKSGIDLNFIDSKLVSSTRKDLAQNDTSIAKQEIQDSHSHCVDASIVFYLANSKIIKGQIEPDYDYFKDIYPKDSDIILPQSKQYLELNQKSQKSKKLFDDSVYSLVYEGKFDEKQKKILTQYELLKENGFVDTHKVFELIFKSFKDKDTIVLKDLKFLDNHLKSYIRKDIFSIFFNEKGELKEAKELKSATKNIDKFYTILSQNQDKIYTIKLDEKAKEKKTLQRNKVIELYKEIFYTKNAKPRARGKNRVTFSLPVYAKDAKYAIKRNSGFAGLKNKDIATKTYIDIDSREILKIPYYSTNVLPIRISDILEILSLQSKNAKQIYKIKIQDNLPKQIVSLDFILSQANRHEVLVSFDKSKLEIQNINDDNGENTFIQKYLCDDFKEFLGKPRDNKIEIIKNNDDILAIKYCVESTSKANKEIIVKALSDETPSAGTKRTADGSEFESPKKKRKV

SEQ ID NO: 189 - protein, 1289 aa, synthetic construct
MTGKSLSINIDMGAINNGIFIATCQDDKIIDKNAFDIKFRKGKLNFSKIDRTLRRHTRRSFDRDRFVLRLLGEILPLENLSNNQKEKLFGLFKNRGFNYLNVNFNAEIDSDNLEILNALDRYYFKDCRVLSDFENSISKIFNELENNEILAFLDDQAQILNQAKEHKNKILNKNINAILEFLESIKNESFKNNKHRKSYLKDIKNEIENSFKDIILKLKIFKNSQELYYFIGNIANFQTRILRRYFNAKFDLVFDDAKLKKNILRNINYLDFISTDEKANKNKILENLNAFSTLEFLKNTDPIVTIPPYENAKNKKPQSCQALVINDEKITPSLKDIAHKILSNSNFECLKTDENGVLADNIKDNEIAKYLQRILDISKGILDDKELYPRLLEKDENAKIFAQEIRLNSVELKEFKDFAKKYYDEVNLAKKGIIKNELLKPCCLHTPHKNKNKNALISALFLKSITQKEIENLEDFFANNKISGNQTFKGFFERLSELKKRYQNRFFHILEHEPTKELEGILKNYKKVMEKIVEHNSNFSFKAPFDDSTISTNFNYLTQLGDIIFDEKSRGFAKTCKFHTLENLIRSSAKSAIASRLASNSARLINGKIEMYLDRLAHEIIKKIDFTDIYNVQINVEMNKFNFESNLSKLGLAKERQKDEESFICPYSGAKISQTNCEYDHILPRSKGLYNSLANLIPTSSTSNQIKSNTKYLLSNLDENYLKYIFAKTQTTDLNSFKAFIDENISKIDENDFTNFKNLSFFEQIAFRHALFLDTDDNSFKKALRLLKLDTIKTHSNGTQKRFINILIEKISKLTKSGIDLNFIDSKLVSSTRKDLAQNDTSIAKQEIQDSHSHCVDASIVFYLANSKIIKGQIEPDYDYFKDIYPKDSDIILPQSKQYLELNQKSQKSKKLFDDSVYSLVYEGKFDEKQKKILTQYELLKENGFVDTHKVFELIFKSFKDKDTIVLKDLKFLDNHLKSYIRKDIFSIFFNEKGELKEAKELKSATKNIDKFYTILSQNQDKIYTIKLDEKAKEKKTLQRNKVIELYKEIFYTKNAKPRARGKNRVTFSLPVYAKDAKYAIKRNSGFAGLKNKDIATKTYIDIDSREILKIPYYSTNVLPIRISDILEILSLQSKNAKQIYKIKIQDNLPKQIVSLDFILSQANRHEVLVSFDKSKLEIQNINDDNGENTFIQKYLCDDFKEFLGKPRDNKIEIIKNNDDILAIKYCVESTSKANKEIIVKALSDETPSAGSSGSETPGTSESATPESGKRKLITSEEERSPAKRGRKS

SEQ ID NO: 190 - protein, 1279 aa, synthetic construct
MKRTADGSEFESPKKKRKVTGKSLSINIDMGAINNGIFIATCQDDKIIDKNAFDIKFRKGKLNFSKIDRTLRRHTRRSFDRDRFVLRLLGEILPLENLSNNQKEKLFGLFKNRGFNYLNVNFNAEIDSDNLEILNALDRYYFKDCRVLSDFENSISKIFNELENNEILAFLDDQAQILNQAKEHKNKILNKNINAILEFLESIKNESFKNNKHRKSYLKDIKNEIENSFKDIILKLKIFKNSQELYYFIGNIANFQTRILRRYFNAKFDLVFDDAKLKKNILRNINYLDFISTDEKANKNKILENLNAFSTLEFLKNTDPIVTIPPYENAKNKKPQSCQALVINDEKITPSLKDIAHKILSNSNFECLKTDENGVLADNIKDNEIAKYLQRILDISKGILDDKELYPRLLEKDENAKIFAQEIRLNSVELKEFKDFAKKYYDEVNLAKKGIIKNELLKPCCLHTPHKNKNKNALISALFLKSITQKEIENLEDFFANNKISGNQTFKGFFERLSELKKRYQNRFFHILEHEPTKELEGILKNYKKVMEKIVEHNSNFSFKAPFDDSTISTNFNYLTQLGDIIFDEKSRGFAKTCKFHTLENLIRSSAKSAIASRLASNSARLINGKIEMYLDRLAHEIIKKIDFTDIYNVQINVEMNKFNFESNLSKLGLAKERQKDEESFICPYSGAKISQTNCEYDHILPRSKGLYNSLANLIPTSSTSNQIKSNTKYLLSNLDENYLKYIFAKTQTTDLNSFKAFIDENISKIDENDFTNFKNLSFFEQIAFRHALFLDTDDNSFKKALRLLKLDTIKTHSNGTQKRFINILIEKISKLTKSGIDLNFIDSKLVSSTRKDLAQNDTSIAKQEIQDSHSHCVDASIVFYLANSKIIKGQIEPDYDYFKDIYPKDSDIILPQSKQYLELNQKSQKSKKLFDDSVYSLVYEGKFDEKQKKILTQYELLKENGFVDTHKVFELIFKSFKDKDTIVLKDLKFLDNHLKSYIRKDIFSIFFNEKGELKEAKELKSATKNIDKFYTILSQNQDKIYTIKLDEKAKEKKTLQRNKVIELYKEIFYTKNAKPRARGKNRVTFSLPVYAKDAKYAIKRNSGFAGLKNKDIATKTYIDIDSREILKIPYYSTNVLPIRISDILEILSLQSKNAKQIYKIKIQDNLPKQIVSLDFILSQANRHEVLVSFDKSKLEIQNINDDNGENTFIQKYLCDDFKEFLGKPRDNKIEIIKNNDDILAIKYCVESTSKANKEIIVKALSDETPSAGTPAAKRVKLD

SEQ ID NO: 191 - protein, 1277 aa, synthetic construct
MKRTADGSEFESPKKKRKVTGKSLSINIDMGAINNGIFIATCQDDKIIDKNAFDIKFRKGKLNFSKIDRTLRRHTRRSFDRDRFVLRLLGEILPLENLSNNQKEKLFGLFKNRGFNYLNVNFNAEIDSDNLEILNALDRYYFKDCRVLSDFENSISKIFNELENNEILAFLDDQAQILNQAKEHKNKILNKNINAILEFLESIKNESFKNNKHRKSYLKDIKNEIENSFKDIILKLKIFKNSQELYYFIGNIANFQTRILRRYFNAKFDLVFDDAKLKKNILRNINYLDFISTDEKANKNKILENLNAFSTLEFLKNTDPIVTIPPYENAKNKKPQSCQALVINDEKITPSLKDIAHKILSNSNFECLKTDENGVLADNIKDNEIAKYLQRILDISKGILDDKELYPRLLEKDENAKIFAQEIRLNSVELKEFKDFAKKYYDEVNLAKKGIIKNELLKPCCLHTPHKNKNKNALISALFLKSITQKEIENLEDFFANNKISGNQTFKGFFERLSELKKRYQNRFFHILEHEPTKELEGILKNYKKVMEKIVEHNSNFSFKAPFDDSTISTNFNYLTQLGDIIFDEKSRGFAKTCKFHTLENLIRSSAKSAIASRLASNSARLINGKIEMYLDRLAHEIIKKIDFTDIYNVQINVEMNKFNFESNLSKLGLAKERQKDEESFICPYSGAKISQTNCEYDHILPRSKGLYNSLANLIPTSSTSNQIKSNTKYLLSNLDENYLKYIFAKTQTTDLNSFKAFIDENISKIDENDFTNFKNLSFFEQIAFRHALFLDTDDNSFKKALRLLKLDTIKTHSNGTQKRFINILIEKISKLTKSGIDLNFIDSKLVSSTRKDLAQNDTSIAKQEIQDSHSHCVDASIVFYLANSKIIKGQIEPDYDYFKDIYPKDSDIILPQSKQYLELNQKSQKSKKLFDDSVYSLVYEGKFDEKQKKILTQYELLKENGFVDTHKVFELIFKSFKDKDTIVLKDLKFLDNHLKSYIRKDIFSIFFNEKGELKEAKELKSATKNIDKFYTILSQNQDKIYTIKLDEKAKEKKTLQRNKVIELYKEIFYTKNAKPRARGKNRVTFSLPVYAKDAKYAIKRNSGFAGLKNKDIATKTYIDIDSREILKIPYYSTNVLPIRISDILEILSLQSKNAKQIYKIKIQDNLPKQIVSLDFILSQANRHEVLVSFDKSKLEIQNINDDNGENTFIQKYLCDDFKEFLGKPRDNKIEIIKNNDDILAIKYCVESTSKANKEIIVKALSDETPSAGTPKKKRKV

SEQ ID NO: 192 - RNA, 121 nt, synthetic construct
  source 1..121: mol_type = other RNA
cgattaccctgttatccctactgtttcaaaccaagttggattcaacaatctagcttatagcgtttgaaatcaccacaaggtgtcttcatatcggggcaactgcctttggcacccccggtta

SEQ ID NO: 193 - RNA, 108 nt, synthetic construct
  source 1..108: mol_type = other RNA
cgattaccctgttatccctactgtttcaaaccggcacttcggtgccgcgtttgaaatcaccacaaggtgtcttcatatcggggcaactgcctttggcacccccggtta

SEQ ID NO: 194 - RNA, 106 nt, synthetic construct
  source 1..106: mol_type = other RNA
cgattaccctgttatccctactgtttcaaaccggacttcggtccgcgtttgaaatcaccacaaggtgtcttcatatcggggcaactgcctttggcacccccggtta

SEQ ID NO: 195 - RNA, 100 nt, synthetic construct
  source 1..100: mol_type = other RNA
cgattaccctgttatccctactgtttcaaacccttcgggcgtttgaaatcaccacaaggtgtcttcatatcggggcaactgcctttggcacccccggtta

SEQ ID NO: 196 - RNA, 98 nt, synthetic construct
  source 1..98: mol_type = other RNA
cgattaccctgttatccctactgtttcaaaccgaaagcgtttgaaatcaccacaaggtgtcttcatatcggggcaactgcctttggcacccccggtta

SEQ ID NO: 197 - RNA, 113 nt, synthetic construct
  source 1..113: mol_type = other RNA
cgattaccctgttatccctactgtttcaaaccaggcacttcggtgcctatagcgtttgaaatcaccacaaggtgtcttcatatcggggcaactgcctttggcacccccggtta

SEQ ID NO: 198 - RNA, 111 nt, synthetic construct
  source 1..111: mol_type = other RNA
cgattaccctgttatccctactgtttcaaaccaggacttcggtcctatagcgtttgaaatcaccacaaggtgtcttcatatcggggcaactgcctttggcacccccggtta

SEQ ID NO: 199 - RNA, 105 nt, synthetic construct
  source 1..105: mol_type = other RNA
cgattaccctgttatccctactgtttcaaaccacttcggtatagcgtttgaaatcaccacaaggtgtcttcatatcggggcaactgcctttggcacccccggtta

SEQ ID NO: 200 - RNA, 98 nt, synthetic construct
  source 1..98: mol_type = other RNA
cgattaccctgttatccctactgtttcaaaccttcggcgtttgaaatcaccacaaggtgtcttcatatcggggcaactgcctttggcacccccggtta

SEQ ID NO: 201 - RNA, 95 nt, synthetic construct
  source 1..95: mol_type = other RNA
cgattaccctgttatccctactgtttcaaacaaacgtttgaaatcaccacaaggtgtcttcatatcggggcaactgcctttggcacccccggtta

SEQ ID NO: 202 - RNA, 105 nt, synthetic construct
  source 1..105: mol_type = other RNA
cgattaccctgttatccctactgtttcaaacggcacttcggtgccgtttgaaatcaccacaaggtgtcttcatatcggggcaactgcctttggcacccccggtta

SEQ ID NO: 203 - RNA, 97 nt, synthetic construct
  source 1..97: mol_type = other RNA
cgattaccctgttatccctactgtttcaaaccttcgggtttgaaatcaccacaaggtgtcttcatatcggggcaactgcctttggcacccccggtta

SEQ ID NO: 204 - RNA, 126 nt, synthetic construct
  source 1..126: mol_type = other RNA
cgattaccctgttatccctactgtttcaaaccaagttggattcaacaatctagcttatagcgtttgaaatcaccacaaggtgtcttcatatcggggcaactggcacttcggtgccacccccggtta

SEQ ID NO: 205 - RNA, 124 nt, synthetic construct
  source 1..124: mol_type = other RNA
cgattaccctgttatccctactgtttcaaaccaagttggattcaacaatctagcttatagcgtttgaaatcaccacaaggtgtcttcatatcggggcaactggacttcggtccacccccggtta

SEQ ID NO: 206 - RNA, 122 nt, synthetic construct
  source 1..122: mol_type = other RNA
cgattaccctgttatccctactgtttcaaaccaagttggattcaacaatctagcttatagcgtttgaaatcaccacaaggtgtcttcatatcggggcaactgccttcgggcacccccggtta

SEQ ID NO: 207 - RNA, 22 nt, synthetic construct
  source 1..22: mol_type = other RNA
cgattaccctgttatccctact

SEQ ID NO: 208 - protein, 1438 aa, synthetic construct
MKRTADGSEFESPKKKRKVTGTVKSTLAVDMGGRYTGIFSYTTDSGFPKAKEARAYVLNMPDNDALTYSMAARTQTRHRIRSQQRFVLARRLTYILIEGKLKRKLSPREKEAISSLLRRRGYSRLESELDLSVLQGVESGFFKCFLPNFDEDENLLTQWTSLTDGYLQNNSDSRRQIQIFLESSKDSKEFLTVVKSQHQDTKEYKNALKVMRDDAESMIEQSMFGHKHRRLYLEAIAQDIPRDSRLKPIIEAFSGVEKFHHFIGNLSNLQLRALRWYFNDPSMKNNVFDKERLKSVLVRAYQFFHYPKDLTQQRAEVLNAYEGATDILETLQTLNPELTIPPYEDQNNRRPPLDQTLWLSPRLLDQRYGDTWEIWVQNLLRSPLSKGIDENLDTILITTDRKARLLERQSGRLIHYTSQKLYHSYVLQRLLDRTVENDAYLLKTLVSSNRGNSNEIHQAQERLTRDLGSQHIKKFLDFVRQYYDEVDKAKRGLWFIVEKPLMERADIHPPMKNDSVILRLVGNILCVSDLVDLSFWTRKVKGQSTVRSLCTAIEKTRKEYGNSFNYLYQRALYLQSKGKKLSAEDKDFIKLQSNVLLVSDVIAEALDIKEEQKKKFANPFSLAQLYNIIETEKSGFISTTLAAVDENAWRNNLQGKARCVQLCADTVRPFDGALRNILDRQAYEIAKLKAEELLSTELKNQTIDLVVLLESNQFAFSASLAEVKKSANTAAIRQKVAKAQKRQQDRWLSKDERIKSASRGLCPYTGKNLGDKGEVDHIIPRSLSMNYMGSILNSEANLIYCSQEGNQLKLNGRKKLSDLADNYLKVVFGTADRGTICKYIEKSVSELTDAKIVQFELLDRSQQDAVRHALFLEDFSEARRRIIRLLGKINTARVNGTQAWFAKSFITKLRELTKEWCANNQITLAFDLYRLDAQTVSQDYRKKFALINKDWAKPDDKKQPIASHAIDAFCVFAAAKDKRNIANVLGVFDEVAEEQNLKTIAQLMPSEVNLISPKRKSILDKNEVGSRALMKEGIFAEHFLPILVRGDDCRIGFDWSESGSVKVKDADKLFGVLDGLLKQSQKRSVNGFETYTVDRIKAFELLHDVFIRPCSQKMLEQAEVLEKLHYITQNISVTSVYDAVNRQFKCREEILKDKDFDIKVDLGNRFGSAKGKITLPAKREWEKLVNRSELKNLIKDKLSDKGSEKTPDGETLIYDIFRSIPVQKLSHKATRRVWSLPKIPSISSGVRIKRKDSNGNDIYQLYMLNDTKCKGFVVNEKGVIDWSSDLVADLYKQPTLTILNGRYLKADQYVRMDQWYEVDCGRDDVIVKMCPGTSGRRYIEITQSKKQFEDWTGYISGSFWNYPVTIKLSSQQIANFVKNSQMPLLGKPRSGQITVITLGNTLKYWYCVESKNSMMNEAYQKAYLVHFNQGTPKKKRKV

SEQ ID NO: 209 - DNA, 5977 bp, synthetic construct
  source 1..5977: mol_type = other DNA
ccatgtcttcggaaatacaaggacttctgcatccatggagaatgcaaatatgtgaaggagctccgggctccctcctgcatgtaagtgccccttccccagggctgaatctcatcagcacactttgtcagccacgtggctgttcctcgttgtcactgttccttgaattcataatttcacccagtttcttctcaacctctgggcggaagttgggaggaggggaaatatatttttagtcagcggaagccccctcccccctataggatgcaatttcctgtggtatggttttgtgacgtgctttaatccttggggacatttcctgcttgcccagaaatgagcatgtggctaggacagctggcacctgaaggcaggcccttaattcttgcctgatgccctactctgggagggagaagccagtaggaaacatggcagagtgggcttccagggcagagtagagctcctgtgggaaggtaggaagtgcatttggatgcatgatgtataggtatgtgtgtatttgggtttatgtgcatgtaagtgtgcaaatgtggattgactgtgaggcatggcaggactgtacagagagggatcatcatggcggcaggttgaggcctctctttcttcttccttatcccagcaaggacgaggaggtgggagacatggagagtactggcctttggccacgttgtgagagaacaattcctttgtgcagggttcacaggaaatggaacctgacccattaggcatcagcccccggaattctagggcgcagtagtccagggtttccttgatgatgtcatacttatcctgtcccttttttttccacagctgccacccgggttaccatggaaaaaggtgtcatgggctgagcctcccagtggaaaatcgcttatatacctatgaccacacaaccatcctggccgtggtggctgtggtgctgtcatctgtctgtctgctggtcatcgtggggcttctcatgtttaggtaccataggagaggaggttatgatgtggaaaatgaagagaaagtgaagttgggcatgactaattcccactaatgacctaggaacttgtttattgcagcttataatggttacaaataaagcaatagcatcacaaatttcacaaataaagcatttttttcactgcattctagttgtggtttgtccaaactcatcaatgtatcttatcatgtctggatcgcgatcgcagtttgcaggtggcttgactgaaaaaaaaaaagaaaaagaaaacacctactttcctctccatggaaacagcatgccagaaaattttgtggacccttgaaatgagcacacatctcacttgcaaaagcacagcaccagcgccctctgctgtttcctggtttgatttagaactcagagaagctacagtactttctagactaaaataccatgtagagttcaggataatttcagatagacataggcaagcacattttagtacattctgtagtatattccagagtgaaggaaatcaaattaattaagctccggtgcccgtcagtgggcagagcgcacatcgcccacagtccccgagaagttggggggaggggtcggcaattgaaccggtgcctagagaaggtggcgcggggtaaactgggaaagtgatgtcgtgtactggctccgcctttttcccgagggtgggggagaaccgtatataagtgcagtagtcgccgtgaacgttctttttcgcaacgggtttgccgccagaacacaggtaagtgccgtgtgtggttcccgcgggcctggcctctttacgggttatggcccttgcgtgccttgaattacttccacgcccctggctgcagtacgtgattcttgatcccgagcttcgggttggaagtgggtgggagagttcgaggccttgcgcttaaggagccccttcgcctcgtgcttgagttgaggcctggcctgggcgctggggccgccgcgtgcgaatctggtggcaccttcgcgcctgtctcgctgctttcgataagtctctagccatttaaaatttttgatgacctgctgcgacgctttttttctggcaagatagtcttgtaaatgcgggccaagatcgatctgcacactggtatttcggtttttggggccgcgggcggcgacggggcccgtgcgtcccagcgcacatgttcggcgaggcggggcctgcgagcgcggccaccgagaatcggacgggggtagtctcaagctggccggcctgctctggtgcctggcctcgcgccgccgtgtatcgccccgccctgggcggcaaggctggcccggtcggcaccagttgcgtgagcggaaagatggccgcttcccggccctgctgcagggagctcaaaatggaggacgcggcgctcgggagagcgggcgggtgagtcacccacacaaaggaaaagggcctttccgtcctcagccgtcgcttcatgtgactccacggagtaccgggcgccgtccaggcacctcgattagttctcgatcgagcttttggagtacgtcgtctttaggttggggggaggggttttatgcgatggagtttccccacactgagtgggtggagactgaagttaggccagcttggcacttgatgtaattctccttggaatttgccctttttgagtttggatcttggttcattctcaagcctcagacagtggttcaaagtttttttcttccatttcaggtgtcgtgagctagcggttgcccaccctagtcattggaggtgacatccgctagcatgactgaatacaaacccactgtgcggctcgccactcgagacgatgtgcccagggctgtacgcacccttgccgcagcattcgcagattatcccgccacgcgccacaccgttgatcctgatcgccatatcgagagagtcacagagctgcaggaactatttctcacgcgtgtcgggttagacattggcaaggtttgggtggctgacgatggcgccgctgtggccgtgtggactacaccggagtctgtggaagctggggctgtgttcgcagaaataggccctcgaatggccgagttgagcggatcacggttggccgcgcagcaacagatggaaggcctcctggcgccacatagacccaaggaaccagcttggtttctggccaccgtcggtgtcagccctgaccaccagggaaaaggtctgggcagtgccgtagttctgccaggagtggaggcggccgagagggcaggggtgcctgccttcctggagacctccgctccaaggaacctgcccttctacgagcggcttgggtttaccgtgacagcagacgttgaggtccctgaaggaccgaggacctggtgcatgacaagaaagccaggtgctggctccgccaccaatttcagcctgctcaagcaggctggcgacgtggaggaaaacccaggacctgatagcactgaggcagtgatcaaggagttcatgcggttcaaggtgcacatggagggctccatgaacggccacgagttcgagatcgagggcgagggcgagggccgcccctacgagggcacccagaccgccaagctgaaggtgaccaagggtggccccctgcccttctcctgggacatcctgtcccctcagttcatgtacggctccagggccttcatcaagcaccccgccgacatccccgactactataagcagtccttccccgagggcttcaagtgggagcgcgtgatgaacttcgaggacggcggcgccgtgaccgtgacccaggacacctccctggaggacggcaccctgatctacaaggtgaagctccgcggcaccaacttccctcctgacggccccgtaatgcagaagaagacaatgggctgggaagcgtccaccgagcggttgtaccccgaggacggcgtgctgaagggcgacattaagatggccctgcgcctgaaggacggtggccgctacctggcggacttcaagaccacctacaaggccaagaagcccgtgcagatgcccggcgcctacaacgtcgaccgcaagttggacatcacctcccacaacgaggactacaccgtggtggaacagtacgaacgctccgagggccgccactccaccggaggcagtggcggttctaagcttagccatggcttcccgccggaggtggaggagcaggatgatggcacgctgcccatgtcttgtgcccaggagagcgggatggaccgtcaccctgcagcctgtgcttctgctaggatcaatgtgcgcgccgagtagggataacagggtaatcgcgccgaggagggcagagggtccctgctcacctgcggtgacgtggaagagaaccccggccctgccccaggaagcaatagtttctcaacttccgcattcggtcccgtcgcattcagcctgggcctcttgctggtgcttcccgcggcctttcccgccccagtcttcacactcgaagatttcgttggggactggcgacagacagccggctacaacctggaccaagtccttgaacagggaggtgtgtccagtttgtttcagaatctcggggtgtccgtaactccgatccaaaggattgtcctgagcggtgaaaatgggctgaagatcgacatccatgtcatcatcccgtatgaaggtctgagcggcgaccaaatgggccagatcgaaaaaatttttaaggtggtgtaccctgtggatgatcatcactttaaggtgatcctgcactatggcacactggtaatcgacggggttacgccgaacatgatcgactatttcggacggccgtatgaaggcatcgccgtgttcgacggcaaaaagatcactgtaacagggaccctgtggaacggcaacaaaattatcgacgagcgcctgatcaaccccgacggctccctgctgttccgagtaaccatcaacggagtgaccggctggcggctgtgcgaacgcattctggcgtaatgaaataaaggaaatttattttcattgcaatagtgtgttggaattttttgtgtctctcagtttaaacccgctgatcagcctcgactgtgccttctagttgccagccatctgttgtttgcccctcccccgtgccttccttgaccctggaaggtgccactcccactgtcctttcctaataaaatgaggaaattgcatcgcattgtctgagtaggtgtcattctattctggggggtggggtggggcaggacagcaagggggaggattgggaagacaatagcaggcatgctggggatgcggtgggctctatggcttctctcgaggtcaggcaacatcaccccttccctgggtaggtgtgtgggtggaggggctgtgggttccttagcctctctcctaagccaaacccagcaaacggctgccttggcaacccctcagggatgacagcactgccatgctctctggcaggcataatgttgccactgtgcctgaggccaacaccctgcgtcaggctgcaaacatccattcccttccctgtggggagggaggctctgggggccttagtgggagactctggacagggccaagagactgttgtatgcacactgcctccagcctgtcaagaaggcggcgtgcctggcatcccttctactggtgattggtgcagatcccttagctttttaaagcttccttgttttgtctgatcacacacagcagagctgccctgtatttggcagttggcagacagacccatcactccccaccatgtccacagtcacttgtgcatcctttcctataacatccttgtcaggagcttggtattagagggagttgtttaagagtggcatagaaagcccccatattatccttcccaaggtcttgggacagggtgggaaatgttcatcttaaatttgtaaaatggcatcattagtacagggtgaagaaggtgactcaagtagtcaaggtggattgaggtcaggaatctgtctataccagattggtcctgggcattttggtggatggatgtggggcttgcactgtgtggttgagaggccttataaggttgccctcctgga

SEQ ID NO: 210 - RNA, 98 nt, synthetic construct; identical to SEQ ID NO: 200
  source 1..98: mol_type = other RNA

SEQ ID NO: 211 - RNA, 109 nt, synthetic construct
  source 1..109: mol_type = other RNA
gtgcgcgccgagtagggataacgtttcagttgaaagaagtcactcttaaagtgagctgaaatcactaaaaattaagattgaacccggctactgactctgtcatccgggt

SEQ ID NO: 212 - RNA, 100 nt, synthetic construct
  source 1..100: mol_type = other RNA
attaccctgttatccctactgttttagagctagaaatagcaagttaaaataaggctagtccgttatcaacttgaaaaagtggcaccgagtcggtgctttt

SEQ ID NO: 213 - RNA, 98 nt, synthetic construct
  source 1..98: mol_type = other RNA
tccaggttccacgggatgctctgtttcaaaccttcggcgtttgaaatcaccacaaggtgtcttcatatcggggcaactgcctttggcacccccggtta

SEQ ID NO: 214 - RNA, 109 nt, synthetic construct
  source 1..109: mol_type = other RNA
tccaggttccacgggatgctctgtttcagttgaaagaagtcactcttaaagtgagctgaaatcactaaaaattaagattgaacccggctactgactctgtcatccgggt

SEQ ID NO: 215 - RNA, 100 nt, synthetic construct
  source 1..100: mol_type = other RNA
caggttccacgggatgctctgttttagagctagaaatagcaagttaaaataaggctagtccgttatcaacttgaaaaagtggcaccgagtcggtgctttt